European Patent Application EP 4 144 751 A1, published March 8, 2023. Title: New Coronavirus Vaccine and Method of obtaining a Virus vaccine. Applicant: Max-Delbrück-Centrum für Molekulare Medizin in der Helmholtz-Gemeinschaft. The sequence listing filed with the application follows.

SEQUENCE LISTING (259 sequences)

SEQ ID NO: 1 - protein, 223 aa, SARS coronavirus
  wildtype receptor binding domain of SARS-CoV-2 Wuhan variant
RVQPTESIVRFPNITNLCPFGEVFNATRFASVYAWNRKRISNCVADYSVLYNSASFSTFKCYGVSPTKLNDLCFTNVYADSFVIRGDEVRQIAPGQTGKIADYNYKLPDDFTGCVIAWNSNNLDSKVGGNYNYLYRLFRKSNLKPFERDISTEIYQAGSTPCNGVEGFNCYFPLQSYGFQPTNGVGYQPYRVVVLSFELLHAPATVCGPKKSTNLVKNKCVNF

SEQ ID NO: 2 - protein, 223 aa, Artificial Sequence
  mutant receptor binding domain of SARS-CoV-2 Wuhan variant comprising substitution G184E
RVQPTESIVRFPNITNLCPFGEVFNATRFASVYAWNRKRISNCVADYSVLYNSASFSTFKCYGVSPTKLNDLCFTNVYADSFVIRGDEVRQIAPGQTGKIADYNYKLPDDFTGCVIAWNSNNLDSKVGGNYNYLYRLFRKSNLKPFERDISTEIYQAGSTPCNGVEGFNCYFPLQSYGFQPTNEVGYQPYRVVVLSFELLHAPATVCGPKKSTNLVKNKCVNF

SEQ ID NO: 3 - protein, 223 aa, Artificial Sequence
  mutant receptor binding domain of SARS-CoV-2 Wuhan variant comprising substitution G184A
RVQPTESIVRFPNITNLCPFGEVFNATRFASVYAWNRKRISNCVADYSVLYNSASFSTFKCYGVSPTKLNDLCFTNVYADSFVIRGDEVRQIAPGQTGKIADYNYKLPDDFTGCVIAWNSNNLDSKVGGNYNYLYRLFRKSNLKPFERDISTEIYQAGSTPCNGVEGFNCYFPLQSYGFQPTNAVGYQPYRVVVLSFELLHAPATVCGPKKSTNLVKNKCVNF

SEQ ID NO: 4 - protein, 223 aa, Artificial Sequence
  mutant receptor binding domain of SARS-CoV-2 Wuhan variant comprising substitution G184C
RVQPTESIVRFPNITNLCPFGEVFNATRFASVYAWNRKRISNCVADYSVLYNSASFSTFKCYGVSPTKLNDLCFTNVYADSFVIRGDEVRQIAPGQTGKIADYNYKLPDDFTGCVIAWNSNNLDSKVGGNYNYLYRLFRKSNLKPFERDISTEIYQAGSTPCNGVEGFNCYFPLQSYGFQPTNCVGYQPYRVVVLSFELLHAPATVCGPKKSTNLVKNKCVNF

SEQ ID NO: 5 - protein, 223 aa, Artificial Sequence
  mutant receptor binding domain of SARS-CoV-2 Wuhan variant comprising substitution G184D
RVQPTESIVRFPNITNLCPFGEVFNATRFASVYAWNRKRISNCVADYSVLYNSASFSTFKCYGVSPTKLNDLCFTNVYADSFVIRGDEVRQIAPGQTGKIADYNYKLPDDFTGCVIAWNSNNLDSKVGGNYNYLYRLFRKSNLKPFERDISTEIYQAGSTPCNGVEGFNCYFPLQSYGFQPTNDVGYQPYRVVVLSFELLHAPATVCGPKKSTNLVKNKCVNF

SEQ ID NO: 6 - protein, 223 aa, Artificial Sequence
  mutant receptor binding domain of SARS-CoV-2 Wuhan variant comprising substitution G184F
RVQPTESIVRFPNITNLCPFGEVFNATRFASVYAWNRKRISNCVADYSVLYNSASFSTFKCYGVSPTKLNDLCFTNVYADSFVIRGDEVRQIAPGQTGKIADYNYKLPDDFTGCVIAWNSNNLDSKVGGNYNYLYRLFRKSNLKPFERDISTEIYQAGSTPCNGVEGFNCYFPLQSYGFQPTNFVGYQPYRVVVLSFELLHAPATVCGPKKSTNLVKNKCVNF

SEQ ID NO: 7 - protein, 223 aa, Artificial Sequence
  mutant receptor binding domain of SARS-CoV-2 Wuhan variant comprising substitution G184H
RVQPTESIVRFPNITNLCPFGEVFNATRFASVYAWNRKRISNCVADYSVLYNSASFSTFKCYGVSPTKLNDLCFTNVYADSFVIRGDEVRQIAPGQTGKIADYNYKLPDDFTGCVIAWNSNNLDSKVGGNYNYLYRLFRKSNLKPFERDISTEIYQAGSTPCNGVEGFNCYFPLQSYGFQPTNHVGYQPYRVVVLSFELLHAPATVCGPKKSTNLVKNKCVNF

SEQ ID NO: 8 - protein, 223 aa, Artificial Sequence
  mutant receptor binding domain of SARS-CoV-2 Wuhan variant comprising substitution G184I
RVQPTESIVRFPNITNLCPFGEVFNATRFASVYAWNRKRISNCVADYSVLYNSASFSTFKCYGVSPTKLNDLCFTNVYADSFVIRGDEVRQIAPGQTGKIADYNYKLPDDFTGCVIAWNSNNLDSKVGGNYNYLYRLFRKSNLKPFERDISTEIYQAGSTPCNGVEGFNCYFPLQSYGFQPTNIVGYQPYRVVVLSFELLHAPATVCGPKKSTNLVKNKCVNF

SEQ ID NO: 9 - protein, 223 aa, Artificial Sequence
  mutant receptor binding domain of SARS-CoV-2 Wuhan variant comprising substitution G184K
RVQPTESIVRFPNITNLCPFGEVFNATRFASVYAWNRKRISNCVADYSVLYNSASFSTFKCYGVSPTKLNDLCFTNVYADSFVIRGDEVRQIAPGQTGKIADYNYKLPDDFTGCVIAWNSNNLDSKVGGNYNYLYRLFRKSNLKPFERDISTEIYQAGSTPCNGVEGFNCYFPLQSYGFQPTNKVGYQPYRVVVLSFELLHAPATVCGPKKSTNLVKNKCVNF

SEQ ID NO: 10 - protein, 223 aa, Artificial Sequence
  mutant receptor binding domain of SARS-CoV-2 Wuhan variant comprising substitution G184L
RVQPTESIVRFPNITNLCPFGEVFNATRFASVYAWNRKRISNCVADYSVLYNSASFSTFKCYGVSPTKLNDLCFTNVYADSFVIRGDEVRQIAPGQTGKIADYNYKLPDDFTGCVIAWNSNNLDSKVGGNYNYLYRLFRKSNLKPFERDISTEIYQAGSTPCNGVEGFNCYFPLQSYGFQPTNLVGYQPYRVVVLSFELLHAPATVCGPKKSTNLVKNKCVNF

SEQ ID NO: 11 - protein, 223 aa, Artificial Sequence
  mutant receptor binding domain of SARS-CoV-2 Wuhan variant comprising substitution G184M
RVQPTESIVRFPNITNLCPFGEVFNATRFASVYAWNRKRISNCVADYSVLYNSASFSTFKCYGVSPTKLNDLCFTNVYADSFVIRGDEVRQIAPGQTGKIADYNYKLPDDFTGCVIAWNSNNLDSKVGGNYNYLYRLFRKSNLKPFERDISTEIYQAGSTPCNGVEGFNCYFPLQSYGFQPTNMVGYQPYRVVVLSFELLHAPATVCGPKKSTNLVKNKCVNF

SEQ ID NO: 12 - protein, 223 aa, Artificial Sequence
  mutant receptor binding domain of SARS-CoV-2 Wuhan variant comprising substitution G184N
RVQPTESIVRFPNITNLCPFGEVFNATRFASVYAWNRKRISNCVADYSVLYNSASFSTFKCYGVSPTKLNDLCFTNVYADSFVIRGDEVRQIAPGQTGKIADYNYKLPDDFTGCVIAWNSNNLDSKVGGNYNYLYRLFRKSNLKPFERDISTEIYQAGSTPCNGVEGFNCYFPLQSYGFQPTNNVGYQPYRVVVLSFELLHAPATVCGPKKSTNLVKNKCVNF

SEQ ID NO: 13 - protein, 223 aa, Artificial Sequence
  mutant receptor binding domain of SARS-CoV-2 Wuhan variant comprising substitution G184P
RVQPTESIVRFPNITNLCPFGEVFNATRFASVYAWNRKRISNCVADYSVLYNSASFSTFKCYGVSPTKLNDLCFTNVYADSFVIRGDEVRQIAPGQTGKIADYNYKLPDDFTGCVIAWNSNNLDSKVGGNYNYLYRLFRKSNLKPFERDISTEIYQAGSTPCNGVEGFNCYFPLQSYGFQPTNPVGYQPYRVVVLSFELLHAPATVCGPKKSTNLVKNKCVNF

SEQ ID NO: 14 - protein, 223 aa, Artificial Sequence
  mutant receptor binding domain of SARS-CoV-2 Wuhan variant comprising substitution G184Q
RVQPTESIVRFPNITNLCPFGEVFNATRFASVYAWNRKRISNCVADYSVLYNSASFSTFKCYGVSPTKLNDLCFTNVYADSFVIRGDEVRQIAPGQTGKIADYNYKLPDDFTGCVIAWNSNNLDSKVGGNYNYLYRLFRKSNLKPFERDISTEIYQAGSTPCNGVEGFNCYFPLQSYGFQPTNQVGYQPYRVVVLSFELLHAPATVCGPKKSTNLVKNKCVNF

SEQ ID NO: 15 - protein, 223 aa, Artificial Sequence
  mutant receptor binding domain of SARS-CoV-2 Wuhan variant comprising substitution G184R
RVQPTESIVRFPNITNLCPFGEVFNATRFASVYAWNRKRISNCVADYSVLYNSASFSTFKCYGVSPTKLNDLCFTNVYADSFVIRGDEVRQIAPGQTGKIADYNYKLPDDFTGCVIAWNSNNLDSKVGGNYNYLYRLFRKSNLKPFERDISTEIYQAGSTPCNGVEGFNCYFPLQSYGFQPTNRVGYQPYRVVVLSFELLHAPATVCGPKKSTNLVKNKCVNF

SEQ ID NO: 16 - protein, 223 aa, Artificial Sequence
  mutant receptor binding domain of SARS-CoV-2 Wuhan variant comprising substitution G184S
RVQPTESIVRFPNITNLCPFGEVFNATRFASVYAWNRKRISNCVADYSVLYNSASFSTFKCYGVSPTKLNDLCFTNVYADSFVIRGDEVRQIAPGQTGKIADYNYKLPDDFTGCVIAWNSNNLDSKVGGNYNYLYRLFRKSNLKPFERDISTEIYQAGSTPCNGVEGFNCYFPLQSYGFQPTNSVGYQPYRVVVLSFELLHAPATVCGPKKSTNLVKNKCVNF

SEQ ID NO: 17 - protein, 223 aa, Artificial Sequence
  mutant receptor binding domain of SARS-CoV-2 Wuhan variant comprising substitution G184T
RVQPTESIVRFPNITNLCPFGEVFNATRFASVYAWNRKRISNCVADYSVLYNSASFSTFKCYGVSPTKLNDLCFTNVYADSFVIRGDEVRQIAPGQTGKIADYNYKLPDDFTGCVIAWNSNNLDSKVGGNYNYLYRLFRKSNLKPFERDISTEIYQAGSTPCNGVEGFNCYFPLQSYGFQPTNTVGYQPYRVVVLSFELLHAPATVCGPKKSTNLVKNKCVNF

SEQ ID NO: 18 - protein, 223 aa, Artificial Sequence
  mutant receptor binding domain of SARS-CoV-2 Wuhan variant comprising substitution G184V
RVQPTESIVRFPNITNLCPFGEVFNATRFASVYAWNRKRISNCVADYSVLYNSASFSTFKCYGVSPTKLNDLCFTNVYADSFVIRGDEVRQIAPGQTGKIADYNYKLPDDFTGCVIAWNSNNLDSKVGGNYNYLYRLFRKSNLKPFERDISTEIYQAGSTPCNGVEGFNCYFPLQSYGFQPTNVVGYQPYRVVVLSFELLHAPATVCGPKKSTNLVKNKCVNF

SEQ ID NO: 19 - protein, 223 aa, Artificial Sequence
  mutant receptor binding domain of SARS-CoV-2 Wuhan variant comprising substitution G184W
RVQPTESIVRFPNITNLCPFGEVFNATRFASVYAWNRKRISNCVADYSVLYNSASFSTFKCYGVSPTKLNDLCFTNVYADSFVIRGDEVRQIAPGQTGKIADYNYKLPDDFTGCVIAWNSNNLDSKVGGNYNYLYRLFRKSNLKPFERDISTEIYQAGSTPCNGVEGFNCYFPLQSYGFQPTNWVGYQPYRVVVLSFELLHAPATVCGPKKSTNLVKNKCVNF

SEQ ID NO: 20 - protein, 223 aa, Artificial Sequence
  mutant receptor binding domain of SARS-CoV-2 Wuhan variant comprising substitution G184Y
RVQPTESIVRFPNITNLCPFGEVFNATRFASVYAWNRKRISNCVADYSVLYNSASFSTFKCYGVSPTKLNDLCFTNVYADSFVIRGDEVRQIAPGQTGKIADYNYKLPDDFTGCVIAWNSNNLDSKVGGNYNYLYRLFRKSNLKPFERDISTEIYQAGSTPCNGVEGFNCYFPLQSYGFQPTNYVGYQPYRVVVLSFELLHAPATVCGPKKSTNLVKNKCVNF

SEQ ID NO: 21 - protein, 223 aa, Artificial Sequence
  mutant receptor binding domain of SARS-CoV-2 Wuhan variant comprising substitution Y187A
RVQPTESIVRFPNITNLCPFGEVFNATRFASVYAWNRKRISNCVADYSVLYNSASFSTFKCYGVSPTKLNDLCFTNVYADSFVIRGDEVRQIAPGQTGKIADYNYKLPDDFTGCVIAWNSNNLDSKVGGNYNYLYRLFRKSNLKPFERDISTEIYQAGSTPCNGVEGFNCYFPLQSYGFQPTNGVGAQPYRVVVLSFELLHAPATVCGPKKSTNLVKNKCVNF

SEQ ID NO: 22 - protein, 223 aa, Artificial Sequence
  mutant receptor binding domain of SARS-CoV-2 Wuhan variant comprising substitution Y187C
RVQPTESIVRFPNITNLCPFGEVFNATRFASVYAWNRKRISNCVADYSVLYNSASFSTFKCYGVSPTKLNDLCFTNVYADSFVIRGDEVRQIAPGQTGKIADYNYKLPDDFTGCVIAWNSNNLDSKVGGNYNYLYRLFRKSNLKPFERDISTEIYQAGSTPCNGVEGFNCYFPLQSYGFQPTNGVGCQPYRVVVLSFELLHAPATVCGPKKSTNLVKNKCVNF

SEQ ID NO: 23 - protein, 223 aa, Artificial Sequence
  mutant receptor binding domain of SARS-CoV-2 Wuhan variant comprising substitution Y187D
RVQPTESIVRFPNITNLCPFGEVFNATRFASVYAWNRKRISNCVADYSVLYNSASFSTFKCYGVSPTKLNDLCFTNVYADSFVIRGDEVRQIAPGQTGKIADYNYKLPDDFTGCVIAWNSNNLDSKVGGNYNYLYRLFRKSNLKPFERDISTEIYQAGSTPCNGVEGFNCYFPLQSYGFQPTNGVGDQPYRVVVLSFELLHAPATVCGPKKSTNLVKNKCVNF

SEQ ID NO: 24 - protein, 223 aa, Artificial Sequence
  mutant receptor binding domain of SARS-CoV-2 Wuhan variant comprising substitution Y187E
RVQPTESIVRFPNITNLCPFGEVFNATRFASVYAWNRKRISNCVADYSVLYNSASFSTFKCYGVSPTKLNDLCFTNVYADSFVIRGDEVRQIAPGQTGKIADYNYKLPDDFTGCVIAWNSNNLDSKVGGNYNYLYRLFRKSNLKPFERDISTEIYQAGSTPCNGVEGFNCYFPLQSYGFQPTNGVGEQPYRVVVLSFELLHAPATVCGPKKSTNLVKNKCVNF

SEQ ID NO: 25 - protein, 223 aa, Artificial Sequence
  mutant receptor binding domain of SARS-CoV-2 Wuhan variant comprising substitution Y187G
RVQPTESIVRFPNITNLCPFGEVFNATRFASVYAWNRKRISNCVADYSVLYNSASFSTFKCYGVSPTKLNDLCFTNVYADSFVIRGDEVRQIAPGQTGKIADYNYKLPDDFTGCVIAWNSNNLDSKVGGNYNYLYRLFRKSNLKPFERDISTEIYQAGSTPCNGVEGFNCYFPLQSYGFQPTNGVGGQPYRVVVLSFELLHAPATVCGPKKSTNLVKNKCVNF

SEQ ID NO: 26 - protein, 223 aa, Artificial Sequence
  mutant receptor binding domain of SARS-CoV-2 Wuhan variant comprising substitution Y187I
RVQPTESIVRFPNITNLCPFGEVFNATRFASVYAWNRKRISNCVADYSVLYNSASFSTFKCYGVSPTKLNDLCFTNVYADSFVIRGDEVRQIAPGQTGKIADYNYKLPDDFTGCVIAWNSNNLDSKVGGNYNYLYRLFRKSNLKPFERDISTEIYQAGSTPCNGVEGFNCYFPLQSYGFQPTNGVGIQPYRVVVLSFELLHAPATVCGPKKSTNLVKNKCVNF

SEQ ID NO: 27 - protein, 223 aa, Artificial Sequence
  mutant receptor binding domain of SARS-CoV-2 Wuhan variant comprising substitution Y187L
RVQPTESIVRFPNITNLCPFGEVFNATRFASVYAWNRKRISNCVADYSVLYNSASFSTFKCYGVSPTKLNDLCFTNVYADSFVIRGDEVRQIAPGQTGKIADYNYKLPDDFTGCVIAWNSNNLDSKVGGNYNYLYRLFRKSNLKPFERDISTEIYQAGSTPCNGVEGFNCYFPLQSYGFQPTNGVGLQPYRVVVLSFELLHAPATVCGPKKSTNLVKNKCVNF

SEQ ID NO: 28 - protein, 223 aa, Artificial Sequence
  mutant receptor binding domain of SARS-CoV-2 Wuhan variant comprising substitution Y187K
RVQPTESIVRFPNITNLCPFGEVFNATRFASVYAWNRKRISNCVADYSVLYNSASFSTFKCYGVSPTKLNDLCFTNVYADSFVIRGDEVRQIAPGQTGKIADYNYKLPDDFTGCVIAWNSNNLDSKVGGNYNYLYRLFRKSNLKPFERDISTEIYQAGSTPCNGVEGFNCYFPLQSYGFQPTNGVGKQPYRVVVLSFELLHAPATVCGPKKSTNLVKNKCVNF

SEQ ID NO: 29 - protein, 223 aa, Artificial Sequence
  mutant receptor binding domain of SARS-CoV-2 Wuhan variant comprising substitution Y187M
RVQPTESIVRFPNITNLCPFGEVFNATRFASVYAWNRKRISNCVADYSVLYNSASFSTFKCYGVSPTKLNDLCFTNVYADSFVIRGDEVRQIAPGQTGKIADYNYKLPDDFTGCVIAWNSNNLDSKVGGNYNYLYRLFRKSNLKPFERDISTEIYQAGSTPCNGVEGFNCYFPLQSYGFQPTNGVGMQPYRVVVLSFELLHAPATVCGPKKSTNLVKNKCVNF

SEQ ID NO: 30 - protein, 223 aa, Artificial Sequence
  mutant receptor binding domain of SARS-CoV-2 Wuhan variant comprising substitution Y187N
RVQPTESIVRFPNITNLCPFGEVFNATRFASVYAWNRKRISNCVADYSVLYNSASFSTFKCYGVSPTKLNDLCFTNVYADSFVIRGDEVRQIAPGQTGKIADYNYKLPDDFTGCVIAWNSNNLDSKVGGNYNYLYRLFRKSNLKPFERDISTEIYQAGSTPCNGVEGFNCYFPLQSYGFQPTNGVGNQPYRVVVLSFELLHAPATVCGPKKSTNLVKNKCVNF

SEQ ID NO: 31 - protein, 223 aa, Artificial Sequence
  mutant receptor binding domain of SARS-CoV-2 Wuhan variant comprising substitution Y187Q
RVQPTESIVRFPNITNLCPFGEVFNATRFASVYAWNRKRISNCVADYSVLYNSASFSTFKCYGVSPTKLNDLCFTNVYADSFVIRGDEVRQIAPGQTGKIADYNYKLPDDFTGCVIAWNSNNLDSKVGGNYNYLYRLFRKSNLKPFERDISTEIYQAGSTPCNGVEGFNCYFPLQSYGFQPTNGVGQQPYRVVVLSFELLHAPATVCGPKKSTNLVKNKCVNF

SEQ ID NO: 32 - protein, 222 aa, Artificial Sequence
  mutant receptor binding domain of SARS-CoV-2 Wuhan variant comprising substitution Y187R
VQPTESIVRFPNITNLCPFGEVFNATRFASVYAWNRKRISNCVADYSVLYNSASFSTFKCYGVSPTKLNDLCFTNVYADSFVIRGDEVRQIAPGQTGKIADYNYKLPDDFTGCVIAWNSNNLDSKVGGNYNYLYRLFRKSNLKPFERDISTEIYQAGSTPCNGVEGFNCYFPLQSYGFQPTNGVGRQPYRVVVLSFELLHAPATVCGPKKSTNLVKNKCVNF

SEQ ID NO: 33 - protein, 223 aa, Artificial Sequence
  mutant receptor binding domain of SARS-CoV-2 Wuhan variant comprising substitution Y187S
RVQPTESIVRFPNITNLCPFGEVFNATRFASVYAWNRKRISNCVADYSVLYNSASFSTFKCYGVSPTKLNDLCFTNVYADSFVIRGDEVRQIAPGQTGKIADYNYKLPDDFTGCVIAWNSNNLDSKVGGNYNYLYRLFRKSNLKPFERDISTEIYQAGSTPCNGVEGFNCYFPLQSYGFQPTNGVGSQPYRVVVLSFELLHAPATVCGPKKSTNLVKNKCVNF

SEQ ID NO: 34 - protein, 223 aa, Artificial Sequence
  mutant receptor binding domain of SARS-CoV-2 Wuhan variant comprising substitution Y187T
RVQPTESIVRFPNITNLCPFGEVFNATRFASVYAWNRKRISNCVADYSVLYNSASFSTFKCYGVSPTKLNDLCFTNVYADSFVIRGDEVRQIAPGQTGKIADYNYKLPDDFTGCVIAWNSNNLDSKVGGNYNYLYRLFRKSNLKPFERDISTEIYQAGSTPCNGVEGFNCYFPLQSYGFQPTNGVGTQPYRVVVLSFELLHAPATVCGPKKSTNLVKNKCVNF

SEQ ID NO: 35 - protein, 223 aa, Artificial Sequence
  mutant receptor binding domain of SARS-CoV-2 Wuhan variant comprising substitution Y187V
RVQPTESIVRFPNITNLCPFGEVFNATRFASVYAWNRKRISNCVADYSVLYNSASFSTFKCYGVSPTKLNDLCFTNVYADSFVIRGDEVRQIAPGQTGKIADYNYKLPDDFTGCVIAWNSNNLDSKVGGNYNYLYRLFRKSNLKPFERDISTEIYQAGSTPCNGVEGFNCYFPLQSYGFQPTNGVGVQPYRVVVLSFELLHAPATVCGPKKSTNLVKNKCVNF

SEQ ID NO: 36 - protein, 223 aa, Artificial Sequence
  mutant receptor binding domain of SARS-CoV-2 Wuhan variant comprising substitution F138A
RVQPTESIVRFPNITNLCPFGEVFNATRFASVYAWNRKRISNCVADYSVLYNSASFSTFKCYGVSPTKLNDLCFTNVYADSFVIRGDEVRQIAPGQTGKIADYNYKLPDDFTGCVIAWNSNNLDSKVGGNYNYLYRLARKSNLKPFERDISTEIYQAGSTPCNGVEGFNCYFPLQSYGFQPTNGVGYQPYRVVVLSFELLHAPATVCGPKKSTNLVKNKCVNF

SEQ ID NO: 37 - protein, 223 aa, Artificial Sequence
  mutant receptor binding domain of SARS-CoV-2 Wuhan variant comprising substitution F138C
RVQPTESIVRFPNITNLCPFGEVFNATRFASVYAWNRKRISNCVADYSVLYNSASFSTFKCYGVSPTKLNDLCFTNVYADSFVIRGDEVRQIAPGQTGKIADYNYKLPDDFTGCVIAWNSNNLDSKVGGNYNYLYRLCRKSNLKPFERDISTEIYQAGSTPCNGVEGFNCYFPLQSYGFQPTNGVGYQPYRVVVLSFELLHAPATVCGPKKSTNLVKNKCVNF

SEQ ID NO: 38 - protein, 223 aa, Artificial Sequence
  mutant receptor binding domain of SARS-CoV-2 Wuhan variant comprising substitution F138E
RVQPTESIVRFPNITNLCPFGEVFNATRFASVYAWNRKRISNCVADYSVLYNSASFSTFKCYGVSPTKLNDLCFTNVYADSFVIRGDEVRQIAPGQTGKIADYNYKLPDDFTGCVIAWNSNNLDSKVGGNYNYLYRLERKSNLKPFERDISTEIYQAGSTPCNGVEGFNCYFPLQSYGFQPTNGVGYQPYRVVVLSFELLHAPATVCGPKKSTNLVKNKCVNF

SEQ ID NO: 39 - protein, 223 aa, Artificial Sequence
  mutant receptor binding domain of SARS-CoV-2 Wuhan variant comprising substitution F138G
RVQPTESIVRFPNITNLCPFGEVFNATRFASVYAWNRKRISNCVADYSVLYNSASFSTFKCYGVSPTKLNDLCFTNVYADSFVIRGDEVRQIAPGQTGKIADYNYKLPDDFTGCVIAWNSNNLDSKVGGNYNYLYRLGRKSNLKPFERDISTEIYQAGSTPCNGVEGFNCYFPLQSYGFQPTNGVGYQPYRVVVLSFELLHAPATVCGPKKSTNLVKNKCVNF

SEQ ID NO: 40 - protein, 223 aa, Artificial Sequence
  mutant receptor binding domain of SARS-CoV-2 Wuhan variant comprising substitution F138I
RVQPTESIVRFPNITNLCPFGEVFNATRFASVYAWNRKRISNCVADYSVLYNSASFSTFKCYGVSPTKLNDLCFTNVYADSFVIRGDEVRQIAPGQTGKIADYNYKLPDDFTGCVIAWNSNNLDSKVGGNYNYLYRLIRKSNLKPFERDISTEIYQAGSTPCNGVEGFNCYFPLQSYGFQPTNGVGYQPYRVVVLSFELLHAPATVCGPKKSTNLVKNKCVNF

SEQ ID NO: 41 - protein, 223 aa, Artificial Sequence
  mutant receptor binding domain of SARS-CoV-2 Wuhan variant comprising substitution F138K
RVQPTESIVRFPNITNLCPFGEVFNATRFASVYAWNRKRISNCVADYSVLYNSASFSTFKCYGVSPTKLNDLCFTNVYADSFVIRGDEVRQIAPGQTGKIADYNYKLPDDFTGCVIAWNSNNLDSKVGGNYNYLYRLKRKSNLKPFERDISTEIYQAGSTPCNGVEGFNCYFPLQSYGFQPTNGVGYQPYRVVVLSFELLHAPATVCGPKKSTNLVKNKCVNF

SEQ ID NO: 42 - protein, 223 aa, Artificial Sequence
  mutant receptor binding domain of SARS-CoV-2 Wuhan variant comprising substitution F138N
RVQPTESIVRFPNITNLCPFGEVFNATRFASVYAWNRKRISNCVADYSVLYNSASFSTFKCYGVSPTKLNDLCFTNVYADSFVIRGDEVRQIAPGQTGKIADYNYKLPDDFTGCVIAWNSNNLDSKVGGNYNYLYRLNRKSNLKPFERDISTEIYQAGSTPCNGVEGFNCYFPLQSYGFQPTNGVGYQPYRVVVLSFELLHAPATVCGPKKSTNLVKNKCVNF

SEQ ID NO: 43 - protein, 223 aa, Artificial Sequence
  mutant receptor binding domain of SARS-CoV-2 Wuhan variant comprising substitution F138Q
RVQPTESIVRFPNITNLCPFGEVFNATRFASVYAWNRKRISNCVADYSVLYNSASFSTFKCYGVSPTKLNDLCFTNVYADSFVIRGDEVRQIAPGQTGKIADYNYKLPDDFTGCVIAWNSNNLDSKVGGNYNYLYRLQRKSNLKPFERDISTEIYQAGSTPCNGVEGFNCYFPLQSYGFQPTNGVGYQPYRVVVLSFELLHAPATVCGPKKSTNLVKNKCVNF

SEQ ID NO: 44 - protein, 223 aa, Artificial Sequence
  mutant receptor binding domain of SARS-CoV-2 Wuhan variant comprising substitution F138R
RVQPTESIVRFPNITNLCPFGEVFNATRFASVYAWNRKRISNCVADYSVLYNSASFSTFKCYGVSPTKLNDLCFTNVYADSFVIRGDEVRQIAPGQTGKIADYNYKLPDDFTGCVIAWNSNNLDSKVGGNYNYLYRLRRKSNLKPFERDISTEIYQAGSTPCNGVEGFNCYFPLQSYGFQPTNGVGYQPYRVVVLSFELLHAPATVCGPKKSTNLVKNKCVNF

SEQ ID NO: 45 - protein, 223 aa, Artificial Sequence
  mutant receptor binding domain of SARS-CoV-2 Wuhan variant comprising substitution F138S
RVQPTESIVRFPNITNLCPFGEVFNATRFASVYAWNRKRISNCVADYSVLYNSASFSTFKCYGVSPTKLNDLCFTNVYADSFVIRGDEVRQIAPGQTGKIADYNYKLPDDFTGCVIAWNSNNLDSKVGGNYNYLYRLSRKSNLKPFERDISTEIYQAGSTPCNGVEGFNCYFPLQSYGFQPTNGVGYQPYRVVVLSFELLHAPATVCGPKKSTNLVKNKCVNF

SEQ ID NO: 46 - protein, 223 aa, Artificial Sequence
  mutant receptor binding domain of SARS-CoV-2 Wuhan variant comprising substitution F138T
RVQPTESIVRFPNITNLCPFGEVFNATRFASVYAWNRKRISNCVADYSVLYNSASFSTFKCYGVSPTKLNDLCFTNVYADSFVIRGDEVRQIAPGQTGKIADYNYKLPDDFTGCVIAWNSNNLDSKVGGNYNYLYRLTRKSNLKPFERDISTEIYQAGSTPCNGVEGFNCYFPLQSYGFQPTNGVGYQPYRVVVLSFELLHAPATVCGPKKSTNLVKNKCVNF

SEQ ID NO: 47 - protein, 223 aa, Artificial Sequence
  mutant receptor binding domain of SARS-CoV-2 Wuhan variant comprising substitution F138W
RVQPTESIVRFPNITNLCPFGEVFNATRFASVYAWNRKRISNCVADYSVLYNSASFSTFKCYGVSPTKLNDLCFTNVYADSFVIRGDEVRQIAPGQTGKIADYNYKLPDDFTGCVIAWNSNNLDSKVGGNYNYLYRLWRKSNLKPFERDISTEIYQAGSTPCNGVEGFNCYFPLQSYGFQPTNGVGYQPYRVVVLSFELLHAPATVCGPKKSTNLVKNKCVNF

SEQ ID NO: 48 - protein, 223 aa, Artificial Sequence
  mutant receptor binding domain of SARS-CoV-2 Wuhan variant comprising substitution F138Y
RVQPTESIVRFPNITNLCPFGEVFNATRFASVYAWNRKRISNCVADYSVLYNSASFSTFKCYGVSPTKLNDLCFTNVYADSFVIRGDEVRQIAPGQTGKIADYNYKLPDDFTGCVIAWNSNNLDSKVGGNYNYLYRLYRKSNLKPFERDISTEIYQAGSTPCNGVEGFNCYFPLQSYGFQPTNGVGYQPYRVVVLSFELLHAPATVCGPKKSTNLVKNKCVNF

SEQ ID NO: 49 - protein, 223 aa, Artificial Sequence
  mutant receptor binding domain of SARS-CoV-2 Wuhan variant comprising substitution F168C
RVQPTESIVRFPNITNLCPFGEVFNATRFASVYAWNRKRISNCVADYSVLYNSASFSTFKCYGVSPTKLNDLCFTNVYADSFVIRGDEVRQIAPGQTGKIADYNYKLPDDFTGCVIAWNSNNLDSKVGGNYNYLYRLFRKSNLKPFERDISTEIYQAGSTPCNGVEGCNCYFPLQSYGFQPTNGVGYQPYRVVVLSFELLHAPATVCGPKKSTNLVKNKCVNF

SEQ ID NO: 50 - protein, 223 aa, Artificial Sequence
  mutant receptor binding domain of SARS-CoV-2 Wuhan variant comprising substitution F168D
RVQPTESIVRFPNITNLCPFGEVFNATRFASVYAWNRKRISNCVADYSVLYNSASFSTFKCYGVSPTKLNDLCFTNVYADSFVIRGDEVRQIAPGQTGKIADYNYKLPDDFTGCVIAWNSNNLDSKVGGNYNYLYRLFRKSNLKPFERDISTEIYQAGSTPCNGVEGDNCYFPLQSYGFQPTNGVGYQPYRVVVLSFELLHAPATVCGPKKSTNLVKNKCVNF

SEQ ID NO: 51 - protein, 223 aa, Artificial Sequence
  mutant receptor binding domain of SARS-CoV-2 Wuhan variant comprising substitution F168E
RVQPTESIVRFPNITNLCPFGEVFNATRFASVYAWNRKRISNCVADYSVLYNSASFSTFKCYGVSPTKLNDLCFTNVYADSFVIRGDEVRQIAPGQTGKIADYNYKLPDDFTGCVIAWNSNNLDSKVGGNYNYLYRLFRKSNLKPFERDISTEIYQAGSTPCNGVEGENCYFPLQSYGFQPTNGVGYQPYRVVVLSFELLHAPATVCGPKKSTNLVKNKCVNF

SEQ ID NO: 52 - protein, 223 aa, Artificial Sequence
  mutant receptor binding domain of SARS-CoV-2 Wuhan variant comprising substitution L137D
RVQPTESIVRFPNITNLCPFGEVFNATRFASVYAWNRKRISNCVADYSVLYNSASFSTFKCYGVSPTKLNDLCFTNVYADSFVIRGDEVRQIAPGQTGKIADYNYKLPDDFTGCVIAWNSNNLDSKVGGNYNYLYRDFRKSNLKPFERDISTEIYQAGSTPCNGVEGFNCYFPLQSYGFQPTNGVGYQPYRVVVLSFELLHAPATVCGPKKSTNLVKNKCVNF

SEQ ID NO: 53 - protein, 223 aa, Artificial Sequence
  mutant receptor binding domain of SARS-CoV-2 Wuhan variant comprising substitution L137E
RVQPTESIVRFPNITNLCPFGEVFNATRFASVYAWNRKRISNCVADYSVLYNSASFSTFKCYGVSPTKLNDLCFTNVYADSFVIRGDEVRQIAPGQTGKIADYNYKLPDDFTGCVIAWNSNNLDSKVGGNYNYLYREFRKSNLKPFERDISTEIYQAGSTPCNGVEGFNCYFPLQSYGFQPTNGVGYQPYRVVVLSFELLHAPATVCGPKKSTNLVKNKCVNF

SEQ ID NO: 54 - protein, 223 aa, Artificial Sequence
  mutant receptor binding domain of SARS-CoV-2 Wuhan variant comprising substitution L137K
RVQPTESIVRFPNITNLCPFGEVFNATRFASVYAWNRKRISNCVADYSVLYNSASFSTFKCYGVSPTKLNDLCFTNVYADSFVIRGDEVRQIAPGQTGKIADYNYKLPDDFTGCVIAWNSNNLDSKVGGNYNYLYRKFRKSNLKPFERDISTEIYQAGSTPCNGVEGFNCYFPLQSYGFQPTNGVGYQPYRVVVLSFELLHAPATVCGPKKSTNLVKNKCVNF

SEQ ID NO: 55 - protein, 223 aa, Artificial Sequence
  mutant receptor binding domain of SARS-CoV-2 Wuhan variant comprising substitution L137R
RVQPTESIVRFPNITNLCPFGEVFNATRFASVYAWNRKRISNCVADYSVLYNSASFSTFKCYGVSPTKLNDLCFTNVYADSFVIRGDEVRQIAPGQTGKIADYNYKLPDDFTGCVIAWNSNNLDSKVGGNYNYLYRRFRKSNLKPFERDISTEIYQAGSTPCNGVEGFNCYFPLQSYGFQPTNGVGYQPYRVVVLSFELLHAPATVCGPKKSTNLVKNKCVNF

SEQ ID NO: 56 - protein, 223 aa, Artificial Sequence
  mutant receptor binding domain of SARS-CoV-2 Wuhan variant comprising substitution L137Y
RVQPTESIVRFPNITNLCPFGEVFNATRFASVYAWNRKRISNCVADYSVLYNSASFSTFKCYGVSPTKLNDLCFTNVYADSFVIRGDEVRQIAPGQTGKIADYNYKLPDDFTGCVIAWNSNNLDSKVGGNYNYLYRYFRKSNLKPFERDISTEIYQAGSTPCNGVEGFNCYFPLQSYGFQPTNGVGYQPYRVVVLSFELLHAPATVCGPKKSTNLVKNKCVNF

SEQ ID NO: 57 - protein, 223 aa, Artificial Sequence
  mutant receptor binding domain of SARS-CoV-2 Wuhan variant comprising substitution Q180C
RVQPTESIVRFPNITNLCPFGEVFNATRFASVYAWNRKRISNCVADYSVLYNSASFSTFKCYGVSPTKLNDLCFTNVYADSFVIRGDEVRQIAPGQTGKIADYNYKLPDDFTGCVIAWNSNNLDSKVGGNYNYLYRLFRKSNLKPFERDISTEIYQAGSTPCNGVEGFNCYFPLQSYGFCPTNGVGYQPYRVVVLSFELLHAPATVCGPKKSTNLVKNKCVNF

SEQ ID NO: 58 - protein, 223 aa, Artificial Sequence
  mutant receptor binding domain of SARS-CoV-2 Wuhan variant comprising substitution Q180D
RVQPTESIVRFPNITNLCPFGEVFNATRFASVYAWNRKRISNCVADYSVLYNSASFSTFKCYGVSPTKLNDLCFTNVYADSFVIRGDEVRQIAPGQTGKIADYNYKLPDDFTGCVIAWNSNNLDSKVGGNYNYLYRLFRKSNLKPFERDISTEIYQAGSTPCNGVEGFNCYFPLQSYGFDPTNGVGYQPYRVVVLSFELLHAPATVCGPKKSTNLVKNKCVNF

SEQ ID NO: 59 - protein, 223 aa, Artificial Sequence
  mutant receptor binding domain of SARS-CoV-2 Wuhan variant comprising substitution Q180I
RVQPTESIVRFPNITNLCPFGEVFNATRFASVYAWNRKRISNCVADYSVLYNSASFSTFKCYGVSPTKLNDLCFTNVYADSFVIRGDEVRQIAPGQTGKIADYNYKLPDDFTGCVIAWNSNNLDSKVGGNYNYLYRLFRKSNLKPFERDISTEIYQAGSTPCNGVEGFNCYFPLQSYGFIPTNGVGYQPYRVVVLSFELLHAPATVCGPKKSTNLVKNKCVNF

SEQ ID NO: 60 - protein, 223 aa, Artificial Sequence
  mutant receptor binding domain of SARS-CoV-2 Wuhan variant comprising substitution Q180K
RVQPTESIVRFPNITNLCPFGEVFNATRFASVYAWNRKRISNCVADYSVLYNSASFSTFKCYGVSPTKLNDLCFTNVYADSFVIRGDEVRQIAPGQTGKIADYNYKLPDDFTGCVIAWNSNNLDSKVGGNYNYLYRLFRKSNLKPFERDISTEIYQAGSTPCNGVEGFNCYFPLQSYGFKPTNGVGYQPYRVVVLSFELLHAPATVCGPKKSTNLVKNKCVNF

SEQ ID NO: 61 - protein, 223 aa, Artificial Sequence
  mutant receptor binding domain of SARS-CoV-2 Wuhan variant comprising substitution Q180L
RVQPTESIVRFPNITNLCPFGEVFNATRFASVYAWNRKRISNCVADYSVLYNSASFSTFKCYGVSPTKLNDLCFTNVYADSFVIRGDEVRQIAPGQTGKIADYNYKLPDDFTGCVIAWNSNNLDSKVGGNYNYLYRLFRKSNLKPFERDISTEIYQAGSTPCNGVEGFNCYFPLQSYGFLPTNGVGYQPYRVVVLSFELLHAPATVCGPKKSTNLVKNKCVNF

SEQ ID NO: 62 - protein, 223 aa, Artificial Sequence
  mutant receptor binding domain of SARS-CoV-2 Wuhan variant comprising substitution Q180V
RVQPTESIVRFPNITNLCPFGEVFNATRFASVYAWNRKRISNCVADYSVLYNSASFSTFKCYGVSPTKLNDLCFTNVYADSFVIRGDEVRQIAPGQTGKIADYNYKLPDDFTGCVIAWNSNNLDSKVGGNYNYLYRLFRKSNLKPFERDISTEIYQAGSTPCNGVEGFNCYFPLQSYGFVPTNGVGYQPYRVVVLSFELLHAPATVCGPKKSTNLVKNKCVNF

SEQ ID NO: 63 - protein, 223 aa, Artificial Sequence
  mutant receptor binding domain of SARS-CoV-2 Wuhan variant comprising substitution S55N
RVQPTESIVRFPNITNLCPFGEVFNATRFASVYAWNRKRISNCVADYSVLYNSANFSTFKCYGVSPTKLNDLCFTNVYADSFVIRGDEVRQIAPGQTGKIADYNYKLPDDFTGCVIAWNSNNLDSKVGGNYNYLYRLFRKSNLKPFERDISTEIYQAGSTPCNGVEGFNCYFPLQSYGFQPTNGVGYQPYRVVVLSFELLHAPATVCGPKKSTNLVKNKCVNF

SEQ ID NO: 64 - protein, 223 aa, Artificial Sequence
  mutant receptor binding domain of SARS-CoV-2 Wuhan variant comprising substitution Y131A
RVQPTESIVRFPNITNLCPFGEVFNATRFASVYAWNRKRISNCVADYSVLYNSASFSTFKCYGVSPTKLNDLCFTNVYADSFVIRGDEVRQIAPGQTGKIADYNYKLPDDFTGCVIAWNSNNLDSKVGGNANYLYRLFRKSNLKPFERDISTEIYQAGSTPCNGVEGFNCYFPLQSYGFQPTNGVGYQPYRVVVLSFELLHAPATVCGPKKSTNLVKNKCVNF

SEQ ID NO: 65 - protein, 223 aa, Artificial Sequence
  mutant receptor binding domain of SARS-CoV-2 Wuhan variant comprising substitution Y131C
RVQPTESIVRFPNITNLCPFGEVFNATRFASVYAWNRKRISNCVADYSVLYNSASFSTFKCYGVSPTKLNDLCFTNVYADSFVIRGDEVRQIAPGQTGKIADYNYKLPDDFTGCVIAWNSNNLDSKVGGNCNYLYRLFRKSNLKPFERDISTEIYQAGSTPCNGVEGFNCYFPLQSYGFQPTNGVGYQPYRVVVLSFELLHAPATVCGPKKSTNLVKNKCVNF

SEQ ID NO: 66 - protein, 223 aa, Artificial Sequence
  mutant receptor binding domain of SARS-CoV-2 Wuhan variant comprising substitution Y131D
RVQPTESIVRFPNITNLCPFGEVFNATRFASVYAWNRKRISNCVADYSVLYNSASFSTFKCYGVSPTKLNDLCFTNVYADSFVIRGDEVRQIAPGQTGKIADYNYKLPDDFTGCVIAWNSNNLDSKVGGNDNYLYRLFRKSNLKPFERDISTEIYQAGSTPCNGVEGFNCYFPLQSYGFQPTNGVGYQPYRVVVLSFELLHAPATVCGPKKSTNLVKNKCVNF

SEQ ID NO: 67 - protein, 223 aa, Artificial Sequence
  mutant receptor binding domain of SARS-CoV-2 Wuhan variant comprising substitution Y131E
RVQPTESIVRFPNITNLCPFGEVFNATRFASVYAWNRKRISNCVADYSVLYNSASFSTFKCYGVSPTKLNDLCFTNVYADSFVIRGDEVRQIAPGQTGKIADYNYKLPDDFTGCVIAWNSNNLDSKVGGNENYLYRLFRKSNLKPFERDISTEIYQAGSTPCNGVEGFNCYFPLQSYGFQPTNGVGYQPYRVVVLSFELLHAPATVCGPKKSTNLVKNKCVNF

SEQ ID NO: 68 - protein, 223 aa, Artificial Sequence
  mutant receptor binding domain of SARS-CoV-2 Wuhan variant comprising substitution Y131F
RVQPTESIVRFPNITNLCPFGEVFNATRFASVYAWNRKRISNCVADYSVLYNSASFSTFKCYGVSPTKLNDLCFTNVYADSFVIRGDEVRQIAPGQTGKIADYNYKLPDDFTGCVIAWNSNNLDSKVGGNFNYLYRLFRKSNLKPFERDISTEIYQAGSTPCNGVEGFNCYFPLQSYGFQPTNGVGYQPYRVVVLSFELLHAPATVCGPKKSTNLVKNKCVNF

SEQ ID NO: 69 - protein, 223 aa, Artificial Sequence
  mutant receptor binding domain of SARS-CoV-2 Wuhan variant comprising substitution Y131G
RVQPTESIVRFPNITNLCPFGEVFNATRFASVYAWNRKRISNCVADYSVLYNSASFSTFKCYGVSPTKLNDLCFTNVYADSFVIRGDEVRQIAPGQTGKIADYNYKLPDDFTGCVIAWNSNNLDSKVGGNGNYLYRLFRKSNLKPFERDISTEIYQAGSTPCNGVEGFNCYFPLQSYGFQPTNGVGYQPYRVVVLSFELLHAPATVCGPKKSTNLVKNKCVNF

SEQ ID NO: 70 - protein, 223 aa, Artificial Sequence
  mutant receptor binding domain of SARS-CoV-2 Wuhan variant comprising substitution Y131H
RVQPTESIVRFPNITNLCPFGEVFNATRFASVYAWNRKRISNCVADYSVLYNSASFSTFKCYGVSPTKLNDLCFTNVYADSFVIRGDEVRQIAPGQTGKIADYNYKLPDDFTGCVIAWNSNNLDSKVGGNHNYLYRLFRKSNLKPFERDISTEIYQAGSTPCNGVEGFNCYFPLQSYGFQPTNGVGYQPYRVVVLSFELLHAPATVCGPKKSTNLVKNKCVNF

SEQ ID NO: 71 - protein, 223 aa, Artificial Sequence
  mutant receptor binding domain of SARS-CoV-2 Wuhan variant comprising substitution Y131I
RVQPTESIVRFPNITNLCPFGEVFNATRFASVYAWNRKRISNCVADYSVLYNSASFSTFKCYGVSPTKLNDLCFTNVYADSFVIRGDEVRQIAPGQTGKIADYNYKLPDDFTGCVIAWNSNNLDSKVGGNINYLYRLFRKSNLKPFERDISTEIYQAGSTPCNGVEGFNCYFPLQSYGFQPTNGVGYQPYRVVVLSFELLHAPATVCGPKKSTNLVKNKCVNF

SEQ ID NO: 72 - protein, 223 aa, Artificial Sequence
  mutant receptor binding domain of SARS-CoV-2 Wuhan variant comprising substitution Y131L
RVQPTESIVRFPNITNLCPFGEVFNATRFASVYAWNRKRISNCVADYSVLYNSASFSTFKCYGVSPTKLNDLCFTNVYADSFVIRGDEVRQIAPGQTGKIADYNYKLPDDFTGCVIAWNSNNLDSKVGGNLNYLYRLFRKSNLKPFERDISTEIYQAGSTPCNGVEGFNCYFPLQSYGFQPTNGVGYQPYRVVVLSFELLHAPATVCGPKKSTNLVKNKCVNF

SEQ ID NO: 73 - protein, 223 aa, Artificial Sequence
  mutant receptor binding domain of SARS-CoV-2 Wuhan variant comprising substitution Y131M
RVQPTESIVRFPNITNLCPFGEVFNATRFASVYAWNRKRISNCVADYSVLYNSASFSTFKCYGVSPTKLNDLCFTNVYADSFVIRGDEVRQIAPGQTGKIADYNYKLPDDFTGCVIAWNSNNLDSKVGGNMNYLYRLFRKSNLKPFERDISTEIYQAGSTPCNGVEGFNCYFPLQSYGFQPTNGVGYQPYRVVVLSFELLHAPATVCGPKKSTNLVKNKCVNF

SEQ ID NO: 74 - protein, 223 aa, Artificial Sequence
  mutant receptor binding domain of SARS-CoV-2 Wuhan variant comprising substitution Y131N
RVQPTESIVRFPNITNLCPFGEVFNATRFASVYAWNRKRISNCVADYSVLYNSASFSTFKCYGVSPTKLNDLCFTNVYADSFVIRGDEVRQIAPGQTGKIADYNYKLPDDFTGCVIAWNSNNLDSKVGGNNNYLYRLFRKSNLKPFERDISTEIYQAGSTPCNGVEGFNCYFPLQSYGFQPTNGVGYQPYRVVVLSFELLHAPATVCGPKKSTNLVKNKCVNF

SEQ ID NO: 75 - protein, 223 aa, Artificial Sequence
  mutant receptor binding domain of SARS-CoV-2 Wuhan variant comprising substitution Y131P
RVQPTESIVRFPNITNLCPFGEVFNATRFASVYAWNRKRISNCVADYSVLYNSASFSTFKCYGVSPTKLNDLCFTNVYADSFVIRGDEVRQIAPGQTGKIADYNYKLPDDFTGCVIAWNSNNLDSKVGGNPNYLYRLFRKSNLKPFERDISTEIYQAGSTPCNGVEGFNCYFPLQSYGFQPTNGVGYQPYRVVVLSFELLHAPATVCGPKKSTNLVKNKCVNF

SEQ ID NO: 76 - protein, 223 aa, Artificial Sequence
  mutant receptor binding domain of SARS-CoV-2 Wuhan variant comprising substitution Y131Q
RVQPTESIVRFPNITNLCPFGEVFNATRFASVYAWNRKRISNCVADYSVLYNSASFSTFKCYGVSPTKLNDLCFTNVYADSFVIRGDEVRQIAPGQTGKIADYNYKLPDDFTGCVIAWNSNNLDSKVGGNQNYLYRLFRKSNLKPFERDISTEIYQAGSTPCNGVEGFNCYFPLQSYGFQPTNGVGYQPYRVVVLSFELLHAPATVCGPKKSTNLVKNKCVNF

SEQ ID NO: 77 - protein, 223 aa, Artificial Sequence
  mutant receptor binding domain of SARS-CoV-2 Wuhan variant comprising substitution Y131S
RVQPTESIVRFPNITNLCPFGEVFNATRFASVYAWNRKRISNCVADYSVLYNSASFSTFKCYGVSPTKLNDLCFTNVYADSFVIRGDEVRQIAPGQTGKIADYNYKLPDDFTGCVIAWNSNNLDSKVGGNSNYLYRLFRKSNLKPFERDISTEIYQAGSTPCNGVEGFNCYFPLQSYGFQPTNGVGYQPYRVVVLSFELLHAPATVCGPKKSTNLVKNKCVNF

SEQ ID NO: 78 - protein, 223 aa, Artificial Sequence
  mutant receptor binding domain of SARS-CoV-2 Wuhan variant comprising substitution Y131T
RVQPTESIVRFPNITNLCPFGEVFNATRFASVYAWNRKRISNCVADYSVLYNSASFSTFKCYGVSPTKLNDLCFTNVYADSFVIRGDEVRQIAPGQTGKIADYNYKLPDDFTGCVIAWNSNNLDSKVGGNTNYLYRLFRKSNLKPFERDISTEIYQAGSTPCNGVEGFNCYFPLQSYGFQPTNGVGYQPYRVVVLSFELLHAPATVCGPKKSTNLVKNKCVNF

SEQ ID NO: 79 - protein, 223 aa, Artificial Sequence
  mutant receptor binding domain of SARS-CoV-2 Wuhan variant comprising substitution Y131V
RVQPTESIVRFPNITNLCPFGEVFNATRFASVYAWNRKRISNCVADYSVLYNSASFSTFKCYGVSPTKLNDLCFTNVYADSFVIRGDEVRQIAPGQTGKIADYNYKLPDDFTGCVIAWNSNNLDSKVGGNVNYLYRLFRKSNLKPFERDISTEIYQAGSTPCNGVEGFNCYFPLQSYGFQPTNGVGYQPYRVVVLSFELLHAPATVCGPKKSTNLVKNKCVNF

SEQ ID NO: 80 - protein, 223 aa, Artificial Sequence
  mutant receptor binding domain of SARS-CoV-2 Wuhan variant comprising substitution Y131W
RVQPTESIVRFPNITNLCPFGEVFNATRFASVYAWNRKRISNCVADYSVLYNSASFSTFKCYGVSPTKLNDLCFTNVYADSFVIRGDEVRQIAPGQTGKIADYNYKLPDDFTGCVIAWNSNNLDSKVGGNWNYLYRLFRKSNLKPFERDISTEIYQAGSTPCNGVEGFNCYFPLQSYGFQPTNGVGYQPYRVVVLSFELLHAPATVCGPKKSTNLVKNKCVNF

SEQ ID NO: 81 - protein, 223 aa, Artificial Sequence
  mutant receptor binding domain of SARS-CoV-2 Wuhan variant comprising substitution Y171A
RVQPTESIVRFPNITNLCPFGEVFNATRFASVYAWNRKRISNCVADYSVLYNSASFSTFKCYGVSPTKLNDLCFTNVYADSFVIRGDEVRQIAPGQTGKIADYNYKLPDDFTGCVIAWNSNNLDSKVGGNYNYLYRLFRKSNLKPFERDISTEIYQAGSTPCNGVEGFNCAFPLQSYGFQPTNGVGYQPYRVVVLSFELLHAPATVCGPKKSTNLVKNKCVNF

SEQ ID NO: 82 - protein, 223 aa, Artificial Sequence
  mutant receptor binding domain of SARS-CoV-2 Wuhan variant comprising substitution Y171C
RVQPTESIVRFPNITNLCPFGEVFNATRFASVYAWNRKRISNCVADYSVLYNSASFSTFKCYGVSPTKLNDLCFTNVYADSFVIRGDEVRQIAPGQTGKIADYNYKLPDDFTGCVIAWNSNNLDSKVGGNYNYLYRLFRKSNLKPFERDISTEIYQAGSTPCNGVEGFNCCFPLQSYGFQPTNGVGYQPYRVVVLSFELLHAPATVCGPKKSTNLVKNKCVNF

SEQ ID NO: 83 - protein, 223 aa, Artificial Sequence
  mutant receptor binding domain of SARS-CoV-2 Wuhan variant comprising substitution Y171E
RVQPTESIVRFPNITNLCPFGEVFNATRFASVYAWNRKRISNCVADYSVLYNSASFSTFKCYGVSPTKLNDLCFTNVYADSFVIRGDEVRQIAPGQTGKIADYNYKLPDDFTGCVIAWNSNNLDSKVGGNYNYLYRLFRKSNLKPFERDISTEIYQAGSTPCNGVEGFNCEFPLQSYGFQPTNGVGYQPYRVVVLSFELLHAPATVCGPKKSTNLVKNKCVNF

SEQ ID NO: 84 - protein, 223 aa, Artificial Sequence
  mutant receptor binding domain of SARS-CoV-2 Wuhan variant comprising substitution Y171I
RVQPTESIVRFPNITNLCPFGEVFNATRFASVYAWNRKRISNCVADYSVLYNSASFSTFKCYGVSPTKLNDLCFTNVYADSFVIRGDEVRQIAPGQTGKIADYNYKLPDDFTGCVIAWNSNNLDSKVGGNYNYLYRLFRKSNLKPFERDISTEIYQAGSTPCNGVEGFNCIFPLQSYGFQPTNGVGYQPYRVVVLSFELLHAPATVCGPKKSTNLVKNKCVNF

SEQ ID NO: 85 - protein, 223 aa, Artificial Sequence
  mutant receptor binding domain of SARS-CoV-2 Wuhan variant comprising substitution Y171K
RVQPTESIVRFPNITNLCPFGEVFNATRFASVYAWNRKRISNCVADYSVLYNSASFSTFKCYGVSPTKLNDLCFTNVYADSFVIRGDEVRQIAPGQTGKIADYNYKLPDDFTGCVIAWNSNNLDSKVGGNYNYLYRLFRKSNLKPFERDISTEIYQAGSTPCNGVEGFNCKFPLQSYGFQPTNGVGYQPYRVVVLSFELLHAPATVCGPKKSTNLVKNKCVNF

SEQ ID NO: 86 - protein, 223 aa, Artificial Sequence
  mutant receptor binding domain of SARS-CoV-2 Wuhan variant comprising substitution Y171L
RVQPTESIVRFPNITNLCPFGEVFNATRFASVYAWNRKRISNCVADYSVLYNSASFSTFKCYGVSPTKLNDLCFTNVYADSFVIRGDEVRQIAPGQTGKIADYNYKLPDDFTGCVIAWNSNNLDSKVGGNYNYLYRLFRKSNLKPFERDISTEIYQAGSTPCNGVEGFNCLFPLQSYGFQPTNGVGYQPYRVVVLSFELLHAPATVCGPKKSTNLVKNKCVNF

SEQ ID NO: 87 - protein, 223 aa, Artificial Sequence
  mutant receptor binding domain of SARS-CoV-2 Wuhan variant comprising substitution Y171M
RVQPTESIVRFPNITNLCPFGEVFNATRFASVYAWNRKRISNCVADYSVLYNSASFSTFKCYGVSPTKLNDLCFTNVYADSFVIRGDEVRQIAPGQTGKIADYNYKLPDDFTGCVIAWNSNNLDSKVGGNYNYLYRLFRKSNLKPFERDISTEIYQAGSTPCNGVEGFNCMFPLQSYGFQPTNGVGYQPYRVVVLSFELLHAPATVCGPKKSTNLVKNKCVNF

SEQ ID NO: 88 - protein, 223 aa, Artificial Sequence
  mutant receptor binding domain of SARS-CoV-2 Wuhan variant comprising substitution Y171N
RVQPTESIVRFPNITNLCPFGEVFNATRFASVYAWNRKRISNCVADYSVLYNSASFSTFKCYGVSPTKLNDLCFTNVYADSFVIRGDEVRQIAPGQTGKIADYNYKLPDDFTGCVIAWNSNNLDSKVGGNYNYLYRLFRKSNLKPFERDISTEIYQAGSTPCNGVEGFNCNFPLQSYGFQPTNGVGYQPYRVVVLSFELLHAPATVCGPKKSTNLVKNKCVNF

SEQ ID NO: 89 - protein, 223 aa, Artificial Sequence
  mutant receptor binding domain of SARS-CoV-2 Wuhan variant comprising substitution Y171P
RVQPTESIVRFPNITNLCPFGEVFNATRFASVYAWNRKRISNCVADYSVLYNSASFSTFKCYGVSPTKLNDLCFTNVYADSFVIRGDEVRQIAPGQTGKIADYNYKLPDDFTGCVIAWNSNNLDSKVGGNYNYLYRLFRKSNLKPFERDISTEIYQAGSTPCNGVEGFNCPFPLQSYGFQPTNGVGYQPYRVVVLSFELLHAPATVCGPKKSTNLVKNKCVNF

SEQ ID NO: 90 - protein, 223 aa, Artificial Sequence
  mutant receptor binding domain of SARS-CoV-2 Wuhan variant comprising substitution Y171Q
RVQPTESIVRFPNITNLCPFGEVFNATRFASVYAWNRKRISNCVADYSVLYNSASFSTFKCYGVSPTKLNDLCFTNVYADSFVIRGDEVRQIAPGQTGKIADYNYKLPDDFTGCVIAWNSNNLDSKVGGNYNYLYRLFRKSNLKPFERDISTEIYQAGSTPCNGVEGFNCQFPLQSYGFQPTNGVGYQPYRVVVLSFELLHAPATVCGPKKSTNLVKNKCVNF

SEQ ID NO: 91 - protein, 223 aa, Artificial Sequence
  mutant receptor binding domain of SARS-CoV-2 Wuhan variant comprising substitution Y171R
RVQPTESIVRFPNITNLCPFGEVFNATRFASVYAWNRKRISNCVADYSVLYNSASFSTFKCYGVSPTKLNDLCFTNVYADSFVIRGDEVRQIAPGQTGKIADYNYKLPDDFTGCVIAWNSNNLDSKVGGNYNYLYRLFRKSNLKPFERDISTEIYQAGSTPCNGVEGFNCRFPLQSYGFQPTNGVGYQPYRVVVLSFELLHAPATVCGPKKSTNLVKNKCVNF

SEQ ID NO: 92 - protein, 223 aa, Artificial Sequence
  mutant receptor binding domain of SARS-CoV-2 Wuhan variant comprising substitution Y171S
RVQPTESIVRFPNITNLCPFGEVFNATRFASVYAWNRKRISNCVADYSVLYNSASFSTFKCYGVSPTKLNDLCFTNVYADSFVIRGDEVRQIAPGQTGKIADYNYKLPDDFTGCVIAWNSNNLDSKVGGNYNYLYRLFRKSNLKPFERDISTEIYQAGSTPCNGVEGFNCSFPLQSYGFQPTNGVGYQPYRVVVLSFELLHAPATVCGPKKSTNLVKNKCVNF

SEQ ID NO: 93 - protein, 223 aa, Artificial Sequence
  mutant receptor binding domain of SARS-CoV-2 Wuhan variant comprising substitution Y171T
RVQPTESIVRFPNITNLCPFGEVFNATRFASVYAWNRKRISNCVADYSVLYNSASFSTFKCYGVSPTKLNDLCFTNVYADSFVIRGDEVRQIAPGQTGKIADYNYKLPDDFTGCVIAWNSNNLDSKVGGNYNYLYRLFRKSNLKPFERDISTEIYQAGSTPCNGVEGFNCTFPLQSYGFQPTNGVGYQPYRVVVLSFELLHAPATVCGPKKSTNLVKNKCVNF

SEQ ID NO: 94 - protein, 223 aa, Artificial Sequence
  mutant receptor binding domain of SARS-CoV-2 Wuhan variant comprising substitution Y171V
RVQPTESIVRFPNITNLCPFGEVFNATRFASVYAWNRKRISNCVADYSVLYNSASFSTFKCYGVSPTKLNDLCFTNVYADSFVIRGDEVRQIAPGQTGKIADYNYKLPDDFTGCVIAWNSNNLDSKVGGNYNYLYRLFRKSNLKPFERDISTEIYQAGSTPCNGVEGFNCVFPLQSYGFQPTNGVGYQPYRVVVLSFELLHAPATVCGPKKSTNLVKNKCVNF

SEQ ID NO: 95 - protein, 223 aa, Artificial Sequence
  mutant receptor binding domain of SARS-CoV-2 Wuhan variant comprising substitution G178R
RVQPTESIVRFPNITNLCPFGEVFNATRFASVYAWNRKRISNCVADYSVLYNSASFSTFKCYGVSPTKLNDLCFTNVYADSFVIRGDEVRQIAPGQTGKIADYNYKLPDDFTGCVIAWNSNNLDSKVGGNYNYLYRLFRKSNLKPFERDISTEIYQAGSTPCNGVEGFNCYFPLQSYRFQPTNGVGYQPYRVVVLSFELLHAPATVCGPKKSTNLVKNKCVNF

SEQ ID NO: 96 - protein, 223 aa, Artificial Sequence
  mutant receptor binding domain of SARS-CoV-2 Wuhan variant comprising substitutions A157R and G184R
RVQPTESIVRFPNITNLCPFGEVFNATRFASVYAWNRKRISNCVADYSVLYNSASFSTFKCYGVSPTKLNDLCFTNVYADSFVIRGDEVRQIAPGQTGKIADYNYKLPDDFTGCVIAWNSNNLDSKVGGNYNYLYRLFRKSNLKPFERDISTEIYQRGSTPCNGVEGFNCYFPLQSYGFQPTNRVGYQPYRVVVLSFELLHAPATVCGPKKSTNLVKNKCVNF

SEQ ID NO: 97 - protein, 223 aa, Artificial Sequence
  mutant receptor binding domain of SARS-CoV-2 Wuhan variant comprising substitutions G178R and G184R
RVQPTESIVRFPNITNLCPFGEVFNATRFASVYAWNRKRISNCVADYSVLYNSASFSTFKCYGVSPTKLNDLCFTNVYADSFVIRGDEVRQIAPGQTGKIADYNYKLPDDFTGCVIAWNSNNLDSKVGGNYNYLYRLFRKSNLKPFERDISTEIYQAGSTPCNGVEGFNCYFPLQSYRFQPTNRVGYQPYRVVVLSFELLHAPATVCGPKKSTNLVKNKCVNF

SEQ ID NO: 98 - protein, 223 aa, Artificial Sequence
  mutant receptor binding domain of SARS-CoV-2 Wuhan variant comprising substitutions A157R, G178R and G184R
RVQPTESIVRFPNITNLCPFGEVFNATRFASVYAWNRKRISNCVADYSVLYNSASFSTFKCYGVSPTKLNDLCFTNVYADSFVIRGDEVRQIAPGQTGKIADYNYKLPDDFTGCVIAWNSNNLDSKVGGNYNYLYRLFRKSNLKPFERDISTEIYQRGSTPCNGVEGFNCYFPLQSYRFQPTNRVGYQPYRVVVLSFELLHAPATVCGPKKSTNLVKNKCVNF

SEQ ID NO: 99 - protein, 223 aa, Artificial Sequence
  mutant receptor binding domain of SARS-CoV-2 Wuhan variant comprising substitutions L137R, A157R and G178R
RVQPTESIVRFPNITNLCPFGEVFNATRFASVYAWNRKRISNCVADYSVLYNSASFSTFKCYGVSPTKLNDLCFTNVYADSFVIRGDEVRQIAPGQTGKIADYNYKLPDDFTGCVIAWNSNNLDSKVGGNYNYLYRRFRKSNLKPFERDISTEIYQRGSTPCNGVEGFNCYFPLQSYRFQPTNGVGYQPYRVVVLSFELLHAPATVCGPKKSTNLVKNKCVNF

SEQ ID NO: 100 - protein, 1273 aa, SARS-CoV-2, Wuhan variant
  wildtype spike protein of SARS-CoV-2 Wuhan variant
MFVFLVLLPLVSSQCVNLTTRTQLPPAYTNSFTRGVYYPDKVFRSSVLHSTQDLFLPFFSNVTWFHAIHVSGTNGTKRFDNPVLPFNDGVYFASTEKSNIIRGWIFGTTLDSKTQSLLIVNNATNVVIKVCEFQFCNDPFLGVYYHKNNKSWMESEFRVYSSANNCTFEYVSQPFLMDLEGKQGNFKNLREFVFKNIDGYFKIYSKHTPINLVRDLPQGFSALEPLVDLPIGINITRFQTLLALHRSYLTPGDSSSGWTAGAAAYYVGYLQPRTFLLKYNENGTITDAVDCALDPLSETKCTLKSFTVEKGIYQTSNFRVQPTESIVRFPNITNLCPFGEVFNATRFASVYAWNRKRISNCVADYSVLYNSASFSTFKCYGVSPTKLNDLCFTNVYADSFVIRGDEVRQIAPGQTGKIADYNYKLPDDFTGCVIAWNSNNLDSKVGGNYNYLYRLFRKSNLKPFERDISTEIYQAGSTPCNGVEGFNCYFPLQSYGFQPTNGVGYQPYRVVVLSFELLHAPATVCGPKKSTNLVKNKCVNFNFNGLTGTGVLTESNKKFLPFQQFGRDIADTTDAVRDPQTLEILDITPCSFGGVSVITPGTNTSNQVAVLYQDVNCTEVPVAIHADQLTPTWRVYSTGSNVFQTRAGCLIGAEHVNNSYECDIPIGAGICASYQTQTNSPRRARSVASQSIIAYTMSLGAENSVAYSNNSIAIPTNFTISVTTEILPVSMTKTSVDCTMYICGDSTECSNLLLQYGSFCTQLNRALTGIAVEQDKNTQEVFAQVKQIYKTPPIKDFGGFNFSQILPDPSKPSKRSFIEDLLFNKVTLADAGFIKQYGDCLGDIAARDLICAQKFNGLTVLPPLLTDEMIAQYTSALLAGTITSGWTFGAGAALQIPFAMQMAYRFNGIGVTQNVLYENQKLIANQFNSAIGKIQDSLSSTASALGKLQDVVNQNAQALNTLVKQLSSNFGAISSVLNDILSRLDKVEAEVQIDRLITGRLQSLQTYVTQQLIRAAEIRASANLAATKMSECVLGQSKRVDFCGKGYHLMSFPQSAPHGVVFLHVTYVPAQEKNFTTAPAICHDGKAHFPREGVFVSNGTHWFVTQRNFYEPQIITTDNTFVSGNCDVVIGIVNNTVYDPLQPELDSFKEELDKYFKNHTSPDVDLGDISGINASVVNIQKEIDRLNEVAKNLNESLIDLQELGKYEQYIKWPWYIWLGFIAGLIAIVMVTIMLCCMTSCCSCLKGCCSCGSCCKFDEDDSEPVLKGVKLHYT

SEQ ID NO: 101 - protein, 1273 aa, Artificial Sequence
  mutant spike protein of SARS-CoV-2 Wuhan variant comprising substitution G502E, 2-P-mutation (substitutions K986P and V987P) and inoperative furin cleavage site (substitution 682-QQAQ-685)
MFVFLVLLPLVSSQCVNLTTRTQLPPAYTNSFTRGVYYPDKVFRSSVLHSTQDLFLPFFSNVTWFHAIHVSGTNGTKRFDNPVLPFNDGVYFASTEKSNIIRGWIFGTTLDSKTQSLLIVNNATNVVIKVCEFQFCNDPFLGVYYHKNNKSWMESEFRVYSSANNCTFEYVSQPFLMDLEGKQGNFKNLREFVFKNIDGYFKIYSKHTPINLVRDLPQGFSALEPLVDLPIGINITRFQTLLALHRSYLTPGDSSSGWTAGAAAYYVGYLQPRTFLLKYNENGTITDAVDCALDPLSETKCTLKSFTVEKGIYQTSNFRVQPTESIVRFPNITNLCPFGEVFNATRFASVYAWNRKRISNCVADYSVLYNSASFSTFKCYGVSPTKLNDLCFTNVYADSFVIRGDEVRQIAPGQTGKIADYNYKLPDDFTGCVIAWNSNNLDSKVGGNYNYLYRLFRKSNLKPFERDISTEIYQAGSTPCNGVEGFNCYFPLQSYGFQPTNEVGYQPYRVVVLSFELLHAPATVCGPKKSTNLVKNKCVNFNFNGLTGTGVLTESNKKFLPFQQFGRDIADTTDAVRDPQTLEILDITPCSFGGVSVITPGTNTSNQVAVLYQDVNCTEVPVAIHADQLTPTWRVYSTGSNVFQTRAGCLIGAEHVNNSYECDIPIGAGICASYQTQTNSPQQAQSVASQSIIAYTMSLGAENSVAYSNNSIAIPTNFTISVTTEILPVSMTKTSVDCTMYICGDSTECSNLLLQYGSFCTQLNRALTGIAVEQDKNTQEVFAQVKQIYKTPPIKDFGGFNFSQILPDPSKPSKRSFIEDLLFNKVTLADAGFIKQYGDCLGDIAARDLICAQKFNGLTVLPPLLTDEMIAQYTSALLAGTITSGWTFGAGAALQIPFAMQMAYRFNGIGVTQNVLYENQKLIANQFNSAIGKIQDSLSSTASALGKLQDVVNQNAQALNTLVKQLSSNFGAISSVLNDILSRLDPPEAEVQIDRLITGRLQSLQTYVTQQLIRAAEIRASANLAATKMSECVLGQSKRVDFCGKGYHLMSFPQSAPHGVVFLHVTYVPAQEKNFTTAPAICHDGKAHFPREGVFVSNGTHWFVTQRNFYEPQIITTDNTFVSGNCDVVIGIVNNTVYDPLQPELDSFKEELDKYFKNHTSPDVDLGDISGINASVVNIQKEIDRLNEVAKNLNESLIDLQELGKYEQYIKWPWYIWLGFIAGLIAIVMVTIMLCCMTSCCSCLKGCCSCGSCCKFDEDDSEPVLKGVKLHYT

SEQ ID NO: 102 - protein, 1273 aa, Artificial Sequence
  mutant spike protein of SARS-CoV-2 Wuhan variant comprising substitution G502A, 2-P-mutation (substitutions K986P and V987P) and inoperative furin cleavage site (substitution 682-QQAQ-685)
MFVFLVLLPLVSSQCVNLTTRTQLPPAYTNSFTRGVYYPDKVFRSSVLHSTQDLFLPFFSNVTWFHAIHVSGTNGTKRFDNPVLPFNDGVYFASTEKSNIIRGWIFGTTLDSKTQSLLIVNNATNVVIKVCEFQFCNDPFLGVYYHKNNKSWMESEFRVYSSANNCTFEYVSQPFLMDLEGKQGNFKNLREFVFKNIDGYFKIYSKHTPINLVRDLPQGFSALEPLVDLPIGINITRFQTLLALHRSYLTPGDSSSGWTAGAAAYYVGYLQPRTFLLKYNENGTITDAVDCALDPLSETKCTLKSFTVEKGIYQTSNFRVQPTESIVRFPNITNLCPFGEVFNATRFASVYAWNRKRISNCVADYSVLYNSASFSTFKCYGVSPTKLNDLCFTNVYADSFVIRGDEVRQIAPGQTGKIADYNYKLPDDFTGCVIAWNSNNLDSKVGGNYNYLYRLFRKSNLKPFERDISTEIYQAGSTPCNGVEGFNCYFPLQSYGFQPTNAVGYQPYRVVVLSFELLHAPATVCGPKKSTNLVKNKCVNFNFNGLTGTGVLTESNKKFLPFQQFGRDIADTTDAVRDPQTLEILDITPCSFGGVSVITPGTNTSNQVAVLYQDVNCTEVPVAIHADQLTPTWRVYSTGSNVFQTRAGCLIGAEHVNNSYECDIPIGAGICASYQTQTNSPQQAQSVASQSIIAYTMSLGAENSVAYSNNSIAIPTNFTISVTTEILPVSMTKTSVDCTMYICGDSTECSNLLLQYGSFCTQLNRALTGIAVEQDKNTQEVFAQVKQIYKTPPIKDFGGFNFSQILPDPSKPSKRSFIEDLLFNKVTLADAGFIKQYGDCLGDIAARDLICAQKFNGLTVLPPLLTDEMIAQYTSALLAGTITSGWTFGAGAALQIPFAMQMAYRFNGIGVTQNVLYENQKLIANQFNSAIGKIQDSLSSTASALGKLQDVVNQNAQALNTLVKQLSSNFGAISSVLNDILSRLDPPEAEVQIDRLITGRLQSLQTYVTQQLIRAAEIRASANLAATKMSECVLGQSKRVDFCGKGYHLMSFPQSAPHGVVFLHVTYVPAQEKNFTTAPAICHDGKAHFPREGVFVSNGTHWFVTQRNFYEPQIITTDNTFVSGNCDVVIGIVNNTVYDPLQPELDSFKEELDKYFKNHTSPDVDLGDISGINASVVNIQKEIDRLNEVAKNLNESLIDLQELGKYEQYIKWPWYIWLGFIAGLIAIVMVTIMLCCMTSCCSCLKGCCSCGSCCKFDEDDSEPVLKGVKLHYT

SEQ ID NO: 103 - protein, 1273 aa, Artificial Sequence
  mutant spike protein of SARS-CoV-2 Wuhan variant comprising substitution G502C, 2-P-mutation (substitutions K986P and V987P) and inoperative furin cleavage site (substitution 682-QQAQ-685)
MFVFLVLLPLVSSQCVNLTTRTQLPPAYTNSFTRGVYYPDKVFRSSVLHSTQDLFLPFFSNVTWFHAIHVSGTNGTKRFDNPVLPFNDGVYFASTEKSNIIRGWIFGTTLDSKTQSLLIVNNATNVVIKVCEFQFCNDPFLGVYYHKNNKSWMESEFRVYSSANNCTFEYVSQPFLMDLEGKQGNFKNLREFVFKNIDGYFKIYSKHTPINLVRDLPQGFSALEPLVDLPIGINITRFQTLLALHRSYLTPGDSSSGWTAGAAAYYVGYLQPRTFLLKYNENGTITDAVDCALDPLSETKCTLKSFTVEKGIYQTSNFRVQPTESIVRFPNITNLCPFGEVFNATRFASVYAWNRKRISNCVADYSVLYNSASFSTFKCYGVSPTKLNDLCFTNVYADSFVIRGDEVRQIAPGQTGKIADYNYKLPDDFTGCVIAWNSNNLDSKVGGNYNYLYRLFRKSNLKPFERDISTEIYQAGSTPCNGVEGFNCYFPLQSYGFQPTNCVGYQPYRVVVLSFELLHAPATVCGPKKSTNLVKNKCVNFNFNGLTGTGVLTESNKKFLPFQQFGRDIADTTDAVRDPQTLEILDITPCSFGGVSVITPGTNTSNQVAVLYQDVNCTEVPVAIHADQLTPTWRVYSTGSNVFQTRAGCLIGAEHVNNSYECDIPIGAGICASYQTQTNSPQQAQSVASQSIIAYTMSLGAENSVAYSNNSIAIPTNFTISVTTEILPVSMTKTSVDCTMYICGDSTECSNLLLQYGSFCTQLNRALTGIAVEQDKNTQEVFAQVKQIYKTPPIKDFGGFNFSQILPDPSKPSKRSFIEDLLFNKVTLADAGFIKQYGDCLGDIAARDLICAQKFNGLTVLPPLLTDEMIAQYTSALLAGTITSGWTFGAGAALQIPFAMQMAYRFNGIGVTQNVLYENQKLIANQFNSAIGKIQDSLSSTASALGKLQDVVNQNAQALNTLVKQLSSNFGAISSVLNDILSRLDPPEAEVQIDRLITGRLQSLQTYVTQQLIRAAEIRASANLAATKMSECVLGQSKRVDFCGKGYHLMSFPQSAPHGVVFLHVTYVPAQEKNFTTAPAICHDGKAHFPREGVFVSNGTHWFVTQRNFYEPQIITTDNTFVSGNCDVVIGIVNNTVYDPLQPELDSFKEELDKYFKNHTSPDVDLGDISGINASVVNIQKEIDRLNEVAKNLNESLIDLQELGKYEQYIKWPWYIWLGFIAGLIAIVMVTIMLCCMTSCCSCLKGCCSCGSCCKFDEDDSEPVLKGVKLHYT

SEQ ID NO: 104 - protein, 1273 aa, Artificial Sequence
  mutant spike protein of SARS-CoV-2 Wuhan variant comprising substitution G502D, 2-P-mutation (substiutions K986P and V987P) and inoperative furin cleavage site (substitution 682-QQAQ-685)
MFVFLVLLPLVSSQCVNLTTRTQLPPAYTNSFTRGVYYPDKVFRSSVLHSTQDLFLPFFSNVTWFHAIHVSGTNGTKRFDNPVLPFNDGVYFASTEKSNIIRGWIFGTTLDSKTQSLLIVNNATNVVIKVCEFQFCNDPFLGVYYHKNNKSWMESEFRVYSSANNCTFEYVSQPFLMDLEGKQGNFKNLREFVFKNIDGYFKIYSKHTPINLVRDLPQGFSALEPLVDLPIGINITRFQTLLALHRSYLTPGDSSSGWTAGAAAYYVGYLQPRTFLLKYNENGTITDAVDCALDPLSETKCTLKSFTVEKGIYQTSNFRVQPTESIVRFPNITNLCPFGEVFNATRFASVYAWNRKRISNCVADYSVLYNSASFSTFKCYGVSPTKLNDLCFTNVYADSFVIRGDEVRQIAPGQTGKIADYNYKLPDDFTGCVIAWNSNNLDSKVGGNYNYLYRLFRKSNLKPFERDISTEIYQAGSTPCNGVEGFNCYFPLQSYGFQPTNDVGYQPYRVVVLSFELLHAPATVCGPKKSTNLVKNKCVNFNFNGLTGTGVLTESNKKFLPFQQFGRDIADTTDAVRDPQTLEILDITPCSFGGVSVITPGTNTSNQVAVLYQDVNCTEVPVAIHADQLTPTWRVYSTGSNVFQTRAGCLIGAEHVNNSYECDIPIGAGICASYQTQTNSPQQAQSVASQSIIAYTMSLGAENSVAYSNNSIAIPTNFTISVTTEILPVSMTKTSVDCTMYICGDSTECSNLLLQYGSFCTQLNRALTGIAVEQDKNTQEVFAQVKQIYKTPPIKDFGGFNFSQILPDPSKPSKRSFIEDLLFNKVTLADAGFIKQYGDCLGDIAARDLICAQKFNGLTVLPPLLTDEMIAQYTSALLAGTITSGWTFGAGAALQIPFAMQMAYRFNGIGVTQNVLYENQKLIANQFNSAIGKIQDSLSSTASALGKLQDVVNQNAQALNTLVKQLSSNFGAISSVLNDILSRLDPPEAEVQIDRLITGRLQSLQTYVTQQLIRAAEIRASANLAATKMSECVLGQSKRVDFCGKGYHLMSFPQSAPHGVVFLHVTYVPAQEKNFTTAPAICHDGKAHFPREGVFVSNGTHWFVTQRNFYEPQIITTDNTFVSGNCDVVIGIVNNTVYDPLQPELDSFKEELDKYFKNHTSPDVDLGDISGINASVVNIQKEIDRLNEVAKNLNESLIDLQELGKYEQYIKWPWYIWLGFIAGLIAIVMVTIMLCCMTSCCSCLKGCCSCGSCCKFDEDDSEPVLKGVKLHYT

SEQ ID NO: 105 - protein, 1273 aa, Artificial Sequence
  mutant spike protein of SARS-CoV-2 Wuhan variant comprising substitution G502F, 2-P-mutation (substiutions K986P and V987P) and inoperative furin cleavage site (substitution 682-QQAQ-685)
MFVFLVLLPLVSSQCVNLTTRTQLPPAYTNSFTRGVYYPDKVFRSSVLHSTQDLFLPFFSNVTWFHAIHVSGTNGTKRFDNPVLPFNDGVYFASTEKSNIIRGWIFGTTLDSKTQSLLIVNNATNVVIKVCEFQFCNDPFLGVYYHKNNKSWMESEFRVYSSANNCTFEYVSQPFLMDLEGKQGNFKNLREFVFKNIDGYFKIYSKHTPINLVRDLPQGFSALEPLVDLPIGINITRFQTLLALHRSYLTPGDSSSGWTAGAAAYYVGYLQPRTFLLKYNENGTITDAVDCALDPLSETKCTLKSFTVEKGIYQTSNFRVQPTESIVRFPNITNLCPFGEVFNATRFASVYAWNRKRISNCVADYSVLYNSASFSTFKCYGVSPTKLNDLCFTNVYADSFVIRGDEVRQIAPGQTGKIADYNYKLPDDFTGCVIAWNSNNLDSKVGGNYNYLYRLFRKSNLKPFERDISTEIYQAGSTPCNGVEGFNCYFPLQSYGFQPTNFVGYQPYRVVVLSFELLHAPATVCGPKKSTNLVKNKCVNFNFNGLTGTGVLTESNKKFLPFQQFGRDIADTTDAVRDPQTLEILDITPCSFGGVSVITPGTNTSNQVAVLYQDVNCTEVPVAIHADQLTPTWRVYSTGSNVFQTRAGCLIGAEHVNNSYECDIPIGAGICASYQTQTNSPQQAQSVASQSIIAYTMSLGAENSVAYSNNSIAIPTNFTISVTTEILPVSMTKTSVDCTMYICGDSTECSNLLLQYGSFCTQLNRALTGIAVEQDKNTQEVFAQVKQIYKTPPIKDFGGFNFSQILPDPSKPSKRSFIEDLLFNKVTLADAGFIKQYGDCLGDIAARDLICAQKFNGLTVLPPLLTDEMIAQYTSALLAGTITSGWTFGAGAALQIPFAMQMAYRFNGIGVTQNVLYENQKLIANQFNSAIGKIQDSLSSTASALGKLQDVVNQNAQALNTLVKQLSSNFGAISSVLNDILSRLDPPEAEVQIDRLITGRLQSLQTYVTQQLIRAAEIRASANLAATKMSECVLGQSKRVDFCGKGYHLMSFPQSAPHGVVFLHVTYVPAQEKNFTTAPAICHDGKAHFPREGVFVSNGTHWFVTQRNFYEPQIITTDNTFVSGNCDVVIGIVNNTVYDPLQPELDSFKEELDKYFKNHTSPDVDLGDISGINASVVNIQKEIDRLNEVAKNLNESLIDLQELGKYEQYIKWPWYIWLGFIAGLIAIVMVTIMLCCMTSCCSCLKGCCSCGSCCKFDEDDSEPVLKGVKLHYT

SEQ ID NO: 106 - protein, 1273 aa, Artificial Sequence
  mutant spike protein of SARS-CoV-2 Wuhan variant comprising substitution G502H, 2-P-mutation (substiutions K986P and V987P) and inoperative furin cleavage site (substitution 682-QQAQ-685)
MFVFLVLLPLVSSQCVNLTTRTQLPPAYTNSFTRGVYYPDKVFRSSVLHSTQDLFLPFFSNVTWFHAIHVSGTNGTKRFDNPVLPFNDGVYFASTEKSNIIRGWIFGTTLDSKTQSLLIVNNATNVVIKVCEFQFCNDPFLGVYYHKNNKSWMESEFRVYSSANNCTFEYVSQPFLMDLEGKQGNFKNLREFVFKNIDGYFKIYSKHTPINLVRDLPQGFSALEPLVDLPIGINITRFQTLLALHRSYLTPGDSSSGWTAGAAAYYVGYLQPRTFLLKYNENGTITDAVDCALDPLSETKCTLKSFTVEKGIYQTSNFRVQPTESIVRFPNITNLCPFGEVFNATRFASVYAWNRKRISNCVADYSVLYNSASFSTFKCYGVSPTKLNDLCFTNVYADSFVIRGDEVRQIAPGQTGKIADYNYKLPDDFTGCVIAWNSNNLDSKVGGNYNYLYRLFRKSNLKPFERDISTEIYQAGSTPCNGVEGFNCYFPLQSYGFQPTNHVGYQPYRVVVLSFELLHAPATVCGPKKSTNLVKNKCVNFNFNGLTGTGVLTESNKKFLPFQQFGRDIADTTDAVRDPQTLEILDITPCSFGGVSVITPGTNTSNQVAVLYQDVNCTEVPVAIHADQLTPTWRVYSTGSNVFQTRAGCLIGAEHVNNSYECDIPIGAGICASYQTQTNSPQQAQSVASQSIIAYTMSLGAENSVAYSNNSIAIPTNFTISVTTEILPVSMTKTSVDCTMYICGDSTECSNLLLQYGSFCTQLNRALTGIAVEQDKNTQEVFAQVKQIYKTPPIKDFGGFNFSQILPDPSKPSKRSFIEDLLFNKVTLADAGFIKQYGDCLGDIAARDLICAQKFNGLTVLPPLLTDEMIAQYTSALLAGTITSGWTFGAGAALQIPFAMQMAYRFNGIGVTQNVLYENQKLIANQFNSAIGKIQDSLSSTASALGKLQDVVNQNAQALNTLVKQLSSNFGAISSVLNDILSRLDPPEAEVQIDRLITGRLQSLQTYVTQQLIRAAEIRASANLAATKMSECVLGQSKRVDFCGKGYHLMSFPQSAPHGVVFLHVTYVPAQEKNFTTAPAICHDGKAHFPREGVFVSNGTHWFVTQRNFYEPQIITTDNTFVSGNCDVVIGIVNNTVYDPLQPELDSFKEELDKYFKNHTSPDVDLGDISGINASVVNIQKEIDRLNEVAKNLNESLIDLQELGKYEQYIKWPWYIWLGFIAGLIAIVMVTIMLCCMTSCCSCLKGCCSCGSCCKFDEDDSEPVLKGVKLHYT

SEQ ID NO: 107 - protein, 1273 aa, Artificial Sequence
  mutant spike protein of SARS-CoV-2 Wuhan variant comprising substitution G502I, 2-P-mutation (substiutions K986P and V987P) and inoperative furin cleavage site (substitution 682-QQAQ-685)
MFVFLVLLPLVSSQCVNLTTRTQLPPAYTNSFTRGVYYPDKVFRSSVLHSTQDLFLPFFSNVTWFHAIHVSGTNGTKRFDNPVLPFNDGVYFASTEKSNIIRGWIFGTTLDSKTQSLLIVNNATNVVIKVCEFQFCNDPFLGVYYHKNNKSWMESEFRVYSSANNCTFEYVSQPFLMDLEGKQGNFKNLREFVFKNIDGYFKIYSKHTPINLVRDLPQGFSALEPLVDLPIGINITRFQTLLALHRSYLTPGDSSSGWTAGAAAYYVGYLQPRTFLLKYNENGTITDAVDCALDPLSETKCTLKSFTVEKGIYQTSNFRVQPTESIVRFPNITNLCPFGEVFNATRFASVYAWNRKRISNCVADYSVLYNSASFSTFKCYGVSPTKLNDLCFTNVYADSFVIRGDEVRQIAPGQTGKIADYNYKLPDDFTGCVIAWNSNNLDSKVGGNYNYLYRLFRKSNLKPFERDISTEIYQAGSTPCNGVEGFNCYFPLQSYGFQPTNIVGYQPYRVVVLSFELLHAPATVCGPKKSTNLVKNKCVNFNFNGLTGTGVLTESNKKFLPFQQFGRDIADTTDAVRDPQTLEILDITPCSFGGVSVITPGTNTSNQVAVLYQDVNCTEVPVAIHADQLTPTWRVYSTGSNVFQTRAGCLIGAEHVNNSYECDIPIGAGICASYQTQTNSPQQAQSVASQSIIAYTMSLGAENSVAYSNNSIAIPTNFTISVTTEILPVSMTKTSVDCTMYICGDSTECSNLLLQYGSFCTQLNRALTGIAVEQDKNTQEVFAQVKQIYKTPPIKDFGGFNFSQILPDPSKPSKRSFIEDLLFNKVTLADAGFIKQYGDCLGDIAARDLICAQKFNGLTVLPPLLTDEMIAQYTSALLAGTITSGWTFGAGAALQIPFAMQMAYRFNGIGVTQNVLYENQKLIANQFNSAIGKIQDSLSSTASALGKLQDVVNQNAQALNTLVKQLSSNFGAISSVLNDILSRLDPPEAEVQIDRLITGRLQSLQTYVTQQLIRAAEIRASANLAATKMSECVLGQSKRVDFCGKGYHLMSFPQSAPHGVVFLHVTYVPAQEKNFTTAPAICHDGKAHFPREGVFVSNGTHWFVTQRNFYEPQIITTDNTFVSGNCDVVIGIVNNTVYDPLQPELDSFKEELDKYFKNHTSPDVDLGDISGINASVVNIQKEIDRLNEVAKNLNESLIDLQELGKYEQYIKWPWYIWLGFIAGLIAIVMVTIMLCCMTSCCSCLKGCCSCGSCCKFDEDDSEPVLKGVKLHYT

SEQ ID NO: 108 - protein, 1273 aa, Artificial Sequence
  mutant spike protein of SARS-CoV-2 Wuhan variant comprising substitution G502K, 2-P-mutation (substiutions K986P and V987P) and inoperative furin cleavage site (substitution 682-QQAQ-685)
MFVFLVLLPLVSSQCVNLTTRTQLPPAYTNSFTRGVYYPDKVFRSSVLHSTQDLFLPFFSNVTWFHAIHVSGTNGTKRFDNPVLPFNDGVYFASTEKSNIIRGWIFGTTLDSKTQSLLIVNNATNVVIKVCEFQFCNDPFLGVYYHKNNKSWMESEFRVYSSANNCTFEYVSQPFLMDLEGKQGNFKNLREFVFKNIDGYFKIYSKHTPINLVRDLPQGFSALEPLVDLPIGINITRFQTLLALHRSYLTPGDSSSGWTAGAAAYYVGYLQPRTFLLKYNENGTITDAVDCALDPLSETKCTLKSFTVEKGIYQTSNFRVQPTESIVRFPNITNLCPFGEVFNATRFASVYAWNRKRISNCVADYSVLYNSASFSTFKCYGVSPTKLNDLCFTNVYADSFVIRGDEVRQIAPGQTGKIADYNYKLPDDFTGCVIAWNSNNLDSKVGGNYNYLYRLFRKSNLKPFERDISTEIYQAGSTPCNGVEGFNCYFPLQSYGFQPTNKVGYQPYRVVVLSFELLHAPATVCGPKKSTNLVKNKCVNFNFNGLTGTGVLTESNKKFLPFQQFGRDIADTTDAVRDPQTLEILDITPCSFGGVSVITPGTNTSNQVAVLYQDVNCTEVPVAIHADQLTPTWRVYSTGSNVFQTRAGCLIGAEHVNNSYECDIPIGAGICASYQTQTNSPQQAQSVASQSIIAYTMSLGAENSVAYSNNSIAIPTNFTISVTTEILPVSMTKTSVDCTMYICGDSTECSNLLLQYGSFCTQLNRALTGIAVEQDKNTQEVFAQVKQIYKTPPIKDFGGFNFSQILPDPSKPSKRSFIEDLLFNKVTLADAGFIKQYGDCLGDIAARDLICAQKFNGLTVLPPLLTDEMIAQYTSALLAGTITSGWTFGAGAALQIPFAMQMAYRFNGIGVTQNVLYENQKLIANQFNSAIGKIQDSLSSTASALGKLQDVVNQNAQALNTLVKQLSSNFGAISSVLNDILSRLDPPEAEVQIDRLITGRLQSLQTYVTQQLIRAAEIRASANLAATKMSECVLGQSKRVDFCGKGYHLMSFPQSAPHGVVFLHVTYVPAQEKNFTTAPAICHDGKAHFPREGVFVSNGTHWFVTQRNFYEPQIITTDNTFVSGNCDVVIGIVNNTVYDPLQPELDSFKEELDKYFKNHTSPDVDLGDISGINASVVNIQKEIDRLNEVAKNLNESLIDLQELGKYEQYIKWPWYIWLGFIAGLIAIVMVTIMLCCMTSCCSCLKGCCSCGSCCKFDEDDSEPVLKGVKLHYT

SEQ ID NO: 109 - protein, 1273 aa, Artificial Sequence
  mutant spike protein of SARS-CoV-2 Wuhan variant comprising substitution G502L, 2-P-mutation (substiutions K986P and V987P) and inoperative furin cleavage site (substitution 682-QQAQ-685)
MFVFLVLLPLVSSQCVNLTTRTQLPPAYTNSFTRGVYYPDKVFRSSVLHSTQDLFLPFFSNVTWFHAIHVSGTNGTKRFDNPVLPFNDGVYFASTEKSNIIRGWIFGTTLDSKTQSLLIVNNATNVVIKVCEFQFCNDPFLGVYYHKNNKSWMESEFRVYSSANNCTFEYVSQPFLMDLEGKQGNFKNLREFVFKNIDGYFKIYSKHTPINLVRDLPQGFSALEPLVDLPIGINITRFQTLLALHRSYLTPGDSSSGWTAGAAAYYVGYLQPRTFLLKYNENGTITDAVDCALDPLSETKCTLKSFTVEKGIYQTSNFRVQPTESIVRFPNITNLCPFGEVFNATRFASVYAWNRKRISNCVADYSVLYNSASFSTFKCYGVSPTKLNDLCFTNVYADSFVIRGDEVRQIAPGQTGKIADYNYKLPDDFTGCVIAWNSNNLDSKVGGNYNYLYRLFRKSNLKPFERDISTEIYQAGSTPCNGVEGFNCYFPLQSYGFQPTNLVGYQPYRVVVLSFELLHAPATVCGPKKSTNLVKNKCVNFNFNGLTGTGVLTESNKKFLPFQQFGRDIADTTDAVRDPQTLEILDITPCSFGGVSVITPGTNTSNQVAVLYQDVNCTEVPVAIHADQLTPTWRVYSTGSNVFQTRAGCLIGAEHVNNSYECDIPIGAGICASYQTQTNSPQQAQSVASQSIIAYTMSLGAENSVAYSNNSIAIPTNFTISVTTEILPVSMTKTSVDCTMYICGDSTECSNLLLQYGSFCTQLNRALTGIAVEQDKNTQEVFAQVKQIYKTPPIKDFGGFNFSQILPDPSKPSKRSFIEDLLFNKVTLADAGFIKQYGDCLGDIAARDLICAQKFNGLTVLPPLLTDEMIAQYTSALLAGTITSGWTFGAGAALQIPFAMQMAYRFNGIGVTQNVLYENQKLIANQFNSAIGKIQDSLSSTASALGKLQDVVNQNAQALNTLVKQLSSNFGAISSVLNDILSRLDPPEAEVQIDRLITGRLQSLQTYVTQQLIRAAEIRASANLAATKMSECVLGQSKRVDFCGKGYHLMSFPQSAPHGVVFLHVTYVPAQEKNFTTAPAICHDGKAHFPREGVFVSNGTHWFVTQRNFYEPQIITTDNTFVSGNCDVVIGIVNNTVYDPLQPELDSFKEELDKYFKNHTSPDVDLGDISGINASVVNIQKEIDRLNEVAKNLNESLIDLQELGKYEQYIKWPWYIWLGFIAGLIAIVMVTIMLCCMTSCCSCLKGCCSCGSCCKFDEDDSEPVLKGVKLHYT

SEQ ID NO: 110 - protein, 1273 aa, Artificial Sequence
  mutant spike protein of SARS-CoV-2 Wuhan variant comprising substitution G502M, 2-P-mutation (substiutions K986P and V987P) and inoperative furin cleavage site (substitution 682-QQAQ-685)
MFVFLVLLPLVSSQCVNLTTRTQLPPAYTNSFTRGVYYPDKVFRSSVLHSTQDLFLPFFSNVTWFHAIHVSGTNGTKRFDNPVLPFNDGVYFASTEKSNIIRGWIFGTTLDSKTQSLLIVNNATNVVIKVCEFQFCNDPFLGVYYHKNNKSWMESEFRVYSSANNCTFEYVSQPFLMDLEGKQGNFKNLREFVFKNIDGYFKIYSKHTPINLVRDLPQGFSALEPLVDLPIGINITRFQTLLALHRSYLTPGDSSSGWTAGAAAYYVGYLQPRTFLLKYNENGTITDAVDCALDPLSETKCTLKSFTVEKGIYQTSNFRVQPTESIVRFPNITNLCPFGEVFNATRFASVYAWNRKRISNCVADYSVLYNSASFSTFKCYGVSPTKLNDLCFTNVYADSFVIRGDEVRQIAPGQTGKIADYNYKLPDDFTGCVIAWNSNNLDSKVGGNYNYLYRLFRKSNLKPFERDISTEIYQAGSTPCNGVEGFNCYFPLQSYGFQPTNMVGYQPYRVVVLSFELLHAPATVCGPKKSTNLVKNKCVNFNFNGLTGTGVLTESNKKFLPFQQFGRDIADTTDAVRDPQTLEILDITPCSFGGVSVITPGTNTSNQVAVLYQDVNCTEVPVAIHADQLTPTWRVYSTGSNVFQTRAGCLIGAEHVNNSYECDIPIGAGICASYQTQTNSPQQAQSVASQSIIAYTMSLGAENSVAYSNNSIAIPTNFTISVTTEILPVSMTKTSVDCTMYICGDSTECSNLLLQYGSFCTQLNRALTGIAVEQDKNTQEVFAQVKQIYKTPPIKDFGGFNFSQILPDPSKPSKRSFIEDLLFNKVTLADAGFIKQYGDCLGDIAARDLICAQKFNGLTVLPPLLTDEMIAQYTSALLAGTITSGWTFGAGAALQIPFAMQMAYRFNGIGVTQNVLYENQKLIANQFNSAIGKIQDSLSSTASALGKLQDVVNQNAQALNTLVKQLSSNFGAISSVLNDILSRLDPPEAEVQIDRLITGRLQSLQTYVTQQLIRAAEIRASANLAATKMSECVLGQSKRVDFCGKGYHLMSFPQSAPHGVVFLHVTYVPAQEKNFTTAPAICHDGKAHFPREGVFVSNGTHWFVTQRNFYEPQIITTDNTFVSGNCDVVIGIVNNTVYDPLQPELDSFKEELDKYFKNHTSPDVDLGDISGINASVVNIQKEIDRLNEVAKNLNESLIDLQELGKYEQYIKWPWYIWLGFIAGLIAIVMVTIMLCCMTSCCSCLKGCCSCGSCCKFDEDDSEPVLKGVKLHYT

SEQ ID NO: 111 - protein, 1273 aa, Artificial Sequence
  mutant spike protein of SARS-CoV-2 Wuhan variant comprising substitution G502N, 2-P-mutation (substiutions K986P and V987P) and inoperative furin cleavage site (substitution 682-QQAQ-685)
MFVFLVLLPLVSSQCVNLTTRTQLPPAYTNSFTRGVYYPDKVFRSSVLHSTQDLFLPFFSNVTWFHAIHVSGTNGTKRFDNPVLPFNDGVYFASTEKSNIIRGWIFGTTLDSKTQSLLIVNNATNVVIKVCEFQFCNDPFLGVYYHKNNKSWMESEFRVYSSANNCTFEYVSQPFLMDLEGKQGNFKNLREFVFKNIDGYFKIYSKHTPINLVRDLPQGFSALEPLVDLPIGINITRFQTLLALHRSYLTPGDSSSGWTAGAAAYYVGYLQPRTFLLKYNENGTITDAVDCALDPLSETKCTLKSFTVEKGIYQTSNFRVQPTESIVRFPNITNLCPFGEVFNATRFASVYAWNRKRISNCVADYSVLYNSASFSTFKCYGVSPTKLNDLCFTNVYADSFVIRGDEVRQIAPGQTGKIADYNYKLPDDFTGCVIAWNSNNLDSKVGGNYNYLYRLFRKSNLKPFERDISTEIYQAGSTPCNGVEGFNCYFPLQSYGFQPTNNVGYQPYRVVVLSFELLHAPATVCGPKKSTNLVKNKCVNFNFNGLTGTGVLTESNKKFLPFQQFGRDIADTTDAVRDPQTLEILDITPCSFGGVSVITPGTNTSNQVAVLYQDVNCTEVPVAIHADQLTPTWRVYSTGSNVFQTRAGCLIGAEHVNNSYECDIPIGAGICASYQTQTNSPQQAQSVASQSIIAYTMSLGAENSVAYSNNSIAIPTNFTISVTTEILPVSMTKTSVDCTMYICGDSTECSNLLLQYGSFCTQLNRALTGIAVEQDKNTQEVFAQVKQIYKTPPIKDFGGFNFSQILPDPSKPSKRSFIEDLLFNKVTLADAGFIKQYGDCLGDIAARDLICAQKFNGLTVLPPLLTDEMIAQYTSALLAGTITSGWTFGAGAALQIPFAMQMAYRFNGIGVTQNVLYENQKLIANQFNSAIGKIQDSLSSTASALGKLQDVVNQNAQALNTLVKQLSSNFGAISSVLNDILSRLDPPEAEVQIDRLITGRLQSLQTYVTQQLIRAAEIRASANLAATKMSECVLGQSKRVDFCGKGYHLMSFPQSAPHGVVFLHVTYVPAQEKNFTTAPAICHDGKAHFPREGVFVSNGTHWFVTQRNFYEPQIITTDNTFVSGNCDVVIGIVNNTVYDPLQPELDSFKEELDKYFKNHTSPDVDLGDISGINASVVNIQKEIDRLNEVAKNLNESLIDLQELGKYEQYIKWPWYIWLGFIAGLIAIVMVTIMLCCMTSCCSCLKGCCSCGSCCKFDEDDSEPVLKGVKLHYT

SEQ ID NO: 112 - protein, 1273 aa, Artificial Sequence
  mutant spike protein of SARS-CoV-2 Wuhan variant comprising substitution G184P, 2-P-mutation (substiutions K986P and V987P) and inoperative furin cleavage site (substitution 682-QQAQ-685)
MFVFLVLLPLVSSQCVNLTTRTQLPPAYTNSFTRGVYYPDKVFRSSVLHSTQDLFLPFFSNVTWFHAIHVSGTNGTKRFDNPVLPFNDGVYFASTEKSNIIRGWIFGTTLDSKTQSLLIVNNATNVVIKVCEFQFCNDPFLGVYYHKNNKSWMESEFRVYSSANNCTFEYVSQPFLMDLEGKQGNFKNLREFVFKNIDGYFKIYSKHTPINLVRDLPQGFSALEPLVDLPIGINITRFQTLLALHRSYLTPGDSSSGWTAGAAAYYVGYLQPRTFLLKYNENGTITDAVDCALDPLSETKCTLKSFTVEKGIYQTSNFRVQPTESIVRFPNITNLCPFGEVFNATRFASVYAWNRKRISNCVADYSVLYNSASFSTFKCYGVSPTKLNDLCFTNVYADSFVIRGDEVRQIAPGQTGKIADYNYKLPDDFTGCVIAWNSNNLDSKVGGNYNYLYRLFRKSNLKPFERDISTEIYQAGSTPCNGVEGFNCYFPLQSYGFQPTNPVGYQPYRVVVLSFELLHAPATVCGPKKSTNLVKNKCVNFNFNGLTGTGVLTESNKKFLPFQQFGRDIADTTDAVRDPQTLEILDITPCSFGGVSVITPGTNTSNQVAVLYQDVNCTEVPVAIHADQLTPTWRVYSTGSNVFQTRAGCLIGAEHVNNSYECDIPIGAGICASYQTQTNSPQQAQSVASQSIIAYTMSLGAENSVAYSNNSIAIPTNFTISVTTEILPVSMTKTSVDCTMYICGDSTECSNLLLQYGSFCTQLNRALTGIAVEQDKNTQEVFAQVKQIYKTPPIKDFGGFNFSQILPDPSKPSKRSFIEDLLFNKVTLADAGFIKQYGDCLGDIAARDLICAQKFNGLTVLPPLLTDEMIAQYTSALLAGTITSGWTFGAGAALQIPFAMQMAYRFNGIGVTQNVLYENQKLIANQFNSAIGKIQDSLSSTASALGKLQDVVNQNAQALNTLVKQLSSNFGAISSVLNDILSRLDPPEAEVQIDRLITGRLQSLQTYVTQQLIRAAEIRASANLAATKMSECVLGQSKRVDFCGKGYHLMSFPQSAPHGVVFLHVTYVPAQEKNFTTAPAICHDGKAHFPREGVFVSNGTHWFVTQRNFYEPQIITTDNTFVSGNCDVVIGIVNNTVYDPLQPELDSFKEELDKYFKNHTSPDVDLGDISGINASVVNIQKEIDRLNEVAKNLNESLIDLQELGKYEQYIKWPWYIWLGFIAGLIAIVMVTIMLCCMTSCCSCLKGCCSCGSCCKFDEDDSEPVLKGVKLHYT

SEQ ID NO: 113 - protein, 1273 aa, Artificial Sequence
  mutant spike protein of SARS-CoV-2 Wuhan variant comprising substitution G502Q, 2-P-mutation (substiutions K986P and V987P) and inoperative furin cleavage site (substitution 682-QQAQ-685)
MFVFLVLLPLVSSQCVNLTTRTQLPPAYTNSFTRGVYYPDKVFRSSVLHSTQDLFLPFFSNVTWFHAIHVSGTNGTKRFDNPVLPFNDGVYFASTEKSNIIRGWIFGTTLDSKTQSLLIVNNATNVVIKVCEFQFCNDPFLGVYYHKNNKSWMESEFRVYSSANNCTFEYVSQPFLMDLEGKQGNFKNLREFVFKNIDGYFKIYSKHTPINLVRDLPQGFSALEPLVDLPIGINITRFQTLLALHRSYLTPGDSSSGWTAGAAAYYVGYLQPRTFLLKYNENGTITDAVDCALDPLSETKCTLKSFTVEKGIYQTSNFRVQPTESIVRFPNITNLCPFGEVFNATRFASVYAWNRKRISNCVADYSVLYNSASFSTFKCYGVSPTKLNDLCFTNVYADSFVIRGDEVRQIAPGQTGKIADYNYKLPDDFTGCVIAWNSNNLDSKVGGNYNYLYRLFRKSNLKPFERDISTEIYQAGSTPCNGVEGFNCYFPLQSYGFQPTNQVGYQPYRVVVLSFELLHAPATVCGPKKSTNLVKNKCVNFNFNGLTGTGVLTESNKKFLPFQQFGRDIADTTDAVRDPQTLEILDITPCSFGGVSVITPGTNTSNQVAVLYQDVNCTEVPVAIHADQLTPTWRVYSTGSNVFQTRAGCLIGAEHVNNSYECDIPIGAGICASYQTQTNSPQQAQSVASQSIIAYTMSLGAENSVAYSNNSIAIPTNFTISVTTEILPVSMTKTSVDCTMYICGDSTECSNLLLQYGSFCTQLNRALTGIAVEQDKNTQEVFAQVKQIYKTPPIKDFGGFNFSQILPDPSKPSKRSFIEDLLFNKVTLADAGFIKQYGDCLGDIAARDLICAQKFNGLTVLPPLLTDEMIAQYTSALLAGTITSGWTFGAGAALQIPFAMQMAYRFNGIGVTQNVLYENQKLIANQFNSAIGKIQDSLSSTASALGKLQDVVNQNAQALNTLVKQLSSNFGAISSVLNDILSRLDPPEAEVQIDRLITGRLQSLQTYVTQQLIRAAEIRASANLAATKMSECVLGQSKRVDFCGKGYHLMSFPQSAPHGVVFLHVTYVPAQEKNFTTAPAICHDGKAHFPREGVFVSNGTHWFVTQRNFYEPQIITTDNTFVSGNCDVVIGIVNNTVYDPLQPELDSFKEELDKYFKNHTSPDVDLGDISGINASVVNIQKEIDRLNEVAKNLNESLIDLQELGKYEQYIKWPWYIWLGFIAGLIAIVMVTIMLCCMTSCCSCLKGCCSCGSCCKFDEDDSEPVLKGVKLHYT

SEQ ID NO: 114 - protein, 1273 aa, Artificial Sequence
  mutant spike protein of SARS-CoV-2 Wuhan variant comprising substitution G502R, 2-P-mutation (substiutions K986P and V987P) and inoperative furin cleavage site (substitution 682-QQAQ-685)
MFVFLVLLPLVSSQCVNLTTRTQLPPAYTNSFTRGVYYPDKVFRSSVLHSTQDLFLPFFSNVTWFHAIHVSGTNGTKRFDNPVLPFNDGVYFASTEKSNIIRGWIFGTTLDSKTQSLLIVNNATNVVIKVCEFQFCNDPFLGVYYHKNNKSWMESEFRVYSSANNCTFEYVSQPFLMDLEGKQGNFKNLREFVFKNIDGYFKIYSKHTPINLVRDLPQGFSALEPLVDLPIGINITRFQTLLALHRSYLTPGDSSSGWTAGAAAYYVGYLQPRTFLLKYNENGTITDAVDCALDPLSETKCTLKSFTVEKGIYQTSNFRVQPTESIVRFPNITNLCPFGEVFNATRFASVYAWNRKRISNCVADYSVLYNSASFSTFKCYGVSPTKLNDLCFTNVYADSFVIRGDEVRQIAPGQTGKIADYNYKLPDDFTGCVIAWNSNNLDSKVGGNYNYLYRLFRKSNLKPFERDISTEIYQAGSTPCNGVEGFNCYFPLQSYGFQPTNRVGYQPYRVVVLSFELLHAPATVCGPKKSTNLVKNKCVNFNFNGLTGTGVLTESNKKFLPFQQFGRDIADTTDAVRDPQTLEILDITPCSFGGVSVITPGTNTSNQVAVLYQDVNCTEVPVAIHADQLTPTWRVYSTGSNVFQTRAGCLIGAEHVNNSYECDIPIGAGICASYQTQTNSPQQAQSVASQSIIAYTMSLGAENSVAYSNNSIAIPTNFTISVTTEILPVSMTKTSVDCTMYICGDSTECSNLLLQYGSFCTQLNRALTGIAVEQDKNTQEVFAQVKQIYKTPPIKDFGGFNFSQILPDPSKPSKRSFIEDLLFNKVTLADAGFIKQYGDCLGDIAARDLICAQKFNGLTVLPPLLTDEMIAQYTSALLAGTITSGWTFGAGAALQIPFAMQMAYRFNGIGVTQNVLYENQKLIANQFNSAIGKIQDSLSSTASALGKLQDVVNQNAQALNTLVKQLSSNFGAISSVLNDILSRLDPPEAEVQIDRLITGRLQSLQTYVTQQLIRAAEIRASANLAATKMSECVLGQSKRVDFCGKGYHLMSFPQSAPHGVVFLHVTYVPAQEKNFTTAPAICHDGKAHFPREGVFVSNGTHWFVTQRNFYEPQIITTDNTFVSGNCDVVIGIVNNTVYDPLQPELDSFKEELDKYFKNHTSPDVDLGDISGINASVVNIQKEIDRLNEVAKNLNESLIDLQELGKYEQYIKWPWYIWLGFIAGLIAIVMVTIMLCCMTSCCSCLKGCCSCGSCCKFDEDDSEPVLKGVKLHYT

SEQ ID NO: 115 - protein, 1273 aa, Artificial Sequence
  mutant spike protein of SARS-CoV-2 Wuhan variant comprising substitution G502S, 2-P-mutation (substiutions K986P and V987P) and inoperative furin cleavage site (substitution 682-QQAQ-685)
MFVFLVLLPLVSSQCVNLTTRTQLPPAYTNSFTRGVYYPDKVFRSSVLHSTQDLFLPFFSNVTWFHAIHVSGTNGTKRFDNPVLPFNDGVYFASTEKSNIIRGWIFGTTLDSKTQSLLIVNNATNVVIKVCEFQFCNDPFLGVYYHKNNKSWMESEFRVYSSANNCTFEYVSQPFLMDLEGKQGNFKNLREFVFKNIDGYFKIYSKHTPINLVRDLPQGFSALEPLVDLPIGINITRFQTLLALHRSYLTPGDSSSGWTAGAAAYYVGYLQPRTFLLKYNENGTITDAVDCALDPLSETKCTLKSFTVEKGIYQTSNFRVQPTESIVRFPNITNLCPFGEVFNATRFASVYAWNRKRISNCVADYSVLYNSASFSTFKCYGVSPTKLNDLCFTNVYADSFVIRGDEVRQIAPGQTGKIADYNYKLPDDFTGCVIAWNSNNLDSKVGGNYNYLYRLFRKSNLKPFERDISTEIYQAGSTPCNGVEGFNCYFPLQSYGFQPTNSVGYQPYRVVVLSFELLHAPATVCGPKKSTNLVKNKCVNFNFNGLTGTGVLTESNKKFLPFQQFGRDIADTTDAVRDPQTLEILDITPCSFGGVSVITPGTNTSNQVAVLYQDVNCTEVPVAIHADQLTPTWRVYSTGSNVFQTRAGCLIGAEHVNNSYECDIPIGAGICASYQTQTNSPQQAQSVASQSIIAYTMSLGAENSVAYSNNSIAIPTNFTISVTTEILPVSMTKTSVDCTMYICGDSTECSNLLLQYGSFCTQLNRALTGIAVEQDKNTQEVFAQVKQIYKTPPIKDFGGFNFSQILPDPSKPSKRSFIEDLLFNKVTLADAGFIKQYGDCLGDIAARDLICAQKFNGLTVLPPLLTDEMIAQYTSALLAGTITSGWTFGAGAALQIPFAMQMAYRFNGIGVTQNVLYENQKLIANQFNSAIGKIQDSLSSTASALGKLQDVVNQNAQALNTLVKQLSSNFGAISSVLNDILSRLDPPEAEVQIDRLITGRLQSLQTYVTQQLIRAAEIRASANLAATKMSECVLGQSKRVDFCGKGYHLMSFPQSAPHGVVFLHVTYVPAQEKNFTTAPAICHDGKAHFPREGVFVSNGTHWFVTQRNFYEPQIITTDNTFVSGNCDVVIGIVNNTVYDPLQPELDSFKEELDKYFKNHTSPDVDLGDISGINASVVNIQKEIDRLNEVAKNLNESLIDLQELGKYEQYIKWPWYIWLGFIAGLIAIVMVTIMLCCMTSCCSCLKGCCSCGSCCKFDEDDSEPVLKGVKLHYT

SEQ ID NO: 116 - protein, 1273 aa, Artificial Sequence
  mutant spike protein of SARS-CoV-2 Wuhan variant comprising substitution G502T, 2-P-mutation (substiutions K986P and V987P) and inoperative furin cleavage site (substitution 682-QQAQ-685)
MFVFLVLLPLVSSQCVNLTTRTQLPPAYTNSFTRGVYYPDKVFRSSVLHSTQDLFLPFFSNVTWFHAIHVSGTNGTKRFDNPVLPFNDGVYFASTEKSNIIRGWIFGTTLDSKTQSLLIVNNATNVVIKVCEFQFCNDPFLGVYYHKNNKSWMESEFRVYSSANNCTFEYVSQPFLMDLEGKQGNFKNLREFVFKNIDGYFKIYSKHTPINLVRDLPQGFSALEPLVDLPIGINITRFQTLLALHRSYLTPGDSSSGWTAGAAAYYVGYLQPRTFLLKYNENGTITDAVDCALDPLSETKCTLKSFTVEKGIYQTSNFRVQPTESIVRFPNITNLCPFGEVFNATRFASVYAWNRKRISNCVADYSVLYNSASFSTFKCYGVSPTKLNDLCFTNVYADSFVIRGDEVRQIAPGQTGKIADYNYKLPDDFTGCVIAWNSNNLDSKVGGNYNYLYRLFRKSNLKPFERDISTEIYQAGSTPCNGVEGFNCYFPLQSYGFQPTNTVGYQPYRVVVLSFELLHAPATVCGPKKSTNLVKNKCVNFNFNGLTGTGVLTESNKKFLPFQQFGRDIADTTDAVRDPQTLEILDITPCSFGGVSVITPGTNTSNQVAVLYQDVNCTEVPVAIHADQLTPTWRVYSTGSNVFQTRAGCLIGAEHVNNSYECDIPIGAGICASYQTQTNSPQQAQSVASQSIIAYTMSLGAENSVAYSNNSIAIPTNFTISVTTEILPVSMTKTSVDCTMYICGDSTECSNLLLQYGSFCTQLNRALTGIAVEQDKNTQEVFAQVKQIYKTPPIKDFGGFNFSQILPDPSKPSKRSFIEDLLFNKVTLADAGFIKQYGDCLGDIAARDLICAQKFNGLTVLPPLLTDEMIAQYTSALLAGTITSGWTFGAGAALQIPFAMQMAYRFNGIGVTQNVLYENQKLIANQFNSAIGKIQDSLSSTASALGKLQDVVNQNAQALNTLVKQLSSNFGAISSVLNDILSRLDPPEAEVQIDRLITGRLQSLQTYVTQQLIRAAEIRASANLAATKMSECVLGQSKRVDFCGKGYHLMSFPQSAPHGVVFLHVTYVPAQEKNFTTAPAICHDGKAHFPREGVFVSNGTHWFVTQRNFYEPQIITTDNTFVSGNCDVVIGIVNNTVYDPLQPELDSFKEELDKYFKNHTSPDVDLGDISGINASVVNIQKEIDRLNEVAKNLNESLIDLQELGKYEQYIKWPWYIWLGFIAGLIAIVMVTIMLCCMTSCCSCLKGCCSCGSCCKFDEDDSEPVLKGVKLHYT

SEQ ID NO: 117 - protein, 1273 aa, Artificial Sequence
  mutant spike protein of SARS-CoV-2 Wuhan variant comprising substitution G502V, 2-P-mutation (substiutions K986P and V987P) and inoperative furin cleavage site (substitution 682-QQAQ-685)
MFVFLVLLPLVSSQCVNLTTRTQLPPAYTNSFTRGVYYPDKVFRSSVLHSTQDLFLPFFSNVTWFHAIHVSGTNGTKRFDNPVLPFNDGVYFASTEKSNIIRGWIFGTTLDSKTQSLLIVNNATNVVIKVCEFQFCNDPFLGVYYHKNNKSWMESEFRVYSSANNCTFEYVSQPFLMDLEGKQGNFKNLREFVFKNIDGYFKIYSKHTPINLVRDLPQGFSALEPLVDLPIGINITRFQTLLALHRSYLTPGDSSSGWTAGAAAYYVGYLQPRTFLLKYNENGTITDAVDCALDPLSETKCTLKSFTVEKGIYQTSNFRVQPTESIVRFPNITNLCPFGEVFNATRFASVYAWNRKRISNCVADYSVLYNSASFSTFKCYGVSPTKLNDLCFTNVYADSFVIRGDEVRQIAPGQTGKIADYNYKLPDDFTGCVIAWNSNNLDSKVGGNYNYLYRLFRKSNLKPFERDISTEIYQAGSTPCNGVEGFNCYFPLQSYGFQPTNVVGYQPYRVVVLSFELLHAPATVCGPKKSTNLVKNKCVNFNFNGLTGTGVLTESNKKFLPFQQFGRDIADTTDAVRDPQTLEILDITPCSFGGVSVITPGTNTSNQVAVLYQDVNCTEVPVAIHADQLTPTWRVYSTGSNVFQTRAGCLIGAEHVNNSYECDIPIGAGICASYQTQTNSPQQAQSVASQSIIAYTMSLGAENSVAYSNNSIAIPTNFTISVTTEILPVSMTKTSVDCTMYICGDSTECSNLLLQYGSFCTQLNRALTGIAVEQDKNTQEVFAQVKQIYKTPPIKDFGGFNFSQILPDPSKPSKRSFIEDLLFNKVTLADAGFIKQYGDCLGDIAARDLICAQKFNGLTVLPPLLTDEMIAQYTSALLAGTITSGWTFGAGAALQIPFAMQMAYRFNGIGVTQNVLYENQKLIANQFNSAIGKIQDSLSSTASALGKLQDVVNQNAQALNTLVKQLSSNFGAISSVLNDILSRLDPPEAEVQIDRLITGRLQSLQTYVTQQLIRAAEIRASANLAATKMSECVLGQSKRVDFCGKGYHLMSFPQSAPHGVVFLHVTYVPAQEKNFTTAPAICHDGKAHFPREGVFVSNGTHWFVTQRNFYEPQIITTDNTFVSGNCDVVIGIVNNTVYDPLQPELDSFKEELDKYFKNHTSPDVDLGDISGINASVVNIQKEIDRLNEVAKNLNESLIDLQELGKYEQYIKWPWYIWLGFIAGLIAIVMVTIMLCCMTSCCSCLKGCCSCGSCCKFDEDDSEPVLKGVKLHYT

SEQ ID NO: 118 - protein, 1273 aa, Artificial Sequence
  mutant spike protein of SARS-CoV-2 Wuhan variant comprising substitution G502W, 2-P-mutation (substiutions K986P and V987P) and inoperative furin cleavage site (substitution 682-QQAQ-685)
MFVFLVLLPLVSSQCVNLTTRTQLPPAYTNSFTRGVYYPDKVFRSSVLHSTQDLFLPFFSNVTWFHAIHVSGTNGTKRFDNPVLPFNDGVYFASTEKSNIIRGWIFGTTLDSKTQSLLIVNNATNVVIKVCEFQFCNDPFLGVYYHKNNKSWMESEFRVYSSANNCTFEYVSQPFLMDLEGKQGNFKNLREFVFKNIDGYFKIYSKHTPINLVRDLPQGFSALEPLVDLPIGINITRFQTLLALHRSYLTPGDSSSGWTAGAAAYYVGYLQPRTFLLKYNENGTITDAVDCALDPLSETKCTLKSFTVEKGIYQTSNFRVQPTESIVRFPNITNLCPFGEVFNATRFASVYAWNRKRISNCVADYSVLYNSASFSTFKCYGVSPTKLNDLCFTNVYADSFVIRGDEVRQIAPGQTGKIADYNYKLPDDFTGCVIAWNSNNLDSKVGGNYNYLYRLFRKSNLKPFERDISTEIYQAGSTPCNGVEGFNCYFPLQSYGFQPTNWVGYQPYRVVVLSFELLHAPATVCGPKKSTNLVKNKCVNFNFNGLTGTGVLTESNKKFLPFQQFGRDIADTTDAVRDPQTLEILDITPCSFGGVSVITPGTNTSNQVAVLYQDVNCTEVPVAIHADQLTPTWRVYSTGSNVFQTRAGCLIGAEHVNNSYECDIPIGAGICASYQTQTNSPQQAQSVASQSIIAYTMSLGAENSVAYSNNSIAIPTNFTISVTTEILPVSMTKTSVDCTMYICGDSTECSNLLLQYGSFCTQLNRALTGIAVEQDKNTQEVFAQVKQIYKTPPIKDFGGFNFSQILPDPSKPSKRSFIEDLLFNKVTLADAGFIKQYGDCLGDIAARDLICAQKFNGLTVLPPLLTDEMIAQYTSALLAGTITSGWTFGAGAALQIPFAMQMAYRFNGIGVTQNVLYENQKLIANQFNSAIGKIQDSLSSTASALGKLQDVVNQNAQALNTLVKQLSSNFGAISSVLNDILSRLDPPEAEVQIDRLITGRLQSLQTYVTQQLIRAAEIRASANLAATKMSECVLGQSKRVDFCGKGYHLMSFPQSAPHGVVFLHVTYVPAQEKNFTTAPAICHDGKAHFPREGVFVSNGTHWFVTQRNFYEPQIITTDNTFVSGNCDVVIGIVNNTVYDPLQPELDSFKEELDKYFKNHTSPDVDLGDISGINASVVNIQKEIDRLNEVAKNLNESLIDLQELGKYEQYIKWPWYIWLGFIAGLIAIVMVTIMLCCMTSCCSCLKGCCSCGSCCKFDEDDSEPVLKGVKLHYT

SEQ ID NO: 119 - protein, 1273 aa, Artificial Sequence
  mutant spike protein of SARS-CoV-2 Wuhan variant comprising substitution G502Y, 2-P-mutation (substiutions K986P and V987P) and inoperative furin cleavage site (substitution 682-QQAQ-685)
MFVFLVLLPLVSSQCVNLTTRTQLPPAYTNSFTRGVYYPDKVFRSSVLHSTQDLFLPFFSNVTWFHAIHVSGTNGTKRFDNPVLPFNDGVYFASTEKSNIIRGWIFGTTLDSKTQSLLIVNNATNVVIKVCEFQFCNDPFLGVYYHKNNKSWMESEFRVYSSANNCTFEYVSQPFLMDLEGKQGNFKNLREFVFKNIDGYFKIYSKHTPINLVRDLPQGFSALEPLVDLPIGINITRFQTLLALHRSYLTPGDSSSGWTAGAAAYYVGYLQPRTFLLKYNENGTITDAVDCALDPLSETKCTLKSFTVEKGIYQTSNFRVQPTESIVRFPNITNLCPFGEVFNATRFASVYAWNRKRISNCVADYSVLYNSASFSTFKCYGVSPTKLNDLCFTNVYADSFVIRGDEVRQIAPGQTGKIADYNYKLPDDFTGCVIAWNSNNLDSKVGGNYNYLYRLFRKSNLKPFERDISTEIYQAGSTPCNGVEGFNCYFPLQSYGFQPTNYVGYQPYRVVVLSFELLHAPATVCGPKKSTNLVKNKCVNFNFNGLTGTGVLTESNKKFLPFQQFGRDIADTTDAVRDPQTLEILDITPCSFGGVSVITPGTNTSNQVAVLYQDVNCTEVPVAIHADQLTPTWRVYSTGSNVFQTRAGCLIGAEHVNNSYECDIPIGAGICASYQTQTNSPQQAQSVASQSIIAYTMSLGAENSVAYSNNSIAIPTNFTISVTTEILPVSMTKTSVDCTMYICGDSTECSNLLLQYGSFCTQLNRALTGIAVEQDKNTQEVFAQVKQIYKTPPIKDFGGFNFSQILPDPSKPSKRSFIEDLLFNKVTLADAGFIKQYGDCLGDIAARDLICAQKFNGLTVLPPLLTDEMIAQYTSALLAGTITSGWTFGAGAALQIPFAMQMAYRFNGIGVTQNVLYENQKLIANQFNSAIGKIQDSLSSTASALGKLQDVVNQNAQALNTLVKQLSSNFGAISSVLNDILSRLDPPEAEVQIDRLITGRLQSLQTYVTQQLIRAAEIRASANLAATKMSECVLGQSKRVDFCGKGYHLMSFPQSAPHGVVFLHVTYVPAQEKNFTTAPAICHDGKAHFPREGVFVSNGTHWFVTQRNFYEPQIITTDNTFVSGNCDVVIGIVNNTVYDPLQPELDSFKEELDKYFKNHTSPDVDLGDISGINASVVNIQKEIDRLNEVAKNLNESLIDLQELGKYEQYIKWPWYIWLGFIAGLIAIVMVTIMLCCMTSCCSCLKGCCSCGSCCKFDEDDSEPVLKGVKLHYT

SEQ ID NO: 120 - protein, 1273 aa, Artificial Sequence
  mutant spike protein of SARS-CoV-2 Wuhan variant comprising substitution Y505A, 2-P-mutation (substiutions K986P and V987P) and inoperative furin cleavage site (substitution 682-QQAQ-685)
MFVFLVLLPLVSSQCVNLTTRTQLPPAYTNSFTRGVYYPDKVFRSSVLHSTQDLFLPFFSNVTWFHAIHVSGTNGTKRFDNPVLPFNDGVYFASTEKSNIIRGWIFGTTLDSKTQSLLIVNNATNVVIKVCEFQFCNDPFLGVYYHKNNKSWMESEFRVYSSANNCTFEYVSQPFLMDLEGKQGNFKNLREFVFKNIDGYFKIYSKHTPINLVRDLPQGFSALEPLVDLPIGINITRFQTLLALHRSYLTPGDSSSGWTAGAAAYYVGYLQPRTFLLKYNENGTITDAVDCALDPLSETKCTLKSFTVEKGIYQTSNFRVQPTESIVRFPNITNLCPFGEVFNATRFASVYAWNRKRISNCVADYSVLYNSASFSTFKCYGVSPTKLNDLCFTNVYADSFVIRGDEVRQIAPGQTGKIADYNYKLPDDFTGCVIAWNSNNLDSKVGGNYNYLYRLFRKSNLKPFERDISTEIYQAGSTPCNGVEGFNCYFPLQSYGFQPTNGVGAQPYRVVVLSFELLHAPATVCGPKKSTNLVKNKCVNFNFNGLTGTGVLTESNKKFLPFQQFGRDIADTTDAVRDPQTLEILDITPCSFGGVSVITPGTNTSNQVAVLYQDVNCTEVPVAIHADQLTPTWRVYSTGSNVFQTRAGCLIGAEHVNNSYECDIPIGAGICASYQTQTNSPQQAQSVASQSIIAYTMSLGAENSVAYSNNSIAIPTNFTISVTTEILPVSMTKTSVDCTMYICGDSTECSNLLLQYGSFCTQLNRALTGIAVEQDKNTQEVFAQVKQIYKTPPIKDFGGFNFSQILPDPSKPSKRSFIEDLLFNKVTLADAGFIKQYGDCLGDIAARDLICAQKFNGLTVLPPLLTDEMIAQYTSALLAGTITSGWTFGAGAALQIPFAMQMAYRFNGIGVTQNVLYENQKLIANQFNSAIGKIQDSLSSTASALGKLQDVVNQNAQALNTLVKQLSSNFGAISSVLNDILSRLDPPEAEVQIDRLITGRLQSLQTYVTQQLIRAAEIRASANLAATKMSECVLGQSKRVDFCGKGYHLMSFPQSAPHGVVFLHVTYVPAQEKNFTTAPAICHDGKAHFPREGVFVSNGTHWFVTQRNFYEPQIITTDNTFVSGNCDVVIGIVNNTVYDPLQPELDSFKEELDKYFKNHTSPDVDLGDISGINASVVNIQKEIDRLNEVAKNLNESLIDLQELGKYEQYIKWPWYIWLGFIAGLIAIVMVTIMLCCMTSCCSCLKGCCSCGSCCKFDEDDSEPVLKGVKLHYT

SEQ ID NO: 121 - protein, 1273 aa, Artificial Sequence
  mutant spike protein of SARS-CoV-2 Wuhan variant comprising substitution Y505C, 2-P-mutation (substiutions K986P and V987P) and inoperative furin cleavage site (substitution 682-QQAQ-685)
MFVFLVLLPLVSSQCVNLTTRTQLPPAYTNSFTRGVYYPDKVFRSSVLHSTQDLFLPFFSNVTWFHAIHVSGTNGTKRFDNPVLPFNDGVYFASTEKSNIIRGWIFGTTLDSKTQSLLIVNNATNVVIKVCEFQFCNDPFLGVYYHKNNKSWMESEFRVYSSANNCTFEYVSQPFLMDLEGKQGNFKNLREFVFKNIDGYFKIYSKHTPINLVRDLPQGFSALEPLVDLPIGINITRFQTLLALHRSYLTPGDSSSGWTAGAAAYYVGYLQPRTFLLKYNENGTITDAVDCALDPLSETKCTLKSFTVEKGIYQTSNFRVQPTESIVRFPNITNLCPFGEVFNATRFASVYAWNRKRISNCVADYSVLYNSASFSTFKCYGVSPTKLNDLCFTNVYADSFVIRGDEVRQIAPGQTGKIADYNYKLPDDFTGCVIAWNSNNLDSKVGGNYNYLYRLFRKSNLKPFERDISTEIYQAGSTPCNGVEGFNCYFPLQSYGFQPTNGVGCQPYRVVVLSFELLHAPATVCGPKKSTNLVKNKCVNFNFNGLTGTGVLTESNKKFLPFQQFGRDIADTTDAVRDPQTLEILDITPCSFGGVSVITPGTNTSNQVAVLYQDVNCTEVPVAIHADQLTPTWRVYSTGSNVFQTRAGCLIGAEHVNNSYECDIPIGAGICASYQTQTNSPQQAQSVASQSIIAYTMSLGAENSVAYSNNSIAIPTNFTISVTTEILPVSMTKTSVDCTMYICGDSTECSNLLLQYGSFCTQLNRALTGIAVEQDKNTQEVFAQVKQIYKTPPIKDFGGFNFSQILPDPSKPSKRSFIEDLLFNKVTLADAGFIKQYGDCLGDIAARDLICAQKFNGLTVLPPLLTDEMIAQYTSALLAGTITSGWTFGAGAALQIPFAMQMAYRFNGIGVTQNVLYENQKLIANQFNSAIGKIQDSLSSTASALGKLQDVVNQNAQALNTLVKQLSSNFGAISSVLNDILSRLDPPEAEVQIDRLITGRLQSLQTYVTQQLIRAAEIRASANLAATKMSECVLGQSKRVDFCGKGYHLMSFPQSAPHGVVFLHVTYVPAQEKNFTTAPAICHDGKAHFPREGVFVSNGTHWFVTQRNFYEPQIITTDNTFVSGNCDVVIGIVNNTVYDPLQPELDSFKEELDKYFKNHTSPDVDLGDISGINASVVNIQKEIDRLNEVAKNLNESLIDLQELGKYEQYIKWPWYIWLGFIAGLIAIVMVTIMLCCMTSCCSCLKGCCSCGSCCKFDEDDSEPVLKGVKLHYT

SEQ ID NO: 122 - protein, 1273 aa, Artificial Sequence
  mutant spike protein of SARS-CoV-2 Wuhan variant comprising substitution Y505D, 2-P-mutation (substiutions K986P and V987P) and inoperative furin cleavage site (substitution 682-QQAQ-685)
MFVFLVLLPLVSSQCVNLTTRTQLPPAYTNSFTRGVYYPDKVFRSSVLHSTQDLFLPFFSNVTWFHAIHVSGTNGTKRFDNPVLPFNDGVYFASTEKSNIIRGWIFGTTLDSKTQSLLIVNNATNVVIKVCEFQFCNDPFLGVYYHKNNKSWMESEFRVYSSANNCTFEYVSQPFLMDLEGKQGNFKNLREFVFKNIDGYFKIYSKHTPINLVRDLPQGFSALEPLVDLPIGINITRFQTLLALHRSYLTPGDSSSGWTAGAAAYYVGYLQPRTFLLKYNENGTITDAVDCALDPLSETKCTLKSFTVEKGIYQTSNFRVQPTESIVRFPNITNLCPFGEVFNATRFASVYAWNRKRISNCVADYSVLYNSASFSTFKCYGVSPTKLNDLCFTNVYADSFVIRGDEVRQIAPGQTGKIADYNYKLPDDFTGCVIAWNSNNLDSKVGGNYNYLYRLFRKSNLKPFERDISTEIYQAGSTPCNGVEGFNCYFPLQSYGFQPTNGVGDQPYRVVVLSFELLHAPATVCGPKKSTNLVKNKCVNFNFNGLTGTGVLTESNKKFLPFQQFGRDIADTTDAVRDPQTLEILDITPCSFGGVSVITPGTNTSNQVAVLYQDVNCTEVPVAIHADQLTPTWRVYSTGSNVFQTRAGCLIGAEHVNNSYECDIPIGAGICASYQTQTNSPQQAQSVASQSIIAYTMSLGAENSVAYSNNSIAIPTNFTISVTTEILPVSMTKTSVDCTMYICGDSTECSNLLLQYGSFCTQLNRALTGIAVEQDKNTQEVFAQVKQIYKTPPIKDFGGFNFSQILPDPSKPSKRSFIEDLLFNKVTLADAGFIKQYGDCLGDIAARDLICAQKFNGLTVLPPLLTDEMIAQYTSALLAGTITSGWTFGAGAALQIPFAMQMAYRFNGIGVTQNVLYENQKLIANQFNSAIGKIQDSLSSTASALGKLQDVVNQNAQALNTLVKQLSSNFGAISSVLNDILSRLDPPEAEVQIDRLITGRLQSLQTYVTQQLIRAAEIRASANLAATKMSECVLGQSKRVDFCGKGYHLMSFPQSAPHGVVFLHVTYVPAQEKNFTTAPAICHDGKAHFPREGVFVSNGTHWFVTQRNFYEPQIITTDNTFVSGNCDVVIGIVNNTVYDPLQPELDSFKEELDKYFKNHTSPDVDLGDISGINASVVNIQKEIDRLNEVAKNLNESLIDLQELGKYEQYIKWPWYIWLGFIAGLIAIVMVTIMLCCMTSCCSCLKGCCSCGSCCKFDEDDSEPVLKGVKLHYT

SEQ ID NO: 123 - protein, 1273 aa, Artificial Sequence
  mutant spike protein of SARS-CoV-2 Wuhan variant comprising substitution Y505E, 2-P-mutation (substiutions K986P and V987P) and inoperative furin cleavage site (substitution 682-QQAQ-685)
MFVFLVLLPLVSSQCVNLTTRTQLPPAYTNSFTRGVYYPDKVFRSSVLHSTQDLFLPFFSNVTWFHAIHVSGTNGTKRFDNPVLPFNDGVYFASTEKSNIIRGWIFGTTLDSKTQSLLIVNNATNVVIKVCEFQFCNDPFLGVYYHKNNKSWMESEFRVYSSANNCTFEYVSQPFLMDLEGKQGNFKNLREFVFKNIDGYFKIYSKHTPINLVRDLPQGFSALEPLVDLPIGINITRFQTLLALHRSYLTPGDSSSGWTAGAAAYYVGYLQPRTFLLKYNENGTITDAVDCALDPLSETKCTLKSFTVEKGIYQTSNFRVQPTESIVRFPNITNLCPFGEVFNATRFASVYAWNRKRISNCVADYSVLYNSASFSTFKCYGVSPTKLNDLCFTNVYADSFVIRGDEVRQIAPGQTGKIADYNYKLPDDFTGCVIAWNSNNLDSKVGGNYNYLYRLFRKSNLKPFERDISTEIYQAGSTPCNGVEGFNCYFPLQSYGFQPTNGVGEQPYRVVVLSFELLHAPATVCGPKKSTNLVKNKCVNFNFNGLTGTGVLTESNKKFLPFQQFGRDIADTTDAVRDPQTLEILDITPCSFGGVSVITPGTNTSNQVAVLYQDVNCTEVPVAIHADQLTPTWRVYSTGSNVFQTRAGCLIGAEHVNNSYECDIPIGAGICASYQTQTNSPQQAQSVASQSIIAYTMSLGAENSVAYSNNSIAIPTNFTISVTTEILPVSMTKTSVDCTMYICGDSTECSNLLLQYGSFCTQLNRALTGIAVEQDKNTQEVFAQVKQIYKTPPIKDFGGFNFSQILPDPSKPSKRSFIEDLLFNKVTLADAGFIKQYGDCLGDIAARDLICAQKFNGLTVLPPLLTDEMIAQYTSALLAGTITSGWTFGAGAALQIPFAMQMAYRFNGIGVTQNVLYENQKLIANQFNSAIGKIQDSLSSTASALGKLQDVVNQNAQALNTLVKQLSSNFGAISSVLNDILSRLDPPEAEVQIDRLITGRLQSLQTYVTQQLIRAAEIRASANLAATKMSECVLGQSKRVDFCGKGYHLMSFPQSAPHGVVFLHVTYVPAQEKNFTTAPAICHDGKAHFPREGVFVSNGTHWFVTQRNFYEPQIITTDNTFVSGNCDVVIGIVNNTVYDPLQPELDSFKEELDKYFKNHTSPDVDLGDISGINASVVNIQKEIDRLNEVAKNLNESLIDLQELGKYEQYIKWPWYIWLGFIAGLIAIVMVTIMLCCMTSCCSCLKGCCSCGSCCKFDEDDSEPVLKGVKLHYT

SEQ ID NO: 124 - protein, 1273 aa, Artificial Sequence
  mutant spike protein of SARS-CoV-2 Wuhan variant comprising substitution Y505G, 2-P-mutation (substiutions K986P and V987P) and inoperative furin cleavage site (substitution 682-QQAQ-685)
MFVFLVLLPLVSSQCVNLTTRTQLPPAYTNSFTRGVYYPDKVFRSSVLHSTQDLFLPFFSNVTWFHAIHVSGTNGTKRFDNPVLPFNDGVYFASTEKSNIIRGWIFGTTLDSKTQSLLIVNNATNVVIKVCEFQFCNDPFLGVYYHKNNKSWMESEFRVYSSANNCTFEYVSQPFLMDLEGKQGNFKNLREFVFKNIDGYFKIYSKHTPINLVRDLPQGFSALEPLVDLPIGINITRFQTLLALHRSYLTPGDSSSGWTAGAAAYYVGYLQPRTFLLKYNENGTITDAVDCALDPLSETKCTLKSFTVEKGIYQTSNFRVQPTESIVRFPNITNLCPFGEVFNATRFASVYAWNRKRISNCVADYSVLYNSASFSTFKCYGVSPTKLNDLCFTNVYADSFVIRGDEVRQIAPGQTGKIADYNYKLPDDFTGCVIAWNSNNLDSKVGGNYNYLYRLFRKSNLKPFERDISTEIYQAGSTPCNGVEGFNCYFPLQSYGFQPTNGVGGQPYRVVVLSFELLHAPATVCGPKKSTNLVKNKCVNFNFNGLTGTGVLTESNKKFLPFQQFGRDIADTTDAVRDPQTLEILDITPCSFGGVSVITPGTNTSNQVAVLYQDVNCTEVPVAIHADQLTPTWRVYSTGSNVFQTRAGCLIGAEHVNNSYECDIPIGAGICASYQTQTNSPQQAQSVASQSIIAYTMSLGAENSVAYSNNSIAIPTNFTISVTTEILPVSMTKTSVDCTMYICGDSTECSNLLLQYGSFCTQLNRALTGIAVEQDKNTQEVFAQVKQIYKTPPIKDFGGFNFSQILPDPSKPSKRSFIEDLLFNKVTLADAGFIKQYGDCLGDIAARDLICAQKFNGLTVLPPLLTDEMIAQYTSALLAGTITSGWTFGAGAALQIPFAMQMAYRFNGIGVTQNVLYENQKLIANQFNSAIGKIQDSLSSTASALGKLQDVVNQNAQALNTLVKQLSSNFGAISSVLNDILSRLDPPEAEVQIDRLITGRLQSLQTYVTQQLIRAAEIRASANLAATKMSECVLGQSKRVDFCGKGYHLMSFPQSAPHGVVFLHVTYVPAQEKNFTTAPAICHDGKAHFPREGVFVSNGTHWFVTQRNFYEPQIITTDNTFVSGNCDVVIGIVNNTVYDPLQPELDSFKEELDKYFKNHTSPDVDLGDISGINASVVNIQKEIDRLNEVAKNLNESLIDLQELGKYEQYIKWPWYIWLGFIAGLIAIVMVTIMLCCMTSCCSCLKGCCSCGSCCKFDEDDSEPVLKGVKLHYT

SEQ ID NO: 125 - protein, 1273 aa, Artificial Sequence
  mutant spike protein of SARS-CoV-2 Wuhan variant comprising substitution Y505I, 2-P-mutation (substiutions K986P and V987P) and inoperative furin cleavage site (substitution 682-QQAQ-685)
MFVFLVLLPLVSSQCVNLTTRTQLPPAYTNSFTRGVYYPDKVFRSSVLHSTQDLFLPFFSNVTWFHAIHVSGTNGTKRFDNPVLPFNDGVYFASTEKSNIIRGWIFGTTLDSKTQSLLIVNNATNVVIKVCEFQFCNDPFLGVYYHKNNKSWMESEFRVYSSANNCTFEYVSQPFLMDLEGKQGNFKNLREFVFKNIDGYFKIYSKHTPINLVRDLPQGFSALEPLVDLPIGINITRFQTLLALHRSYLTPGDSSSGWTAGAAAYYVGYLQPRTFLLKYNENGTITDAVDCALDPLSETKCTLKSFTVEKGIYQTSNFRVQPTESIVRFPNITNLCPFGEVFNATRFASVYAWNRKRISNCVADYSVLYNSASFSTFKCYGVSPTKLNDLCFTNVYADSFVIRGDEVRQIAPGQTGKIADYNYKLPDDFTGCVIAWNSNNLDSKVGGNYNYLYRLFRKSNLKPFERDISTEIYQAGSTPCNGVEGFNCYFPLQSYGFQPTNGVGIQPYRVVVLSFELLHAPATVCGPKKSTNLVKNKCVNFNFNGLTGTGVLTESNKKFLPFQQFGRDIADTTDAVRDPQTLEILDITPCSFGGVSVITPGTNTSNQVAVLYQDVNCTEVPVAIHADQLTPTWRVYSTGSNVFQTRAGCLIGAEHVNNSYECDIPIGAGICASYQTQTNSPQQAQSVASQSIIAYTMSLGAENSVAYSNNSIAIPTNFTISVTTEILPVSMTKTSVDCTMYICGDSTECSNLLLQYGSFCTQLNRALTGIAVEQDKNTQEVFAQVKQIYKTPPIKDFGGFNFSQILPDPSKPSKRSFIEDLLFNKVTLADAGFIKQYGDCLGDIAARDLICAQKFNGLTVLPPLLTDEMIAQYTSALLAGTITSGWTFGAGAALQIPFAMQMAYRFNGIGVTQNVLYENQKLIANQFNSAIGKIQDSLSSTASALGKLQDVVNQNAQALNTLVKQLSSNFGAISSVLNDILSRLDPPEAEVQIDRLITGRLQSLQTYVTQQLIRAAEIRASANLAATKMSECVLGQSKRVDFCGKGYHLMSFPQSAPHGVVFLHVTYVPAQEKNFTTAPAICHDGKAHFPREGVFVSNGTHWFVTQRNFYEPQIITTDNTFVSGNCDVVIGIVNNTVYDPLQPELDSFKEELDKYFKNHTSPDVDLGDISGINASVVNIQKEIDRLNEVAKNLNESLIDLQELGKYEQYIKWPWYIWLGFIAGLIAIVMVTIMLCCMTSCCSCLKGCCSCGSCCKFDEDDSEPVLKGVKLHYT

SEQ ID NO: 126 - protein, 1273 aa, Artificial Sequence
  mutant spike protein of SARS-CoV-2 Wuhan variant comprising substitution Y505L, 2-P-mutation (substiutions K986P and V987P) and inoperative furin cleavage site (substitution 682-QQAQ-685)
MFVFLVLLPLVSSQCVNLTTRTQLPPAYTNSFTRGVYYPDKVFRSSVLHSTQDLFLPFFSNVTWFHAIHVSGTNGTKRFDNPVLPFNDGVYFASTEKSNIIRGWIFGTTLDSKTQSLLIVNNATNVVIKVCEFQFCNDPFLGVYYHKNNKSWMESEFRVYSSANNCTFEYVSQPFLMDLEGKQGNFKNLREFVFKNIDGYFKIYSKHTPINLVRDLPQGFSALEPLVDLPIGINITRFQTLLALHRSYLTPGDSSSGWTAGAAAYYVGYLQPRTFLLKYNENGTITDAVDCALDPLSETKCTLKSFTVEKGIYQTSNFRVQPTESIVRFPNITNLCPFGEVFNATRFASVYAWNRKRISNCVADYSVLYNSASFSTFKCYGVSPTKLNDLCFTNVYADSFVIRGDEVRQIAPGQTGKIADYNYKLPDDFTGCVIAWNSNNLDSKVGGNYNYLYRLFRKSNLKPFERDISTEIYQAGSTPCNGVEGFNCYFPLQSYGFQPTNGVGLQPYRVVVLSFELLHAPATVCGPKKSTNLVKNKCVNFNFNGLTGTGVLTESNKKFLPFQQFGRDIADTTDAVRDPQTLEILDITPCSFGGVSVITPGTNTSNQVAVLYQDVNCTEVPVAIHADQLTPTWRVYSTGSNVFQTRAGCLIGAEHVNNSYECDIPIGAGICASYQTQTNSPQQAQSVASQSIIAYTMSLGAENSVAYSNNSIAIPTNFTISVTTEILPVSMTKTSVDCTMYICGDSTECSNLLLQYGSFCTQLNRALTGIAVEQDKNTQEVFAQVKQIYKTPPIKDFGGFNFSQILPDPSKPSKRSFIEDLLFNKVTLADAGFIKQYGDCLGDIAARDLICAQKFNGLTVLPPLLTDEMIAQYTSALLAGTITSGWTFGAGAALQIPFAMQMAYRFNGIGVTQNVLYENQKLIANQFNSAIGKIQDSLSSTASALGKLQDVVNQNAQALNTLVKQLSSNFGAISSVLNDILSRLDPPEAEVQIDRLITGRLQSLQTYVTQQLIRAAEIRASANLAATKMSECVLGQSKRVDFCGKGYHLMSFPQSAPHGVVFLHVTYVPAQEKNFTTAPAICHDGKAHFPREGVFVSNGTHWFVTQRNFYEPQIITTDNTFVSGNCDVVIGIVNNTVYDPLQPELDSFKEELDKYFKNHTSPDVDLGDISGINASVVNIQKEIDRLNEVAKNLNESLIDLQELGKYEQYIKWPWYIWLGFIAGLIAIVMVTIMLCCMTSCCSCLKGCCSCGSCCKFDEDDSEPVLKGVKLHYT

SEQ ID NO: 127 - protein, 1273 aa, Artificial Sequence
  mutant spike protein of SARS-CoV-2 Wuhan variant comprising substitution Y505K, 2-P-mutation (substiutions K986P and V987P) and inoperative furin cleavage site (substitution 682-QQAQ-685)
MFVFLVLLPLVSSQCVNLTTRTQLPPAYTNSFTRGVYYPDKVFRSSVLHSTQDLFLPFFSNVTWFHAIHVSGTNGTKRFDNPVLPFNDGVYFASTEKSNIIRGWIFGTTLDSKTQSLLIVNNATNVVIKVCEFQFCNDPFLGVYYHKNNKSWMESEFRVYSSANNCTFEYVSQPFLMDLEGKQGNFKNLREFVFKNIDGYFKIYSKHTPINLVRDLPQGFSALEPLVDLPIGINITRFQTLLALHRSYLTPGDSSSGWTAGAAAYYVGYLQPRTFLLKYNENGTITDAVDCALDPLSETKCTLKSFTVEKGIYQTSNFRVQPTESIVRFPNITNLCPFGEVFNATRFASVYAWNRKRISNCVADYSVLYNSASFSTFKCYGVSPTKLNDLCFTNVYADSFVIRGDEVRQIAPGQTGKIADYNYKLPDDFTGCVIAWNSNNLDSKVGGNYNYLYRLFRKSNLKPFERDISTEIYQAGSTPCNGVEGFNCYFPLQSYGFQPTNGVGKQPYRVVVLSFELLHAPATVCGPKKSTNLVKNKCVNFNFNGLTGTGVLTESNKKFLPFQQFGRDIADTTDAVRDPQTLEILDITPCSFGGVSVITPGTNTSNQVAVLYQDVNCTEVPVAIHADQLTPTWRVYSTGSNVFQTRAGCLIGAEHVNNSYECDIPIGAGICASYQTQTNSPQQAQSVASQSIIAYTMSLGAENSVAYSNNSIAIPTNFTISVTTEILPVSMTKTSVDCTMYICGDSTECSNLLLQYGSFCTQLNRALTGIAVEQDKNTQEVFAQVKQIYKTPPIKDFGGFNFSQILPDPSKPSKRSFIEDLLFNKVTLADAGFIKQYGDCLGDIAARDLICAQKFNGLTVLPPLLTDEMIAQYTSALLAGTITSGWTFGAGAALQIPFAMQMAYRFNGIGVTQNVLYENQKLIANQFNSAIGKIQDSLSSTASALGKLQDVVNQNAQALNTLVKQLSSNFGAISSVLNDILSRLDPPEAEVQIDRLITGRLQSLQTYVTQQLIRAAEIRASANLAATKMSECVLGQSKRVDFCGKGYHLMSFPQSAPHGVVFLHVTYVPAQEKNFTTAPAICHDGKAHFPREGVFVSNGTHWFVTQRNFYEPQIITTDNTFVSGNCDVVIGIVNNTVYDPLQPELDSFKEELDKYFKNHTSPDVDLGDISGINASVVNIQKEIDRLNEVAKNLNESLIDLQELGKYEQYIKWPWYIWLGFIAGLIAIVMVTIMLCCMTSCCSCLKGCCSCGSCCKFDEDDSEPVLKGVKLHYT

SEQ ID NO: 128 - protein, 1273 aa, Artificial Sequence
  mutant spike protein of SARS-CoV-2 Wuhan variant comprising substitution Y505M, 2-P-mutation (substiutions K986P and V987P) and inoperative furin cleavage site (substitution 682-QQAQ-685)
MFVFLVLLPLVSSQCVNLTTRTQLPPAYTNSFTRGVYYPDKVFRSSVLHSTQDLFLPFFSNVTWFHAIHVSGTNGTKRFDNPVLPFNDGVYFASTEKSNIIRGWIFGTTLDSKTQSLLIVNNATNVVIKVCEFQFCNDPFLGVYYHKNNKSWMESEFRVYSSANNCTFEYVSQPFLMDLEGKQGNFKNLREFVFKNIDGYFKIYSKHTPINLVRDLPQGFSALEPLVDLPIGINITRFQTLLALHRSYLTPGDSSSGWTAGAAAYYVGYLQPRTFLLKYNENGTITDAVDCALDPLSETKCTLKSFTVEKGIYQTSNFRVQPTESIVRFPNITNLCPFGEVFNATRFASVYAWNRKRISNCVADYSVLYNSASFSTFKCYGVSPTKLNDLCFTNVYADSFVIRGDEVRQIAPGQTGKIADYNYKLPDDFTGCVIAWNSNNLDSKVGGNYNYLYRLFRKSNLKPFERDISTEIYQAGSTPCNGVEGFNCYFPLQSYGFQPTNGVGMQPYRVVVLSFELLHAPATVCGPKKSTNLVKNKCVNFNFNGLTGTGVLTESNKKFLPFQQFGRDIADTTDAVRDPQTLEILDITPCSFGGVSVITPGTNTSNQVAVLYQDVNCTEVPVAIHADQLTPTWRVYSTGSNVFQTRAGCLIGAEHVNNSYECDIPIGAGICASYQTQTNSPQQAQSVASQSIIAYTMSLGAENSVAYSNNSIAIPTNFTISVTTEILPVSMTKTSVDCTMYICGDSTECSNLLLQYGSFCTQLNRALTGIAVEQDKNTQEVFAQVKQIYKTPPIKDFGGFNFSQILPDPSKPSKRSFIEDLLFNKVTLADAGFIKQYGDCLGDIAARDLICAQKFNGLTVLPPLLTDEMIAQYTSALLAGTITSGWTFGAGAALQIPFAMQMAYRFNGIGVTQNVLYENQKLIANQFNSAIGKIQDSLSSTASALGKLQDVVNQNAQALNTLVKQLSSNFGAISSVLNDILSRLDPPEAEVQIDRLITGRLQSLQTYVTQQLIRAAEIRASANLAATKMSECVLGQSKRVDFCGKGYHLMSFPQSAPHGVVFLHVTYVPAQEKNFTTAPAICHDGKAHFPREGVFVSNGTHWFVTQRNFYEPQIITTDNTFVSGNCDVVIGIVNNTVYDPLQPELDSFKEELDKYFKNHTSPDVDLGDISGINASVVNIQKEIDRLNEVAKNLNESLIDLQELGKYEQYIKWPWYIWLGFIAGLIAIVMVTIMLCCMTSCCSCLKGCCSCGSCCKFDEDDSEPVLKGVKLHYT

SEQ ID NO: 129 - protein, 1273 aa, Artificial Sequence
  mutant spike protein of SARS-CoV-2 Wuhan variant comprising substitution Y505N, 2-P-mutation (substiutions K986P and V987P) and inoperative furin cleavage site (substitution 682-QQAQ-685)
MFVFLVLLPLVSSQCVNLTTRTQLPPAYTNSFTRGVYYPDKVFRSSVLHSTQDLFLPFFSNVTWFHAIHVSGTNGTKRFDNPVLPFNDGVYFASTEKSNIIRGWIFGTTLDSKTQSLLIVNNATNVVIKVCEFQFCNDPFLGVYYHKNNKSWMESEFRVYSSANNCTFEYVSQPFLMDLEGKQGNFKNLREFVFKNIDGYFKIYSKHTPINLVRDLPQGFSALEPLVDLPIGINITRFQTLLALHRSYLTPGDSSSGWTAGAAAYYVGYLQPRTFLLKYNENGTITDAVDCALDPLSETKCTLKSFTVEKGIYQTSNFRVQPTESIVRFPNITNLCPFGEVFNATRFASVYAWNRKRISNCVADYSVLYNSASFSTFKCYGVSPTKLNDLCFTNVYADSFVIRGDEVRQIAPGQTGKIADYNYKLPDDFTGCVIAWNSNNLDSKVGGNYNYLYRLFRKSNLKPFERDISTEIYQAGSTPCNGVEGFNCYFPLQSYGFQPTNGVGNQPYRVVVLSFELLHAPATVCGPKKSTNLVKNKCVNFNFNGLTGTGVLTESNKKFLPFQQFGRDIADTTDAVRDPQTLEILDITPCSFGGVSVITPGTNTSNQVAVLYQDVNCTEVPVAIHADQLTPTWRVYSTGSNVFQTRAGCLIGAEHVNNSYECDIPIGAGICASYQTQTNSPQQAQSVASQSIIAYTMSLGAENSVAYSNNSIAIPTNFTISVTTEILPVSMTKTSVDCTMYICGDSTECSNLLLQYGSFCTQLNRALTGIAVEQDKNTQEVFAQVKQIYKTPPIKDFGGFNFSQILPDPSKPSKRSFIEDLLFNKVTLADAGFIKQYGDCLGDIAARDLICAQKFNGLTVLPPLLTDEMIAQYTSALLAGTITSGWTFGAGAALQIPFAMQMAYRFNGIGVTQNVLYENQKLIANQFNSAIGKIQDSLSSTASALGKLQDVVNQNAQALNTLVKQLSSNFGAISSVLNDILSRLDPPEAEVQIDRLITGRLQSLQTYVTQQLIRAAEIRASANLAATKMSECVLGQSKRVDFCGKGYHLMSFPQSAPHGVVFLHVTYVPAQEKNFTTAPAICHDGKAHFPREGVFVSNGTHWFVTQRNFYEPQIITTDNTFVSGNCDVVIGIVNNTVYDPLQPELDSFKEELDKYFKNHTSPDVDLGDISGINASVVNIQKEIDRLNEVAKNLNESLIDLQELGKYEQYIKWPWYIWLGFIAGLIAIVMVTIMLCCMTSCCSCLKGCCSCGSCCKFDEDDSEPVLKGVKLHYT

SEQ ID NO: 130 - protein, 1273 aa, Artificial Sequence
  mutant spike protein of SARS-CoV-2 Wuhan variant comprising substitution Y505Q, 2-P-mutation (substiutions K986P and V987P) and inoperative furin cleavage site (substitution 682-QQAQ-685)
MFVFLVLLPLVSSQCVNLTTRTQLPPAYTNSFTRGVYYPDKVFRSSVLHSTQDLFLPFFSNVTWFHAIHVSGTNGTKRFDNPVLPFNDGVYFASTEKSNIIRGWIFGTTLDSKTQSLLIVNNATNVVIKVCEFQFCNDPFLGVYYHKNNKSWMESEFRVYSSANNCTFEYVSQPFLMDLEGKQGNFKNLREFVFKNIDGYFKIYSKHTPINLVRDLPQGFSALEPLVDLPIGINITRFQTLLALHRSYLTPGDSSSGWTAGAAAYYVGYLQPRTFLLKYNENGTITDAVDCALDPLSETKCTLKSFTVEKGIYQTSNFRVQPTESIVRFPNITNLCPFGEVFNATRFASVYAWNRKRISNCVADYSVLYNSASFSTFKCYGVSPTKLNDLCFTNVYADSFVIRGDEVRQIAPGQTGKIADYNYKLPDDFTGCVIAWNSNNLDSKVGGNYNYLYRLFRKSNLKPFERDISTEIYQAGSTPCNGVEGFNCYFPLQSYGFQPTNGVGQQPYRVVVLSFELLHAPATVCGPKKSTNLVKNKCVNFNFNGLTGTGVLTESNKKFLPFQQFGRDIADTTDAVRDPQTLEILDITPCSFGGVSVITPGTNTSNQVAVLYQDVNCTEVPVAIHADQLTPTWRVYSTGSNVFQTRAGCLIGAEHVNNSYECDIPIGAGICASYQTQTNSPQQAQSVASQSIIAYTMSLGAENSVAYSNNSIAIPTNFTISVTTEILPVSMTKTSVDCTMYICGDSTECSNLLLQYGSFCTQLNRALTGIAVEQDKNTQEVFAQVKQIYKTPPIKDFGGFNFSQILPDPSKPSKRSFIEDLLFNKVTLADAGFIKQYGDCLGDIAARDLICAQKFNGLTVLPPLLTDEMIAQYTSALLAGTITSGWTFGAGAALQIPFAMQMAYRFNGIGVTQNVLYENQKLIANQFNSAIGKIQDSLSSTASALGKLQDVVNQNAQALNTLVKQLSSNFGAISSVLNDILSRLDPPEAEVQIDRLITGRLQSLQTYVTQQLIRAAEIRASANLAATKMSECVLGQSKRVDFCGKGYHLMSFPQSAPHGVVFLHVTYVPAQEKNFTTAPAICHDGKAHFPREGVFVSNGTHWFVTQRNFYEPQIITTDNTFVSGNCDVVIGIVNNTVYDPLQPELDSFKEELDKYFKNHTSPDVDLGDISGINASVVNIQKEIDRLNEVAKNLNESLIDLQELGKYEQYIKWPWYIWLGFIAGLIAIVMVTIMLCCMTSCCSCLKGCCSCGSCCKFDEDDSEPVLKGVKLHYT

SEQ ID NO: 131 - protein, 1273 aa, Artificial Sequence
  mutant spike protein of SARS-CoV-2 Wuhan variant comprising substitution Y505R, 2-P-mutation (substiutions K986P and V987P) and inoperative furin cleavage site (substitution 682-QQAQ-685)
MFVFLVLLPLVSSQCVNLTTRTQLPPAYTNSFTRGVYYPDKVFRSSVLHSTQDLFLPFFSNVTWFHAIHVSGTNGTKRFDNPVLPFNDGVYFASTEKSNIIRGWIFGTTLDSKTQSLLIVNNATNVVIKVCEFQFCNDPFLGVYYHKNNKSWMESEFRVYSSANNCTFEYVSQPFLMDLEGKQGNFKNLREFVFKNIDGYFKIYSKHTPINLVRDLPQGFSALEPLVDLPIGINITRFQTLLALHRSYLTPGDSSSGWTAGAAAYYVGYLQPRTFLLKYNENGTITDAVDCALDPLSETKCTLKSFTVEKGIYQTSNFRVQPTESIVRFPNITNLCPFGEVFNATRFASVYAWNRKRISNCVADYSVLYNSASFSTFKCYGVSPTKLNDLCFTNVYADSFVIRGDEVRQIAPGQTGKIADYNYKLPDDFTGCVIAWNSNNLDSKVGGNYNYLYRLFRKSNLKPFERDISTEIYQAGSTPCNGVEGFNCYFPLQSYGFQPTNGVGRQPYRVVVLSFELLHAPATVCGPKKSTNLVKNKCVNFNFNGLTGTGVLTESNKKFLPFQQFGRDIADTTDAVRDPQTLEILDITPCSFGGVSVITPGTNTSNQVAVLYQDVNCTEVPVAIHADQLTPTWRVYSTGSNVFQTRAGCLIGAEHVNNSYECDIPIGAGICASYQTQTNSPQQAQSVASQSIIAYTMSLGAENSVAYSNNSIAIPTNFTISVTTEILPVSMTKTSVDCTMYICGDSTECSNLLLQYGSFCTQLNRALTGIAVEQDKNTQEVFAQVKQIYKTPPIKDFGGFNFSQILPDPSKPSKRSFIEDLLFNKVTLADAGFIKQYGDCLGDIAARDLICAQKFNGLTVLPPLLTDEMIAQYTSALLAGTITSGWTFGAGAALQIPFAMQMAYRFNGIGVTQNVLYENQKLIANQFNSAIGKIQDSLSSTASALGKLQDVVNQNAQALNTLVKQLSSNFGAISSVLNDILSRLDPPEAEVQIDRLITGRLQSLQTYVTQQLIRAAEIRASANLAATKMSECVLGQSKRVDFCGKGYHLMSFPQSAPHGVVFLHVTYVPAQEKNFTTAPAICHDGKAHFPREGVFVSNGTHWFVTQRNFYEPQIITTDNTFVSGNCDVVIGIVNNTVYDPLQPELDSFKEELDKYFKNHTSPDVDLGDISGINASVVNIQKEIDRLNEVAKNLNESLIDLQELGKYEQYIKWPWYIWLGFIAGLIAIVMVTIMLCCMTSCCSCLKGCCSCGSCCKFDEDDSEPVLKGVKLHYT

SEQ ID NO: 132 - protein, 1273 aa, Artificial Sequence
  mutant spike protein of SARS-CoV-2 Wuhan variant comprising substitution Y505S, 2-P-mutation (substiutions K986P and V987P) and inoperative furin cleavage site (substitution 682-QQAQ-685)
MFVFLVLLPLVSSQCVNLTTRTQLPPAYTNSFTRGVYYPDKVFRSSVLHSTQDLFLPFFSNVTWFHAIHVSGTNGTKRFDNPVLPFNDGVYFASTEKSNIIRGWIFGTTLDSKTQSLLIVNNATNVVIKVCEFQFCNDPFLGVYYHKNNKSWMESEFRVYSSANNCTFEYVSQPFLMDLEGKQGNFKNLREFVFKNIDGYFKIYSKHTPINLVRDLPQGFSALEPLVDLPIGINITRFQTLLALHRSYLTPGDSSSGWTAGAAAYYVGYLQPRTFLLKYNENGTITDAVDCALDPLSETKCTLKSFTVEKGIYQTSNFRVQPTESIVRFPNITNLCPFGEVFNATRFASVYAWNRKRISNCVADYSVLYNSASFSTFKCYGVSPTKLNDLCFTNVYADSFVIRGDEVRQIAPGQTGKIADYNYKLPDDFTGCVIAWNSNNLDSKVGGNYNYLYRLFRKSNLKPFERDISTEIYQAGSTPCNGVEGFNCYFPLQSYGFQPTNGVGSQPYRVVVLSFELLHAPATVCGPKKSTNLVKNKCVNFNFNGLTGTGVLTESNKKFLPFQQFGRDIADTTDAVRDPQTLEILDITPCSFGGVSVITPGTNTSNQVAVLYQDVNCTEVPVAIHADQLTPTWRVYSTGSNVFQTRAGCLIGAEHVNNSYECDIPIGAGICASYQTQTNSPQQAQSVASQSIIAYTMSLGAENSVAYSNNSIAIPTNFTISVTTEILPVSMTKTSVDCTMYICGDSTECSNLLLQYGSFCTQLNRALTGIAVEQDKNTQEVFAQVKQIYKTPPIKDFGGFNFSQILPDPSKPSKRSFIEDLLFNKVTLADAGFIKQYGDCLGDIAARDLICAQKFNGLTVLPPLLTDEMIAQYTSALLAGTITSGWTFGAGAALQIPFAMQMAYRFNGIGVTQNVLYENQKLIANQFNSAIGKIQDSLSSTASALGKLQDVVNQNAQALNTLVKQLSSNFGAISSVLNDILSRLDPPEAEVQIDRLITGRLQSLQTYVTQQLIRAAEIRASANLAATKMSECVLGQSKRVDFCGKGYHLMSFPQSAPHGVVFLHVTYVPAQEKNFTTAPAICHDGKAHFPREGVFVSNGTHWFVTQRNFYEPQIITTDNTFVSGNCDVVIGIVNNTVYDPLQPELDSFKEELDKYFKNHTSPDVDLGDISGINASVVNIQKEIDRLNEVAKNLNESLIDLQELGKYEQYIKWPWYIWLGFIAGLIAIVMVTIMLCCMTSCCSCLKGCCSCGSCCKFDEDDSEPVLKGVKLHYT

SEQ ID NO: 133 - protein, 1273 aa, Artificial Sequence
  mutant spike protein of SARS-CoV-2 Wuhan variant comprising substitution Y505T, 2-P-mutation (substiutions K986P and V987P) and inoperative furin cleavage site (substitution 682-QQAQ-685)
MFVFLVLLPLVSSQCVNLTTRTQLPPAYTNSFTRGVYYPDKVFRSSVLHSTQDLFLPFFSNVTWFHAIHVSGTNGTKRFDNPVLPFNDGVYFASTEKSNIIRGWIFGTTLDSKTQSLLIVNNATNVVIKVCEFQFCNDPFLGVYYHKNNKSWMESEFRVYSSANNCTFEYVSQPFLMDLEGKQGNFKNLREFVFKNIDGYFKIYSKHTPINLVRDLPQGFSALEPLVDLPIGINITRFQTLLALHRSYLTPGDSSSGWTAGAAAYYVGYLQPRTFLLKYNENGTITDAVDCALDPLSETKCTLKSFTVEKGIYQTSNFRVQPTESIVRFPNITNLCPFGEVFNATRFASVYAWNRKRISNCVADYSVLYNSASFSTFKCYGVSPTKLNDLCFTNVYADSFVIRGDEVRQIAPGQTGKIADYNYKLPDDFTGCVIAWNSNNLDSKVGGNYNYLYRLFRKSNLKPFERDISTEIYQAGSTPCNGVEGFNCYFPLQSYGFQPTNGVGTQPYRVVVLSFELLHAPATVCGPKKSTNLVKNKCVNFNFNGLTGTGVLTESNKKFLPFQQFGRDIADTTDAVRDPQTLEILDITPCSFGGVSVITPGTNTSNQVAVLYQDVNCTEVPVAIHADQLTPTWRVYSTGSNVFQTRAGCLIGAEHVNNSYECDIPIGAGICASYQTQTNSPQQAQSVASQSIIAYTMSLGAENSVAYSNNSIAIPTNFTISVTTEILPVSMTKTSVDCTMYICGDSTECSNLLLQYGSFCTQLNRALTGIAVEQDKNTQEVFAQVKQIYKTPPIKDFGGFNFSQILPDPSKPSKRSFIEDLLFNKVTLADAGFIKQYGDCLGDIAARDLICAQKFNGLTVLPPLLTDEMIAQYTSALLAGTITSGWTFGAGAALQIPFAMQMAYRFNGIGVTQNVLYENQKLIANQFNSAIGKIQDSLSSTASALGKLQDVVNQNAQALNTLVKQLSSNFGAISSVLNDILSRLDPPEAEVQIDRLITGRLQSLQTYVTQQLIRAAEIRASANLAATKMSECVLGQSKRVDFCGKGYHLMSFPQSAPHGVVFLHVTYVPAQEKNFTTAPAICHDGKAHFPREGVFVSNGTHWFVTQRNFYEPQIITTDNTFVSGNCDVVIGIVNNTVYDPLQPELDSFKEELDKYFKNHTSPDVDLGDISGINASVVNIQKEIDRLNEVAKNLNESLIDLQELGKYEQYIKWPWYIWLGFIAGLIAIVMVTIMLCCMTSCCSCLKGCCSCGSCCKFDEDDSEPVLKGVKLHYT

SEQ ID NO: 134 - protein, 1273 aa, Artificial Sequence
  mutant spike protein of SARS-CoV-2 Wuhan variant comprising substitution Y505V, 2-P-mutation (substiutions K986P and V987P) and inoperative furin cleavage site (substitution 682-QQAQ-685)
MFVFLVLLPLVSSQCVNLTTRTQLPPAYTNSFTRGVYYPDKVFRSSVLHSTQDLFLPFFSNVTWFHAIHVSGTNGTKRFDNPVLPFNDGVYFASTEKSNIIRGWIFGTTLDSKTQSLLIVNNATNVVIKVCEFQFCNDPFLGVYYHKNNKSWMESEFRVYSSANNCTFEYVSQPFLMDLEGKQGNFKNLREFVFKNIDGYFKIYSKHTPINLVRDLPQGFSALEPLVDLPIGINITRFQTLLALHRSYLTPGDSSSGWTAGAAAYYVGYLQPRTFLLKYNENGTITDAVDCALDPLSETKCTLKSFTVEKGIYQTSNFRVQPTESIVRFPNITNLCPFGEVFNATRFASVYAWNRKRISNCVADYSVLYNSASFSTFKCYGVSPTKLNDLCFTNVYADSFVIRGDEVRQIAPGQTGKIADYNYKLPDDFTGCVIAWNSNNLDSKVGGNYNYLYRLFRKSNLKPFERDISTEIYQAGSTPCNGVEGFNCYFPLQSYGFQPTNGVGVQPYRVVVLSFELLHAPATVCGPKKSTNLVKNKCVNFNFNGLTGTGVLTESNKKFLPFQQFGRDIADTTDAVRDPQTLEILDITPCSFGGVSVITPGTNTSNQVAVLYQDVNCTEVPVAIHADQLTPTWRVYSTGSNVFQTRAGCLIGAEHVNNSYECDIPIGAGICASYQTQTNSPQQAQSVASQSIIAYTMSLGAENSVAYSNNSIAIPTNFTISVTTEILPVSMTKTSVDCTMYICGDSTECSNLLLQYGSFCTQLNRALTGIAVEQDKNTQEVFAQVKQIYKTPPIKDFGGFNFSQILPDPSKPSKRSFIEDLLFNKVTLADAGFIKQYGDCLGDIAARDLICAQKFNGLTVLPPLLTDEMIAQYTSALLAGTITSGWTFGAGAALQIPFAMQMAYRFNGIGVTQNVLYENQKLIANQFNSAIGKIQDSLSSTASALGKLQDVVNQNAQALNTLVKQLSSNFGAISSVLNDILSRLDPPEAEVQIDRLITGRLQSLQTYVTQQLIRAAEIRASANLAATKMSECVLGQSKRVDFCGKGYHLMSFPQSAPHGVVFLHVTYVPAQEKNFTTAPAICHDGKAHFPREGVFVSNGTHWFVTQRNFYEPQIITTDNTFVSGNCDVVIGIVNNTVYDPLQPELDSFKEELDKYFKNHTSPDVDLGDISGINASVVNIQKEIDRLNEVAKNLNESLIDLQELGKYEQYIKWPWYIWLGFIAGLIAIVMVTIMLCCMTSCCSCLKGCCSCGSCCKFDEDDSEPVLKGVKLHYT

SEQ ID NO: 135 - protein, 1273 aa, Artificial Sequence
  mutant spike protein of SARS-CoV-2 Wuhan variant comprising substitution F456A, 2-P-mutation (substiutions K986P and V987P) and inoperative furin cleavage site (substitution 682-QQAQ-685)
MFVFLVLLPLVSSQCVNLTTRTQLPPAYTNSFTRGVYYPDKVFRSSVLHSTQDLFLPFFSNVTWFHAIHVSGTNGTKRFDNPVLPFNDGVYFASTEKSNIIRGWIFGTTLDSKTQSLLIVNNATNVVIKVCEFQFCNDPFLGVYYHKNNKSWMESEFRVYSSANNCTFEYVSQPFLMDLEGKQGNFKNLREFVFKNIDGYFKIYSKHTPINLVRDLPQGFSALEPLVDLPIGINITRFQTLLALHRSYLTPGDSSSGWTAGAAAYYVGYLQPRTFLLKYNENGTITDAVDCALDPLSETKCTLKSFTVEKGIYQTSNFRVQPTESIVRFPNITNLCPFGEVFNATRFASVYAWNRKRISNCVADYSVLYNSASFSTFKCYGVSPTKLNDLCFTNVYADSFVIRGDEVRQIAPGQTGKIADYNYKLPDDFTGCVIAWNSNNLDSKVGGNYNYLYRLARKSNLKPFERDISTEIYQAGSTPCNGVEGFNCYFPLQSYGFQPTNGVGYQPYRVVVLSFELLHAPATVCGPKKSTNLVKNKCVNFNFNGLTGTGVLTESNKKFLPFQQFGRDIADTTDAVRDPQTLEILDITPCSFGGVSVITPGTNTSNQVAVLYQDVNCTEVPVAIHADQLTPTWRVYSTGSNVFQTRAGCLIGAEHVNNSYECDIPIGAGICASYQTQTNSPQQAQSVASQSIIAYTMSLGAENSVAYSNNSIAIPTNFTISVTTEILPVSMTKTSVDCTMYICGDSTECSNLLLQYGSFCTQLNRALTGIAVEQDKNTQEVFAQVKQIYKTPPIKDFGGFNFSQILPDPSKPSKRSFIEDLLFNKVTLADAGFIKQYGDCLGDIAARDLICAQKFNGLTVLPPLLTDEMIAQYTSALLAGTITSGWTFGAGAALQIPFAMQMAYRFNGIGVTQNVLYENQKLIANQFNSAIGKIQDSLSSTASALGKLQDVVNQNAQALNTLVKQLSSNFGAISSVLNDILSRLDPPEAEVQIDRLITGRLQSLQTYVTQQLIRAAEIRASANLAATKMSECVLGQSKRVDFCGKGYHLMSFPQSAPHGVVFLHVTYVPAQEKNFTTAPAICHDGKAHFPREGVFVSNGTHWFVTQRNFYEPQIITTDNTFVSGNCDVVIGIVNNTVYDPLQPELDSFKEELDKYFKNHTSPDVDLGDISGINASVVNIQKEIDRLNEVAKNLNESLIDLQELGKYEQYIKWPWYIWLGFIAGLIAIVMVTIMLCCMTSCCSCLKGCCSCGSCCKFDEDDSEPVLKGVKLHYT

SEQ ID NO: 136 - protein, 1273 aa, Artificial Sequence
  mutant spike protein of SARS-CoV-2 Wuhan variant comprising substitution F456C, 2-P-mutation (substiutions K986P and V987P) and inoperative furin cleavage site (substitution 682-QQAQ-685)
MFVFLVLLPLVSSQCVNLTTRTQLPPAYTNSFTRGVYYPDKVFRSSVLHSTQDLFLPFFSNVTWFHAIHVSGTNGTKRFDNPVLPFNDGVYFASTEKSNIIRGWIFGTTLDSKTQSLLIVNNATNVVIKVCEFQFCNDPFLGVYYHKNNKSWMESEFRVYSSANNCTFEYVSQPFLMDLEGKQGNFKNLREFVFKNIDGYFKIYSKHTPINLVRDLPQGFSALEPLVDLPIGINITRFQTLLALHRSYLTPGDSSSGWTAGAAAYYVGYLQPRTFLLKYNENGTITDAVDCALDPLSETKCTLKSFTVEKGIYQTSNFRVQPTESIVRFPNITNLCPFGEVFNATRFASVYAWNRKRISNCVADYSVLYNSASFSTFKCYGVSPTKLNDLCFTNVYADSFVIRGDEVRQIAPGQTGKIADYNYKLPDDFTGCVIAWNSNNLDSKVGGNYNYLYRLCRKSNLKPFERDISTEIYQAGSTPCNGVEGFNCYFPLQSYGFQPTNGVGYQPYRVVVLSFELLHAPATVCGPKKSTNLVKNKCVNFNFNGLTGTGVLTESNKKFLPFQQFGRDIADTTDAVRDPQTLEILDITPCSFGGVSVITPGTNTSNQVAVLYQDVNCTEVPVAIHADQLTPTWRVYSTGSNVFQTRAGCLIGAEHVNNSYECDIPIGAGICASYQTQTNSPQQAQSVASQSIIAYTMSLGAENSVAYSNNSIAIPTNFTISVTTEILPVSMTKTSVDCTMYICGDSTECSNLLLQYGSFCTQLNRALTGIAVEQDKNTQEVFAQVKQIYKTPPIKDFGGFNFSQILPDPSKPSKRSFIEDLLFNKVTLADAGFIKQYGDCLGDIAARDLICAQKFNGLTVLPPLLTDEMIAQYTSALLAGTITSGWTFGAGAALQIPFAMQMAYRFNGIGVTQNVLYENQKLIANQFNSAIGKIQDSLSSTASALGKLQDVVNQNAQALNTLVKQLSSNFGAISSVLNDILSRLDPPEAEVQIDRLITGRLQSLQTYVTQQLIRAAEIRASANLAATKMSECVLGQSKRVDFCGKGYHLMSFPQSAPHGVVFLHVTYVPAQEKNFTTAPAICHDGKAHFPREGVFVSNGTHWFVTQRNFYEPQIITTDNTFVSGNCDVVIGIVNNTVYDPLQPELDSFKEELDKYFKNHTSPDVDLGDISGINASVVNIQKEIDRLNEVAKNLNESLIDLQELGKYEQYIKWPWYIWLGFIAGLIAIVMVTIMLCCMTSCCSCLKGCCSCGSCCKFDEDDSEPVLKGVKLHYT

SEQ ID NO: 137 - protein, 1273 aa, Artificial Sequence
  mutant spike protein of SARS-CoV-2 Wuhan variant comprising substitution F456YE, 2-P-mutation (substiutions K986P and V987P) and inoperative furin cleavage site (substitution 682-QQAQ-685)
MFVFLVLLPLVSSQCVNLTTRTQLPPAYTNSFTRGVYYPDKVFRSSVLHSTQDLFLPFFSNVTWFHAIHVSGTNGTKRFDNPVLPFNDGVYFASTEKSNIIRGWIFGTTLDSKTQSLLIVNNATNVVIKVCEFQFCNDPFLGVYYHKNNKSWMESEFRVYSSANNCTFEYVSQPFLMDLEGKQGNFKNLREFVFKNIDGYFKIYSKHTPINLVRDLPQGFSALEPLVDLPIGINITRFQTLLALHRSYLTPGDSSSGWTAGAAAYYVGYLQPRTFLLKYNENGTITDAVDCALDPLSETKCTLKSFTVEKGIYQTSNFRVQPTESIVRFPNITNLCPFGEVFNATRFASVYAWNRKRISNCVADYSVLYNSASFSTFKCYGVSPTKLNDLCFTNVYADSFVIRGDEVRQIAPGQTGKIADYNYKLPDDFTGCVIAWNSNNLDSKVGGNYNYLYRLERKSNLKPFERDISTEIYQAGSTPCNGVEGFNCYFPLQSYGFQPTNGVGYQPYRVVVLSFELLHAPATVCGPKKSTNLVKNKCVNFNFNGLTGTGVLTESNKKFLPFQQFGRDIADTTDAVRDPQTLEILDITPCSFGGVSVITPGTNTSNQVAVLYQDVNCTEVPVAIHADQLTPTWRVYSTGSNVFQTRAGCLIGAEHVNNSYECDIPIGAGICASYQTQTNSPQQAQSVASQSIIAYTMSLGAENSVAYSNNSIAIPTNFTISVTTEILPVSMTKTSVDCTMYICGDSTECSNLLLQYGSFCTQLNRALTGIAVEQDKNTQEVFAQVKQIYKTPPIKDFGGFNFSQILPDPSKPSKRSFIEDLLFNKVTLADAGFIKQYGDCLGDIAARDLICAQKFNGLTVLPPLLTDEMIAQYTSALLAGTITSGWTFGAGAALQIPFAMQMAYRFNGIGVTQNVLYENQKLIANQFNSAIGKIQDSLSSTASALGKLQDVVNQNAQALNTLVKQLSSNFGAISSVLNDILSRLDPPEAEVQIDRLITGRLQSLQTYVTQQLIRAAEIRASANLAATKMSECVLGQSKRVDFCGKGYHLMSFPQSAPHGVVFLHVTYVPAQEKNFTTAPAICHDGKAHFPREGVFVSNGTHWFVTQRNFYEPQIITTDNTFVSGNCDVVIGIVNNTVYDPLQPELDSFKEELDKYFKNHTSPDVDLGDISGINASVVNIQKEIDRLNEVAKNLNESLIDLQELGKYEQYIKWPWYIWLGFIAGLIAIVMVTIMLCCMTSCCSCLKGCCSCGSCCKFDEDDSEPVLKGVKLHYT

SEQ ID NO: 138 - protein, 1273 aa, Artificial Sequence
  mutant spike protein of SARS-CoV-2 Wuhan variant comprising substitution F456G, 2-P-mutation (substiutions K986P and V987P) and inoperative furin cleavage site (substitution 682-QQAQ-685)
MFVFLVLLPLVSSQCVNLTTRTQLPPAYTNSFTRGVYYPDKVFRSSVLHSTQDLFLPFFSNVTWFHAIHVSGTNGTKRFDNPVLPFNDGVYFASTEKSNIIRGWIFGTTLDSKTQSLLIVNNATNVVIKVCEFQFCNDPFLGVYYHKNNKSWMESEFRVYSSANNCTFEYVSQPFLMDLEGKQGNFKNLREFVFKNIDGYFKIYSKHTPINLVRDLPQGFSALEPLVDLPIGINITRFQTLLALHRSYLTPGDSSSGWTAGAAAYYVGYLQPRTFLLKYNENGTITDAVDCALDPLSETKCTLKSFTVEKGIYQTSNFRVQPTESIVRFPNITNLCPFGEVFNATRFASVYAWNRKRISNCVADYSVLYNSASFSTFKCYGVSPTKLNDLCFTNVYADSFVIRGDEVRQIAPGQTGKIADYNYKLPDDFTGCVIAWNSNNLDSKVGGNYNYLYRLGRKSNLKPFERDISTEIYQAGSTPCNGVEGFNCYFPLQSYGFQPTNGVGYQPYRVVVLSFELLHAPATVCGPKKSTNLVKNKCVNFNFNGLTGTGVLTESNKKFLPFQQFGRDIADTTDAVRDPQTLEILDITPCSFGGVSVITPGTNTSNQVAVLYQDVNCTEVPVAIHADQLTPTWRVYSTGSNVFQTRAGCLIGAEHVNNSYECDIPIGAGICASYQTQTNSPQQAQSVASQSIIAYTMSLGAENSVAYSNNSIAIPTNFTISVTTEILPVSMTKTSVDCTMYICGDSTECSNLLLQYGSFCTQLNRALTGIAVEQDKNTQEVFAQVKQIYKTPPIKDFGGFNFSQILPDPSKPSKRSFIEDLLFNKVTLADAGFIKQYGDCLGDIAARDLICAQKFNGLTVLPPLLTDEMIAQYTSALLAGTITSGWTFGAGAALQIPFAMQMAYRFNGIGVTQNVLYENQKLIANQFNSAIGKIQDSLSSTASALGKLQDVVNQNAQALNTLVKQLSSNFGAISSVLNDILSRLDPPEAEVQIDRLITGRLQSLQTYVTQQLIRAAEIRASANLAATKMSECVLGQSKRVDFCGKGYHLMSFPQSAPHGVVFLHVTYVPAQEKNFTTAPAICHDGKAHFPREGVFVSNGTHWFVTQRNFYEPQIITTDNTFVSGNCDVVIGIVNNTVYDPLQPELDSFKEELDKYFKNHTSPDVDLGDISGINASVVNIQKEIDRLNEVAKNLNESLIDLQELGKYEQYIKWPWYIWLGFIAGLIAIVMVTIMLCCMTSCCSCLKGCCSCGSCCKFDEDDSEPVLKGVKLHYT

SEQ ID NO: 139 - protein, 1273 aa, Artificial Sequence
  mutant spike protein of SARS-CoV-2 Wuhan variant comprising substitution F456I, 2-P-mutation (substiutions K986P and V987P) and inoperative furin cleavage site (substitution 682-QQAQ-685)
MFVFLVLLPLVSSQCVNLTTRTQLPPAYTNSFTRGVYYPDKVFRSSVLHSTQDLFLPFFSNVTWFHAIHVSGTNGTKRFDNPVLPFNDGVYFASTEKSNIIRGWIFGTTLDSKTQSLLIVNNATNVVIKVCEFQFCNDPFLGVYYHKNNKSWMESEFRVYSSANNCTFEYVSQPFLMDLEGKQGNFKNLREFVFKNIDGYFKIYSKHTPINLVRDLPQGFSALEPLVDLPIGINITRFQTLLALHRSYLTPGDSSSGWTAGAAAYYVGYLQPRTFLLKYNENGTITDAVDCALDPLSETKCTLKSFTVEKGIYQTSNFRVQPTESIVRFPNITNLCPFGEVFNATRFASVYAWNRKRISNCVADYSVLYNSASFSTFKCYGVSPTKLNDLCFTNVYADSFVIRGDEVRQIAPGQTGKIADYNYKLPDDFTGCVIAWNSNNLDSKVGGNYNYLYRLIRKSNLKPFERDISTEIYQAGSTPCNGVEGFNCYFPLQSYGFQPTNGVGYQPYRVVVLSFELLHAPATVCGPKKSTNLVKNKCVNFNFNGLTGTGVLTESNKKFLPFQQFGRDIADTTDAVRDPQTLEILDITPCSFGGVSVITPGTNTSNQVAVLYQDVNCTEVPVAIHADQLTPTWRVYSTGSNVFQTRAGCLIGAEHVNNSYECDIPIGAGICASYQTQTNSPQQAQSVASQSIIAYTMSLGAENSVAYSNNSIAIPTNFTISVTTEILPVSMTKTSVDCTMYICGDSTECSNLLLQYGSFCTQLNRALTGIAVEQDKNTQEVFAQVKQIYKTPPIKDFGGFNFSQILPDPSKPSKRSFIEDLLFNKVTLADAGFIKQYGDCLGDIAARDLICAQKFNGLTVLPPLLTDEMIAQYTSALLAGTITSGWTFGAGAALQIPFAMQMAYRFNGIGVTQNVLYENQKLIANQFNSAIGKIQDSLSSTASALGKLQDVVNQNAQALNTLVKQLSSNFGAISSVLNDILSRLDPPEAEVQIDRLITGRLQSLQTYVTQQLIRAAEIRASANLAATKMSECVLGQSKRVDFCGKGYHLMSFPQSAPHGVVFLHVTYVPAQEKNFTTAPAICHDGKAHFPREGVFVSNGTHWFVTQRNFYEPQIITTDNTFVSGNCDVVIGIVNNTVYDPLQPELDSFKEELDKYFKNHTSPDVDLGDISGINASVVNIQKEIDRLNEVAKNLNESLIDLQELGKYEQYIKWPWYIWLGFIAGLIAIVMVTIMLCCMTSCCSCLKGCCSCGSCCKFDEDDSEPVLKGVKLHYT

SEQ ID NO: 140 - protein, 1273 aa, Artificial Sequence
  mutant spike protein of SARS-CoV-2 Wuhan variant comprising substitution F456K, 2-P-mutation (substiutions K986P and V987P) and inoperative furin cleavage site (substitution 682-QQAQ-685)
MFVFLVLLPLVSSQCVNLTTRTQLPPAYTNSFTRGVYYPDKVFRSSVLHSTQDLFLPFFSNVTWFHAIHVSGTNGTKRFDNPVLPFNDGVYFASTEKSNIIRGWIFGTTLDSKTQSLLIVNNATNVVIKVCEFQFCNDPFLGVYYHKNNKSWMESEFRVYSSANNCTFEYVSQPFLMDLEGKQGNFKNLREFVFKNIDGYFKIYSKHTPINLVRDLPQGFSALEPLVDLPIGINITRFQTLLALHRSYLTPGDSSSGWTAGAAAYYVGYLQPRTFLLKYNENGTITDAVDCALDPLSETKCTLKSFTVEKGIYQTSNFRVQPTESIVRFPNITNLCPFGEVFNATRFASVYAWNRKRISNCVADYSVLYNSASFSTFKCYGVSPTKLNDLCFTNVYADSFVIRGDEVRQIAPGQTGKIADYNYKLPDDFTGCVIAWNSNNLDSKVGGNYNYLYRLKRKSNLKPFERDISTEIYQAGSTPCNGVEGFNCYFPLQSYGFQPTNGVGYQPYRVVVLSFELLHAPATVCGPKKSTNLVKNKCVNFNFNGLTGTGVLTESNKKFLPFQQFGRDIADTTDAVRDPQTLEILDITPCSFGGVSVITPGTNTSNQVAVLYQDVNCTEVPVAIHADQLTPTWRVYSTGSNVFQTRAGCLIGAEHVNNSYECDIPIGAGICASYQTQTNSPQQAQSVASQSIIAYTMSLGAENSVAYSNNSIAIPTNFTISVTTEILPVSMTKTSVDCTMYICGDSTECSNLLLQYGSFCTQLNRALTGIAVEQDKNTQEVFAQVKQIYKTPPIKDFGGFNFSQILPDPSKPSKRSFIEDLLFNKVTLADAGFIKQYGDCLGDIAARDLICAQKFNGLTVLPPLLTDEMIAQYTSALLAGTITSGWTFGAGAALQIPFAMQMAYRFNGIGVTQNVLYENQKLIANQFNSAIGKIQDSLSSTASALGKLQDVVNQNAQALNTLVKQLSSNFGAISSVLNDILSRLDPPEAEVQIDRLITGRLQSLQTYVTQQLIRAAEIRASANLAATKMSECVLGQSKRVDFCGKGYHLMSFPQSAPHGVVFLHVTYVPAQEKNFTTAPAICHDGKAHFPREGVFVSNGTHWFVTQRNFYEPQIITTDNTFVSGNCDVVIGIVNNTVYDPLQPELDSFKEELDKYFKNHTSPDVDLGDISGINASVVNIQKEIDRLNEVAKNLNESLIDLQELGKYEQYIKWPWYIWLGFIAGLIAIVMVTIMLCCMTSCCSCLKGCCSCGSCCKFDEDDSEPVLKGVKLHYT

SEQ ID NO: 141 - protein, 1273 aa, Artificial Sequence
  mutant spike protein of SARS-CoV-2 Wuhan variant comprising substitution F456N, 2-P-mutation (substiutions K986P and V987P) and inoperative furin cleavage site (substitution 682-QQAQ-685)
MFVFLVLLPLVSSQCVNLTTRTQLPPAYTNSFTRGVYYPDKVFRSSVLHSTQDLFLPFFSNVTWFHAIHVSGTNGTKRFDNPVLPFNDGVYFASTEKSNIIRGWIFGTTLDSKTQSLLIVNNATNVVIKVCEFQFCNDPFLGVYYHKNNKSWMESEFRVYSSANNCTFEYVSQPFLMDLEGKQGNFKNLREFVFKNIDGYFKIYSKHTPINLVRDLPQGFSALEPLVDLPIGINITRFQTLLALHRSYLTPGDSSSGWTAGAAAYYVGYLQPRTFLLKYNENGTITDAVDCALDPLSETKCTLKSFTVEKGIYQTSNFRVQPTESIVRFPNITNLCPFGEVFNATRFASVYAWNRKRISNCVADYSVLYNSASFSTFKCYGVSPTKLNDLCFTNVYADSFVIRGDEVRQIAPGQTGKIADYNYKLPDDFTGCVIAWNSNNLDSKVGGNYNYLYRLNRKSNLKPFERDISTEIYQAGSTPCNGVEGFNCYFPLQSYGFQPTNGVGYQPYRVVVLSFELLHAPATVCGPKKSTNLVKNKCVNFNFNGLTGTGVLTESNKKFLPFQQFGRDIADTTDAVRDPQTLEILDITPCSFGGVSVITPGTNTSNQVAVLYQDVNCTEVPVAIHADQLTPTWRVYSTGSNVFQTRAGCLIGAEHVNNSYECDIPIGAGICASYQTQTNSPQQAQSVASQSIIAYTMSLGAENSVAYSNNSIAIPTNFTISVTTEILPVSMTKTSVDCTMYICGDSTECSNLLLQYGSFCTQLNRALTGIAVEQDKNTQEVFAQVKQIYKTPPIKDFGGFNFSQILPDPSKPSKRSFIEDLLFNKVTLADAGFIKQYGDCLGDIAARDLICAQKFNGLTVLPPLLTDEMIAQYTSALLAGTITSGWTFGAGAALQIPFAMQMAYRFNGIGVTQNVLYENQKLIANQFNSAIGKIQDSLSSTASALGKLQDVVNQNAQALNTLVKQLSSNFGAISSVLNDILSRLDPPEAEVQIDRLITGRLQSLQTYVTQQLIRAAEIRASANLAATKMSECVLGQSKRVDFCGKGYHLMSFPQSAPHGVVFLHVTYVPAQEKNFTTAPAICHDGKAHFPREGVFVSNGTHWFVTQRNFYEPQIITTDNTFVSGNCDVVIGIVNNTVYDPLQPELDSFKEELDKYFKNHTSPDVDLGDISGINASVVNIQKEIDRLNEVAKNLNESLIDLQELGKYEQYIKWPWYIWLGFIAGLIAIVMVTIMLCCMTSCCSCLKGCCSCGSCCKFDEDDSEPVLKGVKLHYT

SEQ ID NO: 142 - protein, 1273 aa, Artificial Sequence
  mutant spike protein of SARS-CoV-2 Wuhan variant comprising substitution F456Q, 2-P-mutation (substiutions K986P and V987P) and inoperative furin cleavage site (substitution 682-QQAQ-685)
MFVFLVLLPLVSSQCVNLTTRTQLPPAYTNSFTRGVYYPDKVFRSSVLHSTQDLFLPFFSNVTWFHAIHVSGTNGTKRFDNPVLPFNDGVYFASTEKSNIIRGWIFGTTLDSKTQSLLIVNNATNVVIKVCEFQFCNDPFLGVYYHKNNKSWMESEFRVYSSANNCTFEYVSQPFLMDLEGKQGNFKNLREFVFKNIDGYFKIYSKHTPINLVRDLPQGFSALEPLVDLPIGINITRFQTLLALHRSYLTPGDSSSGWTAGAAAYYVGYLQPRTFLLKYNENGTITDAVDCALDPLSETKCTLKSFTVEKGIYQTSNFRVQPTESIVRFPNITNLCPFGEVFNATRFASVYAWNRKRISNCVADYSVLYNSASFSTFKCYGVSPTKLNDLCFTNVYADSFVIRGDEVRQIAPGQTGKIADYNYKLPDDFTGCVIAWNSNNLDSKVGGNYNYLYRLQRKSNLKPFERDISTEIYQAGSTPCNGVEGFNCYFPLQSYGFQPTNGVGYQPYRVVVLSFELLHAPATVCGPKKSTNLVKNKCVNFNFNGLTGTGVLTESNKKFLPFQQFGRDIADTTDAVRDPQTLEILDITPCSFGGVSVITPGTNTSNQVAVLYQDVNCTEVPVAIHADQLTPTWRVYSTGSNVFQTRAGCLIGAEHVNNSYECDIPIGAGICASYQTQTNSPQQAQSVASQSIIAYTMSLGAENSVAYSNNSIAIPTNFTISVTTEILPVSMTKTSVDCTMYICGDSTECSNLLLQYGSFCTQLNRALTGIAVEQDKNTQEVFAQVKQIYKTPPIKDFGGFNFSQILPDPSKPSKRSFIEDLLFNKVTLADAGFIKQYGDCLGDIAARDLICAQKFNGLTVLPPLLTDEMIAQYTSALLAGTITSGWTFGAGAALQIPFAMQMAYRFNGIGVTQNVLYENQKLIANQFNSAIGKIQDSLSSTASALGKLQDVVNQNAQALNTLVKQLSSNFGAISSVLNDILSRLDPPEAEVQIDRLITGRLQSLQTYVTQQLIRAAEIRASANLAATKMSECVLGQSKRVDFCGKGYHLMSFPQSAPHGVVFLHVTYVPAQEKNFTTAPAICHDGKAHFPREGVFVSNGTHWFVTQRNFYEPQIITTDNTFVSGNCDVVIGIVNNTVYDPLQPELDSFKEELDKYFKNHTSPDVDLGDISGINASVVNIQKEIDRLNEVAKNLNESLIDLQELGKYEQYIKWPWYIWLGFIAGLIAIVMVTIMLCCMTSCCSCLKGCCSCGSCCKFDEDDSEPVLKGVKLHYT

SEQ ID NO: 143 - protein, 1273 aa, Artificial Sequence
  mutant spike protein of SARS-CoV-2 Wuhan variant comprising substitution F456R, 2-P-mutation (substiutions K986P and V987P) and inoperative furin cleavage site (substitution 682-QQAQ-685)
MFVFLVLLPLVSSQCVNLTTRTQLPPAYTNSFTRGVYYPDKVFRSSVLHSTQDLFLPFFSNVTWFHAIHVSGTNGTKRFDNPVLPFNDGVYFASTEKSNIIRGWIFGTTLDSKTQSLLIVNNATNVVIKVCEFQFCNDPFLGVYYHKNNKSWMESEFRVYSSANNCTFEYVSQPFLMDLEGKQGNFKNLREFVFKNIDGYFKIYSKHTPINLVRDLPQGFSALEPLVDLPIGINITRFQTLLALHRSYLTPGDSSSGWTAGAAAYYVGYLQPRTFLLKYNENGTITDAVDCALDPLSETKCTLKSFTVEKGIYQTSNFRVQPTESIVRFPNITNLCPFGEVFNATRFASVYAWNRKRISNCVADYSVLYNSASFSTFKCYGVSPTKLNDLCFTNVYADSFVIRGDEVRQIAPGQTGKIADYNYKLPDDFTGCVIAWNSNNLDSKVGGNYNYLYRLRRKSNLKPFERDISTEIYQAGSTPCNGVEGFNCYFPLQSYGFQPTNGVGYQPYRVVVLSFELLHAPATVCGPKKSTNLVKNKCVNFNFNGLTGTGVLTESNKKFLPFQQFGRDIADTTDAVRDPQTLEILDITPCSFGGVSVITPGTNTSNQVAVLYQDVNCTEVPVAIHADQLTPTWRVYSTGSNVFQTRAGCLIGAEHVNNSYECDIPIGAGICASYQTQTNSPQQAQSVASQSIIAYTMSLGAENSVAYSNNSIAIPTNFTISVTTEILPVSMTKTSVDCTMYICGDSTECSNLLLQYGSFCTQLNRALTGIAVEQDKNTQEVFAQVKQIYKTPPIKDFGGFNFSQILPDPSKPSKRSFIEDLLFNKVTLADAGFIKQYGDCLGDIAARDLICAQKFNGLTVLPPLLTDEMIAQYTSALLAGTITSGWTFGAGAALQIPFAMQMAYRFNGIGVTQNVLYENQKLIANQFNSAIGKIQDSLSSTASALGKLQDVVNQNAQALNTLVKQLSSNFGAISSVLNDILSRLDPPEAEVQIDRLITGRLQSLQTYVTQQLIRAAEIRASANLAATKMSECVLGQSKRVDFCGKGYHLMSFPQSAPHGVVFLHVTYVPAQEKNFTTAPAICHDGKAHFPREGVFVSNGTHWFVTQRNFYEPQIITTDNTFVSGNCDVVIGIVNNTVYDPLQPELDSFKEELDKYFKNHTSPDVDLGDISGINASVVNIQKEIDRLNEVAKNLNESLIDLQELGKYEQYIKWPWYIWLGFIAGLIAIVMVTIMLCCMTSCCSCLKGCCSCGSCCKFDEDDSEPVLKGVKLHYT

SEQ ID NO: 144 - protein, 1273 aa, Artificial Sequence
  mutant spike protein of SARS-CoV-2 Wuhan variant comprising substitution F456S, 2-P-mutation (substiutions K986P and V987P) and inoperative furin cleavage site (substitution 682-QQAQ-685)
MFVFLVLLPLVSSQCVNLTTRTQLPPAYTNSFTRGVYYPDKVFRSSVLHSTQDLFLPFFSNVTWFHAIHVSGTNGTKRFDNPVLPFNDGVYFASTEKSNIIRGWIFGTTLDSKTQSLLIVNNATNVVIKVCEFQFCNDPFLGVYYHKNNKSWMESEFRVYSSANNCTFEYVSQPFLMDLEGKQGNFKNLREFVFKNIDGYFKIYSKHTPINLVRDLPQGFSALEPLVDLPIGINITRFQTLLALHRSYLTPGDSSSGWTAGAAAYYVGYLQPRTFLLKYNENGTITDAVDCALDPLSETKCTLKSFTVEKGIYQTSNFRVQPTESIVRFPNITNLCPFGEVFNATRFASVYAWNRKRISNCVADYSVLYNSASFSTFKCYGVSPTKLNDLCFTNVYADSFVIRGDEVRQIAPGQTGKIADYNYKLPDDFTGCVIAWNSNNLDSKVGGNYNYLYRLSRKSNLKPFERDISTEIYQAGSTPCNGVEGFNCYFPLQSYGFQPTNGVGYQPYRVVVLSFELLHAPATVCGPKKSTNLVKNKCVNFNFNGLTGTGVLTESNKKFLPFQQFGRDIADTTDAVRDPQTLEILDITPCSFGGVSVITPGTNTSNQVAVLYQDVNCTEVPVAIHADQLTPTWRVYSTGSNVFQTRAGCLIGAEHVNNSYECDIPIGAGICASYQTQTNSPQQAQSVASQSIIAYTMSLGAENSVAYSNNSIAIPTNFTISVTTEILPVSMTKTSVDCTMYICGDSTECSNLLLQYGSFCTQLNRALTGIAVEQDKNTQEVFAQVKQIYKTPPIKDFGGFNFSQILPDPSKPSKRSFIEDLLFNKVTLADAGFIKQYGDCLGDIAARDLICAQKFNGLTVLPPLLTDEMIAQYTSALLAGTITSGWTFGAGAALQIPFAMQMAYRFNGIGVTQNVLYENQKLIANQFNSAIGKIQDSLSSTASALGKLQDVVNQNAQALNTLVKQLSSNFGAISSVLNDILSRLDPPEAEVQIDRLITGRLQSLQTYVTQQLIRAAEIRASANLAATKMSECVLGQSKRVDFCGKGYHLMSFPQSAPHGVVFLHVTYVPAQEKNFTTAPAICHDGKAHFPREGVFVSNGTHWFVTQRNFYEPQIITTDNTFVSGNCDVVIGIVNNTVYDPLQPELDSFKEELDKYFKNHTSPDVDLGDISGINASVVNIQKEIDRLNEVAKNLNESLIDLQELGKYEQYIKWPWYIWLGFIAGLIAIVMVTIMLCCMTSCCSCLKGCCSCGSCCKFDEDDSEPVLKGVKLHYT

SEQ ID NO: 145 - protein, 1273 aa, Artificial Sequence
  mutant spike protein of SARS-CoV-2 Wuhan variant comprising substitution F456T, 2-P-mutation (substiutions K986P and V987P) and inoperative furin cleavage site (substitution 682-QQAQ-685)
MFVFLVLLPLVSSQCVNLTTRTQLPPAYTNSFTRGVYYPDKVFRSSVLHSTQDLFLPFFSNVTWFHAIHVSGTNGTKRFDNPVLPFNDGVYFASTEKSNIIRGWIFGTTLDSKTQSLLIVNNATNVVIKVCEFQFCNDPFLGVYYHKNNKSWMESEFRVYSSANNCTFEYVSQPFLMDLEGKQGNFKNLREFVFKNIDGYFKIYSKHTPINLVRDLPQGFSALEPLVDLPIGINITRFQTLLALHRSYLTPGDSSSGWTAGAAAYYVGYLQPRTFLLKYNENGTITDAVDCALDPLSETKCTLKSFTVEKGIYQTSNFRVQPTESIVRFPNITNLCPFGEVFNATRFASVYAWNRKRISNCVADYSVLYNSASFSTFKCYGVSPTKLNDLCFTNVYADSFVIRGDEVRQIAPGQTGKIADYNYKLPDDFTGCVIAWNSNNLDSKVGGNYNYLYRLTRKSNLKPFERDISTEIYQAGSTPCNGVEGFNCYFPLQSYGFQPTNGVGYQPYRVVVLSFELLHAPATVCGPKKSTNLVKNKCVNFNFNGLTGTGVLTESNKKFLPFQQFGRDIADTTDAVRDPQTLEILDITPCSFGGVSVITPGTNTSNQVAVLYQDVNCTEVPVAIHADQLTPTWRVYSTGSNVFQTRAGCLIGAEHVNNSYECDIPIGAGICASYQTQTNSPQQAQSVASQSIIAYTMSLGAENSVAYSNNSIAIPTNFTISVTTEILPVSMTKTSVDCTMYICGDSTECSNLLLQYGSFCTQLNRALTGIAVEQDKNTQEVFAQVKQIYKTPPIKDFGGFNFSQILPDPSKPSKRSFIEDLLFNKVTLADAGFIKQYGDCLGDIAARDLICAQKFNGLTVLPPLLTDEMIAQYTSALLAGTITSGWTFGAGAALQIPFAMQMAYRFNGIGVTQNVLYENQKLIANQFNSAIGKIQDSLSSTASALGKLQDVVNQNAQALNTLVKQLSSNFGAISSVLNDILSRLDPPEAEVQIDRLITGRLQSLQTYVTQQLIRAAEIRASANLAATKMSECVLGQSKRVDFCGKGYHLMSFPQSAPHGVVFLHVTYVPAQEKNFTTAPAICHDGKAHFPREGVFVSNGTHWFVTQRNFYEPQIITTDNTFVSGNCDVVIGIVNNTVYDPLQPELDSFKEELDKYFKNHTSPDVDLGDISGINASVVNIQKEIDRLNEVAKNLNESLIDLQELGKYEQYIKWPWYIWLGFIAGLIAIVMVTIMLCCMTSCCSCLKGCCSCGSCCKFDEDDSEPVLKGVKLHYT

SEQ ID NO: 146 - protein, 1273 aa, Artificial Sequence
  mutant spike protein of SARS-CoV-2 Wuhan variant comprising substitution F456W, 2-P-mutation (substiutions K986P and V987P) and inoperative furin cleavage site (substitution 682-QQAQ-685)
MFVFLVLLPLVSSQCVNLTTRTQLPPAYTNSFTRGVYYPDKVFRSSVLHSTQDLFLPFFSNVTWFHAIHVSGTNGTKRFDNPVLPFNDGVYFASTEKSNIIRGWIFGTTLDSKTQSLLIVNNATNVVIKVCEFQFCNDPFLGVYYHKNNKSWMESEFRVYSSANNCTFEYVSQPFLMDLEGKQGNFKNLREFVFKNIDGYFKIYSKHTPINLVRDLPQGFSALEPLVDLPIGINITRFQTLLALHRSYLTPGDSSSGWTAGAAAYYVGYLQPRTFLLKYNENGTITDAVDCALDPLSETKCTLKSFTVEKGIYQTSNFRVQPTESIVRFPNITNLCPFGEVFNATRFASVYAWNRKRISNCVADYSVLYNSASFSTFKCYGVSPTKLNDLCFTNVYADSFVIRGDEVRQIAPGQTGKIADYNYKLPDDFTGCVIAWNSNNLDSKVGGNYNYLYRLWRKSNLKPFERDISTEIYQAGSTPCNGVEGFNCYFPLQSYGFQPTNGVGYQPYRVVVLSFELLHAPATVCGPKKSTNLVKNKCVNFNFNGLTGTGVLTESNKKFLPFQQFGRDIADTTDAVRDPQTLEILDITPCSFGGVSVITPGTNTSNQVAVLYQDVNCTEVPVAIHADQLTPTWRVYSTGSNVFQTRAGCLIGAEHVNNSYECDIPIGAGICASYQTQTNSPQQAQSVASQSIIAYTMSLGAENSVAYSNNSIAIPTNFTISVTTEILPVSMTKTSVDCTMYICGDSTECSNLLLQYGSFCTQLNRALTGIAVEQDKNTQEVFAQVKQIYKTPPIKDFGGFNFSQILPDPSKPSKRSFIEDLLFNKVTLADAGFIKQYGDCLGDIAARDLICAQKFNGLTVLPPLLTDEMIAQYTSALLAGTITSGWTFGAGAALQIPFAMQMAYRFNGIGVTQNVLYENQKLIANQFNSAIGKIQDSLSSTASALGKLQDVVNQNAQALNTLVKQLSSNFGAISSVLNDILSRLDPPEAEVQIDRLITGRLQSLQTYVTQQLIRAAEIRASANLAATKMSECVLGQSKRVDFCGKGYHLMSFPQSAPHGVVFLHVTYVPAQEKNFTTAPAICHDGKAHFPREGVFVSNGTHWFVTQRNFYEPQIITTDNTFVSGNCDVVIGIVNNTVYDPLQPELDSFKEELDKYFKNHTSPDVDLGDISGINASVVNIQKEIDRLNEVAKNLNESLIDLQELGKYEQYIKWPWYIWLGFIAGLIAIVMVTIMLCCMTSCCSCLKGCCSCGSCCKFDEDDSEPVLKGVKLHYT

SEQ ID NO: 147 - protein, 1273 aa, Artificial Sequence
  mutant spike protein of SARS-CoV-2 Wuhan variant comprising substitution F456Y, 2-P-mutation (substiutions K986P and V987P) and inoperative furin cleavage site (substitution 682-QQAQ-685)
MFVFLVLLPLVSSQCVNLTTRTQLPPAYTNSFTRGVYYPDKVFRSSVLHSTQDLFLPFFSNVTWFHAIHVSGTNGTKRFDNPVLPFNDGVYFASTEKSNIIRGWIFGTTLDSKTQSLLIVNNATNVVIKVCEFQFCNDPFLGVYYHKNNKSWMESEFRVYSSANNCTFEYVSQPFLMDLEGKQGNFKNLREFVFKNIDGYFKIYSKHTPINLVRDLPQGFSALEPLVDLPIGINITRFQTLLALHRSYLTPGDSSSGWTAGAAAYYVGYLQPRTFLLKYNENGTITDAVDCALDPLSETKCTLKSFTVEKGIYQTSNFRVQPTESIVRFPNITNLCPFGEVFNATRFASVYAWNRKRISNCVADYSVLYNSASFSTFKCYGVSPTKLNDLCFTNVYADSFVIRGDEVRQIAPGQTGKIADYNYKLPDDFTGCVIAWNSNNLDSKVGGNYNYLYRLYRKSNLKPFERDISTEIYQAGSTPCNGVEGFNCYFPLQSYGFQPTNGVGYQPYRVVVLSFELLHAPATVCGPKKSTNLVKNKCVNFNFNGLTGTGVLTESNKKFLPFQQFGRDIADTTDAVRDPQTLEILDITPCSFGGVSVITPGTNTSNQVAVLYQDVNCTEVPVAIHADQLTPTWRVYSTGSNVFQTRAGCLIGAEHVNNSYECDIPIGAGICASYQTQTNSPQQAQSVASQSIIAYTMSLGAENSVAYSNNSIAIPTNFTISVTTEILPVSMTKTSVDCTMYICGDSTECSNLLLQYGSFCTQLNRALTGIAVEQDKNTQEVFAQVKQIYKTPPIKDFGGFNFSQILPDPSKPSKRSFIEDLLFNKVTLADAGFIKQYGDCLGDIAARDLICAQKFNGLTVLPPLLTDEMIAQYTSALLAGTITSGWTFGAGAALQIPFAMQMAYRFNGIGVTQNVLYENQKLIANQFNSAIGKIQDSLSSTASALGKLQDVVNQNAQALNTLVKQLSSNFGAISSVLNDILSRLDPPEAEVQIDRLITGRLQSLQTYVTQQLIRAAEIRASANLAATKMSECVLGQSKRVDFCGKGYHLMSFPQSAPHGVVFLHVTYVPAQEKNFTTAPAICHDGKAHFPREGVFVSNGTHWFVTQRNFYEPQIITTDNTFVSGNCDVVIGIVNNTVYDPLQPELDSFKEELDKYFKNHTSPDVDLGDISGINASVVNIQKEIDRLNEVAKNLNESLIDLQELGKYEQYIKWPWYIWLGFIAGLIAIVMVTIMLCCMTSCCSCLKGCCSCGSCCKFDEDDSEPVLKGVKLHYT

SEQ ID NO: 148 - protein, 1273 aa, Artificial Sequence
  mutant spike protein of SARS-CoV-2 Wuhan variant comprising substitution F486C, 2-P-mutation (substiutions K986P and V987P) and inoperative furin cleavage site (substitution 682-QQAQ-685)
MFVFLVLLPLVSSQCVNLTTRTQLPPAYTNSFTRGVYYPDKVFRSSVLHSTQDLFLPFFSNVTWFHAIHVSGTNGTKRFDNPVLPFNDGVYFASTEKSNIIRGWIFGTTLDSKTQSLLIVNNATNVVIKVCEFQFCNDPFLGVYYHKNNKSWMESEFRVYSSANNCTFEYVSQPFLMDLEGKQGNFKNLREFVFKNIDGYFKIYSKHTPINLVRDLPQGFSALEPLVDLPIGINITRFQTLLALHRSYLTPGDSSSGWTAGAAAYYVGYLQPRTFLLKYNENGTITDAVDCALDPLSETKCTLKSFTVEKGIYQTSNFRVQPTESIVRFPNITNLCPFGEVFNATRFASVYAWNRKRISNCVADYSVLYNSASFSTFKCYGVSPTKLNDLCFTNVYADSFVIRGDEVRQIAPGQTGKIADYNYKLPDDFTGCVIAWNSNNLDSKVGGNYNYLYRLFRKSNLKPFERDISTEIYQAGSTPCNGVEGCNCYFPLQSYGFQPTNGVGYQPYRVVVLSFELLHAPATVCGPKKSTNLVKNKCVNFNFNGLTGTGVLTESNKKFLPFQQFGRDIADTTDAVRDPQTLEILDITPCSFGGVSVITPGTNTSNQVAVLYQDVNCTEVPVAIHADQLTPTWRVYSTGSNVFQTRAGCLIGAEHVNNSYECDIPIGAGICASYQTQTNSPQQAQSVASQSIIAYTMSLGAENSVAYSNNSIAIPTNFTISVTTEILPVSMTKTSVDCTMYICGDSTECSNLLLQYGSFCTQLNRALTGIAVEQDKNTQEVFAQVKQIYKTPPIKDFGGFNFSQILPDPSKPSKRSFIEDLLFNKVTLADAGFIKQYGDCLGDIAARDLICAQKFNGLTVLPPLLTDEMIAQYTSALLAGTITSGWTFGAGAALQIPFAMQMAYRFNGIGVTQNVLYENQKLIANQFNSAIGKIQDSLSSTASALGKLQDVVNQNAQALNTLVKQLSSNFGAISSVLNDILSRLDPPEAEVQIDRLITGRLQSLQTYVTQQLIRAAEIRASANLAATKMSECVLGQSKRVDFCGKGYHLMSFPQSAPHGVVFLHVTYVPAQEKNFTTAPAICHDGKAHFPREGVFVSNGTHWFVTQRNFYEPQIITTDNTFVSGNCDVVIGIVNNTVYDPLQPELDSFKEELDKYFKNHTSPDVDLGDISGINASVVNIQKEIDRLNEVAKNLNESLIDLQELGKYEQYIKWPWYIWLGFIAGLIAIVMVTIMLCCMTSCCSCLKGCCSCGSCCKFDEDDSEPVLKGVKLHYT

SEQ ID NO: 149 - protein, 1273 aa, Artificial Sequence
  mutant spike protein of SARS-CoV-2 Wuhan variant comprising substitution F486D, 2-P-mutation (substiutions K986P and V987P) and inoperative furin cleavage site (substitution 682-QQAQ-685)
MFVFLVLLPLVSSQCVNLTTRTQLPPAYTNSFTRGVYYPDKVFRSSVLHSTQDLFLPFFSNVTWFHAIHVSGTNGTKRFDNPVLPFNDGVYFASTEKSNIIRGWIFGTTLDSKTQSLLIVNNATNVVIKVCEFQFCNDPFLGVYYHKNNKSWMESEFRVYSSANNCTFEYVSQPFLMDLEGKQGNFKNLREFVFKNIDGYFKIYSKHTPINLVRDLPQGFSALEPLVDLPIGINITRFQTLLALHRSYLTPGDSSSGWTAGAAAYYVGYLQPRTFLLKYNENGTITDAVDCALDPLSETKCTLKSFTVEKGIYQTSNFRVQPTESIVRFPNITNLCPFGEVFNATRFASVYAWNRKRISNCVADYSVLYNSASFSTFKCYGVSPTKLNDLCFTNVYADSFVIRGDEVRQIAPGQTGKIADYNYKLPDDFTGCVIAWNSNNLDSKVGGNYNYLYRLFRKSNLKPFERDISTEIYQAGSTPCNGVEGDNCYFPLQSYGFQPTNGVGYQPYRVVVLSFELLHAPATVCGPKKSTNLVKNKCVNFNFNGLTGTGVLTESNKKFLPFQQFGRDIADTTDAVRDPQTLEILDITPCSFGGVSVITPGTNTSNQVAVLYQDVNCTEVPVAIHADQLTPTWRVYSTGSNVFQTRAGCLIGAEHVNNSYECDIPIGAGICASYQTQTNSPQQAQSVASQSIIAYTMSLGAENSVAYSNNSIAIPTNFTISVTTEILPVSMTKTSVDCTMYICGDSTECSNLLLQYGSFCTQLNRALTGIAVEQDKNTQEVFAQVKQIYKTPPIKDFGGFNFSQILPDPSKPSKRSFIEDLLFNKVTLADAGFIKQYGDCLGDIAARDLICAQKFNGLTVLPPLLTDEMIAQYTSALLAGTITSGWTFGAGAALQIPFAMQMAYRFNGIGVTQNVLYENQKLIANQFNSAIGKIQDSLSSTASALGKLQDVVNQNAQALNTLVKQLSSNFGAISSVLNDILSRLDPPEAEVQIDRLITGRLQSLQTYVTQQLIRAAEIRASANLAATKMSECVLGQSKRVDFCGKGYHLMSFPQSAPHGVVFLHVTYVPAQEKNFTTAPAICHDGKAHFPREGVFVSNGTHWFVTQRNFYEPQIITTDNTFVSGNCDVVIGIVNNTVYDPLQPELDSFKEELDKYFKNHTSPDVDLGDISGINASVVNIQKEIDRLNEVAKNLNESLIDLQELGKYEQYIKWPWYIWLGFIAGLIAIVMVTIMLCCMTSCCSCLKGCCSCGSCCKFDEDDSEPVLKGVKLHYT

SEQ ID NO: 150 - protein, 1273 aa, Artificial Sequence
  mutant spike protein of SARS-CoV-2 Wuhan variant comprising substitution F486E, 2-P-mutation (substiutions K986P and V987P) and inoperative furin cleavage site (substitution 682-QQAQ-685)
MFVFLVLLPLVSSQCVNLTTRTQLPPAYTNSFTRGVYYPDKVFRSSVLHSTQDLFLPFFSNVTWFHAIHVSGTNGTKRFDNPVLPFNDGVYFASTEKSNIIRGWIFGTTLDSKTQSLLIVNNATNVVIKVCEFQFCNDPFLGVYYHKNNKSWMESEFRVYSSANNCTFEYVSQPFLMDLEGKQGNFKNLREFVFKNIDGYFKIYSKHTPINLVRDLPQGFSALEPLVDLPIGINITRFQTLLALHRSYLTPGDSSSGWTAGAAAYYVGYLQPRTFLLKYNENGTITDAVDCALDPLSETKCTLKSFTVEKGIYQTSNFRVQPTESIVRFPNITNLCPFGEVFNATRFASVYAWNRKRISNCVADYSVLYNSASFSTFKCYGVSPTKLNDLCFTNVYADSFVIRGDEVRQIAPGQTGKIADYNYKLPDDFTGCVIAWNSNNLDSKVGGNYNYLYRLFRKSNLKPFERDISTEIYQAGSTPCNGVEGENCYFPLQSYGFQPTNGVGYQPYRVVVLSFELLHAPATVCGPKKSTNLVKNKCVNFNFNGLTGTGVLTESNKKFLPFQQFGRDIADTTDAVRDPQTLEILDITPCSFGGVSVITPGTNTSNQVAVLYQDVNCTEVPVAIHADQLTPTWRVYSTGSNVFQTRAGCLIGAEHVNNSYECDIPIGAGICASYQTQTNSPQQAQSVASQSIIAYTMSLGAENSVAYSNNSIAIPTNFTISVTTEILPVSMTKTSVDCTMYICGDSTECSNLLLQYGSFCTQLNRALTGIAVEQDKNTQEVFAQVKQIYKTPPIKDFGGFNFSQILPDPSKPSKRSFIEDLLFNKVTLADAGFIKQYGDCLGDIAARDLICAQKFNGLTVLPPLLTDEMIAQYTSALLAGTITSGWTFGAGAALQIPFAMQMAYRFNGIGVTQNVLYENQKLIANQFNSAIGKIQDSLSSTASALGKLQDVVNQNAQALNTLVKQLSSNFGAISSVLNDILSRLDPPEAEVQIDRLITGRLQSLQTYVTQQLIRAAEIRASANLAATKMSECVLGQSKRVDFCGKGYHLMSFPQSAPHGVVFLHVTYVPAQEKNFTTAPAICHDGKAHFPREGVFVSNGTHWFVTQRNFYEPQIITTDNTFVSGNCDVVIGIVNNTVYDPLQPELDSFKEELDKYFKNHTSPDVDLGDISGINASVVNIQKEIDRLNEVAKNLNESLIDLQELGKYEQYIKWPWYIWLGFIAGLIAIVMVTIMLCCMTSCCSCLKGCCSCGSCCKFDEDDSEPVLKGVKLHYT

SEQ ID NO: 151 - protein, 1273 aa, Artificial Sequence
  mutant spike protein of SARS-CoV-2 Wuhan variant comprising substitution L455D, 2-P-mutation (substiutions K986P and V987P) and inoperative furin cleavage site (substitution 682-QQAQ-685)
MFVFLVLLPLVSSQCVNLTTRTQLPPAYTNSFTRGVYYPDKVFRSSVLHSTQDLFLPFFSNVTWFHAIHVSGTNGTKRFDNPVLPFNDGVYFASTEKSNIIRGWIFGTTLDSKTQSLLIVNNATNVVIKVCEFQFCNDPFLGVYYHKNNKSWMESEFRVYSSANNCTFEYVSQPFLMDLEGKQGNFKNLREFVFKNIDGYFKIYSKHTPINLVRDLPQGFSALEPLVDLPIGINITRFQTLLALHRSYLTPGDSSSGWTAGAAAYYVGYLQPRTFLLKYNENGTITDAVDCALDPLSETKCTLKSFTVEKGIYQTSNFRVQPTESIVRFPNITNLCPFGEVFNATRFASVYAWNRKRISNCVADYSVLYNSASFSTFKCYGVSPTKLNDLCFTNVYADSFVIRGDEVRQIAPGQTGKIADYNYKLPDDFTGCVIAWNSNNLDSKVGGNYNYLYRDFRKSNLKPFERDISTEIYQAGSTPCNGVEGFNCYFPLQSYGFQPTNGVGYQPYRVVVLSFELLHAPATVCGPKKSTNLVKNKCVNFNFNGLTGTGVLTESNKKFLPFQQFGRDIADTTDAVRDPQTLEILDITPCSFGGVSVITPGTNTSNQVAVLYQDVNCTEVPVAIHADQLTPTWRVYSTGSNVFQTRAGCLIGAEHVNNSYECDIPIGAGICASYQTQTNSPQQAQSVASQSIIAYTMSLGAENSVAYSNNSIAIPTNFTISVTTEILPVSMTKTSVDCTMYICGDSTECSNLLLQYGSFCTQLNRALTGIAVEQDKNTQEVFAQVKQIYKTPPIKDFGGFNFSQILPDPSKPSKRSFIEDLLFNKVTLADAGFIKQYGDCLGDIAARDLICAQKFNGLTVLPPLLTDEMIAQYTSALLAGTITSGWTFGAGAALQIPFAMQMAYRFNGIGVTQNVLYENQKLIANQFNSAIGKIQDSLSSTASALGKLQDVVNQNAQALNTLVKQLSSNFGAISSVLNDILSRLDPPEAEVQIDRLITGRLQSLQTYVTQQLIRAAEIRASANLAATKMSECVLGQSKRVDFCGKGYHLMSFPQSAPHGVVFLHVTYVPAQEKNFTTAPAICHDGKAHFPREGVFVSNGTHWFVTQRNFYEPQIITTDNTFVSGNCDVVIGIVNNTVYDPLQPELDSFKEELDKYFKNHTSPDVDLGDISGINASVVNIQKEIDRLNEVAKNLNESLIDLQELGKYEQYIKWPWYIWLGFIAGLIAIVMVTIMLCCMTSCCSCLKGCCSCGSCCKFDEDDSEPVLKGVKLHYT

SEQ ID NO: 152 - protein, 1273 aa, Artificial Sequence
  mutant spike protein of SARS-CoV-2 Wuhan variant comprising substitution L455E, 2-P-mutation (substiutions K986P and V987P) and inoperative furin cleavage site (substitution 682-QQAQ-685)
MFVFLVLLPLVSSQCVNLTTRTQLPPAYTNSFTRGVYYPDKVFRSSVLHSTQDLFLPFFSNVTWFHAIHVSGTNGTKRFDNPVLPFNDGVYFASTEKSNIIRGWIFGTTLDSKTQSLLIVNNATNVVIKVCEFQFCNDPFLGVYYHKNNKSWMESEFRVYSSANNCTFEYVSQPFLMDLEGKQGNFKNLREFVFKNIDGYFKIYSKHTPINLVRDLPQGFSALEPLVDLPIGINITRFQTLLALHRSYLTPGDSSSGWTAGAAAYYVGYLQPRTFLLKYNENGTITDAVDCALDPLSETKCTLKSFTVEKGIYQTSNFRVQPTESIVRFPNITNLCPFGEVFNATRFASVYAWNRKRISNCVADYSVLYNSASFSTFKCYGVSPTKLNDLCFTNVYADSFVIRGDEVRQIAPGQTGKIADYNYKLPDDFTGCVIAWNSNNLDSKVGGNYNYLYREFRKSNLKPFERDISTEIYQAGSTPCNGVEGFNCYFPLQSYGFQPTNGVGYQPYRVVVLSFELLHAPATVCGPKKSTNLVKNKCVNFNFNGLTGTGVLTESNKKFLPFQQFGRDIADTTDAVRDPQTLEILDITPCSFGGVSVITPGTNTSNQVAVLYQDVNCTEVPVAIHADQLTPTWRVYSTGSNVFQTRAGCLIGAEHVNNSYECDIPIGAGICASYQTQTNSPQQAQSVASQSIIAYTMSLGAENSVAYSNNSIAIPTNFTISVTTEILPVSMTKTSVDCTMYICGDSTECSNLLLQYGSFCTQLNRALTGIAVEQDKNTQEVFAQVKQIYKTPPIKDFGGFNFSQILPDPSKPSKRSFIEDLLFNKVTLADAGFIKQYGDCLGDIAARDLICAQKFNGLTVLPPLLTDEMIAQYTSALLAGTITSGWTFGAGAALQIPFAMQMAYRFNGIGVTQNVLYENQKLIANQFNSAIGKIQDSLSSTASALGKLQDVVNQNAQALNTLVKQLSSNFGAISSVLNDILSRLDPPEAEVQIDRLITGRLQSLQTYVTQQLIRAAEIRASANLAATKMSECVLGQSKRVDFCGKGYHLMSFPQSAPHGVVFLHVTYVPAQEKNFTTAPAICHDGKAHFPREGVFVSNGTHWFVTQRNFYEPQIITTDNTFVSGNCDVVIGIVNNTVYDPLQPELDSFKEELDKYFKNHTSPDVDLGDISGINASVVNIQKEIDRLNEVAKNLNESLIDLQELGKYEQYIKWPWYIWLGFIAGLIAIVMVTIMLCCMTSCCSCLKGCCSCGSCCKFDEDDSEPVLKGVKLHYT

SEQ ID NO: 153 - protein, 1273 aa, Artificial Sequence
  mutant spike protein of SARS-CoV-2 Wuhan variant comprising substitution L455K, 2-P-mutation (substiutions K986P and V987P) and inoperative furin cleavage site (substitution 682-QQAQ-685)
MFVFLVLLPLVSSQCVNLTTRTQLPPAYTNSFTRGVYYPDKVFRSSVLHSTQDLFLPFFSNVTWFHAIHVSGTNGTKRFDNPVLPFNDGVYFASTEKSNIIRGWIFGTTLDSKTQSLLIVNNATNVVIKVCEFQFCNDPFLGVYYHKNNKSWMESEFRVYSSANNCTFEYVSQPFLMDLEGKQGNFKNLREFVFKNIDGYFKIYSKHTPINLVRDLPQGFSALEPLVDLPIGINITRFQTLLALHRSYLTPGDSSSGWTAGAAAYYVGYLQPRTFLLKYNENGTITDAVDCALDPLSETKCTLKSFTVEKGIYQTSNFRVQPTESIVRFPNITNLCPFGEVFNATRFASVYAWNRKRISNCVADYSVLYNSASFSTFKCYGVSPTKLNDLCFTNVYADSFVIRGDEVRQIAPGQTGKIADYNYKLPDDFTGCVIAWNSNNLDSKVGGNYNYLYRKFRKSNLKPFERDISTEIYQAGSTPCNGVEGFNCYFPLQSYGFQPTNGVGYQPYRVVVLSFELLHAPATVCGPKKSTNLVKNKCVNFNFNGLTGTGVLTESNKKFLPFQQFGRDIADTTDAVRDPQTLEILDITPCSFGGVSVITPGTNTSNQVAVLYQDVNCTEVPVAIHADQLTPTWRVYSTGSNVFQTRAGCLIGAEHVNNSYECDIPIGAGICASYQTQTNSPQQAQSVASQSIIAYTMSLGAENSVAYSNNSIAIPTNFTISVTTEILPVSMTKTSVDCTMYICGDSTECSNLLLQYGSFCTQLNRALTGIAVEQDKNTQEVFAQVKQIYKTPPIKDFGGFNFSQILPDPSKPSKRSFIEDLLFNKVTLADAGFIKQYGDCLGDIAARDLICAQKFNGLTVLPPLLTDEMIAQYTSALLAGTITSGWTFGAGAALQIPFAMQMAYRFNGIGVTQNVLYENQKLIANQFNSAIGKIQDSLSSTASALGKLQDVVNQNAQALNTLVKQLSSNFGAISSVLNDILSRLDPPEAEVQIDRLITGRLQSLQTYVTQQLIRAAEIRASANLAATKMSECVLGQSKRVDFCGKGYHLMSFPQSAPHGVVFLHVTYVPAQEKNFTTAPAICHDGKAHFPREGVFVSNGTHWFVTQRNFYEPQIITTDNTFVSGNCDVVIGIVNNTVYDPLQPELDSFKEELDKYFKNHTSPDVDLGDISGINASVVNIQKEIDRLNEVAKNLNESLIDLQELGKYEQYIKWPWYIWLGFIAGLIAIVMVTIMLCCMTSCCSCLKGCCSCGSCCKFDEDDSEPVLKGVKLHYT

SEQ ID NO: 154 - protein, 1273 aa, Artificial Sequence
  mutant spike protein of SARS-CoV-2 Wuhan variant comprising substitution L455R, 2-P-mutation (substiutions K986P and V987P) and inoperative furin cleavage site (substitution 682-QQAQ-685)
MFVFLVLLPLVSSQCVNLTTRTQLPPAYTNSFTRGVYYPDKVFRSSVLHSTQDLFLPFFSNVTWFHAIHVSGTNGTKRFDNPVLPFNDGVYFASTEKSNIIRGWIFGTTLDSKTQSLLIVNNATNVVIKVCEFQFCNDPFLGVYYHKNNKSWMESEFRVYSSANNCTFEYVSQPFLMDLEGKQGNFKNLREFVFKNIDGYFKIYSKHTPINLVRDLPQGFSALEPLVDLPIGINITRFQTLLALHRSYLTPGDSSSGWTAGAAAYYVGYLQPRTFLLKYNENGTITDAVDCALDPLSETKCTLKSFTVEKGIYQTSNFRVQPTESIVRFPNITNLCPFGEVFNATRFASVYAWNRKRISNCVADYSVLYNSASFSTFKCYGVSPTKLNDLCFTNVYADSFVIRGDEVRQIAPGQTGKIADYNYKLPDDFTGCVIAWNSNNLDSKVGGNYNYLYRRFRKSNLKPFERDISTEIYQAGSTPCNGVEGFNCYFPLQSYGFQPTNGVGYQPYRVVVLSFELLHAPATVCGPKKSTNLVKNKCVNFNFNGLTGTGVLTESNKKFLPFQQFGRDIADTTDAVRDPQTLEILDITPCSFGGVSVITPGTNTSNQVAVLYQDVNCTEVPVAIHADQLTPTWRVYSTGSNVFQTRAGCLIGAEHVNNSYECDIPIGAGICASYQTQTNSPQQAQSVASQSIIAYTMSLGAENSVAYSNNSIAIPTNFTISVTTEILPVSMTKTSVDCTMYICGDSTECSNLLLQYGSFCTQLNRALTGIAVEQDKNTQEVFAQVKQIYKTPPIKDFGGFNFSQILPDPSKPSKRSFIEDLLFNKVTLADAGFIKQYGDCLGDIAARDLICAQKFNGLTVLPPLLTDEMIAQYTSALLAGTITSGWTFGAGAALQIPFAMQMAYRFNGIGVTQNVLYENQKLIANQFNSAIGKIQDSLSSTASALGKLQDVVNQNAQALNTLVKQLSSNFGAISSVLNDILSRLDPPEAEVQIDRLITGRLQSLQTYVTQQLIRAAEIRASANLAATKMSECVLGQSKRVDFCGKGYHLMSFPQSAPHGVVFLHVTYVPAQEKNFTTAPAICHDGKAHFPREGVFVSNGTHWFVTQRNFYEPQIITTDNTFVSGNCDVVIGIVNNTVYDPLQPELDSFKEELDKYFKNHTSPDVDLGDISGINASVVNIQKEIDRLNEVAKNLNESLIDLQELGKYEQYIKWPWYIWLGFIAGLIAIVMVTIMLCCMTSCCSCLKGCCSCGSCCKFDEDDSEPVLKGVKLHYT

SEQ ID NO: 155 - protein, 1273 aa, Artificial Sequence
  mutant spike protein of SARS-CoV-2 Wuhan variant comprising substitution L455Y, 2-P-mutation (substiutions K986P and V987P) and inoperative furin cleavage site (substitution 682-QQAQ-685)
MFVFLVLLPLVSSQCVNLTTRTQLPPAYTNSFTRGVYYPDKVFRSSVLHSTQDLFLPFFSNVTWFHAIHVSGTNGTKRFDNPVLPFNDGVYFASTEKSNIIRGWIFGTTLDSKTQSLLIVNNATNVVIKVCEFQFCNDPFLGVYYHKNNKSWMESEFRVYSSANNCTFEYVSQPFLMDLEGKQGNFKNLREFVFKNIDGYFKIYSKHTPINLVRDLPQGFSALEPLVDLPIGINITRFQTLLALHRSYLTPGDSSSGWTAGAAAYYVGYLQPRTFLLKYNENGTITDAVDCALDPLSETKCTLKSFTVEKGIYQTSNFRVQPTESIVRFPNITNLCPFGEVFNATRFASVYAWNRKRISNCVADYSVLYNSASFSTFKCYGVSPTKLNDLCFTNVYADSFVIRGDEVRQIAPGQTGKIADYNYKLPDDFTGCVIAWNSNNLDSKVGGNYNYLYRYFRKSNLKPFERDISTEIYQAGSTPCNGVEGFNCYFPLQSYGFQPTNGVGYQPYRVVVLSFELLHAPATVCGPKKSTNLVKNKCVNFNFNGLTGTGVLTESNKKFLPFQQFGRDIADTTDAVRDPQTLEILDITPCSFGGVSVITPGTNTSNQVAVLYQDVNCTEVPVAIHADQLTPTWRVYSTGSNVFQTRAGCLIGAEHVNNSYECDIPIGAGICASYQTQTNSPQQAQSVASQSIIAYTMSLGAENSVAYSNNSIAIPTNFTISVTTEILPVSMTKTSVDCTMYICGDSTECSNLLLQYGSFCTQLNRALTGIAVEQDKNTQEVFAQVKQIYKTPPIKDFGGFNFSQILPDPSKPSKRSFIEDLLFNKVTLADAGFIKQYGDCLGDIAARDLICAQKFNGLTVLPPLLTDEMIAQYTSALLAGTITSGWTFGAGAALQIPFAMQMAYRFNGIGVTQNVLYENQKLIANQFNSAIGKIQDSLSSTASALGKLQDVVNQNAQALNTLVKQLSSNFGAISSVLNDILSRLDPPEAEVQIDRLITGRLQSLQTYVTQQLIRAAEIRASANLAATKMSECVLGQSKRVDFCGKGYHLMSFPQSAPHGVVFLHVTYVPAQEKNFTTAPAICHDGKAHFPREGVFVSNGTHWFVTQRNFYEPQIITTDNTFVSGNCDVVIGIVNNTVYDPLQPELDSFKEELDKYFKNHTSPDVDLGDISGINASVVNIQKEIDRLNEVAKNLNESLIDLQELGKYEQYIKWPWYIWLGFIAGLIAIVMVTIMLCCMTSCCSCLKGCCSCGSCCKFDEDDSEPVLKGVKLHYT

SEQ ID NO: 156 - protein, 1273 aa, Artificial Sequence
  mutant spike protein of SARS-CoV-2 Wuhan variant comprising substitution Q498C, 2-P-mutation (substiutions K986P and V987P) and inoperative furin cleavage site (substitution 682-QQAQ-685)
MFVFLVLLPLVSSQCVNLTTRTQLPPAYTNSFTRGVYYPDKVFRSSVLHSTQDLFLPFFSNVTWFHAIHVSGTNGTKRFDNPVLPFNDGVYFASTEKSNIIRGWIFGTTLDSKTQSLLIVNNATNVVIKVCEFQFCNDPFLGVYYHKNNKSWMESEFRVYSSANNCTFEYVSQPFLMDLEGKQGNFKNLREFVFKNIDGYFKIYSKHTPINLVRDLPQGFSALEPLVDLPIGINITRFQTLLALHRSYLTPGDSSSGWTAGAAAYYVGYLQPRTFLLKYNENGTITDAVDCALDPLSETKCTLKSFTVEKGIYQTSNFRVQPTESIVRFPNITNLCPFGEVFNATRFASVYAWNRKRISNCVADYSVLYNSASFSTFKCYGVSPTKLNDLCFTNVYADSFVIRGDEVRQIAPGQTGKIADYNYKLPDDFTGCVIAWNSNNLDSKVGGNYNYLYRLFRKSNLKPFERDISTEIYQAGSTPCNGVEGFNCYFPLQSYGFCPTNGVGYQPYRVVVLSFELLHAPATVCGPKKSTNLVKNKCVNFNFNGLTGTGVLTESNKKFLPFQQFGRDIADTTDAVRDPQTLEILDITPCSFGGVSVITPGTNTSNQVAVLYQDVNCTEVPVAIHADQLTPTWRVYSTGSNVFQTRAGCLIGAEHVNNSYECDIPIGAGICASYQTQTNSPQQAQSVASQSIIAYTMSLGAENSVAYSNNSIAIPTNFTISVTTEILPVSMTKTSVDCTMYICGDSTECSNLLLQYGSFCTQLNRALTGIAVEQDKNTQEVFAQVKQIYKTPPIKDFGGFNFSQILPDPSKPSKRSFIEDLLFNKVTLADAGFIKQYGDCLGDIAARDLICAQKFNGLTVLPPLLTDEMIAQYTSALLAGTITSGWTFGAGAALQIPFAMQMAYRFNGIGVTQNVLYENQKLIANQFNSAIGKIQDSLSSTASALGKLQDVVNQNAQALNTLVKQLSSNFGAISSVLNDILSRLDPPEAEVQIDRLITGRLQSLQTYVTQQLIRAAEIRASANLAATKMSECVLGQSKRVDFCGKGYHLMSFPQSAPHGVVFLHVTYVPAQEKNFTTAPAICHDGKAHFPREGVFVSNGTHWFVTQRNFYEPQIITTDNTFVSGNCDVVIGIVNNTVYDPLQPELDSFKEELDKYFKNHTSPDVDLGDISGINASVVNIQKEIDRLNEVAKNLNESLIDLQELGKYEQYIKWPWYIWLGFIAGLIAIVMVTIMLCCMTSCCSCLKGCCSCGSCCKFDEDDSEPVLKGVKLHYT

SEQ ID NO: 157 - protein, 1273 aa, Artificial Sequence
  mutant spike protein of SARS-CoV-2 Wuhan variant comprising substitution Q498D, 2-P-mutation (substiutions K986P and V987P) and inoperative furin cleavage site (substitution 682-QQAQ-685)
MFVFLVLLPLVSSQCVNLTTRTQLPPAYTNSFTRGVYYPDKVFRSSVLHSTQDLFLPFFSNVTWFHAIHVSGTNGTKRFDNPVLPFNDGVYFASTEKSNIIRGWIFGTTLDSKTQSLLIVNNATNVVIKVCEFQFCNDPFLGVYYHKNNKSWMESEFRVYSSANNCTFEYVSQPFLMDLEGKQGNFKNLREFVFKNIDGYFKIYSKHTPINLVRDLPQGFSALEPLVDLPIGINITRFQTLLALHRSYLTPGDSSSGWTAGAAAYYVGYLQPRTFLLKYNENGTITDAVDCALDPLSETKCTLKSFTVEKGIYQTSNFRVQPTESIVRFPNITNLCPFGEVFNATRFASVYAWNRKRISNCVADYSVLYNSASFSTFKCYGVSPTKLNDLCFTNVYADSFVIRGDEVRQIAPGQTGKIADYNYKLPDDFTGCVIAWNSNNLDSKVGGNYNYLYRLFRKSNLKPFERDISTEIYQAGSTPCNGVEGFNCYFPLQSYGFDPTNGVGYQPYRVVVLSFELLHAPATVCGPKKSTNLVKNKCVNFNFNGLTGTGVLTESNKKFLPFQQFGRDIADTTDAVRDPQTLEILDITPCSFGGVSVITPGTNTSNQVAVLYQDVNCTEVPVAIHADQLTPTWRVYSTGSNVFQTRAGCLIGAEHVNNSYECDIPIGAGICASYQTQTNSPQQAQSVASQSIIAYTMSLGAENSVAYSNNSIAIPTNFTISVTTEILPVSMTKTSVDCTMYICGDSTECSNLLLQYGSFCTQLNRALTGIAVEQDKNTQEVFAQVKQIYKTPPIKDFGGFNFSQILPDPSKPSKRSFIEDLLFNKVTLADAGFIKQYGDCLGDIAARDLICAQKFNGLTVLPPLLTDEMIAQYTSALLAGTITSGWTFGAGAALQIPFAMQMAYRFNGIGVTQNVLYENQKLIANQFNSAIGKIQDSLSSTASALGKLQDVVNQNAQALNTLVKQLSSNFGAISSVLNDILSRLDPPEAEVQIDRLITGRLQSLQTYVTQQLIRAAEIRASANLAATKMSECVLGQSKRVDFCGKGYHLMSFPQSAPHGVVFLHVTYVPAQEKNFTTAPAICHDGKAHFPREGVFVSNGTHWFVTQRNFYEPQIITTDNTFVSGNCDVVIGIVNNTVYDPLQPELDSFKEELDKYFKNHTSPDVDLGDISGINASVVNIQKEIDRLNEVAKNLNESLIDLQELGKYEQYIKWPWYIWLGFIAGLIAIVMVTIMLCCMTSCCSCLKGCCSCGSCCKFDEDDSEPVLKGVKLHYT

SEQ ID NO: 158 - protein, 1273 aa, Artificial Sequence
  mutant spike protein of SARS-CoV-2 Wuhan variant comprising substitution Q498I, 2-P-mutation (substiutions K986P and V987P) and inoperative furin cleavage site (substitution 682-QQAQ-685)
MFVFLVLLPLVSSQCVNLTTRTQLPPAYTNSFTRGVYYPDKVFRSSVLHSTQDLFLPFFSNVTWFHAIHVSGTNGTKRFDNPVLPFNDGVYFASTEKSNIIRGWIFGTTLDSKTQSLLIVNNATNVVIKVCEFQFCNDPFLGVYYHKNNKSWMESEFRVYSSANNCTFEYVSQPFLMDLEGKQGNFKNLREFVFKNIDGYFKIYSKHTPINLVRDLPQGFSALEPLVDLPIGINITRFQTLLALHRSYLTPGDSSSGWTAGAAAYYVGYLQPRTFLLKYNENGTITDAVDCALDPLSETKCTLKSFTVEKGIYQTSNFRVQPTESIVRFPNITNLCPFGEVFNATRFASVYAWNRKRISNCVADYSVLYNSASFSTFKCYGVSPTKLNDLCFTNVYADSFVIRGDEVRQIAPGQTGKIADYNYKLPDDFTGCVIAWNSNNLDSKVGGNYNYLYRLFRKSNLKPFERDISTEIYQAGSTPCNGVEGFNCYFPLQSYGFIPTNGVGYQPYRVVVLSFELLHAPATVCGPKKSTNLVKNKCVNFNFNGLTGTGVLTESNKKFLPFQQFGRDIADTTDAVRDPQTLEILDITPCSFGGVSVITPGTNTSNQVAVLYQDVNCTEVPVAIHADQLTPTWRVYSTGSNVFQTRAGCLIGAEHVNNSYECDIPIGAGICASYQTQTNSPQQAQSVASQSIIAYTMSLGAENSVAYSNNSIAIPTNFTISVTTEILPVSMTKTSVDCTMYICGDSTECSNLLLQYGSFCTQLNRALTGIAVEQDKNTQEVFAQVKQIYKTPPIKDFGGFNFSQILPDPSKPSKRSFIEDLLFNKVTLADAGFIKQYGDCLGDIAARDLICAQKFNGLTVLPPLLTDEMIAQYTSALLAGTITSGWTFGAGAALQIPFAMQMAYRFNGIGVTQNVLYENQKLIANQFNSAIGKIQDSLSSTASALGKLQDVVNQNAQALNTLVKQLSSNFGAISSVLNDILSRLDPPEAEVQIDRLITGRLQSLQTYVTQQLIRAAEIRASANLAATKMSECVLGQSKRVDFCGKGYHLMSFPQSAPHGVVFLHVTYVPAQEKNFTTAPAICHDGKAHFPREGVFVSNGTHWFVTQRNFYEPQIITTDNTFVSGNCDVVIGIVNNTVYDPLQPELDSFKEELDKYFKNHTSPDVDLGDISGINASVVNIQKEIDRLNEVAKNLNESLIDLQELGKYEQYIKWPWYIWLGFIAGLIAIVMVTIMLCCMTSCCSCLKGCCSCGSCCKFDEDDSEPVLKGVKLHYT

SEQ ID NO: 159 - protein, 1273 aa, Artificial Sequence
  mutant spike protein of SARS-CoV-2 Wuhan variant comprising substitution Q498K, 2-P-mutation (substiutions K986P and V987P) and inoperative furin cleavage site (substitution 682-QQAQ-685)
MFVFLVLLPLVSSQCVNLTTRTQLPPAYTNSFTRGVYYPDKVFRSSVLHSTQDLFLPFFSNVTWFHAIHVSGTNGTKRFDNPVLPFNDGVYFASTEKSNIIRGWIFGTTLDSKTQSLLIVNNATNVVIKVCEFQFCNDPFLGVYYHKNNKSWMESEFRVYSSANNCTFEYVSQPFLMDLEGKQGNFKNLREFVFKNIDGYFKIYSKHTPINLVRDLPQGFSALEPLVDLPIGINITRFQTLLALHRSYLTPGDSSSGWTAGAAAYYVGYLQPRTFLLKYNENGTITDAVDCALDPLSETKCTLKSFTVEKGIYQTSNFRVQPTESIVRFPNITNLCPFGEVFNATRFASVYAWNRKRISNCVADYSVLYNSASFSTFKCYGVSPTKLNDLCFTNVYADSFVIRGDEVRQIAPGQTGKIADYNYKLPDDFTGCVIAWNSNNLDSKVGGNYNYLYRLFRKSNLKPFERDISTEIYQAGSTPCNGVEGFNCYFPLQSYGFKPTNGVGYQPYRVVVLSFELLHAPATVCGPKKSTNLVKNKCVNFNFNGLTGTGVLTESNKKFLPFQQFGRDIADTTDAVRDPQTLEILDITPCSFGGVSVITPGTNTSNQVAVLYQDVNCTEVPVAIHADQLTPTWRVYSTGSNVFQTRAGCLIGAEHVNNSYECDIPIGAGICASYQTQTNSPQQAQSVASQSIIAYTMSLGAENSVAYSNNSIAIPTNFTISVTTEILPVSMTKTSVDCTMYICGDSTECSNLLLQYGSFCTQLNRALTGIAVEQDKNTQEVFAQVKQIYKTPPIKDFGGFNFSQILPDPSKPSKRSFIEDLLFNKVTLADAGFIKQYGDCLGDIAARDLICAQKFNGLTVLPPLLTDEMIAQYTSALLAGTITSGWTFGAGAALQIPFAMQMAYRFNGIGVTQNVLYENQKLIANQFNSAIGKIQDSLSSTASALGKLQDVVNQNAQALNTLVKQLSSNFGAISSVLNDILSRLDPPEAEVQIDRLITGRLQSLQTYVTQQLIRAAEIRASANLAATKMSECVLGQSKRVDFCGKGYHLMSFPQSAPHGVVFLHVTYVPAQEKNFTTAPAICHDGKAHFPREGVFVSNGTHWFVTQRNFYEPQIITTDNTFVSGNCDVVIGIVNNTVYDPLQPELDSFKEELDKYFKNHTSPDVDLGDISGINASVVNIQKEIDRLNEVAKNLNESLIDLQELGKYEQYIKWPWYIWLGFIAGLIAIVMVTIMLCCMTSCCSCLKGCCSCGSCCKFDEDDSEPVLKGVKLHYT

SEQ ID NO: 160 - protein, 1273 aa, Artificial Sequence
  mutant spike protein of SARS-CoV-2 Wuhan variant comprising substitution Q498L, 2-P-mutation (substiutions K986P and V987P) and inoperative furin cleavage site (substitution 682-QQAQ-685)
MFVFLVLLPLVSSQCVNLTTRTQLPPAYTNSFTRGVYYPDKVFRSSVLHSTQDLFLPFFSNVTWFHAIHVSGTNGTKRFDNPVLPFNDGVYFASTEKSNIIRGWIFGTTLDSKTQSLLIVNNATNVVIKVCEFQFCNDPFLGVYYHKNNKSWMESEFRVYSSANNCTFEYVSQPFLMDLEGKQGNFKNLREFVFKNIDGYFKIYSKHTPINLVRDLPQGFSALEPLVDLPIGINITRFQTLLALHRSYLTPGDSSSGWTAGAAAYYVGYLQPRTFLLKYNENGTITDAVDCALDPLSETKCTLKSFTVEKGIYQTSNFRVQPTESIVRFPNITNLCPFGEVFNATRFASVYAWNRKRISNCVADYSVLYNSASFSTFKCYGVSPTKLNDLCFTNVYADSFVIRGDEVRQIAPGQTGKIADYNYKLPDDFTGCVIAWNSNNLDSKVGGNYNYLYRLFRKSNLKPFERDISTEIYQAGSTPCNGVEGFNCYFPLQSYGFLPTNGVGYQPYRVVVLSFELLHAPATVCGPKKSTNLVKNKCVNFNFNGLTGTGVLTESNKKFLPFQQFGRDIADTTDAVRDPQTLEILDITPCSFGGVSVITPGTNTSNQVAVLYQDVNCTEVPVAIHADQLTPTWRVYSTGSNVFQTRAGCLIGAEHVNNSYECDIPIGAGICASYQTQTNSPQQAQSVASQSIIAYTMSLGAENSVAYSNNSIAIPTNFTISVTTEILPVSMTKTSVDCTMYICGDSTECSNLLLQYGSFCTQLNRALTGIAVEQDKNTQEVFAQVKQIYKTPPIKDFGGFNFSQILPDPSKPSKRSFIEDLLFNKVTLADAGFIKQYGDCLGDIAARDLICAQKFNGLTVLPPLLTDEMIAQYTSALLAGTITSGWTFGAGAALQIPFAMQMAYRFNGIGVTQNVLYENQKLIANQFNSAIGKIQDSLSSTASALGKLQDVVNQNAQALNTLVKQLSSNFGAISSVLNDILSRLDPPEAEVQIDRLITGRLQSLQTYVTQQLIRAAEIRASANLAATKMSECVLGQSKRVDFCGKGYHLMSFPQSAPHGVVFLHVTYVPAQEKNFTTAPAICHDGKAHFPREGVFVSNGTHWFVTQRNFYEPQIITTDNTFVSGNCDVVIGIVNNTVYDPLQPELDSFKEELDKYFKNHTSPDVDLGDISGINASVVNIQKEIDRLNEVAKNLNESLIDLQELGKYEQYIKWPWYIWLGFIAGLIAIVMVTIMLCCMTSCCSCLKGCCSCGSCCKFDEDDSEPVLKGVKLHYT

SEQ ID NO: 161 - protein, 1273 aa, Artificial Sequence
  mutant spike protein of SARS-CoV-2 Wuhan variant comprising substitution Q498V, 2-P-mutation (substiutions K986P and V987P) and inoperative furin cleavage site (substitution 682-QQAQ-685)
MFVFLVLLPLVSSQCVNLTTRTQLPPAYTNSFTRGVYYPDKVFRSSVLHSTQDLFLPFFSNVTWFHAIHVSGTNGTKRFDNPVLPFNDGVYFASTEKSNIIRGWIFGTTLDSKTQSLLIVNNATNVVIKVCEFQFCNDPFLGVYYHKNNKSWMESEFRVYSSANNCTFEYVSQPFLMDLEGKQGNFKNLREFVFKNIDGYFKIYSKHTPINLVRDLPQGFSALEPLVDLPIGINITRFQTLLALHRSYLTPGDSSSGWTAGAAAYYVGYLQPRTFLLKYNENGTITDAVDCALDPLSETKCTLKSFTVEKGIYQTSNFRVQPTESIVRFPNITNLCPFGEVFNATRFASVYAWNRKRISNCVADYSVLYNSASFSTFKCYGVSPTKLNDLCFTNVYADSFVIRGDEVRQIAPGQTGKIADYNYKLPDDFTGCVIAWNSNNLDSKVGGNYNYLYRLFRKSNLKPFERDISTEIYQAGSTPCNGVEGFNCYFPLQSYGFVPTNGVGYQPYRVVVLSFELLHAPATVCGPKKSTNLVKNKCVNFNFNGLTGTGVLTESNKKFLPFQQFGRDIADTTDAVRDPQTLEILDITPCSFGGVSVITPGTNTSNQVAVLYQDVNCTEVPVAIHADQLTPTWRVYSTGSNVFQTRAGCLIGAEHVNNSYECDIPIGAGICASYQTQTNSPQQAQSVASQSIIAYTMSLGAENSVAYSNNSIAIPTNFTISVTTEILPVSMTKTSVDCTMYICGDSTECSNLLLQYGSFCTQLNRALTGIAVEQDKNTQEVFAQVKQIYKTPPIKDFGGFNFSQILPDPSKPSKRSFIEDLLFNKVTLADAGFIKQYGDCLGDIAARDLICAQKFNGLTVLPPLLTDEMIAQYTSALLAGTITSGWTFGAGAALQIPFAMQMAYRFNGIGVTQNVLYENQKLIANQFNSAIGKIQDSLSSTASALGKLQDVVNQNAQALNTLVKQLSSNFGAISSVLNDILSRLDPPEAEVQIDRLITGRLQSLQTYVTQQLIRAAEIRASANLAATKMSECVLGQSKRVDFCGKGYHLMSFPQSAPHGVVFLHVTYVPAQEKNFTTAPAICHDGKAHFPREGVFVSNGTHWFVTQRNFYEPQIITTDNTFVSGNCDVVIGIVNNTVYDPLQPELDSFKEELDKYFKNHTSPDVDLGDISGINASVVNIQKEIDRLNEVAKNLNESLIDLQELGKYEQYIKWPWYIWLGFIAGLIAIVMVTIMLCCMTSCCSCLKGCCSCGSCCKFDEDDSEPVLKGVKLHYT

SEQ ID NO: 162 - protein, 1273 aa, Artificial Sequence
  mutant spike protein of SARS-CoV-2 Wuhan variant comprising substitution S373N, 2-P-mutation (substiutions K986P and V987P) and inoperative furin cleavage site (substitution 682-QQAQ-685)
MFVFLVLLPLVSSQCVNLTTRTQLPPAYTNSFTRGVYYPDKVFRSSVLHSTQDLFLPFFSNVTWFHAIHVSGTNGTKRFDNPVLPFNDGVYFASTEKSNIIRGWIFGTTLDSKTQSLLIVNNATNVVIKVCEFQFCNDPFLGVYYHKNNKSWMESEFRVYSSANNCTFEYVSQPFLMDLEGKQGNFKNLREFVFKNIDGYFKIYSKHTPINLVRDLPQGFSALEPLVDLPIGINITRFQTLLALHRSYLTPGDSSSGWTAGAAAYYVGYLQPRTFLLKYNENGTITDAVDCALDPLSETKCTLKSFTVEKGIYQTSNFRVQPTESIVRFPNITNLCPFGEVFNATRFASVYAWNRKRISNCVADYSVLYNSANFSTFKCYGVSPTKLNDLCFTNVYADSFVIRGDEVRQIAPGQTGKIADYNYKLPDDFTGCVIAWNSNNLDSKVGGNYNYLYRLFRKSNLKPFERDISTEIYQAGSTPCNGVEGFNCYFPLQSYGFQPTNGVGYQPYRVVVLSFELLHAPATVCGPKKSTNLVKNKCVNFNFNGLTGTGVLTESNKKFLPFQQFGRDIADTTDAVRDPQTLEILDITPCSFGGVSVITPGTNTSNQVAVLYQDVNCTEVPVAIHADQLTPTWRVYSTGSNVFQTRAGCLIGAEHVNNSYECDIPIGAGICASYQTQTNSPQQAQSVASQSIIAYTMSLGAENSVAYSNNSIAIPTNFTISVTTEILPVSMTKTSVDCTMYICGDSTECSNLLLQYGSFCTQLNRALTGIAVEQDKNTQEVFAQVKQIYKTPPIKDFGGFNFSQILPDPSKPSKRSFIEDLLFNKVTLADAGFIKQYGDCLGDIAARDLICAQKFNGLTVLPPLLTDEMIAQYTSALLAGTITSGWTFGAGAALQIPFAMQMAYRFNGIGVTQNVLYENQKLIANQFNSAIGKIQDSLSSTASALGKLQDVVNQNAQALNTLVKQLSSNFGAISSVLNDILSRLDPPEAEVQIDRLITGRLQSLQTYVTQQLIRAAEIRASANLAATKMSECVLGQSKRVDFCGKGYHLMSFPQSAPHGVVFLHVTYVPAQEKNFTTAPAICHDGKAHFPREGVFVSNGTHWFVTQRNFYEPQIITTDNTFVSGNCDVVIGIVNNTVYDPLQPELDSFKEELDKYFKNHTSPDVDLGDISGINASVVNIQKEIDRLNEVAKNLNESLIDLQELGKYEQYIKWPWYIWLGFIAGLIAIVMVTIMLCCMTSCCSCLKGCCSCGSCCKFDEDDSEPVLKGVKLHYT

SEQ ID NO: 163 - protein, 1273 aa, Artificial Sequence
  mutant spike protein of SARS-CoV-2 Wuhan variant comprising substitution Y449A, 2-P-mutation (substiutions K986P and V987P) and inoperative furin cleavage site (substitution 682-QQAQ-685)
MFVFLVLLPLVSSQCVNLTTRTQLPPAYTNSFTRGVYYPDKVFRSSVLHSTQDLFLPFFSNVTWFHAIHVSGTNGTKRFDNPVLPFNDGVYFASTEKSNIIRGWIFGTTLDSKTQSLLIVNNATNVVIKVCEFQFCNDPFLGVYYHKNNKSWMESEFRVYSSANNCTFEYVSQPFLMDLEGKQGNFKNLREFVFKNIDGYFKIYSKHTPINLVRDLPQGFSALEPLVDLPIGINITRFQTLLALHRSYLTPGDSSSGWTAGAAAYYVGYLQPRTFLLKYNENGTITDAVDCALDPLSETKCTLKSFTVEKGIYQTSNFRVQPTESIVRFPNITNLCPFGEVFNATRFASVYAWNRKRISNCVADYSVLYNSASFSTFKCYGVSPTKLNDLCFTNVYADSFVIRGDEVRQIAPGQTGKIADYNYKLPDDFTGCVIAWNSNNLDSKVGGNANYLYRLFRKSNLKPFERDISTEIYQAGSTPCNGVEGFNCYFPLQSYGFQPTNGVGYQPYRVVVLSFELLHAPATVCGPKKSTNLVKNKCVNFNFNGLTGTGVLTESNKKFLPFQQFGRDIADTTDAVRDPQTLEILDITPCSFGGVSVITPGTNTSNQVAVLYQDVNCTEVPVAIHADQLTPTWRVYSTGSNVFQTRAGCLIGAEHVNNSYECDIPIGAGICASYQTQTNSPQQAQSVASQSIIAYTMSLGAENSVAYSNNSIAIPTNFTISVTTEILPVSMTKTSVDCTMYICGDSTECSNLLLQYGSFCTQLNRALTGIAVEQDKNTQEVFAQVKQIYKTPPIKDFGGFNFSQILPDPSKPSKRSFIEDLLFNKVTLADAGFIKQYGDCLGDIAARDLICAQKFNGLTVLPPLLTDEMIAQYTSALLAGTITSGWTFGAGAALQIPFAMQMAYRFNGIGVTQNVLYENQKLIANQFNSAIGKIQDSLSSTASALGKLQDVVNQNAQALNTLVKQLSSNFGAISSVLNDILSRLDPPEAEVQIDRLITGRLQSLQTYVTQQLIRAAEIRASANLAATKMSECVLGQSKRVDFCGKGYHLMSFPQSAPHGVVFLHVTYVPAQEKNFTTAPAICHDGKAHFPREGVFVSNGTHWFVTQRNFYEPQIITTDNTFVSGNCDVVIGIVNNTVYDPLQPELDSFKEELDKYFKNHTSPDVDLGDISGINASVVNIQKEIDRLNEVAKNLNESLIDLQELGKYEQYIKWPWYIWLGFIAGLIAIVMVTIMLCCMTSCCSCLKGCCSCGSCCKFDEDDSEPVLKGVKLHYT

SEQ ID NO: 164 - protein, 1273 aa, Artificial Sequence
  mutant spike protein of SARS-CoV-2 Wuhan variant comprising substitution Y449C, 2-P-mutation (substiutions K986P and V987P) and inoperative furin cleavage site (substitution 682-QQAQ-685)
MFVFLVLLPLVSSQCVNLTTRTQLPPAYTNSFTRGVYYPDKVFRSSVLHSTQDLFLPFFSNVTWFHAIHVSGTNGTKRFDNPVLPFNDGVYFASTEKSNIIRGWIFGTTLDSKTQSLLIVNNATNVVIKVCEFQFCNDPFLGVYYHKNNKSWMESEFRVYSSANNCTFEYVSQPFLMDLEGKQGNFKNLREFVFKNIDGYFKIYSKHTPINLVRDLPQGFSALEPLVDLPIGINITRFQTLLALHRSYLTPGDSSSGWTAGAAAYYVGYLQPRTFLLKYNENGTITDAVDCALDPLSETKCTLKSFTVEKGIYQTSNFRVQPTESIVRFPNITNLCPFGEVFNATRFASVYAWNRKRISNCVADYSVLYNSASFSTFKCYGVSPTKLNDLCFTNVYADSFVIRGDEVRQIAPGQTGKIADYNYKLPDDFTGCVIAWNSNNLDSKVGGNCNYLYRLFRKSNLKPFERDISTEIYQAGSTPCNGVEGFNCYFPLQSYGFQPTNGVGYQPYRVVVLSFELLHAPATVCGPKKSTNLVKNKCVNFNFNGLTGTGVLTESNKKFLPFQQFGRDIADTTDAVRDPQTLEILDITPCSFGGVSVITPGTNTSNQVAVLYQDVNCTEVPVAIHADQLTPTWRVYSTGSNVFQTRAGCLIGAEHVNNSYECDIPIGAGICASYQTQTNSPQQAQSVASQSIIAYTMSLGAENSVAYSNNSIAIPTNFTISVTTEILPVSMTKTSVDCTMYICGDSTECSNLLLQYGSFCTQLNRALTGIAVEQDKNTQEVFAQVKQIYKTPPIKDFGGFNFSQILPDPSKPSKRSFIEDLLFNKVTLADAGFIKQYGDCLGDIAARDLICAQKFNGLTVLPPLLTDEMIAQYTSALLAGTITSGWTFGAGAALQIPFAMQMAYRFNGIGVTQNVLYENQKLIANQFNSAIGKIQDSLSSTASALGKLQDVVNQNAQALNTLVKQLSSNFGAISSVLNDILSRLDPPEAEVQIDRLITGRLQSLQTYVTQQLIRAAEIRASANLAATKMSECVLGQSKRVDFCGKGYHLMSFPQSAPHGVVFLHVTYVPAQEKNFTTAPAICHDGKAHFPREGVFVSNGTHWFVTQRNFYEPQIITTDNTFVSGNCDVVIGIVNNTVYDPLQPELDSFKEELDKYFKNHTSPDVDLGDISGINASVVNIQKEIDRLNEVAKNLNESLIDLQELGKYEQYIKWPWYIWLGFIAGLIAIVMVTIMLCCMTSCCSCLKGCCSCGSCCKFDEDDSEPVLKGVKLHYT

SEQ ID NO: 165 - protein, 1273 aa, Artificial Sequence
  mutant spike protein of SARS-CoV-2 Wuhan variant comprising substitution Y449D, 2-P-mutation (substiutions K986P and V987P) and inoperative furin cleavage site (substitution 682-QQAQ-685)
MFVFLVLLPLVSSQCVNLTTRTQLPPAYTNSFTRGVYYPDKVFRSSVLHSTQDLFLPFFSNVTWFHAIHVSGTNGTKRFDNPVLPFNDGVYFASTEKSNIIRGWIFGTTLDSKTQSLLIVNNATNVVIKVCEFQFCNDPFLGVYYHKNNKSWMESEFRVYSSANNCTFEYVSQPFLMDLEGKQGNFKNLREFVFKNIDGYFKIYSKHTPINLVRDLPQGFSALEPLVDLPIGINITRFQTLLALHRSYLTPGDSSSGWTAGAAAYYVGYLQPRTFLLKYNENGTITDAVDCALDPLSETKCTLKSFTVEKGIYQTSNFRVQPTESIVRFPNITNLCPFGEVFNATRFASVYAWNRKRISNCVADYSVLYNSASFSTFKCYGVSPTKLNDLCFTNVYADSFVIRGDEVRQIAPGQTGKIADYNYKLPDDFTGCVIAWNSNNLDSKVGGNDNYLYRLFRKSNLKPFERDISTEIYQAGSTPCNGVEGFNCYFPLQSYGFQPTNGVGYQPYRVVVLSFELLHAPATVCGPKKSTNLVKNKCVNFNFNGLTGTGVLTESNKKFLPFQQFGRDIADTTDAVRDPQTLEILDITPCSFGGVSVITPGTNTSNQVAVLYQDVNCTEVPVAIHADQLTPTWRVYSTGSNVFQTRAGCLIGAEHVNNSYECDIPIGAGICASYQTQTNSPQQAQSVASQSIIAYTMSLGAENSVAYSNNSIAIPTNFTISVTTEILPVSMTKTSVDCTMYICGDSTECSNLLLQYGSFCTQLNRALTGIAVEQDKNTQEVFAQVKQIYKTPPIKDFGGFNFSQILPDPSKPSKRSFIEDLLFNKVTLADAGFIKQYGDCLGDIAARDLICAQKFNGLTVLPPLLTDEMIAQYTSALLAGTITSGWTFGAGAALQIPFAMQMAYRFNGIGVTQNVLYENQKLIANQFNSAIGKIQDSLSSTASALGKLQDVVNQNAQALNTLVKQLSSNFGAISSVLNDILSRLDPPEAEVQIDRLITGRLQSLQTYVTQQLIRAAEIRASANLAATKMSECVLGQSKRVDFCGKGYHLMSFPQSAPHGVVFLHVTYVPAQEKNFTTAPAICHDGKAHFPREGVFVSNGTHWFVTQRNFYEPQIITTDNTFVSGNCDVVIGIVNNTVYDPLQPELDSFKEELDKYFKNHTSPDVDLGDISGINASVVNIQKEIDRLNEVAKNLNESLIDLQELGKYEQYIKWPWYIWLGFIAGLIAIVMVTIMLCCMTSCCSCLKGCCSCGSCCKFDEDDSEPVLKGVKLHYT

SEQ ID NO: 166 - protein, 1273 aa, Artificial Sequence
  mutant spike protein of SARS-CoV-2 Wuhan variant comprising substitution Y449E, 2-P-mutation (substiutions K986P and V987P) and inoperative furin cleavage site (substitution 682-QQAQ-685)
MFVFLVLLPLVSSQCVNLTTRTQLPPAYTNSFTRGVYYPDKVFRSSVLHSTQDLFLPFFSNVTWFHAIHVSGTNGTKRFDNPVLPFNDGVYFASTEKSNIIRGWIFGTTLDSKTQSLLIVNNATNVVIKVCEFQFCNDPFLGVYYHKNNKSWMESEFRVYSSANNCTFEYVSQPFLMDLEGKQGNFKNLREFVFKNIDGYFKIYSKHTPINLVRDLPQGFSALEPLVDLPIGINITRFQTLLALHRSYLTPGDSSSGWTAGAAAYYVGYLQPRTFLLKYNENGTITDAVDCALDPLSETKCTLKSFTVEKGIYQTSNFRVQPTESIVRFPNITNLCPFGEVFNATRFASVYAWNRKRISNCVADYSVLYNSASFSTFKCYGVSPTKLNDLCFTNVYADSFVIRGDEVRQIAPGQTGKIADYNYKLPDDFTGCVIAWNSNNLDSKVGGNENYLYRLFRKSNLKPFERDISTEIYQAGSTPCNGVEGFNCYFPLQSYGFQPTNGVGYQPYRVVVLSFELLHAPATVCGPKKSTNLVKNKCVNFNFNGLTGTGVLTESNKKFLPFQQFGRDIADTTDAVRDPQTLEILDITPCSFGGVSVITPGTNTSNQVAVLYQDVNCTEVPVAIHADQLTPTWRVYSTGSNVFQTRAGCLIGAEHVNNSYECDIPIGAGICASYQTQTNSPQQAQSVASQSIIAYTMSLGAENSVAYSNNSIAIPTNFTISVTTEILPVSMTKTSVDCTMYICGDSTECSNLLLQYGSFCTQLNRALTGIAVEQDKNTQEVFAQVKQIYKTPPIKDFGGFNFSQILPDPSKPSKRSFIEDLLFNKVTLADAGFIKQYGDCLGDIAARDLICAQKFNGLTVLPPLLTDEMIAQYTSALLAGTITSGWTFGAGAALQIPFAMQMAYRFNGIGVTQNVLYENQKLIANQFNSAIGKIQDSLSSTASALGKLQDVVNQNAQALNTLVKQLSSNFGAISSVLNDILSRLDPPEAEVQIDRLITGRLQSLQTYVTQQLIRAAEIRASANLAATKMSECVLGQSKRVDFCGKGYHLMSFPQSAPHGVVFLHVTYVPAQEKNFTTAPAICHDGKAHFPREGVFVSNGTHWFVTQRNFYEPQIITTDNTFVSGNCDVVIGIVNNTVYDPLQPELDSFKEELDKYFKNHTSPDVDLGDISGINASVVNIQKEIDRLNEVAKNLNESLIDLQELGKYEQYIKWPWYIWLGFIAGLIAIVMVTIMLCCMTSCCSCLKGCCSCGSCCKFDEDDSEPVLKGVKLHYT

SEQ ID NO: 167 - protein, 1273 aa, Artificial Sequence
  mutant spike protein of SARS-CoV-2 Wuhan variant comprising substitution Y449F, 2-P-mutation (substiutions K986P and V987P) and inoperative furin cleavage site (substitution 682-QQAQ-685)
MFVFLVLLPLVSSQCVNLTTRTQLPPAYTNSFTRGVYYPDKVFRSSVLHSTQDLFLPFFSNVTWFHAIHVSGTNGTKRFDNPVLPFNDGVYFASTEKSNIIRGWIFGTTLDSKTQSLLIVNNATNVVIKVCEFQFCNDPFLGVYYHKNNKSWMESEFRVYSSANNCTFEYVSQPFLMDLEGKQGNFKNLREFVFKNIDGYFKIYSKHTPINLVRDLPQGFSALEPLVDLPIGINITRFQTLLALHRSYLTPGDSSSGWTAGAAAYYVGYLQPRTFLLKYNENGTITDAVDCALDPLSETKCTLKSFTVEKGIYQTSNFRVQPTESIVRFPNITNLCPFGEVFNATRFASVYAWNRKRISNCVADYSVLYNSASFSTFKCYGVSPTKLNDLCFTNVYADSFVIRGDEVRQIAPGQTGKIADYNYKLPDDFTGCVIAWNSNNLDSKVGGNFNYLYRLFRKSNLKPFERDISTEIYQAGSTPCNGVEGFNCYFPLQSYGFQPTNGVGYQPYRVVVLSFELLHAPATVCGPKKSTNLVKNKCVNFNFNGLTGTGVLTESNKKFLPFQQFGRDIADTTDAVRDPQTLEILDITPCSFGGVSVITPGTNTSNQVAVLYQDVNCTEVPVAIHADQLTPTWRVYSTGSNVFQTRAGCLIGAEHVNNSYECDIPIGAGICASYQTQTNSPQQAQSVASQSIIAYTMSLGAENSVAYSNNSIAIPTNFTISVTTEILPVSMTKTSVDCTMYICGDSTECSNLLLQYGSFCTQLNRALTGIAVEQDKNTQEVFAQVKQIYKTPPIKDFGGFNFSQILPDPSKPSKRSFIEDLLFNKVTLADAGFIKQYGDCLGDIAARDLICAQKFNGLTVLPPLLTDEMIAQYTSALLAGTITSGWTFGAGAALQIPFAMQMAYRFNGIGVTQNVLYENQKLIANQFNSAIGKIQDSLSSTASALGKLQDVVNQNAQALNTLVKQLSSNFGAISSVLNDILSRLDPPEAEVQIDRLITGRLQSLQTYVTQQLIRAAEIRASANLAATKMSECVLGQSKRVDFCGKGYHLMSFPQSAPHGVVFLHVTYVPAQEKNFTTAPAICHDGKAHFPREGVFVSNGTHWFVTQRNFYEPQIITTDNTFVSGNCDVVIGIVNNTVYDPLQPELDSFKEELDKYFKNHTSPDVDLGDISGINASVVNIQKEIDRLNEVAKNLNESLIDLQELGKYEQYIKWPWYIWLGFIAGLIAIVMVTIMLCCMTSCCSCLKGCCSCGSCCKFDEDDSEPVLKGVKLHYT

SEQ ID NO: 168 - protein, 1273 aa, Artificial Sequence
  mutant spike protein of SARS-CoV-2 Wuhan variant comprising substitution Y449G, 2-P-mutation (substiutions K986P and V987P) and inoperative furin cleavage site (substitution 682-QQAQ-685)
MFVFLVLLPLVSSQCVNLTTRTQLPPAYTNSFTRGVYYPDKVFRSSVLHSTQDLFLPFFSNVTWFHAIHVSGTNGTKRFDNPVLPFNDGVYFASTEKSNIIRGWIFGTTLDSKTQSLLIVNNATNVVIKVCEFQFCNDPFLGVYYHKNNKSWMESEFRVYSSANNCTFEYVSQPFLMDLEGKQGNFKNLREFVFKNIDGYFKIYSKHTPINLVRDLPQGFSALEPLVDLPIGINITRFQTLLALHRSYLTPGDSSSGWTAGAAAYYVGYLQPRTFLLKYNENGTITDAVDCALDPLSETKCTLKSFTVEKGIYQTSNFRVQPTESIVRFPNITNLCPFGEVFNATRFASVYAWNRKRISNCVADYSVLYNSASFSTFKCYGVSPTKLNDLCFTNVYADSFVIRGDEVRQIAPGQTGKIADYNYKLPDDFTGCVIAWNSNNLDSKVGGNGNYLYRLFRKSNLKPFERDISTEIYQAGSTPCNGVEGFNCYFPLQSYGFQPTNGVGYQPYRVVVLSFELLHAPATVCGPKKSTNLVKNKCVNFNFNGLTGTGVLTESNKKFLPFQQFGRDIADTTDAVRDPQTLEILDITPCSFGGVSVITPGTNTSNQVAVLYQDVNCTEVPVAIHADQLTPTWRVYSTGSNVFQTRAGCLIGAEHVNNSYECDIPIGAGICASYQTQTNSPQQAQSVASQSIIAYTMSLGAENSVAYSNNSIAIPTNFTISVTTEILPVSMTKTSVDCTMYICGDSTECSNLLLQYGSFCTQLNRALTGIAVEQDKNTQEVFAQVKQIYKTPPIKDFGGFNFSQILPDPSKPSKRSFIEDLLFNKVTLADAGFIKQYGDCLGDIAARDLICAQKFNGLTVLPPLLTDEMIAQYTSALLAGTITSGWTFGAGAALQIPFAMQMAYRFNGIGVTQNVLYENQKLIANQFNSAIGKIQDSLSSTASALGKLQDVVNQNAQALNTLVKQLSSNFGAISSVLNDILSRLDPPEAEVQIDRLITGRLQSLQTYVTQQLIRAAEIRASANLAATKMSECVLGQSKRVDFCGKGYHLMSFPQSAPHGVVFLHVTYVPAQEKNFTTAPAICHDGKAHFPREGVFVSNGTHWFVTQRNFYEPQIITTDNTFVSGNCDVVIGIVNNTVYDPLQPELDSFKEELDKYFKNHTSPDVDLGDISGINASVVNIQKEIDRLNEVAKNLNESLIDLQELGKYEQYIKWPWYIWLGFIAGLIAIVMVTIMLCCMTSCCSCLKGCCSCGSCCKFDEDDSEPVLKGVKLHYT

SEQ ID NO: 169 - protein, 1273 aa, Artificial Sequence
  mutant spike protein of SARS-CoV-2 Wuhan variant comprising substitution Y449H, 2-P-mutation (substiutions K986P and V987P) and inoperative furin cleavage site (substitution 682-QQAQ-685)
MFVFLVLLPLVSSQCVNLTTRTQLPPAYTNSFTRGVYYPDKVFRSSVLHSTQDLFLPFFSNVTWFHAIHVSGTNGTKRFDNPVLPFNDGVYFASTEKSNIIRGWIFGTTLDSKTQSLLIVNNATNVVIKVCEFQFCNDPFLGVYYHKNNKSWMESEFRVYSSANNCTFEYVSQPFLMDLEGKQGNFKNLREFVFKNIDGYFKIYSKHTPINLVRDLPQGFSALEPLVDLPIGINITRFQTLLALHRSYLTPGDSSSGWTAGAAAYYVGYLQPRTFLLKYNENGTITDAVDCALDPLSETKCTLKSFTVEKGIYQTSNFRVQPTESIVRFPNITNLCPFGEVFNATRFASVYAWNRKRISNCVADYSVLYNSASFSTFKCYGVSPTKLNDLCFTNVYADSFVIRGDEVRQIAPGQTGKIADYNYKLPDDFTGCVIAWNSNNLDSKVGGNHNYLYRLFRKSNLKPFERDISTEIYQAGSTPCNGVEGFNCYFPLQSYGFQPTNGVGYQPYRVVVLSFELLHAPATVCGPKKSTNLVKNKCVNFNFNGLTGTGVLTESNKKFLPFQQFGRDIADTTDAVRDPQTLEILDITPCSFGGVSVITPGTNTSNQVAVLYQDVNCTEVPVAIHADQLTPTWRVYSTGSNVFQTRAGCLIGAEHVNNSYECDIPIGAGICASYQTQTNSPQQAQSVASQSIIAYTMSLGAENSVAYSNNSIAIPTNFTISVTTEILPVSMTKTSVDCTMYICGDSTECSNLLLQYGSFCTQLNRALTGIAVEQDKNTQEVFAQVKQIYKTPPIKDFGGFNFSQILPDPSKPSKRSFIEDLLFNKVTLADAGFIKQYGDCLGDIAARDLICAQKFNGLTVLPPLLTDEMIAQYTSALLAGTITSGWTFGAGAALQIPFAMQMAYRFNGIGVTQNVLYENQKLIANQFNSAIGKIQDSLSSTASALGKLQDVVNQNAQALNTLVKQLSSNFGAISSVLNDILSRLDPPEAEVQIDRLITGRLQSLQTYVTQQLIRAAEIRASANLAATKMSECVLGQSKRVDFCGKGYHLMSFPQSAPHGVVFLHVTYVPAQEKNFTTAPAICHDGKAHFPREGVFVSNGTHWFVTQRNFYEPQIITTDNTFVSGNCDVVIGIVNNTVYDPLQPELDSFKEELDKYFKNHTSPDVDLGDISGINASVVNIQKEIDRLNEVAKNLNESLIDLQELGKYEQYIKWPWYIWLGFIAGLIAIVMVTIMLCCMTSCCSCLKGCCSCGSCCKFDEDDSEPVLKGVKLHYT

SEQ ID NO: 170 - protein, 1273 aa, Artificial Sequence
  mutant spike protein of SARS-CoV-2 Wuhan variant comprising substitution Y449I, 2-P-mutation (substiutions K986P and V987P) and inoperative furin cleavage site (substitution 682-QQAQ-685)
MFVFLVLLPLVSSQCVNLTTRTQLPPAYTNSFTRGVYYPDKVFRSSVLHSTQDLFLPFFSNVTWFHAIHVSGTNGTKRFDNPVLPFNDGVYFASTEKSNIIRGWIFGTTLDSKTQSLLIVNNATNVVIKVCEFQFCNDPFLGVYYHKNNKSWMESEFRVYSSANNCTFEYVSQPFLMDLEGKQGNFKNLREFVFKNIDGYFKIYSKHTPINLVRDLPQGFSALEPLVDLPIGINITRFQTLLALHRSYLTPGDSSSGWTAGAAAYYVGYLQPRTFLLKYNENGTITDAVDCALDPLSETKCTLKSFTVEKGIYQTSNFRVQPTESIVRFPNITNLCPFGEVFNATRFASVYAWNRKRISNCVADYSVLYNSASFSTFKCYGVSPTKLNDLCFTNVYADSFVIRGDEVRQIAPGQTGKIADYNYKLPDDFTGCVIAWNSNNLDSKVGGNINYLYRLFRKSNLKPFERDISTEIYQAGSTPCNGVEGFNCYFPLQSYGFQPTNGVGYQPYRVVVLSFELLHAPATVCGPKKSTNLVKNKCVNFNFNGLTGTGVLTESNKKFLPFQQFGRDIADTTDAVRDPQTLEILDITPCSFGGVSVITPGTNTSNQVAVLYQDVNCTEVPVAIHADQLTPTWRVYSTGSNVFQTRAGCLIGAEHVNNSYECDIPIGAGICASYQTQTNSPQQAQSVASQSIIAYTMSLGAENSVAYSNNSIAIPTNFTISVTTEILPVSMTKTSVDCTMYICGDSTECSNLLLQYGSFCTQLNRALTGIAVEQDKNTQEVFAQVKQIYKTPPIKDFGGFNFSQILPDPSKPSKRSFIEDLLFNKVTLADAGFIKQYGDCLGDIAARDLICAQKFNGLTVLPPLLTDEMIAQYTSALLAGTITSGWTFGAGAALQIPFAMQMAYRFNGIGVTQNVLYENQKLIANQFNSAIGKIQDSLSSTASALGKLQDVVNQNAQALNTLVKQLSSNFGAISSVLNDILSRLDPPEAEVQIDRLITGRLQSLQTYVTQQLIRAAEIRASANLAATKMSECVLGQSKRVDFCGKGYHLMSFPQSAPHGVVFLHVTYVPAQEKNFTTAPAICHDGKAHFPREGVFVSNGTHWFVTQRNFYEPQIITTDNTFVSGNCDVVIGIVNNTVYDPLQPELDSFKEELDKYFKNHTSPDVDLGDISGINASVVNIQKEIDRLNEVAKNLNESLIDLQELGKYEQYIKWPWYIWLGFIAGLIAIVMVTIMLCCMTSCCSCLKGCCSCGSCCKFDEDDSEPVLKGVKLHYT

SEQ ID NO: 171 - protein, 1273 aa, Artificial Sequence
  mutant spike protein of SARS-CoV-2 Wuhan variant comprising substitution Y449L, 2-P-mutation (substiutions K986P and V987P) and inoperative furin cleavage site (substitution 682-QQAQ-685)
MFVFLVLLPLVSSQCVNLTTRTQLPPAYTNSFTRGVYYPDKVFRSSVLHSTQDLFLPFFSNVTWFHAIHVSGTNGTKRFDNPVLPFNDGVYFASTEKSNIIRGWIFGTTLDSKTQSLLIVNNATNVVIKVCEFQFCNDPFLGVYYHKNNKSWMESEFRVYSSANNCTFEYVSQPFLMDLEGKQGNFKNLREFVFKNIDGYFKIYSKHTPINLVRDLPQGFSALEPLVDLPIGINITRFQTLLALHRSYLTPGDSSSGWTAGAAAYYVGYLQPRTFLLKYNENGTITDAVDCALDPLSETKCTLKSFTVEKGIYQTSNFRVQPTESIVRFPNITNLCPFGEVFNATRFASVYAWNRKRISNCVADYSVLYNSASFSTFKCYGVSPTKLNDLCFTNVYADSFVIRGDEVRQIAPGQTGKIADYNYKLPDDFTGCVIAWNSNNLDSKVGGNLNYLYRLFRKSNLKPFERDISTEIYQAGSTPCNGVEGFNCYFPLQSYGFQPTNGVGYQPYRVVVLSFELLHAPATVCGPKKSTNLVKNKCVNFNFNGLTGTGVLTESNKKFLPFQQFGRDIADTTDAVRDPQTLEILDITPCSFGGVSVITPGTNTSNQVAVLYQDVNCTEVPVAIHADQLTPTWRVYSTGSNVFQTRAGCLIGAEHVNNSYECDIPIGAGICASYQTQTNSPQQAQSVASQSIIAYTMSLGAENSVAYSNNSIAIPTNFTISVTTEILPVSMTKTSVDCTMYICGDSTECSNLLLQYGSFCTQLNRALTGIAVEQDKNTQEVFAQVKQIYKTPPIKDFGGFNFSQILPDPSKPSKRSFIEDLLFNKVTLADAGFIKQYGDCLGDIAARDLICAQKFNGLTVLPPLLTDEMIAQYTSALLAGTITSGWTFGAGAALQIPFAMQMAYRFNGIGVTQNVLYENQKLIANQFNSAIGKIQDSLSSTASALGKLQDVVNQNAQALNTLVKQLSSNFGAISSVLNDILSRLDPPEAEVQIDRLITGRLQSLQTYVTQQLIRAAEIRASANLAATKMSECVLGQSKRVDFCGKGYHLMSFPQSAPHGVVFLHVTYVPAQEKNFTTAPAICHDGKAHFPREGVFVSNGTHWFVTQRNFYEPQIITTDNTFVSGNCDVVIGIVNNTVYDPLQPELDSFKEELDKYFKNHTSPDVDLGDISGINASVVNIQKEIDRLNEVAKNLNESLIDLQELGKYEQYIKWPWYIWLGFIAGLIAIVMVTIMLCCMTSCCSCLKGCCSCGSCCKFDEDDSEPVLKGVKLHYT

SEQ ID NO: 172 - protein, 1273 aa, Artificial Sequence
  mutant spike protein of SARS-CoV-2 Wuhan variant comprising substitution Y449M, 2-P-mutation (substiutions K986P and V987P) and inoperative furin cleavage site (substitution 682-QQAQ-685)
MFVFLVLLPLVSSQCVNLTTRTQLPPAYTNSFTRGVYYPDKVFRSSVLHSTQDLFLPFFSNVTWFHAIHVSGTNGTKRFDNPVLPFNDGVYFASTEKSNIIRGWIFGTTLDSKTQSLLIVNNATNVVIKVCEFQFCNDPFLGVYYHKNNKSWMESEFRVYSSANNCTFEYVSQPFLMDLEGKQGNFKNLREFVFKNIDGYFKIYSKHTPINLVRDLPQGFSALEPLVDLPIGINITRFQTLLALHRSYLTPGDSSSGWTAGAAAYYVGYLQPRTFLLKYNENGTITDAVDCALDPLSETKCTLKSFTVEKGIYQTSNFRVQPTESIVRFPNITNLCPFGEVFNATRFASVYAWNRKRISNCVADYSVLYNSASFSTFKCYGVSPTKLNDLCFTNVYADSFVIRGDEVRQIAPGQTGKIADYNYKLPDDFTGCVIAWNSNNLDSKVGGNMNYLYRLFRKSNLKPFERDISTEIYQAGSTPCNGVEGFNCYFPLQSYGFQPTNGVGYQPYRVVVLSFELLHAPATVCGPKKSTNLVKNKCVNFNFNGLTGTGVLTESNKKFLPFQQFGRDIADTTDAVRDPQTLEILDITPCSFGGVSVITPGTNTSNQVAVLYQDVNCTEVPVAIHADQLTPTWRVYSTGSNVFQTRAGCLIGAEHVNNSYECDIPIGAGICASYQTQTNSPQQAQSVASQSIIAYTMSLGAENSVAYSNNSIAIPTNFTISVTTEILPVSMTKTSVDCTMYICGDSTECSNLLLQYGSFCTQLNRALTGIAVEQDKNTQEVFAQVKQIYKTPPIKDFGGFNFSQILPDPSKPSKRSFIEDLLFNKVTLADAGFIKQYGDCLGDIAARDLICAQKFNGLTVLPPLLTDEMIAQYTSALLAGTITSGWTFGAGAALQIPFAMQMAYRFNGIGVTQNVLYENQKLIANQFNSAIGKIQDSLSSTASALGKLQDVVNQNAQALNTLVKQLSSNFGAISSVLNDILSRLDPPEAEVQIDRLITGRLQSLQTYVTQQLIRAAEIRASANLAATKMSECVLGQSKRVDFCGKGYHLMSFPQSAPHGVVFLHVTYVPAQEKNFTTAPAICHDGKAHFPREGVFVSNGTHWFVTQRNFYEPQIITTDNTFVSGNCDVVIGIVNNTVYDPLQPELDSFKEELDKYFKNHTSPDVDLGDISGINASVVNIQKEIDRLNEVAKNLNESLIDLQELGKYEQYIKWPWYIWLGFIAGLIAIVMVTIMLCCMTSCCSCLKGCCSCGSCCKFDEDDSEPVLKGVKLHYT

SEQ ID NO: 173 - protein, 1273 aa, Artificial Sequence
  mutant spike protein of SARS-CoV-2 Wuhan variant comprising substitution Y449N, 2-P-mutation (substiutions K986P and V987P) and inoperative furin cleavage site (substitution 682-QQAQ-685)
MFVFLVLLPLVSSQCVNLTTRTQLPPAYTNSFTRGVYYPDKVFRSSVLHSTQDLFLPFFSNVTWFHAIHVSGTNGTKRFDNPVLPFNDGVYFASTEKSNIIRGWIFGTTLDSKTQSLLIVNNATNVVIKVCEFQFCNDPFLGVYYHKNNKSWMESEFRVYSSANNCTFEYVSQPFLMDLEGKQGNFKNLREFVFKNIDGYFKIYSKHTPINLVRDLPQGFSALEPLVDLPIGINITRFQTLLALHRSYLTPGDSSSGWTAGAAAYYVGYLQPRTFLLKYNENGTITDAVDCALDPLSETKCTLKSFTVEKGIYQTSNFRVQPTESIVRFPNITNLCPFGEVFNATRFASVYAWNRKRISNCVADYSVLYNSASFSTFKCYGVSPTKLNDLCFTNVYADSFVIRGDEVRQIAPGQTGKIADYNYKLPDDFTGCVIAWNSNNLDSKVGGNNNYLYRLFRKSNLKPFERDISTEIYQAGSTPCNGVEGFNCYFPLQSYGFQPTNGVGYQPYRVVVLSFELLHAPATVCGPKKSTNLVKNKCVNFNFNGLTGTGVLTESNKKFLPFQQFGRDIADTTDAVRDPQTLEILDITPCSFGGVSVITPGTNTSNQVAVLYQDVNCTEVPVAIHADQLTPTWRVYSTGSNVFQTRAGCLIGAEHVNNSYECDIPIGAGICASYQTQTNSPQQAQSVASQSIIAYTMSLGAENSVAYSNNSIAIPTNFTISVTTEILPVSMTKTSVDCTMYICGDSTECSNLLLQYGSFCTQLNRALTGIAVEQDKNTQEVFAQVKQIYKTPPIKDFGGFNFSQILPDPSKPSKRSFIEDLLFNKVTLADAGFIKQYGDCLGDIAARDLICAQKFNGLTVLPPLLTDEMIAQYTSALLAGTITSGWTFGAGAALQIPFAMQMAYRFNGIGVTQNVLYENQKLIANQFNSAIGKIQDSLSSTASALGKLQDVVNQNAQALNTLVKQLSSNFGAISSVLNDILSRLDPPEAEVQIDRLITGRLQSLQTYVTQQLIRAAEIRASANLAATKMSECVLGQSKRVDFCGKGYHLMSFPQSAPHGVVFLHVTYVPAQEKNFTTAPAICHDGKAHFPREGVFVSNGTHWFVTQRNFYEPQIITTDNTFVSGNCDVVIGIVNNTVYDPLQPELDSFKEELDKYFKNHTSPDVDLGDISGINASVVNIQKEIDRLNEVAKNLNESLIDLQELGKYEQYIKWPWYIWLGFIAGLIAIVMVTIMLCCMTSCCSCLKGCCSCGSCCKFDEDDSEPVLKGVKLHYT

SEQ ID NO: 174 - protein, 1273 aa, Artificial Sequence
  mutant spike protein of SARS-CoV-2 Wuhan variant comprising substitution Y449P, 2-P-mutation (substiutions K986P and V987P) and inoperative furin cleavage site (substitution 682-QQAQ-685)
MFVFLVLLPLVSSQCVNLTTRTQLPPAYTNSFTRGVYYPDKVFRSSVLHSTQDLFLPFFSNVTWFHAIHVSGTNGTKRFDNPVLPFNDGVYFASTEKSNIIRGWIFGTTLDSKTQSLLIVNNATNVVIKVCEFQFCNDPFLGVYYHKNNKSWMESEFRVYSSANNCTFEYVSQPFLMDLEGKQGNFKNLREFVFKNIDGYFKIYSKHTPINLVRDLPQGFSALEPLVDLPIGINITRFQTLLALHRSYLTPGDSSSGWTAGAAAYYVGYLQPRTFLLKYNENGTITDAVDCALDPLSETKCTLKSFTVEKGIYQTSNFRVQPTESIVRFPNITNLCPFGEVFNATRFASVYAWNRKRISNCVADYSVLYNSASFSTFKCYGVSPTKLNDLCFTNVYADSFVIRGDEVRQIAPGQTGKIADYNYKLPDDFTGCVIAWNSNNLDSKVGGNPNYLYRLFRKSNLKPFERDISTEIYQAGSTPCNGVEGFNCYFPLQSYGFQPTNGVGYQPYRVVVLSFELLHAPATVCGPKKSTNLVKNKCVNFNFNGLTGTGVLTESNKKFLPFQQFGRDIADTTDAVRDPQTLEILDITPCSFGGVSVITPGTNTSNQVAVLYQDVNCTEVPVAIHADQLTPTWRVYSTGSNVFQTRAGCLIGAEHVNNSYECDIPIGAGICASYQTQTNSPQQAQSVASQSIIAYTMSLGAENSVAYSNNSIAIPTNFTISVTTEILPVSMTKTSVDCTMYICGDSTECSNLLLQYGSFCTQLNRALTGIAVEQDKNTQEVFAQVKQIYKTPPIKDFGGFNFSQILPDPSKPSKRSFIEDLLFNKVTLADAGFIKQYGDCLGDIAARDLICAQKFNGLTVLPPLLTDEMIAQYTSALLAGTITSGWTFGAGAALQIPFAMQMAYRFNGIGVTQNVLYENQKLIANQFNSAIGKIQDSLSSTASALGKLQDVVNQNAQALNTLVKQLSSNFGAISSVLNDILSRLDPPEAEVQIDRLITGRLQSLQTYVTQQLIRAAEIRASANLAATKMSECVLGQSKRVDFCGKGYHLMSFPQSAPHGVVFLHVTYVPAQEKNFTTAPAICHDGKAHFPREGVFVSNGTHWFVTQRNFYEPQIITTDNTFVSGNCDVVIGIVNNTVYDPLQPELDSFKEELDKYFKNHTSPDVDLGDISGINASVVNIQKEIDRLNEVAKNLNESLIDLQELGKYEQYIKWPWYIWLGFIAGLIAIVMVTIMLCCMTSCCSCLKGCCSCGSCCKFDEDDSEPVLKGVKLHYT

SEQ ID NO: 175 - protein, 1273 aa, Artificial Sequence
  mutant spike protein of SARS-CoV-2 Wuhan variant comprising substitution Y449Q, 2-P-mutation (substiutions K986P and V987P) and inoperative furin cleavage site (substitution 682-QQAQ-685)
MFVFLVLLPLVSSQCVNLTTRTQLPPAYTNSFTRGVYYPDKVFRSSVLHSTQDLFLPFFSNVTWFHAIHVSGTNGTKRFDNPVLPFNDGVYFASTEKSNIIRGWIFGTTLDSKTQSLLIVNNATNVVIKVCEFQFCNDPFLGVYYHKNNKSWMESEFRVYSSANNCTFEYVSQPFLMDLEGKQGNFKNLREFVFKNIDGYFKIYSKHTPINLVRDLPQGFSALEPLVDLPIGINITRFQTLLALHRSYLTPGDSSSGWTAGAAAYYVGYLQPRTFLLKYNENGTITDAVDCALDPLSETKCTLKSFTVEKGIYQTSNFRVQPTESIVRFPNITNLCPFGEVFNATRFASVYAWNRKRISNCVADYSVLYNSASFSTFKCYGVSPTKLNDLCFTNVYADSFVIRGDEVRQIAPGQTGKIADYNYKLPDDFTGCVIAWNSNNLDSKVGGNQNYLYRLFRKSNLKPFERDISTEIYQAGSTPCNGVEGFNCYFPLQSYGFQPTNGVGYQPYRVVVLSFELLHAPATVCGPKKSTNLVKNKCVNFNFNGLTGTGVLTESNKKFLPFQQFGRDIADTTDAVRDPQTLEILDITPCSFGGVSVITPGTNTSNQVAVLYQDVNCTEVPVAIHADQLTPTWRVYSTGSNVFQTRAGCLIGAEHVNNSYECDIPIGAGICASYQTQTNSPQQAQSVASQSIIAYTMSLGAENSVAYSNNSIAIPTNFTISVTTEILPVSMTKTSVDCTMYICGDSTECSNLLLQYGSFCTQLNRALTGIAVEQDKNTQEVFAQVKQIYKTPPIKDFGGFNFSQILPDPSKPSKRSFIEDLLFNKVTLADAGFIKQYGDCLGDIAARDLICAQKFNGLTVLPPLLTDEMIAQYTSALLAGTITSGWTFGAGAALQIPFAMQMAYRFNGIGVTQNVLYENQKLIANQFNSAIGKIQDSLSSTASALGKLQDVVNQNAQALNTLVKQLSSNFGAISSVLNDILSRLDPPEAEVQIDRLITGRLQSLQTYVTQQLIRAAEIRASANLAATKMSECVLGQSKRVDFCGKGYHLMSFPQSAPHGVVFLHVTYVPAQEKNFTTAPAICHDGKAHFPREGVFVSNGTHWFVTQRNFYEPQIITTDNTFVSGNCDVVIGIVNNTVYDPLQPELDSFKEELDKYFKNHTSPDVDLGDISGINASVVNIQKEIDRLNEVAKNLNESLIDLQELGKYEQYIKWPWYIWLGFIAGLIAIVMVTIMLCCMTSCCSCLKGCCSCGSCCKFDEDDSEPVLKGVKLHYT

SEQ ID NO: 176 - protein, 1273 aa, Artificial Sequence
  mutant spike protein of SARS-CoV-2 Wuhan variant comprising substitution Y449S, 2-P-mutation (substiutions K986P and V987P) and inoperative furin cleavage site (substitution 682-QQAQ-685)
MFVFLVLLPLVSSQCVNLTTRTQLPPAYTNSFTRGVYYPDKVFRSSVLHSTQDLFLPFFSNVTWFHAIHVSGTNGTKRFDNPVLPFNDGVYFASTEKSNIIRGWIFGTTLDSKTQSLLIVNNATNVVIKVCEFQFCNDPFLGVYYHKNNKSWMESEFRVYSSANNCTFEYVSQPFLMDLEGKQGNFKNLREFVFKNIDGYFKIYSKHTPINLVRDLPQGFSALEPLVDLPIGINITRFQTLLALHRSYLTPGDSSSGWTAGAAAYYVGYLQPRTFLLKYNENGTITDAVDCALDPLSETKCTLKSFTVEKGIYQTSNFRVQPTESIVRFPNITNLCPFGEVFNATRFASVYAWNRKRISNCVADYSVLYNSASFSTFKCYGVSPTKLNDLCFTNVYADSFVIRGDEVRQIAPGQTGKIADYNYKLPDDFTGCVIAWNSNNLDSKVGGNSNYLYRLFRKSNLKPFERDISTEIYQAGSTPCNGVEGFNCYFPLQSYGFQPTNGVGYQPYRVVVLSFELLHAPATVCGPKKSTNLVKNKCVNFNFNGLTGTGVLTESNKKFLPFQQFGRDIADTTDAVRDPQTLEILDITPCSFGGVSVITPGTNTSNQVAVLYQDVNCTEVPVAIHADQLTPTWRVYSTGSNVFQTRAGCLIGAEHVNNSYECDIPIGAGICASYQTQTNSPQQAQSVASQSIIAYTMSLGAENSVAYSNNSIAIPTNFTISVTTEILPVSMTKTSVDCTMYICGDSTECSNLLLQYGSFCTQLNRALTGIAVEQDKNTQEVFAQVKQIYKTPPIKDFGGFNFSQILPDPSKPSKRSFIEDLLFNKVTLADAGFIKQYGDCLGDIAARDLICAQKFNGLTVLPPLLTDEMIAQYTSALLAGTITSGWTFGAGAALQIPFAMQMAYRFNGIGVTQNVLYENQKLIANQFNSAIGKIQDSLSSTASALGKLQDVVNQNAQALNTLVKQLSSNFGAISSVLNDILSRLDPPEAEVQIDRLITGRLQSLQTYVTQQLIRAAEIRASANLAATKMSECVLGQSKRVDFCGKGYHLMSFPQSAPHGVVFLHVTYVPAQEKNFTTAPAICHDGKAHFPREGVFVSNGTHWFVTQRNFYEPQIITTDNTFVSGNCDVVIGIVNNTVYDPLQPELDSFKEELDKYFKNHTSPDVDLGDISGINASVVNIQKEIDRLNEVAKNLNESLIDLQELGKYEQYIKWPWYIWLGFIAGLIAIVMVTIMLCCMTSCCSCLKGCCSCGSCCKFDEDDSEPVLKGVKLHYT

SEQ ID NO: 177 - protein, 1273 aa, Artificial Sequence
  mutant spike protein of SARS-CoV-2 Wuhan variant comprising substitution Y449T, 2-P-mutation (substiutions K986P and V987P) and inoperative furin cleavage site (substitution 682-QQAQ-685)
MFVFLVLLPLVSSQCVNLTTRTQLPPAYTNSFTRGVYYPDKVFRSSVLHSTQDLFLPFFSNVTWFHAIHVSGTNGTKRFDNPVLPFNDGVYFASTEKSNIIRGWIFGTTLDSKTQSLLIVNNATNVVIKVCEFQFCNDPFLGVYYHKNNKSWMESEFRVYSSANNCTFEYVSQPFLMDLEGKQGNFKNLREFVFKNIDGYFKIYSKHTPINLVRDLPQGFSALEPLVDLPIGINITRFQTLLALHRSYLTPGDSSSGWTAGAAAYYVGYLQPRTFLLKYNENGTITDAVDCALDPLSETKCTLKSFTVEKGIYQTSNFRVQPTESIVRFPNITNLCPFGEVFNATRFASVYAWNRKRISNCVADYSVLYNSASFSTFKCYGVSPTKLNDLCFTNVYADSFVIRGDEVRQIAPGQTGKIADYNYKLPDDFTGCVIAWNSNNLDSKVGGNTNYLYRLFRKSNLKPFERDISTEIYQAGSTPCNGVEGFNCYFPLQSYGFQPTNGVGYQPYRVVVLSFELLHAPATVCGPKKSTNLVKNKCVNFNFNGLTGTGVLTESNKKFLPFQQFGRDIADTTDAVRDPQTLEILDITPCSFGGVSVITPGTNTSNQVAVLYQDVNCTEVPVAIHADQLTPTWRVYSTGSNVFQTRAGCLIGAEHVNNSYECDIPIGAGICASYQTQTNSPQQAQSVASQSIIAYTMSLGAENSVAYSNNSIAIPTNFTISVTTEILPVSMTKTSVDCTMYICGDSTECSNLLLQYGSFCTQLNRALTGIAVEQDKNTQEVFAQVKQIYKTPPIKDFGGFNFSQILPDPSKPSKRSFIEDLLFNKVTLADAGFIKQYGDCLGDIAARDLICAQKFNGLTVLPPLLTDEMIAQYTSALLAGTITSGWTFGAGAALQIPFAMQMAYRFNGIGVTQNVLYENQKLIANQFNSAIGKIQDSLSSTASALGKLQDVVNQNAQALNTLVKQLSSNFGAISSVLNDILSRLDPPEAEVQIDRLITGRLQSLQTYVTQQLIRAAEIRASANLAATKMSECVLGQSKRVDFCGKGYHLMSFPQSAPHGVVFLHVTYVPAQEKNFTTAPAICHDGKAHFPREGVFVSNGTHWFVTQRNFYEPQIITTDNTFVSGNCDVVIGIVNNTVYDPLQPELDSFKEELDKYFKNHTSPDVDLGDISGINASVVNIQKEIDRLNEVAKNLNESLIDLQELGKYEQYIKWPWYIWLGFIAGLIAIVMVTIMLCCMTSCCSCLKGCCSCGSCCKFDEDDSEPVLKGVKLHYT

SEQ ID NO: 178 - protein, 1273 aa, Artificial Sequence
  mutant spike protein of SARS-CoV-2 Wuhan variant comprising substitution Y449V, 2-P-mutation (substiutions K986P and V987P) and inoperative furin cleavage site (substitution 682-QQAQ-685)
MFVFLVLLPLVSSQCVNLTTRTQLPPAYTNSFTRGVYYPDKVFRSSVLHSTQDLFLPFFSNVTWFHAIHVSGTNGTKRFDNPVLPFNDGVYFASTEKSNIIRGWIFGTTLDSKTQSLLIVNNATNVVIKVCEFQFCNDPFLGVYYHKNNKSWMESEFRVYSSANNCTFEYVSQPFLMDLEGKQGNFKNLREFVFKNIDGYFKIYSKHTPINLVRDLPQGFSALEPLVDLPIGINITRFQTLLALHRSYLTPGDSSSGWTAGAAAYYVGYLQPRTFLLKYNENGTITDAVDCALDPLSETKCTLKSFTVEKGIYQTSNFRVQPTESIVRFPNITNLCPFGEVFNATRFASVYAWNRKRISNCVADYSVLYNSASFSTFKCYGVSPTKLNDLCFTNVYADSFVIRGDEVRQIAPGQTGKIADYNYKLPDDFTGCVIAWNSNNLDSKVGGNVNYLYRLFRKSNLKPFERDISTEIYQAGSTPCNGVEGFNCYFPLQSYGFQPTNGVGYQPYRVVVLSFELLHAPATVCGPKKSTNLVKNKCVNFNFNGLTGTGVLTESNKKFLPFQQFGRDIADTTDAVRDPQTLEILDITPCSFGGVSVITPGTNTSNQVAVLYQDVNCTEVPVAIHADQLTPTWRVYSTGSNVFQTRAGCLIGAEHVNNSYECDIPIGAGICASYQTQTNSPQQAQSVASQSIIAYTMSLGAENSVAYSNNSIAIPTNFTISVTTEILPVSMTKTSVDCTMYICGDSTECSNLLLQYGSFCTQLNRALTGIAVEQDKNTQEVFAQVKQIYKTPPIKDFGGFNFSQILPDPSKPSKRSFIEDLLFNKVTLADAGFIKQYGDCLGDIAARDLICAQKFNGLTVLPPLLTDEMIAQYTSALLAGTITSGWTFGAGAALQIPFAMQMAYRFNGIGVTQNVLYENQKLIANQFNSAIGKIQDSLSSTASALGKLQDVVNQNAQALNTLVKQLSSNFGAISSVLNDILSRLDPPEAEVQIDRLITGRLQSLQTYVTQQLIRAAEIRASANLAATKMSECVLGQSKRVDFCGKGYHLMSFPQSAPHGVVFLHVTYVPAQEKNFTTAPAICHDGKAHFPREGVFVSNGTHWFVTQRNFYEPQIITTDNTFVSGNCDVVIGIVNNTVYDPLQPELDSFKEELDKYFKNHTSPDVDLGDISGINASVVNIQKEIDRLNEVAKNLNESLIDLQELGKYEQYIKWPWYIWLGFIAGLIAIVMVTIMLCCMTSCCSCLKGCCSCGSCCKFDEDDSEPVLKGVKLHYT

SEQ ID NO: 179 - protein, 1273 aa, Artificial Sequence
  mutant spike protein of SARS-CoV-2 Wuhan variant comprising substitution Y449W, 2-P-mutation (substiutions K986P and V987P) and inoperative furin cleavage site (substitution 682-QQAQ-685)
MFVFLVLLPLVSSQCVNLTTRTQLPPAYTNSFTRGVYYPDKVFRSSVLHSTQDLFLPFFSNVTWFHAIHVSGTNGTKRFDNPVLPFNDGVYFASTEKSNIIRGWIFGTTLDSKTQSLLIVNNATNVVIKVCEFQFCNDPFLGVYYHKNNKSWMESEFRVYSSANNCTFEYVSQPFLMDLEGKQGNFKNLREFVFKNIDGYFKIYSKHTPINLVRDLPQGFSALEPLVDLPIGINITRFQTLLALHRSYLTPGDSSSGWTAGAAAYYVGYLQPRTFLLKYNENGTITDAVDCALDPLSETKCTLKSFTVEKGIYQTSNFRVQPTESIVRFPNITNLCPFGEVFNATRFASVYAWNRKRISNCVADYSVLYNSASFSTFKCYGVSPTKLNDLCFTNVYADSFVIRGDEVRQIAPGQTGKIADYNYKLPDDFTGCVIAWNSNNLDSKVGGNWNYLYRLFRKSNLKPFERDISTEIYQAGSTPCNGVEGFNCYFPLQSYGFQPTNGVGYQPYRVVVLSFELLHAPATVCGPKKSTNLVKNKCVNFNFNGLTGTGVLTESNKKFLPFQQFGRDIADTTDAVRDPQTLEILDITPCSFGGVSVITPGTNTSNQVAVLYQDVNCTEVPVAIHADQLTPTWRVYSTGSNVFQTRAGCLIGAEHVNNSYECDIPIGAGICASYQTQTNSPQQAQSVASQSIIAYTMSLGAENSVAYSNNSIAIPTNFTISVTTEILPVSMTKTSVDCTMYICGDSTECSNLLLQYGSFCTQLNRALTGIAVEQDKNTQEVFAQVKQIYKTPPIKDFGGFNFSQILPDPSKPSKRSFIEDLLFNKVTLADAGFIKQYGDCLGDIAARDLICAQKFNGLTVLPPLLTDEMIAQYTSALLAGTITSGWTFGAGAALQIPFAMQMAYRFNGIGVTQNVLYENQKLIANQFNSAIGKIQDSLSSTASALGKLQDVVNQNAQALNTLVKQLSSNFGAISSVLNDILSRLDPPEAEVQIDRLITGRLQSLQTYVTQQLIRAAEIRASANLAATKMSECVLGQSKRVDFCGKGYHLMSFPQSAPHGVVFLHVTYVPAQEKNFTTAPAICHDGKAHFPREGVFVSNGTHWFVTQRNFYEPQIITTDNTFVSGNCDVVIGIVNNTVYDPLQPELDSFKEELDKYFKNHTSPDVDLGDISGINASVVNIQKEIDRLNEVAKNLNESLIDLQELGKYEQYIKWPWYIWLGFIAGLIAIVMVTIMLCCMTSCCSCLKGCCSCGSCCKFDEDDSEPVLKGVKLHYT

SEQ ID NO: 180 - protein, 1273 aa, Artificial Sequence
  mutant spike protein of SARS-CoV-2 Wuhan variant comprising substitution Y489A, 2-P-mutation (substiutions K986P and V987P) and inoperative furin cleavage site (substitution 682-QQAQ-685)
MFVFLVLLPLVSSQCVNLTTRTQLPPAYTNSFTRGVYYPDKVFRSSVLHSTQDLFLPFFSNVTWFHAIHVSGTNGTKRFDNPVLPFNDGVYFASTEKSNIIRGWIFGTTLDSKTQSLLIVNNATNVVIKVCEFQFCNDPFLGVYYHKNNKSWMESEFRVYSSANNCTFEYVSQPFLMDLEGKQGNFKNLREFVFKNIDGYFKIYSKHTPINLVRDLPQGFSALEPLVDLPIGINITRFQTLLALHRSYLTPGDSSSGWTAGAAAYYVGYLQPRTFLLKYNENGTITDAVDCALDPLSETKCTLKSFTVEKGIYQTSNFRVQPTESIVRFPNITNLCPFGEVFNATRFASVYAWNRKRISNCVADYSVLYNSASFSTFKCYGVSPTKLNDLCFTNVYADSFVIRGDEVRQIAPGQTGKIADYNYKLPDDFTGCVIAWNSNNLDSKVGGNYNYLYRLFRKSNLKPFERDISTEIYQAGSTPCNGVEGFNCAFPLQSYGFQPTNGVGYQPYRVVVLSFELLHAPATVCGPKKSTNLVKNKCVNFNFNGLTGTGVLTESNKKFLPFQQFGRDIADTTDAVRDPQTLEILDITPCSFGGVSVITPGTNTSNQVAVLYQDVNCTEVPVAIHADQLTPTWRVYSTGSNVFQTRAGCLIGAEHVNNSYECDIPIGAGICASYQTQTNSPQQAQSVASQSIIAYTMSLGAENSVAYSNNSIAIPTNFTISVTTEILPVSMTKTSVDCTMYICGDSTECSNLLLQYGSFCTQLNRALTGIAVEQDKNTQEVFAQVKQIYKTPPIKDFGGFNFSQILPDPSKPSKRSFIEDLLFNKVTLADAGFIKQYGDCLGDIAARDLICAQKFNGLTVLPPLLTDEMIAQYTSALLAGTITSGWTFGAGAALQIPFAMQMAYRFNGIGVTQNVLYENQKLIANQFNSAIGKIQDSLSSTASALGKLQDVVNQNAQALNTLVKQLSSNFGAISSVLNDILSRLDPPEAEVQIDRLITGRLQSLQTYVTQQLIRAAEIRASANLAATKMSECVLGQSKRVDFCGKGYHLMSFPQSAPHGVVFLHVTYVPAQEKNFTTAPAICHDGKAHFPREGVFVSNGTHWFVTQRNFYEPQIITTDNTFVSGNCDVVIGIVNNTVYDPLQPELDSFKEELDKYFKNHTSPDVDLGDISGINASVVNIQKEIDRLNEVAKNLNESLIDLQELGKYEQYIKWPWYIWLGFIAGLIAIVMVTIMLCCMTSCCSCLKGCCSCGSCCKFDEDDSEPVLKGVKLHYT

SEQ ID NO: 181 - protein, 1273 aa, Artificial Sequence
  mutant spike protein of SARS-CoV-2 Wuhan variant comprising substitution Y489C, 2-P-mutation (substiutions K986P and V987P) and inoperative furin cleavage site (substitution 682-QQAQ-685)
MFVFLVLLPLVSSQCVNLTTRTQLPPAYTNSFTRGVYYPDKVFRSSVLHSTQDLFLPFFSNVTWFHAIHVSGTNGTKRFDNPVLPFNDGVYFASTEKSNIIRGWIFGTTLDSKTQSLLIVNNATNVVIKVCEFQFCNDPFLGVYYHKNNKSWMESEFRVYSSANNCTFEYVSQPFLMDLEGKQGNFKNLREFVFKNIDGYFKIYSKHTPINLVRDLPQGFSALEPLVDLPIGINITRFQTLLALHRSYLTPGDSSSGWTAGAAAYYVGYLQPRTFLLKYNENGTITDAVDCALDPLSETKCTLKSFTVEKGIYQTSNFRVQPTESIVRFPNITNLCPFGEVFNATRFASVYAWNRKRISNCVADYSVLYNSASFSTFKCYGVSPTKLNDLCFTNVYADSFVIRGDEVRQIAPGQTGKIADYNYKLPDDFTGCVIAWNSNNLDSKVGGNYNYLYRLFRKSNLKPFERDISTEIYQAGSTPCNGVEGFNCCFPLQSYGFQPTNGVGYQPYRVVVLSFELLHAPATVCGPKKSTNLVKNKCVNFNFNGLTGTGVLTESNKKFLPFQQFGRDIADTTDAVRDPQTLEILDITPCSFGGVSVITPGTNTSNQVAVLYQDVNCTEVPVAIHADQLTPTWRVYSTGSNVFQTRAGCLIGAEHVNNSYECDIPIGAGICASYQTQTNSPQQAQSVASQSIIAYTMSLGAENSVAYSNNSIAIPTNFTISVTTEILPVSMTKTSVDCTMYICGDSTECSNLLLQYGSFCTQLNRALTGIAVEQDKNTQEVFAQVKQIYKTPPIKDFGGFNFSQILPDPSKPSKRSFIEDLLFNKVTLADAGFIKQYGDCLGDIAARDLICAQKFNGLTVLPPLLTDEMIAQYTSALLAGTITSGWTFGAGAALQIPFAMQMAYRFNGIGVTQNVLYENQKLIANQFNSAIGKIQDSLSSTASALGKLQDVVNQNAQALNTLVKQLSSNFGAISSVLNDILSRLDPPEAEVQIDRLITGRLQSLQTYVTQQLIRAAEIRASANLAATKMSECVLGQSKRVDFCGKGYHLMSFPQSAPHGVVFLHVTYVPAQEKNFTTAPAICHDGKAHFPREGVFVSNGTHWFVTQRNFYEPQIITTDNTFVSGNCDVVIGIVNNTVYDPLQPELDSFKEELDKYFKNHTSPDVDLGDISGINASVVNIQKEIDRLNEVAKNLNESLIDLQELGKYEQYIKWPWYIWLGFIAGLIAIVMVTIMLCCMTSCCSCLKGCCSCGSCCKFDEDDSEPVLKGVKLHYT

SEQ ID NO: 182 - protein, 1273 aa, Artificial Sequence
  mutant spike protein of SARS-CoV-2 Wuhan variant comprising substitution Y489E, 2-P-mutation (substiutions K986P and V987P) and inoperative furin cleavage site (substitution 682-QQAQ-685)
MFVFLVLLPLVSSQCVNLTTRTQLPPAYTNSFTRGVYYPDKVFRSSVLHSTQDLFLPFFSNVTWFHAIHVSGTNGTKRFDNPVLPFNDGVYFASTEKSNIIRGWIFGTTLDSKTQSLLIVNNATNVVIKVCEFQFCNDPFLGVYYHKNNKSWMESEFRVYSSANNCTFEYVSQPFLMDLEGKQGNFKNLREFVFKNIDGYFKIYSKHTPINLVRDLPQGFSALEPLVDLPIGINITRFQTLLALHRSYLTPGDSSSGWTAGAAAYYVGYLQPRTFLLKYNENGTITDAVDCALDPLSETKCTLKSFTVEKGIYQTSNFRVQPTESIVRFPNITNLCPFGEVFNATRFASVYAWNRKRISNCVADYSVLYNSASFSTFKCYGVSPTKLNDLCFTNVYADSFVIRGDEVRQIAPGQTGKIADYNYKLPDDFTGCVIAWNSNNLDSKVGGNYNYLYRLFRKSNLKPFERDISTEIYQAGSTPCNGVEGFNCEFPLQSYGFQPTNGVGYQPYRVVVLSFELLHAPATVCGPKKSTNLVKNKCVNFNFNGLTGTGVLTESNKKFLPFQQFGRDIADTTDAVRDPQTLEILDITPCSFGGVSVITPGTNTSNQVAVLYQDVNCTEVPVAIHADQLTPTWRVYSTGSNVFQTRAGCLIGAEHVNNSYECDIPIGAGICASYQTQTNSPQQAQSVASQSIIAYTMSLGAENSVAYSNNSIAIPTNFTISVTTEILPVSMTKTSVDCTMYICGDSTECSNLLLQYGSFCTQLNRALTGIAVEQDKNTQEVFAQVKQIYKTPPIKDFGGFNFSQILPDPSKPSKRSFIEDLLFNKVTLADAGFIKQYGDCLGDIAARDLICAQKFNGLTVLPPLLTDEMIAQYTSALLAGTITSGWTFGAGAALQIPFAMQMAYRFNGIGVTQNVLYENQKLIANQFNSAIGKIQDSLSSTASALGKLQDVVNQNAQALNTLVKQLSSNFGAISSVLNDILSRLDPPEAEVQIDRLITGRLQSLQTYVTQQLIRAAEIRASANLAATKMSECVLGQSKRVDFCGKGYHLMSFPQSAPHGVVFLHVTYVPAQEKNFTTAPAICHDGKAHFPREGVFVSNGTHWFVTQRNFYEPQIITTDNTFVSGNCDVVIGIVNNTVYDPLQPELDSFKEELDKYFKNHTSPDVDLGDISGINASVVNIQKEIDRLNEVAKNLNESLIDLQELGKYEQYIKWPWYIWLGFIAGLIAIVMVTIMLCCMTSCCSCLKGCCSCGSCCKFDEDDSEPVLKGVKLHYT

SEQ ID NO: 183 - protein, 1273 aa, Artificial Sequence
  mutant spike protein of SARS-CoV-2 Wuhan variant comprising substitution Y489I, 2-P-mutation (substiutions K986P and V987P) and inoperative furin cleavage site (substitution 682-QQAQ-685)
MFVFLVLLPLVSSQCVNLTTRTQLPPAYTNSFTRGVYYPDKVFRSSVLHSTQDLFLPFFSNVTWFHAIHVSGTNGTKRFDNPVLPFNDGVYFASTEKSNIIRGWIFGTTLDSKTQSLLIVNNATNVVIKVCEFQFCNDPFLGVYYHKNNKSWMESEFRVYSSANNCTFEYVSQPFLMDLEGKQGNFKNLREFVFKNIDGYFKIYSKHTPINLVRDLPQGFSALEPLVDLPIGINITRFQTLLALHRSYLTPGDSSSGWTAGAAAYYVGYLQPRTFLLKYNENGTITDAVDCALDPLSETKCTLKSFTVEKGIYQTSNFRVQPTESIVRFPNITNLCPFGEVFNATRFASVYAWNRKRISNCVADYSVLYNSASFSTFKCYGVSPTKLNDLCFTNVYADSFVIRGDEVRQIAPGQTGKIADYNYKLPDDFTGCVIAWNSNNLDSKVGGNYNYLYRLFRKSNLKPFERDISTEIYQAGSTPCNGVEGFNCIFPLQSYGFQPTNGVGYQPYRVVVLSFELLHAPATVCGPKKSTNLVKNKCVNFNFNGLTGTGVLTESNKKFLPFQQFGRDIADTTDAVRDPQTLEILDITPCSFGGVSVITPGTNTSNQVAVLYQDVNCTEVPVAIHADQLTPTWRVYSTGSNVFQTRAGCLIGAEHVNNSYECDIPIGAGICASYQTQTNSPQQAQSVASQSIIAYTMSLGAENSVAYSNNSIAIPTNFTISVTTEILPVSMTKTSVDCTMYICGDSTECSNLLLQYGSFCTQLNRALTGIAVEQDKNTQEVFAQVKQIYKTPPIKDFGGFNFSQILPDPSKPSKRSFIEDLLFNKVTLADAGFIKQYGDCLGDIAARDLICAQKFNGLTVLPPLLTDEMIAQYTSALLAGTITSGWTFGAGAALQIPFAMQMAYRFNGIGVTQNVLYENQKLIANQFNSAIGKIQDSLSSTASALGKLQDVVNQNAQALNTLVKQLSSNFGAISSVLNDILSRLDPPEAEVQIDRLITGRLQSLQTYVTQQLIRAAEIRASANLAATKMSECVLGQSKRVDFCGKGYHLMSFPQSAPHGVVFLHVTYVPAQEKNFTTAPAICHDGKAHFPREGVFVSNGTHWFVTQRNFYEPQIITTDNTFVSGNCDVVIGIVNNTVYDPLQPELDSFKEELDKYFKNHTSPDVDLGDISGINASVVNIQKEIDRLNEVAKNLNESLIDLQELGKYEQYIKWPWYIWLGFIAGLIAIVMVTIMLCCMTSCCSCLKGCCSCGSCCKFDEDDSEPVLKGVKLHYT

SEQ ID NO: 184 - protein, 1273 aa, Artificial Sequence
  mutant spike protein of SARS-CoV-2 Wuhan variant comprising substitution Y489K, 2-P-mutation (substiutions K986P and V987P) and inoperative furin cleavage site (substitution 682-QQAQ-685)
MFVFLVLLPLVSSQCVNLTTRTQLPPAYTNSFTRGVYYPDKVFRSSVLHSTQDLFLPFFSNVTWFHAIHVSGTNGTKRFDNPVLPFNDGVYFASTEKSNIIRGWIFGTTLDSKTQSLLIVNNATNVVIKVCEFQFCNDPFLGVYYHKNNKSWMESEFRVYSSANNCTFEYVSQPFLMDLEGKQGNFKNLREFVFKNIDGYFKIYSKHTPINLVRDLPQGFSALEPLVDLPIGINITRFQTLLALHRSYLTPGDSSSGWTAGAAAYYVGYLQPRTFLLKYNENGTITDAVDCALDPLSETKCTLKSFTVEKGIYQTSNFRVQPTESIVRFPNITNLCPFGEVFNATRFASVYAWNRKRISNCVADYSVLYNSASFSTFKCYGVSPTKLNDLCFTNVYADSFVIRGDEVRQIAPGQTGKIADYNYKLPDDFTGCVIAWNSNNLDSKVGGNYNYLYRLFRKSNLKPFERDISTEIYQAGSTPCNGVEGFNCKFPLQSYGFQPTNGVGYQPYRVVVLSFELLHAPATVCGPKKSTNLVKNKCVNFNFNGLTGTGVLTESNKKFLPFQQFGRDIADTTDAVRDPQTLEILDITPCSFGGVSVITPGTNTSNQVAVLYQDVNCTEVPVAIHADQLTPTWRVYSTGSNVFQTRAGCLIGAEHVNNSYECDIPIGAGICASYQTQTNSPQQAQSVASQSIIAYTMSLGAENSVAYSNNSIAIPTNFTISVTTEILPVSMTKTSVDCTMYICGDSTECSNLLLQYGSFCTQLNRALTGIAVEQDKNTQEVFAQVKQIYKTPPIKDFGGFNFSQILPDPSKPSKRSFIEDLLFNKVTLADAGFIKQYGDCLGDIAARDLICAQKFNGLTVLPPLLTDEMIAQYTSALLAGTITSGWTFGAGAALQIPFAMQMAYRFNGIGVTQNVLYENQKLIANQFNSAIGKIQDSLSSTASALGKLQDVVNQNAQALNTLVKQLSSNFGAISSVLNDILSRLDPPEAEVQIDRLITGRLQSLQTYVTQQLIRAAEIRASANLAATKMSECVLGQSKRVDFCGKGYHLMSFPQSAPHGVVFLHVTYVPAQEKNFTTAPAICHDGKAHFPREGVFVSNGTHWFVTQRNFYEPQIITTDNTFVSGNCDVVIGIVNNTVYDPLQPELDSFKEELDKYFKNHTSPDVDLGDISGINASVVNIQKEIDRLNEVAKNLNESLIDLQELGKYEQYIKWPWYIWLGFIAGLIAIVMVTIMLCCMTSCCSCLKGCCSCGSCCKFDEDDSEPVLKGVKLHYT

SEQ ID NO: 185 - protein, 1273 aa, Artificial Sequence
  mutant spike protein of SARS-CoV-2 Wuhan variant comprising substitution Y489L, 2-P-mutation (substiutions K986P and V987P) and inoperative furin cleavage site (substitution 682-QQAQ-685)
MFVFLVLLPLVSSQCVNLTTRTQLPPAYTNSFTRGVYYPDKVFRSSVLHSTQDLFLPFFSNVTWFHAIHVSGTNGTKRFDNPVLPFNDGVYFASTEKSNIIRGWIFGTTLDSKTQSLLIVNNATNVVIKVCEFQFCNDPFLGVYYHKNNKSWMESEFRVYSSANNCTFEYVSQPFLMDLEGKQGNFKNLREFVFKNIDGYFKIYSKHTPINLVRDLPQGFSALEPLVDLPIGINITRFQTLLALHRSYLTPGDSSSGWTAGAAAYYVGYLQPRTFLLKYNENGTITDAVDCALDPLSETKCTLKSFTVEKGIYQTSNFRVQPTESIVRFPNITNLCPFGEVFNATRFASVYAWNRKRISNCVADYSVLYNSASFSTFKCYGVSPTKLNDLCFTNVYADSFVIRGDEVRQIAPGQTGKIADYNYKLPDDFTGCVIAWNSNNLDSKVGGNYNYLYRLFRKSNLKPFERDISTEIYQAGSTPCNGVEGFNCLFPLQSYGFQPTNGVGYQPYRVVVLSFELLHAPATVCGPKKSTNLVKNKCVNFNFNGLTGTGVLTESNKKFLPFQQFGRDIADTTDAVRDPQTLEILDITPCSFGGVSVITPGTNTSNQVAVLYQDVNCTEVPVAIHADQLTPTWRVYSTGSNVFQTRAGCLIGAEHVNNSYECDIPIGAGICASYQTQTNSPQQAQSVASQSIIAYTMSLGAENSVAYSNNSIAIPTNFTISVTTEILPVSMTKTSVDCTMYICGDSTECSNLLLQYGSFCTQLNRALTGIAVEQDKNTQEVFAQVKQIYKTPPIKDFGGFNFSQILPDPSKPSKRSFIEDLLFNKVTLADAGFIKQYGDCLGDIAARDLICAQKFNGLTVLPPLLTDEMIAQYTSALLAGTITSGWTFGAGAALQIPFAMQMAYRFNGIGVTQNVLYENQKLIANQFNSAIGKIQDSLSSTASALGKLQDVVNQNAQALNTLVKQLSSNFGAISSVLNDILSRLDPPEAEVQIDRLITGRLQSLQTYVTQQLIRAAEIRASANLAATKMSECVLGQSKRVDFCGKGYHLMSFPQSAPHGVVFLHVTYVPAQEKNFTTAPAICHDGKAHFPREGVFVSNGTHWFVTQRNFYEPQIITTDNTFVSGNCDVVIGIVNNTVYDPLQPELDSFKEELDKYFKNHTSPDVDLGDISGINASVVNIQKEIDRLNEVAKNLNESLIDLQELGKYEQYIKWPWYIWLGFIAGLIAIVMVTIMLCCMTSCCSCLKGCCSCGSCCKFDEDDSEPVLKGVKLHYT

SEQ ID NO: 186 - protein, 1273 aa, Artificial Sequence
  mutant spike protein of SARS-CoV-2 Wuhan variant comprising substitution Y489M, 2-P-mutation (substiutions K986P and V987P) and inoperative furin cleavage site (substitution 682-QQAQ-685)
MFVFLVLLPLVSSQCVNLTTRTQLPPAYTNSFTRGVYYPDKVFRSSVLHSTQDLFLPFFSNVTWFHAIHVSGTNGTKRFDNPVLPFNDGVYFASTEKSNIIRGWIFGTTLDSKTQSLLIVNNATNVVIKVCEFQFCNDPFLGVYYHKNNKSWMESEFRVYSSANNCTFEYVSQPFLMDLEGKQGNFKNLREFVFKNIDGYFKIYSKHTPINLVRDLPQGFSALEPLVDLPIGINITRFQTLLALHRSYLTPGDSSSGWTAGAAAYYVGYLQPRTFLLKYNENGTITDAVDCALDPLSETKCTLKSFTVEKGIYQTSNFRVQPTESIVRFPNITNLCPFGEVFNATRFASVYAWNRKRISNCVADYSVLYNSASFSTFKCYGVSPTKLNDLCFTNVYADSFVIRGDEVRQIAPGQTGKIADYNYKLPDDFTGCVIAWNSNNLDSKVGGNYNYLYRLFRKSNLKPFERDISTEIYQAGSTPCNGVEGFNCMFPLQSYGFQPTNGVGYQPYRVVVLSFELLHAPATVCGPKKSTNLVKNKCVNFNFNGLTGTGVLTESNKKFLPFQQFGRDIADTTDAVRDPQTLEILDITPCSFGGVSVITPGTNTSNQVAVLYQDVNCTEVPVAIHADQLTPTWRVYSTGSNVFQTRAGCLIGAEHVNNSYECDIPIGAGICASYQTQTNSPQQAQSVASQSIIAYTMSLGAENSVAYSNNSIAIPTNFTISVTTEILPVSMTKTSVDCTMYICGDSTECSNLLLQYGSFCTQLNRALTGIAVEQDKNTQEVFAQVKQIYKTPPIKDFGGFNFSQILPDPSKPSKRSFIEDLLFNKVTLADAGFIKQYGDCLGDIAARDLICAQKFNGLTVLPPLLTDEMIAQYTSALLAGTITSGWTFGAGAALQIPFAMQMAYRFNGIGVTQNVLYENQKLIANQFNSAIGKIQDSLSSTASALGKLQDVVNQNAQALNTLVKQLSSNFGAISSVLNDILSRLDPPEAEVQIDRLITGRLQSLQTYVTQQLIRAAEIRASANLAATKMSECVLGQSKRVDFCGKGYHLMSFPQSAPHGVVFLHVTYVPAQEKNFTTAPAICHDGKAHFPREGVFVSNGTHWFVTQRNFYEPQIITTDNTFVSGNCDVVIGIVNNTVYDPLQPELDSFKEELDKYFKNHTSPDVDLGDISGINASVVNIQKEIDRLNEVAKNLNESLIDLQELGKYEQYIKWPWYIWLGFIAGLIAIVMVTIMLCCMTSCCSCLKGCCSCGSCCKFDEDDSEPVLKGVKLHYT

SEQ ID NO: 187 - protein, 1273 aa, Artificial Sequence
  mutant spike protein of SARS-CoV-2 Wuhan variant comprising substitution Y489N, 2-P-mutation (substiutions K986P and V987P) and inoperative furin cleavage site (substitution 682-QQAQ-685)
MFVFLVLLPLVSSQCVNLTTRTQLPPAYTNSFTRGVYYPDKVFRSSVLHSTQDLFLPFFSNVTWFHAIHVSGTNGTKRFDNPVLPFNDGVYFASTEKSNIIRGWIFGTTLDSKTQSLLIVNNATNVVIKVCEFQFCNDPFLGVYYHKNNKSWMESEFRVYSSANNCTFEYVSQPFLMDLEGKQGNFKNLREFVFKNIDGYFKIYSKHTPINLVRDLPQGFSALEPLVDLPIGINITRFQTLLALHRSYLTPGDSSSGWTAGAAAYYVGYLQPRTFLLKYNENGTITDAVDCALDPLSETKCTLKSFTVEKGIYQTSNFRVQPTESIVRFPNITNLCPFGEVFNATRFASVYAWNRKRISNCVADYSVLYNSASFSTFKCYGVSPTKLNDLCFTNVYADSFVIRGDEVRQIAPGQTGKIADYNYKLPDDFTGCVIAWNSNNLDSKVGGNYNYLYRLFRKSNLKPFERDISTEIYQAGSTPCNGVEGFNCNFPLQSYGFQPTNGVGYQPYRVVVLSFELLHAPATVCGPKKSTNLVKNKCVNFNFNGLTGTGVLTESNKKFLPFQQFGRDIADTTDAVRDPQTLEILDITPCSFGGVSVITPGTNTSNQVAVLYQDVNCTEVPVAIHADQLTPTWRVYSTGSNVFQTRAGCLIGAEHVNNSYECDIPIGAGICASYQTQTNSPQQAQSVASQSIIAYTMSLGAENSVAYSNNSIAIPTNFTISVTTEILPVSMTKTSVDCTMYICGDSTECSNLLLQYGSFCTQLNRALTGIAVEQDKNTQEVFAQVKQIYKTPPIKDFGGFNFSQILPDPSKPSKRSFIEDLLFNKVTLADAGFIKQYGDCLGDIAARDLICAQKFNGLTVLPPLLTDEMIAQYTSALLAGTITSGWTFGAGAALQIPFAMQMAYRFNGIGVTQNVLYENQKLIANQFNSAIGKIQDSLSSTASALGKLQDVVNQNAQALNTLVKQLSSNFGAISSVLNDILSRLDPPEAEVQIDRLITGRLQSLQTYVTQQLIRAAEIRASANLAATKMSECVLGQSKRVDFCGKGYHLMSFPQSAPHGVVFLHVTYVPAQEKNFTTAPAICHDGKAHFPREGVFVSNGTHWFVTQRNFYEPQIITTDNTFVSGNCDVVIGIVNNTVYDPLQPELDSFKEELDKYFKNHTSPDVDLGDISGINASVVNIQKEIDRLNEVAKNLNESLIDLQELGKYEQYIKWPWYIWLGFIAGLIAIVMVTIMLCCMTSCCSCLKGCCSCGSCCKFDEDDSEPVLKGVKLHYT

SEQ ID NO: 188 - protein, 1273 aa, Artificial Sequence
  mutant spike protein of SARS-CoV-2 Wuhan variant comprising substitution Y489P, 2-P-mutation (substiutions K986P and V987P) and inoperative furin cleavage site (substitution 682-QQAQ-685)
MFVFLVLLPLVSSQCVNLTTRTQLPPAYTNSFTRGVYYPDKVFRSSVLHSTQDLFLPFFSNVTWFHAIHVSGTNGTKRFDNPVLPFNDGVYFASTEKSNIIRGWIFGTTLDSKTQSLLIVNNATNVVIKVCEFQFCNDPFLGVYYHKNNKSWMESEFRVYSSANNCTFEYVSQPFLMDLEGKQGNFKNLREFVFKNIDGYFKIYSKHTPINLVRDLPQGFSALEPLVDLPIGINITRFQTLLALHRSYLTPGDSSSGWTAGAAAYYVGYLQPRTFLLKYNENGTITDAVDCALDPLSETKCTLKSFTVEKGIYQTSNFRVQPTESIVRFPNITNLCPFGEVFNATRFASVYAWNRKRISNCVADYSVLYNSASFSTFKCYGVSPTKLNDLCFTNVYADSFVIRGDEVRQIAPGQTGKIADYNYKLPDDFTGCVIAWNSNNLDSKVGGNYNYLYRLFRKSNLKPFERDISTEIYQAGSTPCNGVEGFNCPFPLQSYGFQPTNGVGYQPYRVVVLSFELLHAPATVCGPKKSTNLVKNKCVNFNFNGLTGTGVLTESNKKFLPFQQFGRDIADTTDAVRDPQTLEILDITPCSFGGVSVITPGTNTSNQVAVLYQDVNCTEVPVAIHADQLTPTWRVYSTGSNVFQTRAGCLIGAEHVNNSYECDIPIGAGICASYQTQTNSPQQAQSVASQSIIAYTMSLGAENSVAYSNNSIAIPTNFTISVTTEILPVSMTKTSVDCTMYICGDSTECSNLLLQYGSFCTQLNRALTGIAVEQDKNTQEVFAQVKQIYKTPPIKDFGGFNFSQILPDPSKPSKRSFIEDLLFNKVTLADAGFIKQYGDCLGDIAARDLICAQKFNGLTVLPPLLTDEMIAQYTSALLAGTITSGWTFGAGAALQIPFAMQMAYRFNGIGVTQNVLYENQKLIANQFNSAIGKIQDSLSSTASALGKLQDVVNQNAQALNTLVKQLSSNFGAISSVLNDILSRLDPPEAEVQIDRLITGRLQSLQTYVTQQLIRAAEIRASANLAATKMSECVLGQSKRVDFCGKGYHLMSFPQSAPHGVVFLHVTYVPAQEKNFTTAPAICHDGKAHFPREGVFVSNGTHWFVTQRNFYEPQIITTDNTFVSGNCDVVIGIVNNTVYDPLQPELDSFKEELDKYFKNHTSPDVDLGDISGINASVVNIQKEIDRLNEVAKNLNESLIDLQELGKYEQYIKWPWYIWLGFIAGLIAIVMVTIMLCCMTSCCSCLKGCCSCGSCCKFDEDDSEPVLKGVKLHYT

SEQ ID NO: 189 - protein, 1273 aa, Artificial Sequence
  mutant spike protein of SARS-CoV-2 Wuhan variant comprising substitution Y489Q, 2-P-mutation (substitutions K986P and V987P) and inoperative furin cleavage site (substitution 682-QQAQ-685)
MFVFLVLLPLVSSQCVNLTTRTQLPPAYTNSFTRGVYYPDKVFRSSVLHSTQDLFLPFFSNVTWFHAIHVSGTNGTKRFDNPVLPFNDGVYFASTEKSNIIRGWIFGTTLDSKTQSLLIVNNATNVVIKVCEFQFCNDPFLGVYYHKNNKSWMESEFRVYSSANNCTFEYVSQPFLMDLEGKQGNFKNLREFVFKNIDGYFKIYSKHTPINLVRDLPQGFSALEPLVDLPIGINITRFQTLLALHRSYLTPGDSSSGWTAGAAAYYVGYLQPRTFLLKYNENGTITDAVDCALDPLSETKCTLKSFTVEKGIYQTSNFRVQPTESIVRFPNITNLCPFGEVFNATRFASVYAWNRKRISNCVADYSVLYNSASFSTFKCYGVSPTKLNDLCFTNVYADSFVIRGDEVRQIAPGQTGKIADYNYKLPDDFTGCVIAWNSNNLDSKVGGNYNYLYRLFRKSNLKPFERDISTEIYQAGSTPCNGVEGFNCQFPLQSYGFQPTNGVGYQPYRVVVLSFELLHAPATVCGPKKSTNLVKNKCVNFNFNGLTGTGVLTESNKKFLPFQQFGRDIADTTDAVRDPQTLEILDITPCSFGGVSVITPGTNTSNQVAVLYQDVNCTEVPVAIHADQLTPTWRVYSTGSNVFQTRAGCLIGAEHVNNSYECDIPIGAGICASYQTQTNSPQQAQSVASQSIIAYTMSLGAENSVAYSNNSIAIPTNFTISVTTEILPVSMTKTSVDCTMYICGDSTECSNLLLQYGSFCTQLNRALTGIAVEQDKNTQEVFAQVKQIYKTPPIKDFGGFNFSQILPDPSKPSKRSFIEDLLFNKVTLADAGFIKQYGDCLGDIAARDLICAQKFNGLTVLPPLLTDEMIAQYTSALLAGTITSGWTFGAGAALQIPFAMQMAYRFNGIGVTQNVLYENQKLIANQFNSAIGKIQDSLSSTASALGKLQDVVNQNAQALNTLVKQLSSNFGAISSVLNDILSRLDPPEAEVQIDRLITGRLQSLQTYVTQQLIRAAEIRASANLAATKMSECVLGQSKRVDFCGKGYHLMSFPQSAPHGVVFLHVTYVPAQEKNFTTAPAICHDGKAHFPREGVFVSNGTHWFVTQRNFYEPQIITTDNTFVSGNCDVVIGIVNNTVYDPLQPELDSFKEELDKYFKNHTSPDVDLGDISGINASVVNIQKEIDRLNEVAKNLNESLIDLQELGKYEQYIKWPWYIWLGFIAGLIAIVMVTIMLCCMTSCCSCLKGCCSCGSCCKFDEDDSEPVLKGVKLHYT

SEQ ID NO: 190 - protein, 1273 aa, Artificial Sequence
  mutant spike protein of SARS-CoV-2 Wuhan variant comprising substitution Y489R, 2-P-mutation (substitutions K986P and V987P) and inoperative furin cleavage site (substitution 682-QQAQ-685)
MFVFLVLLPLVSSQCVNLTTRTQLPPAYTNSFTRGVYYPDKVFRSSVLHSTQDLFLPFFSNVTWFHAIHVSGTNGTKRFDNPVLPFNDGVYFASTEKSNIIRGWIFGTTLDSKTQSLLIVNNATNVVIKVCEFQFCNDPFLGVYYHKNNKSWMESEFRVYSSANNCTFEYVSQPFLMDLEGKQGNFKNLREFVFKNIDGYFKIYSKHTPINLVRDLPQGFSALEPLVDLPIGINITRFQTLLALHRSYLTPGDSSSGWTAGAAAYYVGYLQPRTFLLKYNENGTITDAVDCALDPLSETKCTLKSFTVEKGIYQTSNFRVQPTESIVRFPNITNLCPFGEVFNATRFASVYAWNRKRISNCVADYSVLYNSASFSTFKCYGVSPTKLNDLCFTNVYADSFVIRGDEVRQIAPGQTGKIADYNYKLPDDFTGCVIAWNSNNLDSKVGGNYNYLYRLFRKSNLKPFERDISTEIYQAGSTPCNGVEGFNCRFPLQSYGFQPTNGVGYQPYRVVVLSFELLHAPATVCGPKKSTNLVKNKCVNFNFNGLTGTGVLTESNKKFLPFQQFGRDIADTTDAVRDPQTLEILDITPCSFGGVSVITPGTNTSNQVAVLYQDVNCTEVPVAIHADQLTPTWRVYSTGSNVFQTRAGCLIGAEHVNNSYECDIPIGAGICASYQTQTNSPQQAQSVASQSIIAYTMSLGAENSVAYSNNSIAIPTNFTISVTTEILPVSMTKTSVDCTMYICGDSTECSNLLLQYGSFCTQLNRALTGIAVEQDKNTQEVFAQVKQIYKTPPIKDFGGFNFSQILPDPSKPSKRSFIEDLLFNKVTLADAGFIKQYGDCLGDIAARDLICAQKFNGLTVLPPLLTDEMIAQYTSALLAGTITSGWTFGAGAALQIPFAMQMAYRFNGIGVTQNVLYENQKLIANQFNSAIGKIQDSLSSTASALGKLQDVVNQNAQALNTLVKQLSSNFGAISSVLNDILSRLDPPEAEVQIDRLITGRLQSLQTYVTQQLIRAAEIRASANLAATKMSECVLGQSKRVDFCGKGYHLMSFPQSAPHGVVFLHVTYVPAQEKNFTTAPAICHDGKAHFPREGVFVSNGTHWFVTQRNFYEPQIITTDNTFVSGNCDVVIGIVNNTVYDPLQPELDSFKEELDKYFKNHTSPDVDLGDISGINASVVNIQKEIDRLNEVAKNLNESLIDLQELGKYEQYIKWPWYIWLGFIAGLIAIVMVTIMLCCMTSCCSCLKGCCSCGSCCKFDEDDSEPVLKGVKLHYT

SEQ ID NO: 191 - protein, 1273 aa, Artificial Sequence
  mutant spike protein of SARS-CoV-2 Wuhan variant comprising substitution Y489S, 2-P-mutation (substitutions K986P and V987P) and inoperative furin cleavage site (substitution 682-QQAQ-685)
MFVFLVLLPLVSSQCVNLTTRTQLPPAYTNSFTRGVYYPDKVFRSSVLHSTQDLFLPFFSNVTWFHAIHVSGTNGTKRFDNPVLPFNDGVYFASTEKSNIIRGWIFGTTLDSKTQSLLIVNNATNVVIKVCEFQFCNDPFLGVYYHKNNKSWMESEFRVYSSANNCTFEYVSQPFLMDLEGKQGNFKNLREFVFKNIDGYFKIYSKHTPINLVRDLPQGFSALEPLVDLPIGINITRFQTLLALHRSYLTPGDSSSGWTAGAAAYYVGYLQPRTFLLKYNENGTITDAVDCALDPLSETKCTLKSFTVEKGIYQTSNFRVQPTESIVRFPNITNLCPFGEVFNATRFASVYAWNRKRISNCVADYSVLYNSASFSTFKCYGVSPTKLNDLCFTNVYADSFVIRGDEVRQIAPGQTGKIADYNYKLPDDFTGCVIAWNSNNLDSKVGGNYNYLYRLFRKSNLKPFERDISTEIYQAGSTPCNGVEGFNCSFPLQSYGFQPTNGVGYQPYRVVVLSFELLHAPATVCGPKKSTNLVKNKCVNFNFNGLTGTGVLTESNKKFLPFQQFGRDIADTTDAVRDPQTLEILDITPCSFGGVSVITPGTNTSNQVAVLYQDVNCTEVPVAIHADQLTPTWRVYSTGSNVFQTRAGCLIGAEHVNNSYECDIPIGAGICASYQTQTNSPQQAQSVASQSIIAYTMSLGAENSVAYSNNSIAIPTNFTISVTTEILPVSMTKTSVDCTMYICGDSTECSNLLLQYGSFCTQLNRALTGIAVEQDKNTQEVFAQVKQIYKTPPIKDFGGFNFSQILPDPSKPSKRSFIEDLLFNKVTLADAGFIKQYGDCLGDIAARDLICAQKFNGLTVLPPLLTDEMIAQYTSALLAGTITSGWTFGAGAALQIPFAMQMAYRFNGIGVTQNVLYENQKLIANQFNSAIGKIQDSLSSTASALGKLQDVVNQNAQALNTLVKQLSSNFGAISSVLNDILSRLDPPEAEVQIDRLITGRLQSLQTYVTQQLIRAAEIRASANLAATKMSECVLGQSKRVDFCGKGYHLMSFPQSAPHGVVFLHVTYVPAQEKNFTTAPAICHDGKAHFPREGVFVSNGTHWFVTQRNFYEPQIITTDNTFVSGNCDVVIGIVNNTVYDPLQPELDSFKEELDKYFKNHTSPDVDLGDISGINASVVNIQKEIDRLNEVAKNLNESLIDLQELGKYEQYIKWPWYIWLGFIAGLIAIVMVTIMLCCMTSCCSCLKGCCSCGSCCKFDEDDSEPVLKGVKLHYT

SEQ ID NO: 192 - protein, 1273 aa, Artificial Sequence
  mutant spike protein of SARS-CoV-2 Wuhan variant comprising substitution Y489T, 2-P-mutation (substitutions K986P and V987P) and inoperative furin cleavage site (substitution 682-QQAQ-685)
MFVFLVLLPLVSSQCVNLTTRTQLPPAYTNSFTRGVYYPDKVFRSSVLHSTQDLFLPFFSNVTWFHAIHVSGTNGTKRFDNPVLPFNDGVYFASTEKSNIIRGWIFGTTLDSKTQSLLIVNNATNVVIKVCEFQFCNDPFLGVYYHKNNKSWMESEFRVYSSANNCTFEYVSQPFLMDLEGKQGNFKNLREFVFKNIDGYFKIYSKHTPINLVRDLPQGFSALEPLVDLPIGINITRFQTLLALHRSYLTPGDSSSGWTAGAAAYYVGYLQPRTFLLKYNENGTITDAVDCALDPLSETKCTLKSFTVEKGIYQTSNFRVQPTESIVRFPNITNLCPFGEVFNATRFASVYAWNRKRISNCVADYSVLYNSASFSTFKCYGVSPTKLNDLCFTNVYADSFVIRGDEVRQIAPGQTGKIADYNYKLPDDFTGCVIAWNSNNLDSKVGGNYNYLYRLFRKSNLKPFERDISTEIYQAGSTPCNGVEGFNCTFPLQSYGFQPTNGVGYQPYRVVVLSFELLHAPATVCGPKKSTNLVKNKCVNFNFNGLTGTGVLTESNKKFLPFQQFGRDIADTTDAVRDPQTLEILDITPCSFGGVSVITPGTNTSNQVAVLYQDVNCTEVPVAIHADQLTPTWRVYSTGSNVFQTRAGCLIGAEHVNNSYECDIPIGAGICASYQTQTNSPQQAQSVASQSIIAYTMSLGAENSVAYSNNSIAIPTNFTISVTTEILPVSMTKTSVDCTMYICGDSTECSNLLLQYGSFCTQLNRALTGIAVEQDKNTQEVFAQVKQIYKTPPIKDFGGFNFSQILPDPSKPSKRSFIEDLLFNKVTLADAGFIKQYGDCLGDIAARDLICAQKFNGLTVLPPLLTDEMIAQYTSALLAGTITSGWTFGAGAALQIPFAMQMAYRFNGIGVTQNVLYENQKLIANQFNSAIGKIQDSLSSTASALGKLQDVVNQNAQALNTLVKQLSSNFGAISSVLNDILSRLDPPEAEVQIDRLITGRLQSLQTYVTQQLIRAAEIRASANLAATKMSECVLGQSKRVDFCGKGYHLMSFPQSAPHGVVFLHVTYVPAQEKNFTTAPAICHDGKAHFPREGVFVSNGTHWFVTQRNFYEPQIITTDNTFVSGNCDVVIGIVNNTVYDPLQPELDSFKEELDKYFKNHTSPDVDLGDISGINASVVNIQKEIDRLNEVAKNLNESLIDLQELGKYEQYIKWPWYIWLGFIAGLIAIVMVTIMLCCMTSCCSCLKGCCSCGSCCKFDEDDSEPVLKGVKLHYT

SEQ ID NO: 193 - protein, 1273 aa, Artificial Sequence
  mutant spike protein of SARS-CoV-2 Wuhan variant comprising substitution Y489V, 2-P-mutation (substitutions K986P and V987P) and inoperative furin cleavage site (substitution 682-QQAQ-685)
MFVFLVLLPLVSSQCVNLTTRTQLPPAYTNSFTRGVYYPDKVFRSSVLHSTQDLFLPFFSNVTWFHAIHVSGTNGTKRFDNPVLPFNDGVYFASTEKSNIIRGWIFGTTLDSKTQSLLIVNNATNVVIKVCEFQFCNDPFLGVYYHKNNKSWMESEFRVYSSANNCTFEYVSQPFLMDLEGKQGNFKNLREFVFKNIDGYFKIYSKHTPINLVRDLPQGFSALEPLVDLPIGINITRFQTLLALHRSYLTPGDSSSGWTAGAAAYYVGYLQPRTFLLKYNENGTITDAVDCALDPLSETKCTLKSFTVEKGIYQTSNFRVQPTESIVRFPNITNLCPFGEVFNATRFASVYAWNRKRISNCVADYSVLYNSASFSTFKCYGVSPTKLNDLCFTNVYADSFVIRGDEVRQIAPGQTGKIADYNYKLPDDFTGCVIAWNSNNLDSKVGGNYNYLYRLFRKSNLKPFERDISTEIYQAGSTPCNGVEGFNCVFPLQSYGFQPTNGVGYQPYRVVVLSFELLHAPATVCGPKKSTNLVKNKCVNFNFNGLTGTGVLTESNKKFLPFQQFGRDIADTTDAVRDPQTLEILDITPCSFGGVSVITPGTNTSNQVAVLYQDVNCTEVPVAIHADQLTPTWRVYSTGSNVFQTRAGCLIGAEHVNNSYECDIPIGAGICASYQTQTNSPQQAQSVASQSIIAYTMSLGAENSVAYSNNSIAIPTNFTISVTTEILPVSMTKTSVDCTMYICGDSTECSNLLLQYGSFCTQLNRALTGIAVEQDKNTQEVFAQVKQIYKTPPIKDFGGFNFSQILPDPSKPSKRSFIEDLLFNKVTLADAGFIKQYGDCLGDIAARDLICAQKFNGLTVLPPLLTDEMIAQYTSALLAGTITSGWTFGAGAALQIPFAMQMAYRFNGIGVTQNVLYENQKLIANQFNSAIGKIQDSLSSTASALGKLQDVVNQNAQALNTLVKQLSSNFGAISSVLNDILSRLDPPEAEVQIDRLITGRLQSLQTYVTQQLIRAAEIRASANLAATKMSECVLGQSKRVDFCGKGYHLMSFPQSAPHGVVFLHVTYVPAQEKNFTTAPAICHDGKAHFPREGVFVSNGTHWFVTQRNFYEPQIITTDNTFVSGNCDVVIGIVNNTVYDPLQPELDSFKEELDKYFKNHTSPDVDLGDISGINASVVNIQKEIDRLNEVAKNLNESLIDLQELGKYEQYIKWPWYIWLGFIAGLIAIVMVTIMLCCMTSCCSCLKGCCSCGSCCKFDEDDSEPVLKGVKLHYT

SEQ ID NO: 194 - protein, 240 aa, MERS-CoV
  wildtype receptor bindung domain of MERS-CoV
EAKPSGSVVEQAEGVECDFSPLLSGTPPQVYNFKRLVFTNCNYNLTKLLSLFSVNDFTCSQISPAAIASNCYSSLILDYFSYPLSMKSDLSVSSAGPISQFNYKQSFSNPTCLILATVPHNLTTITKPLKYSYINKCSRLLSDDRTEVPQLVNANQYSPCVSIVPSTVWEDGDYYRKQLSPLEGGGWLVASGSTVAMTEQLQMGFGITVQYGTDTNSVCPKLEFANDTKIASQLGNCVEY

SEQ ID NO: 195 - protein, 240 aa, Artificial Sequence
  mutant receptor binding domain of MERS-CoV comprising substitution D144A
EAKPSGSVVEQAEGVECDFSPLLSGTPPQVYNFKRLVFTNCNYNLTKLLSLFSVNDFTCSQISPAAIASNCYSSLILDYFSYPLSMKSDLSVSSAGPISQFNYKQSFSNPTCLILATVPHNLTTITKPLKYSYINKCSRLLSDARTEVPQLVNANQYSPCVSIVPSTVWEDGDYYRKQLSPLEGGGWLVASGSTVAMTEQLQMGFGITVQYGTDTNSVCPKLEFANDTKIASQLGNCVEY

SEQ ID NO: 196 - protein, 240 aa, Artificial Sequence
  mutant receptor binding domain of MERS-CoV comprising substitution D171K
EAKPSGSVVEQAEGVECDFSPLLSGTPPQVYNFKRLVFTNCNYNLTKLLSLFSVNDFTCSQISPAAIASNCYSSLILDYFSYPLSMKSDLSVSSAGPISQFNYKQSFSNPTCLILATVPHNLTTITKPLKYSYINKCSRLLSDDRTEVPQLVNANQYSPCVSIVPSTVWEKGDYYRKQLSPLEGGGWLVASGSTVAMTEQLQMGFGITVQYGTDTNSVCPKLEFANDTKIASQLGNCVEY

SEQ ID NO: 197 - protein, 240 aa, Artificial Sequence
  mutant receptor binding domain of MERS-CoV comprising substitution D173K
EAKPSGSVVEQAEGVECDFSPLLSGTPPQVYNFKRLVFTNCNYNLTKLLSLFSVNDFTCSQISPAAIASNCYSSLILDYFSYPLSMKSDLSVSSAGPISQFNYKQSFSNPTCLILATVPHNLTTITKPLKYSYINKCSRLLSDDRTEVPQLVNANQYSPCVSIVPSTVWEDGKYYRKQLSPLEGGGWLVASGSTVAMTEQLQMGFGITVQYGTDTNSVCPKLEFANDTKIASQLGNCVEY

SEQ ID NO: 198 - protein, 240 aa, Artificial Sequence
  mutant receptor binding domain of MERS-CoV comprising substitution E170R
EAKPSGSVVEQAEGVECDFSPLLSGTPPQVYNFKRLVFTNCNYNLTKLLSLFSVNDFTCSQISPAAIASNCYSSLILDYFSYPLSMKSDLSVSSAGPISQFNYKQSFSNPTCLILATVPHNLTTITKPLKYSYINKCSRLLSDDRTEVPQLVNANQYSPCVSIVPSTVWRDGDYYRKQLSPLEGGGWLVASGSTVAMTEQLQMGFGITVQYGTDTNSVCPKLEFANDTKIASQLGNCVEY

SEQ ID NO: 199 - protein, 240 aa, Artificial Sequence
  mutant receptor binding domain of MERS-CoV comprising substitution L140A
EAKPSGSVVEQAEGVECDFSPLLSGTPPQVYNFKRLVFTNCNYNLTKLLSLFSVNDFTCSQISPAAIASNCYSSLILDYFSYPLSMKSDLSVSSAGPISQFNYKQSFSNPTCLILATVPHNLTTITKPLKYSYINKCSRALSDDRTEVPQLVNANQYSPCVSIVPSTVWEDGDYYRKQLSPLEGGGWLVASGSTVAMTEQLQMGFGITVQYGTDTNSVCPKLEFANDTKIASQLGNCVEY

SEQ ID NO: 200 - protein, 1353 aa, MERS-CoV
  wildtype spike protein of MERS-CoV
MIHSVFLLMFLLTPTESYVDVGPDSVKSACIEVDIQQTFFDKTWPRPIDVSKADGIIYPQGRTYSNITITYQGLFPYQGDHGDMYVYSAGHATGTTPQKLFVANYSQDVKQFANGFVVRIGAAANSTGTVIISPSTSATIRKIYPAFMLGSSVGNFSDGKMGRFFNHTLVLLPDGCGTLLRAFYCILEPRSGNHCPAGNSYTSFATYHTPATDCSDGNYNRNASLNSFKEYFNLRNCTFMYTYNITEDEILEWFGITQTAQGVHLFSSRYVDLYGGNMFQFATLPVYDTIKYYSIIPHSIRSIQSDRKAWAAFYVYKLQPLTFLLDFSVDGYIRRAIDCGFNDLSQLHCSYESFDVESGVYSVSSFEAKPSGSVVEQAEGVECDFSPLLSGTPPQVYNFKRLVFTNCNYNLTKLLSLFSVNDFTCSQISPAAIASNCYSSLILDYFSYPLSMKSDLSVSSAGPISQFNYKQSFSNPTCLILATVPHNLTTITKPLKYSYINKCSRLLSDDRTEVPQLVNANQYSPCVSIVPSTVWEDGDYYRKQLSPLEGGGWLVASGSTVAMTEQLQMGFGITVQYGTDTNSVCPKLEFANDTKIASQLGNCVEYSLYGVSGRGVFQNCTAVGVRQQRFVYDAYQNLVGYYSDDGNYYCLRACVSVPVSVIYDKETKTHATLFGSVACEHISSTMSQYSRSTRSMLKRRDSTYGPLQTPVGCVLGLVNSSLFVEDCKLPLGQSLCALPDTPSTLTPRSVRSVPGEMRLASIAFNHPIQVDQLNSSYFKLSIPTNFSFGVTQEYIQTTIQKVTVDCKQYVCNGFQKCEQLLREYGQFCSKINQALHGANLRQDDSVRNLFASVKSSQSSPIIPGFGGDFNLTLLEPVSISTGSRSARSAIEDLLFDKVTIADPGYMQGYDDCMQQGPASARDLICAQYVAGYKVLPPLMDVNMEAAYTSSLLGSIAGVGWTAGLSSFAAIPFAQSIFYRLNGVGITQQVLSENQKLIANKFNQALGAMQTGFTTTNEAFRKVQDAVNNNAQALSKLASELSNTFGAISASIGDIIQRLDVLEQDAQIDRLINGRLTTLNAFVAQQLVRSESAALSAQLAKDKVNECVKAQSKRSGFCGQGTHIVSFVVNAPNGLYFMHVGYYPSNHIEVVSAYGLCDAANPTNCIAPVNGYFIKTNNTRIVDEWSYTGSSFYAPEPITSLNTKYVAPHVTYQNISTNLPPPLLGNSTGIDFQDELDEFFKNVSTSIPNFGSLTQINTTLLDLTYEMLSLQQVVKALNESYIDLKELGNYTYYNKWPWYIWLGFIAGLVALALCVFFILCCTGCGTNCMGKLKCNRCCDRYEEYDLEPHKVHVH

SEQ ID NO: 201 - protein, 1353 aa, Artificial Sequence
  mutant spike protein of MERS-CoV-2 comprising substitution D510A, 2-P-mutation (substiutions V1060P and L1061P) and inoperative furin cleavage site (substitution 748-ASVG-751)
MIHSVFLLMFLLTPTESYVDVGPDSVKSACIEVDIQQTFFDKTWPRPIDVSKADGIIYPQGRTYSNITITYQGLFPYQGDHGDMYVYSAGHATGTTPQKLFVANYSQDVKQFANGFVVRIGAAANSTGTVIISPSTSATIRKIYPAFMLGSSVGNFSDGKMGRFFNHTLVLLPDGCGTLLRAFYCILEPRSGNHCPAGNSYTSFATYHTPATDCSDGNYNRNASLNSFKEYFNLRNCTFMYTYNITEDEILEWFGITQTAQGVHLFSSRYVDLYGGNMFQFATLPVYDTIKYYSIIPHSIRSIQSDRKAWAAFYVYKLQPLTFLLDFSVDGYIRRAIDCGFNDLSQLHCSYESFDVESGVYSVSSFEAKPSGSVVEQAEGVECDFSPLLSGTPPQVYNFKRLVFTNCNYNLTKLLSLFSVNDFTCSQISPAAIASNCYSSLILDYFSYPLSMKSDLSVSSAGPISQFNYKQSFSNPTCLILATVPHNLTTITKPLKYSYINKCSRLLSDARTEVPQLVNANQYSPCVSIVPSTVWEDGDYYRKQLSPLEGGGWLVASGSTVAMTEQLQMGFGITVQYGTDTNSVCPKLEFANDTKIASQLGNCVEYSLYGVSGRGVFQNCTAVGVRQQRFVYDAYQNLVGYYSDDGNYYCLRACVSVPVSVIYDKETKTHATLFGSVACEHISSTMSQYSRSTRSMLKRRDSTYGPLQTPVGCVLGLVNSSLFVEDCKLPLGQSLCALPDTPSTLTPASVGSVPGEMRLASIAFNHPIQVDQLNSSYFKLSIPTNFSFGVTQEYIQTTIQKVTVDCKQYVCNGFQKCEQLLREYGQFCSKINQALHGANLRQDDSVRNLFASVKSSQSSPIIPGFGGDFNLTLLEPVSISTGSRSARSAIEDLLFDKVTIADPGYMQGYDDCMQQGPASARDLICAQYVAGYKVLPPLMDVNMEAAYTSSLLGSIAGVGWTAGLSSFAAIPFAQSIFYRLNGVGITQQVLSENQKLIANKFNQALGAMQTGFTTTNEAFRKVQDAVNNNAQALSKLASELSNTFGAISASIGDIIQRLDPPEQDAQIDRLINGRLTTLNAFVAQQLVRSESAALSAQLAKDKVNECVKAQSKRSGFCGQGTHIVSFVVNAPNGLYFMHVGYYPSNHIEVVSAYGLCDAANPTNCIAPVNGYFIKTNNTRIVDEWSYTGSSFYAPEPITSLNTKYVAPHVTYQNISTNLPPPLLGNSTGIDFQDELDEFFKNVSTSIPNFGSLTQINTTLLDLTYEMLSLQQVVKALNESYIDLKELGNYTYYNKWPWYIWLGFIAGLVALALCVFFILCCTGCGTNCMGKLKCNRCCDRYEEYDLEPHKVHVH

SEQ ID NO: 202 - protein, 1353 aa, Artificial Sequence
  mutant spike protein of MERS-CoV-2 comprising substitution D537K, 2-P-mutation (substiutions V1060P and L1061P) and inoperative furin cleavage site (substitution 748-ASVG-751)
MIHSVFLLMFLLTPTESYVDVGPDSVKSACIEVDIQQTFFDKTWPRPIDVSKADGIIYPQGRTYSNITITYQGLFPYQGDHGDMYVYSAGHATGTTPQKLFVANYSQDVKQFANGFVVRIGAAANSTGTVIISPSTSATIRKIYPAFMLGSSVGNFSDGKMGRFFNHTLVLLPDGCGTLLRAFYCILEPRSGNHCPAGNSYTSFATYHTPATDCSDGNYNRNASLNSFKEYFNLRNCTFMYTYNITEDEILEWFGITQTAQGVHLFSSRYVDLYGGNMFQFATLPVYDTIKYYSIIPHSIRSIQSDRKAWAAFYVYKLQPLTFLLDFSVDGYIRRAIDCGFNDLSQLHCSYESFDVESGVYSVSSFEAKPSGSVVEQAEGVECDFSPLLSGTPPQVYNFKRLVFTNCNYNLTKLLSLFSVNDFTCSQISPAAIASNCYSSLILDYFSYPLSMKSDLSVSSAGPISQFNYKQSFSNPTCLILATVPHNLTTITKPLKYSYINKCSRLLSDDRTEVPQLVNANQYSPCVSIVPSTVWEKGDYYRKQLSPLEGGGWLVASGSTVAMTEQLQMGFGITVQYGTDTNSVCPKLEFANDTKIASQLGNCVEYSLYGVSGRGVFQNCTAVGVRQQRFVYDAYQNLVGYYSDDGNYYCLRACVSVPVSVIYDKETKTHATLFGSVACEHISSTMSQYSRSTRSMLKRRDSTYGPLQTPVGCVLGLVNSSLFVEDCKLPLGQSLCALPDTPSTLTPASVGSVPGEMRLASIAFNHPIQVDQLNSSYFKLSIPTNFSFGVTQEYIQTTIQKVTVDCKQYVCNGFQKCEQLLREYGQFCSKINQALHGANLRQDDSVRNLFASVKSSQSSPIIPGFGGDFNLTLLEPVSISTGSRSARSAIEDLLFDKVTIADPGYMQGYDDCMQQGPASARDLICAQYVAGYKVLPPLMDVNMEAAYTSSLLGSIAGVGWTAGLSSFAAIPFAQSIFYRLNGVGITQQVLSENQKLIANKFNQALGAMQTGFTTTNEAFRKVQDAVNNNAQALSKLASELSNTFGAISASIGDIIQRLDPPEQDAQIDRLINGRLTTLNAFVAQQLVRSESAALSAQLAKDKVNECVKAQSKRSGFCGQGTHIVSFVVNAPNGLYFMHVGYYPSNHIEVVSAYGLCDAANPTNCIAPVNGYFIKTNNTRIVDEWSYTGSSFYAPEPITSLNTKYVAPHVTYQNISTNLPPPLLGNSTGIDFQDELDEFFKNVSTSIPNFGSLTQINTTLLDLTYEMLSLQQVVKALNESYIDLKELGNYTYYNKWPWYIWLGFIAGLVALALCVFFILCCTGCGTNCMGKLKCNRCCDRYEEYDLEPHKVHVH

SEQ ID NO: 203 - protein, 1353 aa, Artificial Sequence
  mutant spike protein of MERS-CoV-2 comprising substitution D539K, 2-P-mutation (substiutions V1060P and L1061P) and inoperative furin cleavage site (substitution 748-ASVG-751)
MIHSVFLLMFLLTPTESYVDVGPDSVKSACIEVDIQQTFFDKTWPRPIDVSKADGIIYPQGRTYSNITITYQGLFPYQGDHGDMYVYSAGHATGTTPQKLFVANYSQDVKQFANGFVVRIGAAANSTGTVIISPSTSATIRKIYPAFMLGSSVGNFSDGKMGRFFNHTLVLLPDGCGTLLRAFYCILEPRSGNHCPAGNSYTSFATYHTPATDCSDGNYNRNASLNSFKEYFNLRNCTFMYTYNITEDEILEWFGITQTAQGVHLFSSRYVDLYGGNMFQFATLPVYDTIKYYSIIPHSIRSIQSDRKAWAAFYVYKLQPLTFLLDFSVDGYIRRAIDCGFNDLSQLHCSYESFDVESGVYSVSSFEAKPSGSVVEQAEGVECDFSPLLSGTPPQVYNFKRLVFTNCNYNLTKLLSLFSVNDFTCSQISPAAIASNCYSSLILDYFSYPLSMKSDLSVSSAGPISQFNYKQSFSNPTCLILATVPHNLTTITKPLKYSYINKCSRLLSDDRTEVPQLVNANQYSPCVSIVPSTVWEDGKYYRKQLSPLEGGGWLVASGSTVAMTEQLQMGFGITVQYGTDTNSVCPKLEFANDTKIASQLGNCVEYSLYGVSGRGVFQNCTAVGVRQQRFVYDAYQNLVGYYSDDGNYYCLRACVSVPVSVIYDKETKTHATLFGSVACEHISSTMSQYSRSTRSMLKRRDSTYGPLQTPVGCVLGLVNSSLFVEDCKLPLGQSLCALPDTPSTLTPASVGSVPGEMRLASIAFNHPIQVDQLNSSYFKLSIPTNFSFGVTQEYIQTTIQKVTVDCKQYVCNGFQKCEQLLREYGQFCSKINQALHGANLRQDDSVRNLFASVKSSQSSPIIPGFGGDFNLTLLEPVSISTGSRSARSAIEDLLFDKVTIADPGYMQGYDDCMQQGPASARDLICAQYVAGYKVLPPLMDVNMEAAYTSSLLGSIAGVGWTAGLSSFAAIPFAQSIFYRLNGVGITQQVLSENQKLIANKFNQALGAMQTGFTTTNEAFRKVQDAVNNNAQALSKLASELSNTFGAISASIGDIIQRLDPPEQDAQIDRLINGRLTTLNAFVAQQLVRSESAALSAQLAKDKVNECVKAQSKRSGFCGQGTHIVSFVVNAPNGLYFMHVGYYPSNHIEVVSAYGLCDAANPTNCIAPVNGYFIKTNNTRIVDEWSYTGSSFYAPEPITSLNTKYVAPHVTYQNISTNLPPPLLGNSTGIDFQDELDEFFKNVSTSIPNFGSLTQINTTLLDLTYEMLSLQQVVKALNESYIDLKELGNYTYYNKWPWYIWLGFIAGLVALALCVFFILCCTGCGTNCMGKLKCNRCCDRYEEYDLEPHKVHVH

SEQ ID NO: 204 - protein, 1353 aa, Artificial Sequence
  mutant spike protein of MERS-CoV-2 comprising substitution E536R, 2-P-mutation (substiutions V1060P and L1061P) and inoperative furin cleavage site (substitution 748-ASVG-751)
MIHSVFLLMFLLTPTESYVDVGPDSVKSACIEVDIQQTFFDKTWPRPIDVSKADGIIYPQGRTYSNITITYQGLFPYQGDHGDMYVYSAGHATGTTPQKLFVANYSQDVKQFANGFVVRIGAAANSTGTVIISPSTSATIRKIYPAFMLGSSVGNFSDGKMGRFFNHTLVLLPDGCGTLLRAFYCILEPRSGNHCPAGNSYTSFATYHTPATDCSDGNYNRNASLNSFKEYFNLRNCTFMYTYNITEDEILEWFGITQTAQGVHLFSSRYVDLYGGNMFQFATLPVYDTIKYYSIIPHSIRSIQSDRKAWAAFYVYKLQPLTFLLDFSVDGYIRRAIDCGFNDLSQLHCSYESFDVESGVYSVSSFEAKPSGSVVEQAEGVECDFSPLLSGTPPQVYNFKRLVFTNCNYNLTKLLSLFSVNDFTCSQISPAAIASNCYSSLILDYFSYPLSMKSDLSVSSAGPISQFNYKQSFSNPTCLILATVPHNLTTITKPLKYSYINKCSRLLSDDRTEVPQLVNANQYSPCVSIVPSTVWRDGDYYRKQLSPLEGGGWLVASGSTVAMTEQLQMGFGITVQYGTDTNSVCPKLEFANDTKIASQLGNCVEYSLYGVSGRGVFQNCTAVGVRQQRFVYDAYQNLVGYYSDDGNYYCLRACVSVPVSVIYDKETKTHATLFGSVACEHISSTMSQYSRSTRSMLKRRDSTYGPLQTPVGCVLGLVNSSLFVEDCKLPLGQSLCALPDTPSTLTPASVGSVPGEMRLASIAFNHPIQVDQLNSSYFKLSIPTNFSFGVTQEYIQTTIQKVTVDCKQYVCNGFQKCEQLLREYGQFCSKINQALHGANLRQDDSVRNLFASVKSSQSSPIIPGFGGDFNLTLLEPVSISTGSRSARSAIEDLLFDKVTIADPGYMQGYDDCMQQGPASARDLICAQYVAGYKVLPPLMDVNMEAAYTSSLLGSIAGVGWTAGLSSFAAIPFAQSIFYRLNGVGITQQVLSENQKLIANKFNQALGAMQTGFTTTNEAFRKVQDAVNNNAQALSKLASELSNTFGAISASIGDIIQRLDPPEQDAQIDRLINGRLTTLNAFVAQQLVRSESAALSAQLAKDKVNECVKAQSKRSGFCGQGTHIVSFVVNAPNGLYFMHVGYYPSNHIEVVSAYGLCDAANPTNCIAPVNGYFIKTNNTRIVDEWSYTGSSFYAPEPITSLNTKYVAPHVTYQNISTNLPPPLLGNSTGIDFQDELDEFFKNVSTSIPNFGSLTQINTTLLDLTYEMLSLQQVVKALNESYIDLKELGNYTYYNKWPWYIWLGFIAGLVALALCVFFILCCTGCGTNCMGKLKCNRCCDRYEEYDLEPHKVHVH

SEQ ID NO: 205 - protein, 1353 aa, Artificial Sequence
  mutant spike protein of MERS-CoV-2 comprising substitution L506A, 2-P-mutation (substiutions V1060P and L1061P) and inoperative furin cleavage site (substitution 748-ASVG-751)
MIHSVFLLMFLLTPTESYVDVGPDSVKSACIEVDIQQTFFDKTWPRPIDVSKADGIIYPQGRTYSNITITYQGLFPYQGDHGDMYVYSAGHATGTTPQKLFVANYSQDVKQFANGFVVRIGAAANSTGTVIISPSTSATIRKIYPAFMLGSSVGNFSDGKMGRFFNHTLVLLPDGCGTLLRAFYCILEPRSGNHCPAGNSYTSFATYHTPATDCSDGNYNRNASLNSFKEYFNLRNCTFMYTYNITEDEILEWFGITQTAQGVHLFSSRYVDLYGGNMFQFATLPVYDTIKYYSIIPHSIRSIQSDRKAWAAFYVYKLQPLTFLLDFSVDGYIRRAIDCGFNDLSQLHCSYESFDVESGVYSVSSFEAKPSGSVVEQAEGVECDFSPLLSGTPPQVYNFKRLVFTNCNYNLTKLLSLFSVNDFTCSQISPAAIASNCYSSLILDYFSYPLSMKSDLSVSSAGPISQFNYKQSFSNPTCLILATVPHNLTTITKPLKYSYINKCSRALSDDRTEVPQLVNANQYSPCVSIVPSTVWEDGDYYRKQLSPLEGGGWLVASGSTVAMTEQLQMGFGITVQYGTDTNSVCPKLEFANDTKIASQLGNCVEYSLYGVSGRGVFQNCTAVGVRQQRFVYDAYQNLVGYYSDDGNYYCLRACVSVPVSVIYDKETKTHATLFGSVACEHISSTMSQYSRSTRSMLKRRDSTYGPLQTPVGCVLGLVNSSLFVEDCKLPLGQSLCALPDTPSTLTPASVGSVPGEMRLASIAFNHPIQVDQLNSSYFKLSIPTNFSFGVTQEYIQTTIQKVTVDCKQYVCNGFQKCEQLLREYGQFCSKINQALHGANLRQDDSVRNLFASVKSSQSSPIIPGFGGDFNLTLLEPVSISTGSRSARSAIEDLLFDKVTIADPGYMQGYDDCMQQGPASARDLICAQYVAGYKVLPPLMDVNMEAAYTSSLLGSIAGVGWTAGLSSFAAIPFAQSIFYRLNGVGITQQVLSENQKLIANKFNQALGAMQTGFTTTNEAFRKVQDAVNNNAQALSKLASELSNTFGAISASIGDIIQRLDPPEQDAQIDRLINGRLTTLNAFVAQQLVRSESAALSAQLAKDKVNECVKAQSKRSGFCGQGTHIVSFVVNAPNGLYFMHVGYYPSNHIEVVSAYGLCDAANPTNCIAPVNGYFIKTNNTRIVDEWSYTGSSFYAPEPITSLNTKYVAPHVTYQNISTNLPPPLLGNSTGIDFQDELDEFFKNVSTSIPNFGSLTQINTTLLDLTYEMLSLQQVVKALNESYIDLKELGNYTYYNKWPWYIWLGFIAGLVALALCVFFILCCTGCGTNCMGKLKCNRCCDRYEEYDLEPHKVHVH

SEQ ID NO: 206 - DNA, 73 bp, Artificial Sequence
  forward primer
ctgcaaccggtgtacattctgaggtgcagctgctggagagcggcggcggcctggtgaagcccggcggcagcct

SEQ ID NO: 207 - DNA, 120 bp, Artificial Sequence
  forward primer
ggtgaagcccggcggcagcctgaggctgagctgcgaggccagcggcctgaccttcagcaacgtgtggatgagctgggtgaggcaggcccccggcaagggcctggagtgggtgggcaggat

SEQ ID NO: 208 - DNA, 120 bp, Artificial Sequence
  reverse primer
tgcaggtacacggtgttcttgctgtcgtccctgctcagggtgaacctgcccttcacgggggcgccgtagtcggtggtggcgccctcgctcttcctcttgatcctgcccacccactccagg

SEQ ID NO: 209 - DNA, 120 bp, Artificial Sequence
  reverse primer
ccagtagtcgaagtagtagctgctgctccacacgtcgccgcccctggtcagggtgctgcagtagtacacggcggtgtcgtcgatcttcaggctgttcatctgcaggtacacggtgttctt

SEQ ID NO: 210 - DNA, 69 bp, Artificial Sequence
  reverse primer
ctaggtcccttggtcgacgcgctgctcacggtcaccagggcgccctggccccagtagtcgaagtagtag

SEQ ID NO: 211 - DNA, 95 bp, Artificial Sequence
  forward primer
ctgcaaccggtgtacattcacagagcgccctgacccagcccgccagcgtgagcggcagccccggccagagcatcaccatcagctgcaccggcacc

SEQ ID NO: 212 - DNA, 120 bp, Artificial Sequence
  forward primer
accatcagctgcaccggcaccagcagcgacgtgggcacctacgacctggtgagctggtaccagcagcaccccggcaagagccccaagctgatgatctacgccgacatcaagaggcccagc

SEQ ID NO: 213 - DNA, 93 bp, Artificial Sequence
  reverse primer
ctgggggcggccaccgtacgggtcaccttggtgccgccgccgaagatcacgctggtgctgctgccggcgtacaggcagcagtagtagtcggcc

SEQ ID NO: 214 - DNA, 120 bp, Artificial Sequence
  reverse primer
ggcagcagtagtagtcggcctcgtcggcgctctgcaggccgctgatggtcaggctggcggtgttgccgctcttgctgccgctgaacctgtggctcacgccgctgggcctcttgatgtcgg

SEQ ID NO: 215 - DNA, 105 bp, Artificial Sequence
  forward primer
ctgcaaccggtgtacattctcaggtgcagctgcaggagagcggcggcggcctggtgaagcccggcggcagcctgaagctgagctgcgccgccagcggcttcacct

SEQ ID NO: 216 - DNA, 120 bp, Artificial Sequence
  forward primer
gcgccgccagcggcttcaccttcagcagctacaccatgagctgggtgaggcagacccccgacaagaggctggagtgggtggccaccatcagcagcggcggcagctacacctactaccccg

SEQ ID NO: 217 - DNA, 104 bp, Artificial Sequence
  reverse primer
ctaggtcccttggtcgacgcgctgctcacggtcaccatggtgccctggccccagtagtcgtagtcgttgccgtccctggcgcagtagtacatggcggtgtcctc

SEQ ID NO: 218 - DNA, 120 bp, Artificial Sequence
  reverse primer
tagtacatggcggtgtcctcgctcttcaggctgctcatctgcaggtacagggtgttcttggcgttgtccctgctgatggtgaacctgcccttcacgctgtcggggtagtaggtgtagctg

SEQ ID NO: 219 - DNA, 92 bp, Artificial Sequence
  forward primer
ctgcaaccggtgtacattcagacatccagctgacccagagccccagcagcctgagcgccagcatcggcgacagggtgaccatcacctgccag

SEQ ID NO: 220 - DNA, 120 bp, Artificial Sequence
  forward primer
agggtgaccatcacctgccaggccagccaggacatcagcaactacctgaactggtaccagcagaggcccggccaggcccccaagctgctgatctactacaccagcaggctgcacagcggc

SEQ ID NO: 221 - DNA, 90 bp, Artificial Sequence
  reverse primer
ctgggggcggccaccgtacgcttgatctccaccctggtgccgccgccgaaggtcctgggcagggtgttgccctgctggcagaagtaggtg

SEQ ID NO: 222 - DNA, 120 bp, Artificial Sequence
  reverse primer
cctgctggcagaagtaggtgccgatgtcctcggcctggaagctgttgatggcgatggtgaagctggtgccgctgcccctgccgctgaacctgctgggcacgccgctgtgcagcctgctgg

SEQ ID NO: 223 - DNA, 105 bp, Artificial Sequence
  forward primer
ctgcaaccggtgtacattctgaggtgaagctggtggagagcggcggcggcctggtgaagcccggcggcagcctgaagctgagctgcgccgccagcggcttcacct

SEQ ID NO: 224 - DNA, 120 bp, Artificial Sequence
  forward primer
gcgccgccagcggcttcaccttcagcagctacgccatgagctgggtgaggcagacccccgagaagaggctggagtgggtggccaccatcagcagcggcggcacctacacctactaccccg

SEQ ID NO: 225 - DNA, 104 bp, Artificial Sequence
  reverse primer
ctaggtcccttggtcgacgcgctgctcacggtcacgctggtgccctggccccagtagtccatgctgttgccgtccctcacgcagtagtacatggcggtgtcctc

SEQ ID NO: 226 - DNA, 120 bp, Artificial Sequence
  reverse primer
tagtacatggcggtgtcctcgctcctcaggctgctcatctgcaggtacagggtgttctcggcgttgtccctgctgatggtgaacctgcccttcacgctgtcggggtagtaggtgtaggtg

SEQ ID NO: 227 - DNA, 92 bp, Artificial Sequence
  forward primer
ctgcaaccggtgtacattcagacatccagatgacccagaccaccagcagcctgagcgccagcctgggcgacagggtgaccatcatctgcagg

SEQ ID NO: 228 - DNA, 117 bp, Artificial Sequence
  forward primer
agggtgaccatcatctgcagggccagccaggacatcaacaactacctgaactggtaccagaagcccgacggcaccgtgaagctgctgatctactacaccagcaggctgcacagcggc

SEQ ID NO: 229 - DNA, 90 bp, Artificial Sequence
  reverse primer
ctgggggcggccaccgtacgcctcagctccagcttggtgccggcgccgaaggtggggggcagggtgttggcctgctggcagaagtaggtg

SEQ ID NO: 230 - DNA, 120 bp, Artificial Sequence
  reverse primer
cctgctggcagaagtaggtggcgatgtcctcctgctccaggttgctgatggtcaggctgtagtcgctgccgctgccgctgccgctgaacctgctgggcacgccgctgtgcagcctgctgg

SEQ ID NO: 231 - DNA, 99 bp, Artificial Sequence
  forward primer
ctgcaaccggtgtacattctgaggtgcagctggtggagagcggcggcggcctggtgcagcccggcaggagcctgaggctgagctgcgccgccagcggct

SEQ ID NO: 232 - DNA, 120 bp, Artificial Sequence
  forward primer
tgagctgcgccgccagcggcttcaccttcagcaactacgccatgtactgggtgaggcaggcccccggcaagggcctggagtgggtggccctgatcagctacgacatcagcaccgactact

SEQ ID NO: 233 - DNA, 98 bp, Artificial Sequence
  reverse primer
ctaggtcccttggtcgacgcgctgctcacggtcaccagggtgccctggccccagtagtaggtgttggtgcagtagtacagggcggtgtcctcggtcct

SEQ ID NO: 234 - DNA, 120 bp, Artificial Sequence
  reverse primer
agggcggtgtcctcggtcctcaggttgttcatctgcaggtagatggtgttcttgctgttgtccctgctgatggtgaacctgcccttcacgctgtcggcgtagtagtcggtgctgatgtcg

SEQ ID NO: 235 - DNA, 96 bp, Artificial Sequence
  forward primer
ctgcaaccggtgtacattcacagagcgtgctgacccagagccccagcgccagcggcacccccggccagagggtgaccatcagctgcagcggcagca

SEQ ID NO: 236 - DNA, 120 bp, Artificial Sequence
  forward primer
ccatcagctgcagcggcagcagcagcaacatcggcaacaactacgtgtactggtaccagcagctgcccggcaccgcccccaagctgctgatctactggaacgaccagaggcccagcggcg

SEQ ID NO: 237 - DNA, 95 bp, Artificial Sequence
  reverse primer
ctgggggcggccaccgtacgcagcacggtcagctgggtgccgccgccgaacacggcgccgctcaggctgtcgtcccaggcggcgcagtagtagtc

SEQ ID NO: 238 - DNA, 120 bp, Artificial Sequence
  reverse primer
caggcggcgcagtagtagtcggcctcgtcctcgctcctcaggccgctgatggccaggctggcgctggtgccgctcttgctgccgctgaacctgtcgggcacgccgctgggcctctggtcg

SEQ ID NO: 239 - protein, 127 aa, Artificial Sequence
  LCA60 heavy chain insert
EVQLLESGGGLVKPGGSLRLSCEASGLTFSNVWMSWVRQAPGKGLEWVGRIKRKSEGATTDYGAPVKGRFTLSRDDSKNTVYLQMNSLKIDDTAVYYCSTLTRGGDVWSSSYYFDYWGQGALVTVSS

SEQ ID NO: 240 - protein, 109 aa, Artificial Sequence
  LCA60 light chain insert
QSALTQPASVSGSPGQSITISCTGTSSDVGTYDLVSWYQQHPGKSPKLMIYADIKRPSGVSHRFSGSKSGNTASLTISGLQSADEADYYCCLYAGSSTSVIFGGGTKVT

SEQ ID NO: 241 - protein, 116 aa, Artificial Sequence
  4C2h heavy chain insert
QVQLQESGGGLVKPGGSLKLSCAASGFTFSSYTMSWVRQTPDKRLEWVATISSGGSYTYYPDSVKGRFTISRDNAKNTLYLQMSSLKSEDTAMYYCARDGNDYDYWGQGTMVTVSS

SEQ ID NO: 242 - protein, 107 aa, Artificial Sequence
  4C2h light chain insert
DIQLTQSPSSLSASIGDRVTITCQASQDISNYLNWYQQRPGQAPKLLIYYTSRLHSGVPSRFSGRGSGTSFTIAINSFQAEDIGTYFCQQGNTLPRTFGGGTRVEIK

SEQ ID NO: 243 - protein, 116 aa, Artificial Sequence
  D12 heavy chain insert
EVKLVESGGGLVKPGGSLKLSCAASGFTFSSYAMSWVRQTPEKRLEWVATISSGGTYTYYPDSVKGRFTISRDNAENTLYLQMSSLRSEDTAMYYCVRDGNSMDYWGQGTSVTVSS

SEQ ID NO: 244 - protein, 107 aa, Artificial Sequence
  D12 light chain insert
DIQMTQTTSSLSASLGDRVTIICRASQDINNYLNWYQQKPDGTVKLLIYYTSRLHSGVPSRFSGSGSGSDYSLTISNLEQEDIATYFCQQANTLPPTFGAGTKLELR

SEQ ID NO: 245 - protein, 112 aa, Artificial Sequence
  MERS-4V2 heavy chain insert
EVQLVESGGGLVQPGRSLRLSCAASGFTFSNYAMYWVRQAPGKGLEWVALISYDISTDYYADSVKGRFTISRDNSKNTIYLQMNNLRTEDTALYYCTNTYYWGQGTLVTVSS

SEQ ID NO: 246 - protein, 110 aa, Artificial Sequence
  MERS-4V2 light chain insert
QSVLTQSPSASGTPGQRVTISCSGSSSNIGNNYVYWYQQLPGTAPKLLIYWNDQRPSGVPDRFSGSKSGTSASLAISGLRSEDEADYYCAAWDDSLSGAVFGGGTQLTVL

SEQ ID NO: 247 - DNA, 25 bp, Artificial Sequence
  forward primer
gacgcccgcaccgaggtgccccagc

SEQ ID NO: 248 - DNA, 25 bp, Artificial Sequence
  revers primer
agacagcagcctggagcacttattg

SEQ ID NO: 249 - DNA, 24 bp, Artificial Sequence
  forward primer
accgtgtggagggacggcgattac

SEQ ID NO: 250 - DNA, 20 bp, Artificial Sequence
  forward primer
agaaggcacgatgctcacgc

SEQ ID NO: 251 - DNA, 25 bp, Artificial Sequence
  forward primer
gagaagggcgattactataggaagc

SEQ ID NO: 252 - DNA, 22 bp, Artificial Sequence
  MERS_RBD_D537K rev
ccacacggtagaaggcacgatg

SEQ ID NO: 253 - DNA, 27 bp, Artificial Sequence
  forward primer
ggcaagtactataggaagcagctgagc

SEQ ID NO: 254 - DNA, 22 bp, Artificial Sequence
  reverse primer
gtcctcccacacggtagaaggc

SEQ ID NO: 255 - DNA, 3771 bp, Artificial Sequence
  mutant spike protein of SARS-CoV-2 Wuhan variant comprising substitution G502R, 2-P-mutation and inoperative furin cleavage site)
atgtttgtcttcctggtcctgctgcctctggtctcctctcagtgcgtgaacctgactactagaactcagctgcctcccgcttacaccaatagcttcaccaggggcgtgtactatccagacaaggtgtttcgcagctccgtgctgcactccacacaggatctgtttctgcccttcttttctaacgtgacctggttccacgccatccacgtgtccggcaccaatggcacaaagaggttcgacaatccagtgctgccctttaacgatggcgtgtacttcgcctccaccgagaagtctaacatcatccgcggctggatctttggcaccacactggacagcaagacacagtccctgctgatcgtgaacaatgccaccaacgtggtcatcaaggtgtgcgagttccagttttgtaatgatcctttcctgggcgtgtactatcacaagaacaataagtcttggatggagagcgagtttagggtgtactctagcgccaacaattgcacatttgagtatgtgagccagccattcctgatggacctggagggcaagcagggcaatttcaagaacctgcgggagttcgtgtttaagaatatcgatggctacttcaaaatctactccaagcacacccccatcaacctggtgcgggacctgccacagggcttctctgccctggagcctctggtggatctgccaatcggcatcaacatcaccaggtttcagacactgctggccctgcaccgcagctacctgacacctggcgactcctctagcggatggaccgcaggagctgccgcctactatgtgggctacctgcagccaaggaccttcctgctgaagtataacgagaatggcaccatcacagacgcagtggattgcgccctggaccccctgtctgagacaaagtgtacactgaagagctttaccgtggagaagggcatctaccagacaagcaatttccgggtgcagcccaccgagtccatcgtgagatttccaaatatcacaaacctgtgcccctttggcgaggtgttcaacgccacccgcttcgccagcgtgtatgcctggaataggaagcgcatctccaactgcgtggccgactattctgtgctgtacaactccgcctctttcagcacctttaagtgttacggcgtgagccctacaaagctgaatgacctgtgctttaccaacgtgtatgccgattccttcgtgatcaggggcgacgaggtgcgccagatcgcaccaggacagacaggcaagatcgccgactacaattataagctgcccgacgatttcaccggctgcgtgatcgcctggaactctaacaatctggatagcaaagtgggcggcaactacaattatctgtaccggctgtttagaaagtctaatctgaagcctttcgagagggacatctccacagaaatctaccaggccggctctaccccatgcaatggcgtggagggctttaactgttatttccccctgcagtcctacggcttccagcctacaaacgatgtgggctatcagccataccgcgtggtggtgctgtcttttgagctgctgcacgcaccagcaacagtgtgcggacctaagaagagcaccaatctggtgaagaacaagtgcgtgaacttcaacttcaacggcctgaccggcacaggcgtgctgaccgagagcaacaagaagttcctgccctttcagcagttcggccgggacatcgcagataccacagacgccgtgcgggacccccagaccctggagatcctggacatcacaccttgctccttcggcggcgtgtctgtgatcacacctggcaccaatacatccaaccaggtggccgtgctgtaccaggacgtgaattgtaccgaggtgccagtggccatccacgccgatcagctgacccccacatggagggtgtatagcaccggctccaacgtgttccagacacgcgccggatgcctgatcggagcagagcacgtgaacaatagctacgagtgcgacatccccatcggcgccggcatctgtgcctcctatcagacccagacaaactcccctaggagagcccggtctgtggcctcccagtctatcatcgcctacaccatgagcctgggcgccgagaacagcgtggcctattctaacaatagcatcgccatccccaccaacttcacaatcagcgtgaccacagagatcctgcctgtgagcatgaccaagacatccgtggactgcacaatgtacatctgtggcgattccaccgagtgctctaacctgctgctgcagtatggctccttttgtacccagctgaatagagccctgacaggcatcgccgtggagcaggacaagaacacacaggaggtgttcgcccaggtgaagcaaatctacaagaccccccctatcaaggactttggcggcttcaacttcagccagatcctgcccgatccttccaagccatctaagcggagctttatcgaggacctgctgttcaacaaggtgaccctggccgatgccggcttcatcaagcagtacggcgattgcctgggcgacatcgcagcccgggacctgatctgcgcccagaagtttaatggcctgaccgtgctgccacccctgctgacagatgagatgatcgcccagtatacatctgccctgctggccggcaccatcacaagcggatggaccttcggcgcaggagccgccctgcagatcccctttgccatgcagatggcctacagattcaacggcatcggcgtgacccagaatgtgctgtatgagaaccagaagctgatcgccaatcagtttaacagcgccatcggcaagatccaggactctctgtcctctacagccagcgccctgggcaagctgcaggatgtggtgaatcagaacgcccaggccctgaataccctggtgaagcagctgagcagcaacttcggcgccatctctagcgtgctgaatgacatcctgagccggctggaccccccagaggcagaggtgcagatcgaccggctgatcacaggcagactgcagtccctgcagacctacgtgacacagcagctgatcagggcagcagagatcagggcctctgccaatctggccgccaccaagatgagcgagtgcgtgctgggccagtccaagagagtggacttttgtggcaagggctaccacctgatgagcttcccacagtccgccccccacggcgtggtgtttctgcacgtgacctatgtgcctgcccaggagaagaacttcaccacagccccagccatctgccacgatggcaaggcacactttccccgggagggcgtgttcgtgagcaacggcacccactggtttgtgacacagagaaatttctatgagcctcagatcatcaccacagacaataccttcgtgagcggcaactgtgacgtggtcatcggcatcgtgaacaataccgtgtacgatcctctgcagccagagctggactcttttaaggaggagctggataagtatttcaagaaccacaccagccccgacgtggatctgggcgacatctctggcatcaatgccagcgtggtgaacatccagaaggagatcgacaggctgaatgaggtggccaagaatctgaacgagagcctgatcgatctgcaggagctgggcaagtatgagcagtccggccgcgagaacctgtacttccagggaggaggaggctctggatatatcccagaggcacctcgggatggacaggcctacgtgagaaaagacggcgagtgggtcctgctgagtaccttcctggggcatcatcatcatcaccattaa

SEQ ID NO: 256 - DNA, 3771 bp, Artificial Sequence
  mutant spike protein of SARS-CoV-2 Wuhan variant comprising substitution L455R, 2-P-mutation and inoperative furin cleavage site)
atgtttgtcttcctggtcctgctgcctctggtctcctctcagtgcgtgaacctgactactagaactcagctgcctcccgcttacaccaatagcttcaccaggggcgtgtactatccagacaaggtgtttcgcagctccgtgctgcactccacacaggatctgtttctgcccttcttttctaacgtgacctggttccacgccatccacgtgtccggcaccaatggcacaaagaggttcgacaatccagtgctgccctttaacgatggcgtgtacttcgcctccaccgagaagtctaacatcatccgcggctggatctttggcaccacactggacagcaagacacagtccctgctgatcgtgaacaatgccaccaacgtggtcatcaaggtgtgcgagttccagttttgtaatgatcctttcctgggcgtgtactatcacaagaacaataagtcttggatggagagcgagtttagggtgtactctagcgccaacaattgcacatttgagtatgtgagccagccattcctgatggacctggagggcaagcagggcaatttcaagaacctgcgggagttcgtgtttaagaatatcgatggctacttcaaaatctactccaagcacacccccatcaacctggtgcgggacctgccacagggcttctctgccctggagcctctggtggatctgccaatcggcatcaacatcaccaggtttcagacactgctggccctgcaccgcagctacctgacacctggcgactcctctagcggatggaccgcaggagctgccgcctactatgtgggctacctgcagccaaggaccttcctgctgaagtataacgagaatggcaccatcacagacgcagtggattgcgccctggaccccctgtctgagacaaagtgtacactgaagagctttaccgtggagaagggcatctaccagacaagcaatttccgggtgcagcccaccgagtccatcgtgagatttccaaatatcacaaacctgtgcccctttggcgaggtgttcaacgccacccgcttcgccagcgtgtatgcctggaataggaagcgcatctccaactgcgtggccgactattctgtgctgtacaactccgcctctttcagcacctttaagtgttacggcgtgagccctacaaagctgaatgacctgtgctttaccaacgtgtatgccgattccttcgtgatcaggggcgacgaggtgcgccagatcgcaccaggacagacaggcaagatcgccgactacaattataagctgcccgacgatttcaccggctgcgtgatcgcctggaactctaacaatctggatagcaaagtgggcggcaactacaattatctgtaccggcgttttagaaagtctaatctgaagcctttcgagagggacatctccacagaaatctaccaggccggctctaccccatgcaatggcgtggagggctttaactgttatttccccctgcagtcctacggcttccagcctacaaacggcgtgggctatcagccataccgcgtggtggtgctgtcttttgagctgctgcacgcaccagcaacagtgtgcggacctaagaagagcaccaatctggtgaagaacaagtgcgtgaacttcaacttcaacggcctgaccggcacaggcgtgctgaccgagagcaacaagaagttcctgccctttcagcagttcggccgggacatcgcagataccacagacgccgtgcgggacccccagaccctggagatcctggacatcacaccttgctccttcggcggcgtgtctgtgatcacacctggcaccaatacatccaaccaggtggccgtgctgtaccaggacgtgaattgtaccgaggtgccagtggccatccacgccgatcagctgacccccacatggagggtgtatagcaccggctccaacgtgttccagacacgcgccggatgcctgatcggagcagagcacgtgaacaatagctacgagtgcgacatccccatcggcgccggcatctgtgcctcctatcagacccagacaaactcccctaggagagcccggtctgtggcctcccagtctatcatcgcctacaccatgagcctgggcgccgagaacagcgtggcctattctaacaatagcatcgccatccccaccaacttcacaatcagcgtgaccacagagatcctgcctgtgagcatgaccaagacatccgtggactgcacaatgtacatctgtggcgattccaccgagtgctctaacctgctgctgcagtatggctccttttgtacccagctgaatagagccctgacaggcatcgccgtggagcaggacaagaacacacaggaggtgttcgcccaggtgaagcaaatctacaagaccccccctatcaaggactttggcggcttcaacttcagccagatcctgcccgatccttccaagccatctaagcggagctttatcgaggacctgctgttcaacaaggtgaccctggccgatgccggcttcatcaagcagtacggcgattgcctgggcgacatcgcagcccgggacctgatctgcgcccagaagtttaatggcctgaccgtgctgccacccctgctgacagatgagatgatcgcccagtatacatctgccctgctggccggcaccatcacaagcggatggaccttcggcgcaggagccgccctgcagatcccctttgccatgcagatggcctacagattcaacggcatcggcgtgacccagaatgtgctgtatgagaaccagaagctgatcgccaatcagtttaacagcgccatcggcaagatccaggactctctgtcctctacagccagcgccctgggcaagctgcaggatgtggtgaatcagaacgcccaggccctgaataccctggtgaagcagctgagcagcaacttcggcgccatctctagcgtgctgaatgacatcctgagccggctggaccccccagaggcagaggtgcagatcgaccggctgatcacaggcagactgcagtccctgcagacctacgtgacacagcagctgatcagggcagcagagatcagggcctctgccaatctggccgccaccaagatgagcgagtgcgtgctgggccagtccaagagagtggacttttgtggcaagggctaccacctgatgagcttcccacagtccgccccccacggcgtggtgtttctgcacgtgacctatgtgcctgcccaggagaagaacttcaccacagccccagccatctgccacgatggcaaggcacactttccccgggagggcgtgttcgtgagcaacggcacccactggtttgtgacacagagaaatttctatgagcctcagatcatcaccacagacaataccttcgtgagcggcaactgtgacgtggtcatcggcatcgtgaacaataccgtgtacgatcctctgcagccagagctggactcttttaaggaggagctggataagtatttcaagaaccacaccagccccgacgtggatctgggcgacatctctggcatcaatgccagcgtggtgaacatccagaaggagatcgacaggctgaatgaggtggccaagaatctgaacgagagcctgatcgatctgcaggagctgggcaagtatgagcagtccggccgcgagaacctgtacttccagggaggaggaggctctggatatatcccagaggcacctcgggatggacaggcctacgtgagaaaagacggcgagtgggtcctgctgagtaccttcctggggcatcatcatcatcaccattaa

SEQ ID NO: 257 - DNA, 669 bp, Artificial Sequence
  mutant RBD of SARS-CoV-2 Wuhan variant comprising substitution G184R
cgggtgcagcccaccgagtccatcgtgagatttccaaatatcacaaacctgtgcccctttggcgaggtgttcaacgccacccgcttcgccagcgtgtatgcctggaataggaagcgcatctccaactgcgtggccgactattctgtgctgtacaactccgcctctttcagcacctttaagtgttacggcgtgagccctacaaagctgaatgacctgtgctttaccaacgtgtatgccgattccttcgtgatcaggggcgacgaggtgcgccagatcgcaccaggacagacaggcaagatcgccgactacaattataagctgcccgacgatttcaccggctgcgtgatcgcctggaactctaacaatctggatagcaaagtgggcggcaactacaattatctgtaccggctgtttagaaagtctaatctgaagcctttcgagagggacatctccacagaaatctaccaggccggctctaccccatgcaatggcgtggagggctttaactgttatttccccctgcagtcctacggcttccagcctacaaaccgtgtgggctatcagccataccgcgtggtggtgctgtcttttgagctgctgcacgcaccagcaacagtgtgcggacctaagaagagcaccaatctggtgaagaacaagtgcgtgaacttc

SEQ ID NO: 258 - DNA, 669 bp, Artificial Sequence
  mutant RBD of SARS-CoV-2 Wuhan variant comprising substitution L137R
cgggtgcagcccaccgagtccatcgtgagatttccaaatatcacaaacctgtgcccctttggcgaggtgttcaacgccacccgcttcgccagcgtgtatgcctggaataggaagcgcatctccaactgcgtggccgactattctgtgctgtacaactccgcctctttcagcacctttaagtgttacggcgtgagccctacaaagctgaatgacctgtgctttaccaacgtgtatgccgattccttcgtgatcaggggcgacgaggtgcgccagatcgcaccaggacagacaggcaagatcgccgactacaattataagctgcccgacgatttcaccggctgcgtgatcgcctggaactctaacaatctggatagcaaagtgggcggcaactacaattatctgtaccggcgttttagaaagtctaatctgaagcctttcgagagggacatctccacagaaatctaccaggccggctctaccccatgcaatggcgtggagggctttaactgttatttccccctgcagtcctacggcttccagcctacaaacggcgtgggctatcagccataccgcgtggtggtgctgtcttttgagctgctgcacgcaccagcaacagtgtgcggacctaagaagagcaccaatctggtgaagaacaagtgcgtgaacttc

SEQ ID NO: 259 - protein, 1256 aa, Artificial Sequence
  wildtype spike protein of SARS-CoV-2 Whuhan variant comprising 2-P-mutation (substitutions K986P and V987P) and His-tag
MFVFLVLLPLVSSQCVNLTTRTQLPPAYTNSFTRGVYYPDKVFRSSVLHSTQDLFLPFFSNVTWFHAIHVSGTNGTKRFDNPVLPFNDGVYFASTEKSNIIRGWIFGTTLDSKTQSLLIVNNATNVVIKVCEFQFCNDPFLGVYYHKNNKSWMESEFRVYSSANNCTFEYVSQPFLMDLEGKQGNFKNLREFVFKNIDGYFKIYSKHTPINLVRDLPQGFSALEPLVDLPIGINITRFQTLLALHRSYLTPGDSSSGWTAGAAAYYVGYLQPRTFLLKYNENGTITDAVDCALDPLSETKCTLKSFTVEKGIYQTSNFRVQPTESIVRFPNITNLCPFGEVFNATRFASVYAWNRKRISNCVADYSVLYNSASFSTFKCYGVSPTKLNDLCFTNVYADSFVIRGDEVRQIAPGQTGKIADYNYKLPDDFTGCVIAWNSNNLDSKVGGNYNYLYRLFRKSNLKPFERDISTEIYQAGSTPCNGVEGFNCYFPLQSYGFQPTNGVGYQPYRVVVLSFELLHAPATVCGPKKSTNLVKNKCVNFNFNGLTGTGVLTESNKKFLPFQQFGRDIADTTDAVRDPQTLEILDITPCSFGGVSVITPGTNTSNQVAVLYQDVNCTEVPVAIHADQLTPTWRVYSTGSNVFQTRAGCLIGAEHVNNSYECDIPIGAGICASYQTQTNSPRRARSVASQSIIAYTMSLGAENSVAYSNNSIAIPTNFTISVTTEILPVSMTKTSVDCTMYICGDSTECSNLLLQYGSFCTQLNRALTGIAVEQDKNTQEVFAQVKQIYKTPPIKDFGGFNFSQILPDPSKPSKRSFIEDLLFNKVTLADAGFIKQYGDCLGDIAARDLICAQKFNGLTVLPPLLTDEMIAQYTSALLAGTITSGWTFGAGAALQIPFAMQMAYRFNGIGVTQNVLYENQKLIANQFNSAIGKIQDSLSSTASALGKLQDVVNQNAQALNTLVKQLSSNFGAISSVLNDILSRLDPPEAEVQIDRLITGRLQSLQTYVTQQLIRAAEIRASANLAATKMSECVLGQSKRVDFCGKGYHLMSFPQSAPHGVVFLHVTYVPAQEKNFTTAPAICHDGKAHFPREGVFVSNGTHWFVTQRNFYEPQIITTDNTFVSGNCDVVIGIVNNTVYDPLQPELDSFKEELDKYFKNHTSPDVDLGDISGINASVVNIQKEIDRLNEVAKNLNESLIDLQELGKYEQSGRENLYFQGGGGSGYIPEAPRDGQAYVRKDGEWVLLSTFLGHHHHHH